European Patent Specification EP 4 294 375 B1, published April 1, 2026. Title: METHODS OF LOADING EXTRACELLULAR VESICLES. Applicant: Codiak BioSciences, Inc. The sequence listing filed with the application follows.

SEQUENCE LISTING (112 sequences)

SEQ ID NO: 1 - skipped

SEQ ID NO: 2 - DNA, 16010 bp, Artificial Sequence
  STAT6 pre-mRNA transcript
agagctccagggagggacctgggtagaaggagaagccggaaacagcgggctggggcagccactgcttacactgaagagggaggacgggagaggagtgtgtgtgtgtgtgtgtgtgtgtgtgtgtatgtatgtgtgtgctttatcttatttttctttttggtggtggtggtggaaggggggaggtgctagcagggccagccttgaactcgctggacagagctacagacctatggggcctggaagtgcccgctgagaaagggagaagacagcagaggggttgccgaggtgaggggttgcctccgaggtgggtgcgggggcctctatgagtgcatgggggtggattcgtggggggagctctcgggatcctcccctggctgggtggatggtccccaagagatggtttcagctagtgttggtggctggtggcactgggttttagcagtttcgaactcctggaggaatctgggagggtccaggcctcagtactcccctcccccatgggtcacgttttcacagcctcacccctgcacccccagggccatggaaagtcagggaaaggaggtgaaggagtgcccctctgccctgagtcgggggaagtggccgcccctccctggaaggttgatgccagagggcagtggatccttgttaaacccctatcctgccctccactaaaggttcctgttcaagggtgtggctggggcgtgagcaagccccagatgtagacctcatggtggcccagacgagggggaatttccccctcaaaactgctccacgcttggctgctgtagacgctgagatttcccagcggcggcgccgagttaaccctcctcgtgctgaactggctccacctccccgcctgcccccaccgccacattcacgcattgggcaactcagagaagctgttttaactttcgatcctgtggtcccacaatcagaggactcgggcagataggggttgagataagcgagtttaggccaccaagcgggcggacgaggatcccagaccttgcgcttcccttctgagtttgggaggtaacactggccccgcccctcacgccgtggctcctccctcccttccccttcaaggggctgaagacaaaaggtgcccctgtcctggtcaagccaatcgacccagccttgttatgggttggggtggggagaaatgtgtcctcctgatggctggggaagaagaggggttggatatttctagccagggccatgccaggaggctggtcactctgcaaggggatgcagaggaaagcggtgcccactcactccagaggacctttctctcttgggctagagaaaggcctattggaggaacctgagcaggaggggtaaggattctgccttgaggagaaaagagctggggtaagtgggcactggaggaaagaggggcatgaaggtcttggagcagaaacgtccagagaagggacctctccattttccatccctctgagaggcctgggagaggtgagaggctgaacgtgcaacaggaggacttggggttactgggtttggggagacctggggagttgtcatcccatcctctccctcatctctgggagagggatattatgagaaacgtgaactgagaggcccctgggaaaccactggttacccagtcctccctgaacctggaaatggggatgcaaccccctcttctacttccctgtcccctcctctcctttctacctgttttcgtctctcatctttgccttctagccctccagcttcctctctcttctaggctctttcctcctagcttactaaacccgccttttttccagtctcttccatcctcttccttagttctctctactttccttttccacctctcctccttcaagtctcctcccaccttcccccacttcttaggatgatcagatttgcccctggaagggatcctaacaacacagtgcgatggttaatccccactcagattcaaagcctgctttccaaactcacttactgagtggccttgggcagagtagagaaactccttaagcctcagtttcttcatctataaaatgggatattatatattttaaaaagtgtcgtgaggcctgaaggagataatacactgagtgtaatgcctcatacacagtaagtgcttaacaaatagtagctgttattactctcccatcctcttcatcatctagccttgtggttttcatttttattttatttcatttatttatttatttattttgaggcagagtctctctctgtcgcccaggctggagtgcagtggctcgatctctgctcactgcaagctccgccccccaggttcacgccattctgtcacctcagcctccccagtagctgggactacaggcgctcgccaccacgccctgctaattttgtttttgtatttttagtagagatggggtttcactgtgttagccaggatggtcttgatctcctgacctcgtgatctgcccgcctcggcctcccaaagcgctgggattacaggcatgagccactgcgcctggccgagccttgtggttttcaaattatctcatggagtcctagaattttgagaggtttgtctagggatgcctttggcgtcaggaggtggggagagggaagtagaagcagtcgagtttcaggctttccatgcttgctttcaacagggcatcttcggtttcgtaccttttatgtaattgagattccacagattaaaagctgacattgcctaccgctttaaaaagtttggaaagttttccactcatctaacactcatattttatagatgagaagatcgaagcccacaaagggaaggctctttgcccacagaaccagagccaggtctagagctgcaactaaatcctctgccactctaagagagctctcgctctactgccctgtctccctttgcctccccatccctctggctacagctcagctcttcccacccctgtgtctatcactgaaggagttacccccatctcaggcattgactcaggatgcccctggtttaaggtggtctggccatgagtggtggtggggacggtccctaggagggctatctatgggaggtccctggctgccccaggagataggccaagtttcttgggcacccctcagagtggccttatttttctcctccaggcaacctccaagtcccagatcatgtctctgtggggtctggtctccaagatgcccccagaaaaagtgcagcggctctatgtcgactttccccaacacctgcggcatcttctgggtgactggctggagagccagccctggtgagtcctggctgctccctgctggtcccccaagtcttccctaactcatcttccttctccttagatttttctcccctcacccatggattcagaacttgagacctgttattccatgtgtagtgacctagatttagcagggagtctgtgccccatcaagaccaggctatgaatgttgacagatggagaccccatctcttaggaggctgagccgaagaggaggggggtttgggctgggacaaaggcacttctcataacagctagaagactgggaaacaaggcgcatgggtgaaagctacagagggcctagatggagaataaggagcgagaaaggaactgctgagcttttggctgtggggtaaagggtcaggagagctgaggaagccctggcctgaggtagcctcatcctgatcttcctgcagggagttcctggtcggctccgacgccttctgctgcaacttggctagtgccctactttcagacactgtccagcaccttcaggcctcggtgggagagcagggggaggggagcaccatcttgcaacacatcagcacccttgaggtggggcaggaggggaggggacaaggctgggtggggctgaggttgaactgggttgagcattgggccctggaagaaaattggttggatgctggaagcaaattggtgttcctgtggttaactgctagctagcaggcaaattagattttaaaagcatgcaaatgcacaaaaacttctggagtctacagttgtgcttccttatagtatatgtgtgaatgcaggcctggggattggagggattgaaggacatgggtaagagcaaagctcactgtttaccaccctcatttctgtagagcatatatcagagggaccccctgaagctggtggccactttcagacaaatacttcaaggagagaaaaaagctgttatggaacaggtattgtgatattccacctcccaccccaactcaatcccctgagactttggcctgagccatgacaaactagaaagaatttgaacctcagtaaaggctcagtgttctaggcccaggaatgaccaaaggaggttcctagggtcagagtgaaccccaagtcaagctcagggaatctttctatgagggactgaaggtaagaggccggggagaacagagcaagggataaggagctgattctgctaggagcaaggtcttatctccacgatattccaaaaggtcaggaagaactgccaaaggggagaggggaacaagaaaacgctatctgcagagcagagagtggaggccaggtatagagggatgagcagagtgtttcacttcttggcatctgtccttcctgtgtagttccgccacttgccaatgcctttccactggaagcaggaagaactcaagtttaagacaggcttgcggaggctgcagcaccgagtaggggagatccaccttctccgagaagccctgcagaagggggctgaggctggccaaggtgggggccagggtggttctggggagtgtgtaggagtggttgcctcttggatctcaaccttatctgaacctctaatctgtctgcacccttgatttctgcccccaaccctcagtgtctctgcacagcttgatagaaactcctgctaatgggactgggccaagtgaggtgagtaatgggctgacaggtggagaccttggtcaaagtgcagctggagggatggaagctagacctcagaaagacacaggctgaagtagggcaagggaatgccagaggagtgagaaaaagagccgtatcccaggagctgggtgtggaggcagcgtgaggccctggctcaggcccctctctgcccataggccctggccatgctactgcaggagaccactggagagctagaggcagccaaagccctagtgctgaagaggatccagatttggaaacggcagcagcagctggcagggaatggcgcaccgtttgaggagagcctggccccactccaggagaggttgggctagggctgatggggaagagggggcaagctgggggtgggcagctgaccctgctgaaggccctacaggtgagagaaagaagccaggcgggagggccttggagtggaccaagatgcataaaagccagttccagcggggctgtgcacactgtcgttcaggtcgcatcctgtacaagtgggcctagtggaggggcacaagcggggactcatccaacccaggcttctctcctcaagccccatgcctagaggaataggagggcttttccatttggtttattgggtgggaacactttccaatttgccacaaagcactgtaagtggtggcagttgtcctgggtgcaagagccgtcgggggagaggcagctgggtttccacagggggtgtaggcactgagaatgaacctcccacccagaccctaggccaacagatcacagaacccccttcagcccaggtgccttgcagccacacccactacccaccccacttctccacacatgatagcctttctccctgggtataggggaagggggtctgggccggagcaagcagccttaatcctgtgccccctgaccactgtcctggccccaggtgtgaaagcctggtggacatttattcccagctacagcaggaggtaggggcggctggtggggagcttgagcccaagacccgggcatcgctgactggccggctggatgaagtcctgagaaccctcgtcaccaggtattccccgggagctcccagtctggcctagaacagacctcgggaagaaaagaagggggctagagctgtggggagggcaccagcagggacctagcccccaactccccttgtgtcctcctcactcccagttgcttcctggtggagaagcagcccccccaggtactgaagactcagaccaagttccaggctggagttcgattcctgttgggcttgaggttcctgggggccccagccaagcctccgctggtcagggccgacatggtgacagagaagcaggcgcgggagctgagtgtgcctcagggtcctggggctggagcgtaagctgggattggacctggggttggagaagggctgttagggtgatggaggcagcctggagggctggcactgaaaagagcaagggatggggagggagggccatgggatgtggagaccctgaatggtcaaggcagaggaaagggagggacccatttagggctggaatggggtgggggcatcatgatttggccaagatggggactcctcccttaagaacccaaacagagacatggagatttagggctggtgacagtgggtagtctacactcacccatgcactcgccacacctgacgacagtgagatgagctcgttcacactctgacctcccctggcagagaaagcactggagaaatcatcaacaacactgtgcccttggagaacagcattcctgggaactgctgctctgccctgttcaagaacctggtgaggggctttggggtgcagtgaggggggcaccactaggagactgtgggactctccttggagaggatgtcaggaagcccaggaggagcggtctctgtcctcatgacctcgcccttgctctccctcaccccacccacagcttctcaagaagatcaagcggtgtgagcggaagggcactgagtctgtcacagaggagaagtgcgctgtgctcttctctgccagcttcacacttggccccggcaaactccccatccagctccaggtgaaccgtggcccagccctgccccaatctgggaccccgagtcctcctccaatgccacacacaagggccctggaccctcacctcttgtgactgccccataccccatgtgtctgggattcatgcacactggggcccgggtgagtgggggtgagcaagagcatggagtgcacagggcagggaatggtagtggatagcagcaaacacttcggaagcacttcctatagaccagggcactctattaaatgatacatacgcacatgcgtgccagcacacacacgtctggttttcacaataacattatgaggtaggcagtattatcagcctcattttatagataaggacattgagacagagagtttaagtagtttgtcccagtcacacagctaagtgttggagctggtatttgaaacctggaggtctggttccatagcgatgactaataaccacttctctacggtgaggccctgattgagcttcagaacgcatttaataacatggcatgagctttttgattatgatgtgtgagtccaataacttctctgagtgctcagagccagtcccctgaggaaacttcttgcttcactaagaaacccctgtccggctgggcatggtggctcaagcctgtaatcccagcactttgggaggccgaggtgggtagatcacaaggtcaggagttcaagaccagcctggccaatatggtgaaaccccgtctccactaaaaatacaaaaattagctgggcgtggtggtgcaggcctgtagtcccagctgctcgggaggctaagcaggagaatcgcttgaacccaggaggcggaggttgcagtgagccaagattgcgccactgcccttcagcctgggcgacagagcaagactatgtctcaaaaacaaaacaaaacaactcagcactttgggaggccaaggtaggaggatcgcttgagcctgcaagtttaagaccagcctgggctacatagggagatccaatctctacaaaaaataaaaaattggccgggcatggtggctcacgcctgtaatcccagcactttgggaggccaaggcgggcggatcatgaggtcaggaaatcgagaccatcctggctaacacggtgaaacctcgtatctactaaaaatacaaaaaattagccaggcatggtggcgggcgcctgagtcccagctactcgggaggctgaagcaggagaatggcgtgaacctgggagggagagcttgcagtgagccaagatcgcgccactgcactccagcctgagtgacagagcgagactctgtctcaaaaataaataaataaataattagctggattaggtggtacatttctgtagttccagctattcaggaggctgaggtggaaggatcacttgagccctgaaggctgaggctgcagtgagctgagattgcactactgcactccagcctgggcaacagagtgagatactatctaaaaaaaaaaaaaaaaaaaaaaaaaaaaaaaaaaaaaaaaaaaaaaaaaggaaagaaagaaagaaaagaaacccctgtcctcaccctcttcaggccctgtctctgcccctggtggtcatcgtccatggcaaccaagacaacaatgccaaagccactatcctgtgggacaatgccttctctgagatggtgaggaaagtcctggagttggagggaacaggggcagggtgggttctaacatgggcagtggtgcaggcctgctgatggggtggtgggcatgtttaaatgggtgtgaccttaacactttctcatgggcctgctttcgtgcttctgacctcttttcaccccagtcttaacaactatcaggccacagcactgtaacctagaaaaaacagcatgtttgtgagcgatatcaggggctgtggaggggtaggccacaggcaggtgggagggatgaaggccggcccgaggaataacaagacggtagcctgcagtgctctcttcttcccccttctccccaggaccgcgtgccctttgtggtggctgagcgggtgccctgggagaagatgtgtgaaactctgaacctgaagttcatggctgaggtggggaccaaccgggggctgctcccagagcacttcctcttcctggcccagaagatcttcaatgacaacagcctcagtatggaggccttccagcaccgttctgtgtcctggtcgcagttcaacaaggtcattctcctgccctttggacctcccacccccaagctcttcatccctggggcactcagggcctgctcagcctccatgcagggaccttccactggattctccacagtgccccctcaggtcctttaggaaggcctgtcatggaccagggaggaaaaaccccaggcctgggggttggctctggagatgcgttctctgacatccctgaggttttggtctgggggccatctgtccttcctctttaccagtgacttgcatgactcacccaggttgtgtgtaaacagagctctgattcaaagtgactttgacctgttggaaaaatagttcctggccgggcacagcggctcatgcctgtaatcccagtctttgacatgccggggtgggtggatcacctgaggtcaggagtttgagaccagcctggccaacatggtgaaactccatctctactaaaaatacaaaaattagccagttgcggtggcacatgcctgtaatcccagctacatgggaggctgacgcaggagaattgcttgaacccaggaggtggaggttgcagtgagctgagatcataccactgcactcaagcctgggtgacagagcaagactctgtctcaaaaaaaaaaaaaaaaaaaggccaggcatggtggttcatgcctgtaatcccagcactttgggaggccgagacggatagatcacctgaggtcaggagttcgagaccagcctggccaacatggcaaaaccccgtctctactaaaaacaaaaaaatagccaggagtggtcgtttgcgtctgtaatcccagctactcggctgaggcaggaggtgaacccaggaggtagaggctgcagggaagatgaaaccattgcactccagcctgggcaagactctgtatcaaaaaaaaaaaaaaaaaaggctaggtgtggtggctcacacctgtaatcccagcactttgggaggctgaggcgggcggatcacaaggtcaagagatcgagaccatcctgaccaacatggtgaaaccccgtctctactaaaaatacaaaaattacctgggcatggtggcgcatgcctgtagtcccaactactcgggaggctgaggcaggagaatcacttgaacctgggaggcagaggttgcagcgagccaagattgtgccactgcactccagcctgccaacagaatgagattctgtctaaaaaaaaaaagaaagaaagaaagaaagaaaaagaattcctgttgcaaaaactgaacaaaatcccacagggacatgtgcagtaataccagctaccacgtgttgacagcttatatgccaggcgctgtgcttaacaccttatgtatgttatctcacttaatcctcccaacatctctttgaggtagatactattattatccccattttacagatgaggaatctgatgctcagagggttatgtagtttgttcaagttcccaaagcaggtgagtgccatggctaggagagaaccacatatttctgactcttgctcttttattttatgttatattatgttattttatgttttggtttttttttcttttctttctttctttctttctttctttctttctttctttctttctttctctttctttctttctttctttctttctttctttctttctttctttctttctttctttctttctctttctctttctctctttttctttcttttgtgtgagacagaatctttaaagagaagaaagaaatgctcatgtgaccagagggtgtgttagctaaagggagcaagacagtcacacccagcaggttaccttcctttgggcgtcacctctgccacacctccttagggagagggtgtagcatagtagttaagaggggctccagggccagaatgcctgggtttaaatcctagctctgcctcttaccagctatgtagacctgggcaagtcattcgacgtttttggacttccatttcttcatctgtaagatggaattattataatccctacttccatagcctggtaaagagcaaataaatatatggaaaggcttgaaatagtggctggcacgtgtaagcattaggattggtcgttgtcattgatggagtctcaggttcggtctgatcctcagccctgtgattctgtcgtgagggcactcacagctcactgcctgccctaaacaggctccagctctggccctccctcggctcacacctttccccctctccccctaggagatcctgctgggccgtggcttcaccttttggcagtggtttgatggtgtcctggacctcaccaaacgctgtctccggagctactggtctgaccggtgagtccccaccctgggtagtctgagcagccatacaccagtcacctccatactcactgcccatgccccatcctctccttcatcccggccaggctgatcattggcttcatcagcaaacagtacgttactagccttcttctcaatgagcccgacggaacctttctcctccgcttcagcgactcagagattgggggcatcaccattgcccatgtcatccggggccaggatggtgaggccaccccagccagtcctctgtctctgtgcctgtgccctctggggtttcttctgggaatgaaatgtcctgaccttcctgatgccgatcctgatcttcaggaagttcttccagcttctcttcttccttctgtggtctaaatgttcaccttctcactgtgagctctgtgggaacggagactagtgggtctctctccctcaggagccccaccctaggtcctctctcccttgccttggtggagtgagaacaggtcttatggtaggggttggggaaggggaagaaagtccggacagagggatctcagggtctccttcctaccataggctctccacagatagagaacatccagccattctctgccaaagacctgtccattcgctcactgggggaccgaatccgggatcttgctcagctcaaaaatctctatcccaagaagcccaaggatgaggctttccggagccactacaagcgtgagctggaactggcagctctgattccttcctgtcacccacttcctccctgctccccgctgccctcctctccctgcccgcgtgtcatcctgatgtcactccctatttcatagctgtgcttctcttacttccccatgatccatgcccaccttttccacctcccttcctccctaaccccagagcactccatggctgtcttttccttctcacaacagctgaacagatgggtaaggatggcaggggttatgtcccagctaccatcaagatgaccgtggaaaggtgagtgtggtggtatggacagtgggtaggtcaggggcttagtgcttatctgcaggaaggaggggtggcatcaacccttggtcagtcacatgtacctccttccctcctccagggaccaaccacttcctaccccagagctccagatgcctaccatggtgccttcttatgaccttggaatggcccctgattcctccatgagcatgcagcttggcccagatatggtgtaaggagctggaaagacaggaatgggagtggtctgtgcagatgggctaatcttagcatgggcagctgggagagctggcactgggggctgaacagggaatcttcctttccatgagagggacacctgttcaaaagcagggtgtggtggtgtccaggagaagggctggcatcagggggtctgttttctttccccaggccccaggtgtacccaccacactctcactccatccccccgtatcaaggcctctccccagaagaatcagtcaacgtgttgtcagccttccaggagtaagtgaaaaacctcatggggataccatcccactctaagggggtgggcatttgaattgttagaagaggctcttctgtgagaaaggagcagcaaatgctaacagcctgtcttcttctcttctgtccactctaatgagggggtagtagttaagatctggactgcctaggtttgaattctagctccaccacttactggtttggggcaaattacttagcctttggtgccttatctgcacaatgggggataataatgctaataataataacctacctcactgcattattgtggagattaaatgagttcataacacttaaaaagctgagcatagtgcatggctcatagcaaaagctgtgtaagtccagtcgtggatcacttaatgaaggagcattttctgtctttggcagtttcataattatgcgaataccattgagtataattacacaaacctagatggtatagactactatacactgaggctatattgtgtagcctattgatcctagctttaaacccgagcagcatgatactgttctgaatagtataaggaaatagtaacataatggtaaatatttgtgtgataggaattttcagcttgattataattttttttttttgagacagggtctcactcactggagtgcagtggtgcgatcttagctccctgcaacctccgcctcttgggctcgagcaatcctcctgctgtagtgcaccacgacactcggctaattcttttttaagatttttctgcagacaaggtctcacttactgcccaagctggtctcaaactcctgggcttaagtgatcctcccacctcggcctcccaaagcgttaggattacaggcgtgagtcactctgcctggccttgattataatcttatgggaccactgtggtctgtagttgacagaaatgtcgttaatgtggtgcatgactgttattattattttctgtcctgcccctgagagccactgtcacttctctgctgtattggtttttgtttactcatctgttttggccttgaaatggcctagacatttttcttcccgaagtatgacactcgggtgcttattaacttagtcaagacacaacatctcccttcccagaaggtgaggcgggagtgaggacttggggacttaagaactaccaaagttcagagtccaaagaaacattagaaattggctaatccacccccataacacgcacattttacagatgagaagactgagctcagagcatagaaatagcttgcccaggccatgactaagtcaggataaggagctggagcttgtttcctcactcagtggtcctgactttgcaccactctgcatttgcctagcctgccttcctctaactgtgctctccctacttccaggcctcacctgcagatgccccccagcctgggccagatgagcctgccctttgaccagcctcacccccagtgagtgacaaagcccctcctgaccccatgtgcctcttctttcctggccttgccccgctctccttatttccattgctggttcctggcaggggcctgctgccgtgccagcctcaggagcatgctgtgtccagccctgaccccctgctctgctcagatgtgaccatggtggaagacagctgcctgagccagccagtgacagcgtttcctcagggcacttggtgagtggcagcttgggagtggaggctgggtggcatctaggggagtgggcgccatgcctactccactgcttctcccatctccttgcaggattggtgaagacatattccctcctctgctgcctcccactgaacaggacctcactaagcttctcctggaggggcaaggggagtcggggggagggtccttgggggcacagcccctcctgcagccctcccactatgggcaatctgggatctcaatgtcccacatggacctaagggccaaccccagttggtgatcccagctggagggagaacccaaagagacagctcttctactacccccacagacctgctctggacacttgctcatgccctgccaagcagcagatggggagggtgccctcctatccccacctactcctgggtcaggaggaaaagactaacaggagaatgcacagtgggtggagccaatccactccttcctttctatcattcccctgcccacctccttccagcactgactggaagggaagttcaggctctgagacacaccccaacatgcctgcacctgcagcgcgcacacgcacgcacacacacatacagagctctctgagggtgatggggctgagcaggaggggggctgggtaagagcacaggttagggcatggaaggcttctccgcccattctgacccagggcctaggacggataggcaggaacatacagacacatttacactagaggccagggatagaggatattgggtctcagccctaggggaatgggaagcagctcaagggaccctgggtgggagcataggaggggtctggacatgtggttactagtacaggttttgccctgattaaaaaatctcccaaagccccaaattcctgttagccaggtggaggcttctgatacgtgtatgagactatgcaaaagtacaagggctgagattcttcgtgtatagctgtgtgaacgtgtatgtacctaggatatgttaaatgtatagctggcaccttagttgcatgaccacatagaacatgtgtctatctgcttttgcctacgtgacaacacaaatttgggagggtgagacactgcacagaagacagcagcaagtgtgctggcctctctgacatatgctaacccccaaatactctgaatttggagtctgactgtgcccaagtgggtccaagtggctgtgacatctacgtatggctccacacctccaatgctgcctgggagccagggtgagagtctgggtccaggcctggccatgtggccctccagtgtatgagagggccctgcctgctgcatcttttctgttgccccatccaccgccagcttcccttcactcccctatcccattctccctctcaaggcaggggtcatagatcctaagccataaaataaattttattccaaaataacaaaataaataatctactgtacacaatctgaaaagaaa

SEQ ID NO: 3 - protein, 847 aa, Artificial Sequence
  STAT6 Amino Acid
MSLWGLVSKMPPEKVQRLYVDFPQHLRHLLGDWLESQPWEFLVGSDAFCCNLASALLSDTVQHLQASVGEQGEGSTILQHISTLESIYQRDPLKLVATFRQILQGEKKAVMEQFRHLPMPFHWKQEELKFKTGLRRLQHRVGEIHLLREALQKGAEAGQVSLHSLIETPANGTGPSEALAMLLQETTGELEAAKALVLKRIQIWKRQQQLAGNGAPFEESLAPLQERCESLVDIYSQLQQEVGAAGGELEPKTRASLTGRLDEVLRTLVTSCFLVEKQPPQVLKTQTKFQAGVRFLLGLRFLGAPAKPPLVRADMVTEKQARELSVPQGPGAGAESTGEIINNTVPLENSIPGNCCSALFKNLLLKKIKRCERKGTESVTEEKCAVLFSASFTLGPGKLPIQLQALSLPLVVIVHGNQDNNAKATILWDNAFSEMDRVPFVVAERVPWEKMCETLNLKFMAEVGTNRGLLPEHFLFLAQKIFNDNSLSMEAFQHRSVSWSQFNKEILLGRGFTFWQWFDGVLDLTKRCLRSYWSDRLIIGFISKQYVTSLLLNEPDGTFLLRFSDSEIGGITIAHVIRGQDGSPQIENIQPFSAKDLSIRSLGDRIRDLAQLKNLYPKKPKDEAFRSHYKPEQMGKDGRGYVPATIKMTVERDQPLPTPELQMPTMVPSYDLGMAPDSSMSMQLGPDMVPQVYPPHSHSIPPYQGLSPEESVNVLSAFQEPHLQMPPSLGQMSLPFDQPHPQGLLPCQPQEHAVSSPDPLLCSDVTMVEDSCLSQPVTAFPQGTWIGEDIFPPLLPPTEQDLTKLLLEGQGESGGGSLGAQPLLQPSHYGQSGISMSHMDLRANPSW

SEQ ID NO: 4 - DNA, 3963 bp, Artificial Sequence
  STAT6 NM_003153.5
ggggcagccactgcttacactgaagagggaggacgggagaggagtgtgtgtgtgtgtgtgtgtgtgtgtgtgtatgtatgtgtgtgctttatcttatttttctttttggtggtggtggtggaaggggggaggtgctagcagggccagccttgaactcgctggacagagctacagacctatggggcctggaagtgcccgctgagaaagggagaagacagcagaggggttgccgaggcaacctccaagtcccagatcatgtctctgtggggtctggtctccaagatgcccccagaaaaagtgcagcggctctatgtcgactttccccaacacctgcggcatcttctgggtgactggctggagagccagccctgggagttcctggtcggctccgacgccttctgctgcaacttggctagtgccctactttcagacactgtccagcaccttcaggcctcggtgggagagcagggggaggggagcaccatcttgcaacacatcagcacccttgagagcatatatcagagggaccccctgaagctggtggccactttcagacaaatacttcaaggagagaaaaaagctgttatggaacagttccgccacttgccaatgcctttccactggaagcaggaagaactcaagtttaagacaggcttgcggaggctgcagcaccgagtaggggagatccaccttctccgagaagccctgcagaagggggctgaggctggccaagtgtctctgcacagcttgatagaaactcctgctaatgggactgggccaagtgaggccctggccatgctactgcaggagaccactggagagctagaggcagccaaagccctagtgctgaagaggatccagatttggaaacggcagcagcagctggcagggaatggcgcaccgtttgaggagagcctggccccactccaggagaggtgtgaaagcctggtggacatttattcccagctacagcaggaggtaggggcggctggtggggagcttgagcccaagacccgggcatcgctgactggccggctggatgaagtcctgagaaccctcgtcaccagttgcttcctggtggagaagcagcccccccaggtactgaagactcagaccaagttccaggctggagttcgattcctgttgggcttgaggttcctgggggccccagccaagcctccgctggtcagggccgacatggtgacagagaagcaggcgcgggagctgagtgtgcctcagggtcctggggctggagcagaaagcactggagaaatcatcaacaacactgtgcccttggagaacagcattcctgggaactgctgctctgccctgttcaagaacctgcttctcaagaagatcaagcggtgtgagcggaagggcactgagtctgtcacagaggagaagtgcgctgtgctcttctctgccagcttcacacttggccccggcaaactccccatccagctccaggccctgtctctgcccctggtggtcatcgtccatggcaaccaagacaacaatgccaaagccactatcctgtgggacaatgccttctctgagatggaccgcgtgccctttgtggtggctgagcgggtgccctgggagaagatgtgtgaaactctgaacctgaagttcatggctgaggtggggaccaaccgggggctgctcccagagcacttcctcttcctggcccagaagatcttcaatgacaacagcctcagtatggaggccttccagcaccgttctgtgtcctggtcgcagttcaacaaggagatcctgctgggccgtggcttcaccttttggcagtggtttgatggtgtcctggacctcaccaaacgctgtctccggagctactggtctgaccggctgatcattggcttcatcagcaaacagtacgttactagccttcttctcaatgagcccgacggaacctttctcctccgcttcagcgactcagagattgggggcatcaccattgcccatgtcatccggggccaggatggctctccacagatagagaacatccagccattctctgccaaagacctgtccattcgctcactgggggaccgaatccgggatcttgctcagctcaaaaatctctatcccaagaagcccaaggatgaggctttccggagccactacaagcctgaacagatgggtaaggatggcaggggttatgtcccagctaccatcaagatgaccgtggaaagggaccaaccacttcctaccccagagctccagatgcctaccatggtgccttcttatgaccttggaatggcccctgattcctccatgagcatgcagcttggcccagatatggtgccccaggtgtacccaccacactctcactccatccccccgtatcaaggcctctccccagaagaatcagtcaacgtgttgtcagccttccaggagcctcacctgcagatgccccccagcctgggccagatgagcctgccctttgaccagcctcacccccagggcctgctgccgtgccagcctcaggagcatgctgtgtccagccctgaccccctgctctgctcagatgtgaccatggtggaagacagctgcctgagccagccagtgacagcgtttcctcagggcacttggattggtgaagacatattccctcctctgctgcctcccactgaacaggacctcactaagcttctcctggaggggcaaggggagtcggggggagggtccttgggggcacagcccctcctgcagccctcccactatgggcaatctgggatctcaatgtcccacatggacctaagggccaaccccagttggtgatcccagctggagggagaacccaaagagacagctcttctactacccccacagacctgctctggacacttgctcatgccctgccaagcagcagatggggagggtgccctcctatccccacctactcctgggtcaggaggaaaagactaacaggagaatgcacagtgggtggagccaatccactccttcctttctatcattcccctgcccacctccttccagcactgactggaagggaagttcaggctctgagacacaccccaacatgcctgcacctgcagcgcgcacacgcacgcacacacacatacagagctctctgagggtgatggggctgagcaggaggggggctgggtaagagcacaggttagggcatggaaggcttctccgcccattctgacccagggcctaggacggataggcaggaacatacagacacatttacactagaggccagggatagaggatattgggtctcagccctaggggaatgggaagcagctcaagggaccctgggtgggagcataggaggggtctggacatgtggttactagtacaggttttgccctgattaaaaaatctcccaaagccccaaattcctgttagccaggtggaggcttctgatacgtgtatgagactatgcaaaagtacaagggctgagattcttcgtgtatagctgtgtgaacgtgtatgtacctaggatatgttaaatgtatagctggcaccttagttgcatgaccacatagaacatgtgtctatctgcttttgcctacgtgacaacacaaatttgggagggtgagacactgcacagaagacagcagcaagtgtgctggcctctctgacatatgctaacccccaaatactctgaatttggagtctgactgtgcccaagtgggtccaagtggctgtgacatctacgtatggctccacacctccaatgctgcctgggagccagggtgagagtctgggtccaggcctggccatgtggccctccagtgtatgagagggccctgcctgctgcatcttttctgttgccccatccaccgccagcttcccttcactcccctatcccattctccctctcaaggcaggggtcatagatcctaagccataaaataaattttattccaaaataacaaaataaataatctactgtacacaatctgaaaa

SEQ ID NO: 5 - protein, 673 aa, Artificial Sequence
  STAT6 Iso 2
MEQALAMLLQETTGELEAAKALVLKRIQIWKRQQQLAGNGAPFEESLAPLQERCESLVDIYSQLQQEVGAAGGELEPKTRASLTGRLDEVLRTLVTSCFLVEKQPPQVLKTQTKFQAGVRFLLGLRFLGAPAKPPLVRADMVTEKQARELSVPQGPGAGAESTGEIINNTVPLENSIPGNCCSALFKNLLLKKIKRCERKGTESVTEEKCAVLFSASFTLGPGKLPIQLQALSLPLVVIVHGNQDNNAKATILWDNAFSEMDRVPFVVAERVPWEKMCETLNLKFMAEVGTNRGLLPEHFLFLAQKIFNDNSLSMEAFQHRSVSWSQFNKEILLGRGFTFWQWFDGVLDLTKRCLRSYWSDRLIIGFISKQYVTSLLLNEPDGTFLLRFSDSEIGGITIAHVIRGQDGSPQIENIQPFSAKDLSIRSLGDRIRDLAQLKNLYPKKPKDEAFRSHYKPEQMGKDGRGYVPATIKMTVERDQPLPTPELQMPTMVPSYDLGMAPDSSMSMQLGPDMVPQVYPPHSHSIPPYQGLSPEESVNVLSAFQEPHLQMPPSLGQMSLPFDQPHPQGLLPCQPQEHAVSSPDPLLCSDVTMVEDSCLSQPVTAFPQGTWIGEDIFPPLLPPTEQDLTKLLLEGQGESGGGSLGAQPLLQPSHYGQSGISMSHMDLRANPSW

SEQ ID NO: 6 - protein, 737 aa, Artificial Sequence
  STAT6 Iso 3
MEQFRHLPMPFHWKQEELKFKTGLRRLQHRVGEIHLLREALQKGAEAGQVSLHSLIETPANGTGPSEALAMLLQETTGELEAAKALVLKRIQIWKRQQQLAGNGAPFEESLAPLQERCESLVDIYSQLQQEVGAAGGELEPKTRASLTGRLDEVLRTLVTSCFLVEKQPPQVLKTQTKFQAGVRFLLGLRFLGAPAKPPLVRADMVTEKQARELSVPQGPGAGAESTGEIINNTVPLENSIPGNCCSALFKNLLLKKIKRCERKGTESVTEEKCAVLFSASFTLGPGKLPIQLQALSLPLVVIVHGNQDNNAKATILWDNAFSEMDRVPFVVAERVPWEKMCETLNLKFMAEVGTNRGLLPEHFLFLAQKIFNDNSLSMEAFQHRSVSWSQFNKEILLGRGFTFWQWFDGVLDLTKRCLRSYWSDRLIIGFISKQYVTSLLLNEPDGTFLLRFSDSEIGGITIAHVIRGQDGSPQIENIQPFSAKDLSIRSLGDRIRDLAQLKNLYPKKPKDEAFRSHYKPEQMGKDGRGYVPATIKMTVERDQPLPTPELQMPTMVPSYDLGMAPDSSMSMQLGPDMVPQVYPPHSHSIPPYQGLSPEESVNVLSAFQEPHLQMPPSLGQMSLPFDQPHPQGLLPCQPQEHAVSSPDPLLCSDVTMVEDSCLSQPVTAFPQGTWIGEDIFPPLLPPTEQDLTKLLLEGQGESGGGSLGAQPLLQPSHYGQSGISMSHMDLRANPSW

SEQ ID NO: 7 - DNA, 32730 bp, Artificial Sequence
  KRAS G12D genomic sequence
gattttcctaggcggcggccgcggcggcggaggcagcagcggcggcggcagtggcggcggcgaaggtggcggcggctcggccagtactcccggcccccgccatttcggactgggagcgagcgcggcgcaggcactgaaggcggcggcggggccagaggctcagcggctcccaggtgcgggagagaggtacggagcggaccacccctcctgggcccctgcccgggtcccgaccctctttgccggcgccgggcggggccggcggcgagtgaatgaattaggggtccccggaggggcgggtggggggcgcgggcgcggggtcggggcgggctgggtgagaggggtctgcaggggggaggcgcgcggacgcggcggcgcggggagtgaggaatgggcggtgcggggctgaggagggtgaggctggaggcggtcgccgctggtgctgcttcctggacggggaaccccttccttcctcctccccgagagccgcggctggaggcttctggggagaaactcgggccgggccggctgcccctcggagcggtggggtgcggtggaggttactcccgcggcgccccggcctcccctccccctctccccgctcccgcacctcttgcctccctttccagcactcggctgcctcggtccagccttccctgctgcatttggcatctctaggacgaaggtataaacttctccctcgagcgcaggctggacggatagtggtccttttccgtgtgtaggggatgtgtgagtaagaggggaggtcacgttttggaagagcataggaaagtgcttagagaccactgtttgaggttattgtgtttggaaaaaaatgcatctgcctccgagttcctgaatgctcccctcccccatgtatgggctgtgacattgctgtggccacaaaggaggaggtggaggtagagatggtggaagaacaggtggccaacaccctacacgtagagcctgtgacctacagtgaaaaggaaaaagttaatcccagatggtctgttttgcttggtcaagttaaacccgaagaaaacccgcagagcagaagcaaggctttttccttgctagttgagtgtagacagcaatagcaaaaatagtacttgaagtttaatttacctgttcttgtcctttcccctatttcttatgtattaccctcatcccctcgtctcttttatactaccctcattttgcagatgtgttctacatctcaagagttattacagtactccaaaacagcacttacatgattttttaaacttacagaggaattgtagcaatccaccagctaaccgcctgaaatagacttaaacatgtgcatctcctttttttttttttttttgagacacagtctcgctctgttgcccaggctggagtgcaatggcgcggtatcggctcactgaaacctccgcctcctgggttcaagcaattctcctgcctcagcctcccgagtagctgggactagtaggtgcacgccaccatgcccagctaatttttgtatttttagtagagacagagtttcatcatgttggtcaggatggtctccatctgctctgttgcccaggctggagtgcagtggcgccgtctcggctcactgcaacctctgcctcctgcattcaagcaattctcctgcctcagcctcccgaataactgggattacaggtgtctgctgccatgcccggctaattttttgtatttttagtagagacgggggtttcaccatgttggtcaggctggtctagaactcctgacctcgtgatctgcccgcctcggcctcccacagtggcatgtgcatcttatagctgaagtctaagccttcttaaatcttgagatccatcaaaacagacaggttttctaattgttatacaatgtatatgttatgtttataatagaaatcattttacaaataagttataaatgggaaaggtctatttgtaattatcagctcagaattaaccataaaactggtgtcactgaagtgactgaggtccaaaatgctgactctgcatgttatagactacagatatcaaatatggttgctaacaatagtttactttgagactgtagccatccacagtatatttgcttttaagagatggtagatggtaattcagttttatgaaaaataaaaatgaattttcttccattacaaaattgttggattcgagtccagtccactccttactagcttttctaactctcggtgagggatcccctcccagcccatgatcttcatttggtaagactcctttggaacccagttctctctagtggatttaaatgtgatttggttttaaaaatctcattcaaggaattttttttttttctggaaacaaccaccgcataaacaagtaaaccggaagatacatgtggctctgaattcatatatatacacaaactctaatccaatgtctgtccacagtatttcctaggctagtaaactttttggccttaacgacccctctaccctctttgtttttttgagagagagagtctcactctgtcacccaggccggaatgcagtggcgcgatctcggcccgctactacctccgactctcaggctcaagcgattctcccgcctcagcttcccgagtagccgggattacaggctcccgccaccgggctaattgtatttttagatacgggatttcaccatgttggccaggctggtctcgacctcctgacctcaggtgatccgcccgcctaagcctcccaaagtgctgggattacaggccaccacacccggcctacactcttaaaaattatcgaaggggccgggcacattggctcttatctgtaatcccagcactttgggagactgaggcgggaggatcgcttgaggccaggagttggagaccagcgtactcaacatagtgagaccttgttataaagaaaaaaaaaatccaggattaaaaaaaatctttgatttgtttgggatttattaatatttaccgtattggaaattaaaacaattttttaaaatgtattcatttaaaaataataagcccattacttggtaacatgaataaaatattttatgaaaaataactattttccaaaacaaaaccaaaacttagaaaagtggtattgtttcacacttcagtaaatctctttaatgatgtggcttaatagaagatatggattcttatatctgcatctgcattcaatctattatgatcacacatctggaaaacttgtgaaagaatgggagttaaaagggtaaaggacatcttaatgttattatgaaaacagttttgacctcttgcacaccagaaaagtcttagtaacctgaggggttcctagaccacattttgagaactgttttaggctatgcaaactggttggggggaggttggggtaggcagagagctagaagatacattttagtgtaattctcctcatctattcctaattgctttggcctacatttgaaataaagcgtggaggcaaacgggataagatacatgtttgtagtggttgttaacttcaccctagacaagcagccaataagtctaggtagagcagagtaaggcggggaactatgccgtgaccgtgtgtgatacaatttttctagcctgtggtgctttttgcggcagggcttaggagtaaggttagtatgttatcatttgggaaaccaaattattattttgggtcttcagtcaattatgatgctgtgtatatttagtgtttatctacaatatatgcacattcattaatttggagctactcatcctataataaatagttgtgcatttactcccatttttttctgcatttctctccttatttataattatgtgttacatgagggaaaggaggtgaaattaaacattcatattatttcaaaaaatttgaaacaactaactaaaaaatatgttttattttctgtatggtgtttgttatacaatctgtcaatattcatgcacctcttgggagacagtgtatgaaaagcaaagagtaacagtcacatggattactgattactgagatatattcacttgcatctttttttttttttgagacggagtggctctgtcgcccaggctggagtgcagtggcgtgatctcggctcactgcaagctccgcctcctgggttcacgccattcttctgcctcagcctcccaagtagctgggactacaggcgcccgccaccacgcccggctaatttttttatatttttagtagagacggggtttcaccgggttagccaggatggtcttgatctcctgacctcgtgatccaccctcctcggcctcccaaagtgctaggattataggcgtgagccaccgtgcccggctcacttgcatctcttaacagctgttttcttactaaaaacagtgtttatctctaatctttttgtttgtttgtttgttttgagatggagtcttactccgtcacccaatctggagtgcagtggcgtgatctgggctcactgcaacctctgcctcccgggttcaagtgattctccttcctcagcctccccagtagctaggactacaggagagcgccaccacgcctgattaatttttgtatttttagtagagagagggtttcaccatattggccaggctggtcttgaactcctggcctcaggtgatccacccgccttggcctctgaaagtgctgggattacaggcatgagccgccgcacccggctttctaatctttatctttttttgtgcagcggtgatacaggattatgtattgtactgaacagttaattcggagttctcttggtttttagctttattttccccagagatttttttttttttttttttttttgagacggagtcttgctctatcgccaggctggagtgcagtggcgccatctcggctcattgcaacctcggactcctattttccccagagatatttcacacattaaaatgtcgtcaaatattgttcttctttgcctcagtgtttaaatttttatttccccatgacacaatccagctttatttgacactcattctctcaactctcatctgattcttactgttaatatttatccaagagaactactgccatgatgctttaaaagtttttctgtagctgttgcatattgacttctaacacttagaggtgggggtccactaggaaaactgtaacaataagagtggagatagctgtcagcaacttttgtgagggtgtgctacagggtgtagagcactgtgaagtctctacatgagtgaagtcatgatatgatcctttgagagcctttagccgccgcagaacagcagtctggctatttagatagaacaacttgattttaagataaaagaactgtctatgtagcatttatgcatttttcttaagcgtcgatggaggagtttgtaaatgaagtacagttcattacgatacacgtctgcagtcaactggaattttcatgattgaattttgtaaggtattttgaaataatttttcatataaaggtgagtttgtattaaaaggtactggtggagtatttgatagtgtattaaccttatgtgtgacatgttctaatatagtcacattttcattatttttattataaggcctgctgaaaatgactgaatataaacttgtggtagttggagctgatggcgtaggcaagagtgccttgacgatacagctaattcagaatcattttgtggacgaatatgatccaacaatagaggtaaatcttgttttaatatgcatattactggtgcaggaccattctttgatacagataaaggtttctctgaccattttcatgagtacttattacaagataattatgctgaaagttaagttatctgaaatgtaccttgggtttcaagttatatgtaaccattaatatgggaactttactttccttgggagtatgtcagggtccatgatgttcactctctgtgcattttgattggaagtgtatttcagagtttcgtgagagggtagaaatttgtatcctatctggacctaaaagacaatctttttattgtaacttttatttttatgggtttcttggtattgtgacatcatatgtaaaggttagatttaattgtactagtgaaatataattgtttgatggttgatttttttaaacttcatcagcagtattttcctatcttcttctcaacattagagaacctacaactaccggataaattttacaaaatgaattatttgcctaaggtgtggtttatataaaggtactattaccaactttacctttgctttgttgtcatttttaaatttactcaaggaaatactaggatttaaaaaaaaattccttgagtaaatttaaattgttatcatgtttttgaggattattttcagatttttttagtttaatgaaaatttaccaaagtaaagaccagcagcagaatgataagtaaagacctgtaagacaccttgaaggtcatggagtagaacttccatcccaagcagatgaggatttatttaatctcaaagacctccaggaggggacattccccaactgtccttgttaactcattttcagaacatatttattagcatattttacatgtaatttggatcttcatgttaaatttaacatcagtggagatggaaaataagcatatcgccttgtctttgaaatagccctatattgttagattgtttcttaggcttctttaccctgggttaagcagtcctaatactttagcatttattctacatctagtgtactaatttaaaaaaatcagttctgaaaaatttctaagaactttcttcaagttccaagctgtgaaatctagaacaggtcaaagtgccttattaacgtactgtactgtgtagtgtcttgaagagacactttgcgctgaggcaagttctgagggcattgggtggccttgggaagatatttatgcagtttagaacctggagaattgattagataactaatcataaggaaacgtcacatatttttggtactataaaaaagtggagaaataatgcctatttgcaaagatttgatttaaacatagaaacaactttatttggcttccaattttaagaatttacagcagtaaaggggaacagtctaattgaagtagactgcctatgcaatagtctctgtatatttacttttgacaagttaattcaatgtgtactatagttttgtttctttgaagaggtttgaatagtgcacccattttaatctgtattgcaaattcagggttacttggcagactctactatttaaatcagatgtaaaaggaagttttaatataattcactttatgcctgaaagttttcctgggattttggaaggtgattttactggaaatgctgtctgtcttccctgaaaatctgagaaattccattacactttgtttccaatcagaggtcatgagtgctatatgagtatatacagcatgacgtcatgaatgtgataaagtgggttaggaaaccttttgctaatgattgttaaaatgcaatataaatgttgaagaaataaagctaacagttaagcctttatttgggcggaaggctgaaaaagtttataaacttaaacctataactctgcttatgatttctgccaaaccagaagacttgactctgggaagcattggttacctgtgaactttgaaactgacggtccctgacgtagtttagtcacctgggaaaaggtatctgagattatctcttatctcccaagttacagtgagtctctgagggaactgacacattacattaagttcttggtgtagttaaactgtaagaaaggcaggagaacttagtagttaaatagttggttaaatggaaatgctgactccatgttattgtaaaaagttaaaaatttaggaggatatggggatttcactgccattgcaggttttgattggtatttaccaatccgtgtgggtcagagagaaaattagaaaggatatgactgcacattttggaattattagcagtttttctacatttaaaatggaaataaattttttaaaaatttaaatcaagtaatactgtattttttggtgatttagatttttcaaaatttacactaagagatagtaaggagggtggctattgtttctttcaataatgtctctgagaggttgtaactcatctaaggatacgtagctaataagtggtaggatttcaatttaaattctctgagaccaagttaagtagaatttgcactgtactcttgtataactttttaaaactgaaaattagctatctttcaaattaagaaaatatttactaatggagactaattcagatttgtaagtataccaaaatttgaacttagcctgctatctaatggcaacttagtggcagaggtatgatgtaaaatcattcaggtatgacacatagatggagtatgtttgtattcgaggctgtgcacataatcacctttacttgtattgtgaagtatatattgttatcttttatgaagcccactaaagagataatgaaatacctcgttattagggcaagattattgaaaactcaaaatagcccccaaacacaatacttggctagaaatatatacctttatagttcagagatcatttattatcaaaaccctgaagttttttttctaaggtaaaatttggtggaagaggaaaagtctcgttttaaaaaaatgtaggtagttacagagatcagaatgattagttgatcacttaccaaatatatattaagtatctactgtatataatatgctagtaagaataaatatagcaggaagtattttttcccaggctctaattgtttgacatcagcatgcttttattgtggcacttataattcagttcaagtattatgcccctctttgatggaacagtttcctattcagtaaggaagaccagattaatcattggattggtttgtttcatctttagtgttctgagctgtagagtatttatttaccaaggtttattttaatttttattttatttttatttttccatgttcattgtagaattcattttacctacgaatgaagtatgtagattatagagagaaaatttgtaaaattaaactgatactgaagactggtataagaaaagccttatgtaatttgtaagctgctattcttctgagtttatacatatatctttagtaatcaatgagggatggttgggtgactgccctccaggggacatttggcaacatctggagatgtttttggttgccacaacttggggagagagtactgctactggcatctattgagtagatgctattactttaaatggcaaagctgcagttacctttgcaccaacctaatattaaacttcctgcagtgcacgggaaagcccccacaacagggttatctgaccccaaacctcaatggtgttaagatccaaaccttgatatgttaacctgtagctttaaacatcctttaaattgtcaaattcatgtccctgacataaggtttatgttagattttcaagtataacaaagatttaaactttaacttttgtacgttaatgatatgttagcttactccagtcttctattaaaacattctgtttttaaaatcagagacacacagcaattttataaatcatttctcttcaaggctgtgaagctctccccacttttgtgagtgccctctactggtcaaattatttgctttataacaagtaacagtgaaatcctaagtttgtgtagtttcgctgtttaaattatgggtggcatcaatttataaatatattcgttttatttaaaagtcttatatgattgatttcgtatcatttttgctctctgctaatattaatataaagattactgtctgtattagttaggcctaactaagtaggtgagtatagtgaactaagaaaggaaacgaggcagtatataagaaaatagggtggttcagttgttaacacttactgagcttactttgttgaagggactaaaaggcagcagtgtggctctctgagcttctttgcatgcactcaggagctgcttaatggagtccaaggcttggtggtgtgttacaggggatgataggagggtcctattcagaagtggcaaattgtgaaagtgcacattttgtagagttttataggactgtagaatagttgtgagcacctgatttttagaataaacagaaaactcaggtactgtatttaggtcaaattaagaataagtatttattaagacctgaatataaaactttactggtcatggtttttttctaccttgggtttttataaatccaaagatttaaaaacatacaaatggaagttggtaatggaattaagtgaaaggaaaaaatgattttatggtttggaatctcctaagattctggttttaacaatacaactaattccttaatcctagaaatgttcttcactgcccactttgtaccatgcagtcttcctgtgggctagagatacactgaggcgcaaaacagaccagattcctgccttcatggagcttattagttttaggtatctctagatttcttgtaatacctattacaatgcctgcacatcagttcattcatgtgggttcaacgtagtactcagtacatggcaaattcaagttttacttttcggaacttcatggatttttttcctcagaatatcttttatccataattggttgaatctgtagatgcagtacccatggatatggatggcccactttattttgaagagcagtgtttctaggcaatcatgctaattatatatgacttaatttagaggctttatacttaagagcattacatttctggcgtctcttaaccattattatttcataatgtgtaggttatggaacagttaaattattgggatcttaatatagaaattagtagaaataagccagatatggtggctcatgcctgtaatcttagcactttgggaggctgaggctattcgctgtactattttttactacttttctataggtttgaaattttttcaaaataaaacattgaaaaaagtaaggtaggtagtgtgtccctccttaatcctttcaaatattttattttcactatttctattaatttttttttttgtttttgagatggagtctcgctctgttgcccaggctggagtgcagtggcgcgatcttggctcactgcagcctccacctcctgggttccagccattctcctgcctcagcctcctgggtagctggtattacaggcatgcaccaccacacccaattactttttgtatttttagtagagacggggtttcaccatgttggccaggctagtctcgaactcctgacctcgtgatctgcccgcctcagcagtgtcactgcttctagaccgttttcaaggcacagagcttagaaatgcatgttactaagaaatcaagagttaactatttttcaccttctttctcccgcagtgagaaccctggttctaccctgtttctccttgtgtaaattttaatgctaaactatacacttgtgaaataaaaatgataatgtcattcttaaattatggatcttgcagtgttatctaagtaacatagattgagtgatttaactttaggtttccttatttgtggaatttggataaatatttttcacccttgagaaaagtgagactcctttctcatcatcagagtatccttaaaccattaaggcaaacatttgggaaaaaactgagctatctggctgcataaaaattaagttttctttaacaaagatagaagacaaatgaaaacctagaaaaaccatttggttcaagtaacaggaagctatcttatatatgaattagagaaaagcaaacacacaaatagaaaaaaagggatggggggtactaaagatataaatagcttgtctaccaaaaaagaaataaaataaataacatgaacatataaaaagacacttacttcatgaatgtgatgcaagttcaaacaataaataacatttctgtactttcatattggctaaggttaaaatgataactgctaggaagggtatggagaagtgtgcgccttgcactgtagtgggagtatagaccctcagactttatggaggtcagtctggaaatatgtttcaaaatgtaaactacatgtcctttgaccaggtaattcaacttcttgaaatttatccaaggatttaattggataaatgtttaagatgtatatataagaatgtttactgcagtgttgtttatgattttaaaaaaatggaaatcatcttcatgtctaccaatagagaatgggtgaataaattatggtatgtccatatatacaaattacatagttgttggaaatattaggtagatttagatatactgatgttcaaaaatgtccattatgtaagtgaagctgggtcacagcaccttgtgttgagtatgatttcatctagaaacaaaattactccctcatcctttgttgtgttttagttttttaaaataagcttataccattgggctgggggaaaagtaaatactcgttttggagagagaaaagggcactaaagtttcagataccgttagattatttcatgcttatttttcaagcctcaataaattacataattcacatgtagtcttggattaaggaaattgctattaaggctaaataaataatatgagaggtatataatataaaatatgaacattatattggcattaagattggatccacggtcattccagcctctcattcttacctggacttcaagtgatcacttgtgggcaaatgccatctgacttgaacaggttacacatgtatgctcattatatcgttattttcaaaatttgtcatataaattttccttgagttcattcagatttttgaactagttttttctcttgggagtagtacacacttaattctctctagtactaagctaatgttcaccattcttataattttaagtatccagcatttagtaaagaagtctttgttttctttatccttacttttagtgaatgtcttagtttttaattgaaaattctgccatgaaaataagctctttaacatcttcactccctaatcaaaacagaaatccttcatagccttcagttgtagctatccttccctgtgatttgtccagctccattatatttattttgaaatatggtgaccagttttgcaaaattatttcaactgtaggtgcccagtgattttgtaaggagaagatactgtttctgaacagttctcagtagccagtggcctgcccctactttttggcctgcgtgtagtatataaaataatgcagttaactttttatagcacttttcattttataaagagattttcatggtctttaatattaatctatgtataaagtcctgtatgcagttttacctactttcacagctgaaggaacaatagcttagagaagatgtgagataaagtagtttgcccaagcccatagcacaaataagtgaagttcttcggctgtccatggatcgaagactcccaagtctatctctagcctggacttctgtcctgagcaccagacatgtatgtatatcaagatgcctgcaggtcatatccaccaggacaacccatgagtacagggaattcaacatgcccaatatcactcatcttttccttcgccctcccctttgtactcatcccctgtcggtaagctctgttattttaaaaaattgaaatgtattcacatagcatacaatttacacttttcaagtgtacatggtttttagtatattcacaagggttgtgcagtcattactactaattccagaatgttattatcaccccaaaagtcccacatccattagcagccactccccaatcccttctcccaccagcctctaaaaactgctaatttttccatctctgtggatttgtccactctgattatttcatataaagagaatcgtacagacgtggccttttgtgtctggcatcctccacacaggatgatattttcagagttcgtctatgtttttgcttgttgatcattccttcattcctttttctggctgaataatactctgttatatggatataccttattttgtttatctgttcatttgatgggcatttgagtgatttcctctttttggcaattttgaataatgccactataaacatttatgtacacgtttttgtgtgaccatatgttttcacttctctcgggtgtatatctaaggtacagttgctgggttatatggtagctctgtctttgactttttgaggaactgccaagtggttttggtagtgattgtactgtttacattcctaccaacaattttacctaagtatttctcaaatctatttaatcttttcggtccatactgctgttgctgccttagttcagattttgtcatttcttgtaataattcgtagctcatctcccagtctctgctcccctctctccctccctcccccttcttctctctcttatttccacccatttttaacatttatagaagtcaaaagtctagttcagaaagcagaaaccatactagatatttcagcacagagaactaattaggtgttggaagactgaaaggcaaaaaaacactgaagtaacacagtaacatcaagaatgggcactactcctaagattcagggaatgctgggaagatttggggtttatcagaactggaagctcagaggaggggccccttgtcgctgaggcttaatccctgcagaggtgcctttggctgctactggtgaatctgagtgggtatgatgagtcagtgtctgggaagggccaaaacattttgtccctttctataatttgtcatgataatgctagtaatgaatctgatctcccttcctattttaaaaaccttttagtgattttgtataggatgaagtttaaaactccttacttaatatacacatgaccctccgtaagctggcccctgcttgattgtccagtttcacttcttggtgcttattctaaggcctctaagccttagagatcctctaagcctttgagatccccaaaccctggactgcggactggtacccacctgtgtggcctgtgaggaactgggctgcacagccggaaggaggtgagcattacttgccttagctcctgtcagatcggcagcattagattctaataggagcgtgaaccgtgttgtgaactgcccatgcaaggatctaggttgcatactccttaggagaatctaactaatgcttgatggtctgaggtgaaacagtttcatcctgaaatcacccccaactcggtccttggaaaaattgtcttccacgaaactggtccctgatgccggaaaagttggggaccgctgttctaagctaaagttatatggagctccttggttctgtgtcctcaacatgctgttctatgttttttacattctgtttgctccttcctgcttggaatgtccttcccctccccgtctttcttaatgcatacaaagttgatctctcctgtgtgccaccattgtacttcgtcttgcatatggtgttacattcattttattttaattatttatttacgttcatgtctcttccactcaccttagttgcttgaggtcagaaactatataatgtgtgacacggaatgtgacacctagattttcaataagtgtttctatgatacaagggagactgatgtgggtagatgggaatgaactcatcaacctctgtttacataccctaaattccctgtttcttccctattataattctgacagtctacaaccgtctttgatggcttataaacggaaagtgcggaacacatcattctacagtgaatttaaataacctttcggaagagtaacgtaaagtacttgagcattaattgagtaaaagtttctcatcttttcctacaggtgttattaagcagtatgtaaaaagtccttacaatacttaatacattaagaaaacatacaatttcaagaggaaatccccgagtaatacattattgacattttcagcagttctagttatattgagaagagcatctcatggaattggcagaatgaagatggagattaaatgagatgatgtttgtaatatgcttatgacagtatctggcatataagtaagggctcagtaaatgttgactgctgtaattactattaatagtaatatgattacctttagtaaaagttattagtttctttaggttttttgtttactacaatatagtaaacaaaatctatacttggaatgtatatattgttttgttttgatacatggaatatgtctctgtgtcagagtcactgcctgagttggaaaacccatactcgagtatgttaaaaggtgaacacactgaataatttagttattaattataatggaaaaatgacaaacttgatgttctggttaatgaggttatcttatcttgaatgagttagcttttaaattcctcaaaataaaggcatttaataaaccaggaaacacttcattaaaaaaattatgcaagtcagtgtaaaagaagattaaaattccacatgggcaaaggacacacgttggcgataaatatgcagataagaaaaaaaacctatataacattattactcctcaaagaaattggtatgaaaacaataaaaatgtgtagcttatcaaaccaacaaaaatttaaaaatatgaaatccattttaagtaatgataaaatgggtgcactcttagtgctttatagaatagtagtataatgaacctcatgtgtgtaccaaccagctctttcatatcttaacatttagcaacatttgatttagctctttcttttttccaagatagaaaagttaatattgttgaagactcctgcattcttttccctagtcttattttcttccctcccataaatgtgttaaaatctctgtgtgtattgttttggttgtatttttacataaaactttacatattatataaaatttaattgaaggtaaaatttattaaattattcttaatatatattgtaatttaaaaattaacagcttcattgtcttgataaaatttatggtatcttaaacatgtgcttgtttttctaagagaacattgaaacatagattttaaaacaaattgttgaaagattaaaaaatctgcctttgcacactgttacattgaaagtggggcatttgtcgtgaacattcatttcaaatatgtagtatcttcagaatatttgagaaggatttgtattatataattgaaaaatctgttaaattgtatttatgttaactgcttaattctaataaaatttccattcattttttagtatctgcatatatttacatcaaatggattcattcacttatttaagaggcagtactaattacctatagcgttcaagactgttaggtagagggtgtgtagtggtgagtacaacaggcgtgagccctaccaacacggagtttaaagcctagtagaggatatagacttaaacaatttcacaagtaaatacataattacaaattataatacatgctatgaaggaaacataggaggtaccagagaaggaagagtgctttgcatttttatttttaagaccgaagagtgctattggaggactttgagcaagtgaatgacatgatctaacctaccttcgttcattcattcattcattcattttcttccttcctggctcaagcagtcctcccacctgagctccccaaatagctgggactacaggtacacactaccacacctaatttttttttgtattttttgtatttttgatgggattttaccatgttggccaggctggtcttgaactcttgacctcaggtgatccacctgtctcggcctcccaaggtgttgggattataggtgcctagcccatggtgcctagccctaacctacatttataaactatcacttgctgctgtgtggagactatattgtgagattaacagcagggatacctgctaggaagcaattgctgcagattgcctgagacaaaatagttatcatggactagggggatggtggtggtggtggtggtaggtggttggatgtaggatatattttgaagataggtaaatggtgcaagattatgggtcagttttaaatgcttaagtaaattttctttgtaagacattttaggatgccatgttaagaatctctttataactgtcatttaaaaaaaaaccacatattttcttagcataatttcccatagtaacattactatgtcaaaggctatgaacatttgaatgactttagataaatactgtaattgctttccaaaaatattgtgcttattatgtcaccagaaatgtttgaattctgtctacaattcagtcttgccagtatagtacatttcatttagaaaaattttttactatgtagatggaaaaaataatattttagctgggagtggggggactatggggaataactttccttcatttaatattttattgtgagttagtttaagttactttattttatcgtagtttcctaaggctacaaattagtaaccttggtaacttatgtacctaatttaaaagtttacttttttgaaaggctggaaatactaattaaaaacgtaacaccttcatccttgtctttgctccattattaactagtttcattacagaatctctgtgttttaaaatcagatgggttttcataaccagtactttctcagagtggtaaatttaaaaaaatatataaagagaataaataatatttgttgagaatacttcaaataatgtgaagagttattaacttacagcaggagttggcaaacttttctataaagggccatatgggtctttgtcacaaagtcttgggtttttgtttttgtttttttaaacagctatttaactattcctagctaatgggcaatacaaaaacagtgggcaagatttggcctgtgggcagtagcttgctgaaaccttatttagactctaaattttttgaaagagtctacattgatgcatatttttttttcttcctccaaatacagttgacccttgaacaacatgcgtttgagtgaccatgggtccacttgtgatacacgtttttttcccaaccaaatgcagatatggagggctgacttttcatatacctggatgttcctgggccaactgtaggactagaggctgggggggtcttggaaccaatgccgtgtgtataccagggatgactgtttcttatggcctgacctgaagttggaacagaatctttattaatatataatttttgttgcgtttgttttctctttatatttatccattctttttagatcgtatttcatttaacactttttcttctttagtttttaccaagttgcactgaaaatagctcagtgactaattgcacttctaagagtgaggaccctagttaaaattaactctaaaaatactgaatttttaacctaaaccttttatttctaatcaacagtattatttatgagtaggttatagattactttgaaacggaatgtgtctcagaactttgctatcgatatttttaaggtctggtagggaaaagataataggaatgagatttatcagtgaataggggactgctttcccagtttctcggtcgcactggtgtattcaccatggaagcatcttatgaaatatgtacataaactactaatatcccacattacaggttgactattctttatctgaaatgcttaggacctagaagtatttttggattttggtttttcagagtagggatactcagcctacattggtaagtaaagaatgtgaggtgacaggctgggcgcgatggttgacgcctgtaatcccagcactttgggaggccgaggcggatcacctgaggtcaggagttgaagaccagcctggccaatctgtactaaaaatacaaaaattagctggacacagtggcacgtgccagtagtcccagctactcaggaggctgaggtaggagaatcgcttgaacctgggaggcggaggttgcagtgactcgagatcgtgtcactgccctccagcctaggcaacagagcaagactccatctcaaaaaaaaaaaaaaaaaaaaaaaaaaagaatgtgaggtggcagcaataggtaggaagagtctttggtcagctttacatgctctgtagccatgcctgggtaatgggttgactctaagactctgtgctttgctcccacctcctgctttttcattactctttagaatggtttttaatttgtgatctataggagttctttcaagtatttaataagagaataggctaaattaagtaaatgtcaactgaatgctcaaatctctactaaagagcctcttatttagaaaataaatatccatcttttttttctgactggtgagataattaatttttattacagatggtttggaaaataccatatgctttaaaagataagcacaaaattatagtctaatatgtaggttttcatactttaaaaaattgaaaaccaaagaaaaacatttaacatagcatctagtacaaagaaaagagataagcaagagataaatgtcttttttgggacagagttttgctgttgttgcccaggctggagtgcaatggcacaatctcagctcaccgtaacctccacctcccgggttcaagtgattctcctgcctcagcctcccgagtagctgggattacagtcatgcaccaccaggcccaggtaattttgtatgtttagtagagatggggtttctccgtgttggtcaggctgatctcaaactcccgacctcaggtgatctgcccaccttggcctcccaaagtgctgggattacagacatgagccatcgcacccggccaagataaatgtcttttaaattatctccattaaagacataacctttataacattttgatgtatatattaccagtttttaaacacatagtagatttgtataaatacataaacacatattattgtgatcatgctgcacttagacatctttatattctccttatactgtaaacattttgaaatactttactaacaacatttgtaatgaccattctttctctctttctccctctgatagaatggtctacagagtaattcataaactaaacatactttagaggctgggcgcagtggctcatgcctgtaatcccagcactttgagaggctgaggcgtgcagatcacgaggtcaggagttagagaccagcctgactaacatggtgaaaccccatctctactaaaaaaacagtacaaaaattagccgggcgtggtggcgtgcacctagaatcccagctactcaagaggctgaggcaggagaatcactcgagcccaggaggcagaggttgtagtgagccgagattgcaccacagcactccagcctgggcgacagagcgagactccatctcaaaaaaaaaaaaaaaagatacattaatactatagcctacatgtggaacattaagaaaataattgcttttatgtttatgctttatacctgttgttagccctgcttcttatttcatgatttcatggcttcacattgtaacatccctttaccatattttttgaggactgttttggcagaatgtgtgaaatcttgagcagaagtattacccaaaagtcagaagaaaatcagatttttatttcaagattctgttaaagttacccactcccttcttttacttaatcttatagttgcagttctctctctttttagaaaagaaaaaagaggcccctcaggatttgcagatgaaacaatattgctctttagagatatccatctggctgttagattatttttccacagttttcagaagtggatgaggccattagaatcttgagtattgcccatttccttatgtgtgcctttgactatagataaaatagatgcatgacaattatttataagttgattgatttttcttgtcatttaaatcatcttgaataatagagttggtagagctatcccatttttgaaattattttgttttgtcaataactttttgttaccagcatgtacacttgcattgttgactctccatataatacctttaaaaaatttttttttgtggtaaaatatgcataacataaagtttaccatggtagttttctttcatttgttttgtttttgtttttttgagacggagccttgctctgttgccaggctggagtgcagtggagcgatcttggctcactgcaacctccgcctcccgggttcaagcaattcccctgcctcagcctcctgagtagctgggactacaggcgcccgccaccacgcccggctaatattttgtattttaatagagatggggtttcaccatgttggccaggatgttcttgatctcctgacctcatgatccgcccacctcggcctcccaaagtgttgggattgcaagtgtgagccaccgcgcctagaccatggtagttaattttaagtgttcaattcagtgaccttaagtgtgttcataatgttgtgcaaccatcaccatgttgtctaaccattagcactatctgttttgagaacttttttttatcatcccaaattagaattctgtacctgtcaaatagtccccagtaatcctccctcccccagcccctggtaatctgtagtctacttttcgtctttttgaatttgcctattttaggttcctcatataagtggaattatgtggtatttgtccttttgtgttggcttacttcatttagcataatgttttcaaggttcatctgtgttgtagcatgtatatacaggttgaagcatccgttatccaaaatggttgtgaccagaagtggtttggatttcagattttttttttggattttggaatattcatagatacttaactggttcagcatccctcgtccaaaaatccaaaatcagatggagctcagtggctcatgcttgtaatcccaacacgttgggtggccaaggcaggaggatcgcttgagcccaggagttcaaccagcctgagcaacacaagaccctatctctccaaaaaaaaaaaaaaaaaaaaaaagatgaaagaaaaaaaaatccaaaatcaaatgctccagtgagcatttccttttagcatcatgtcaggctctaaaagttacaggttttggagcattttggatttcagatttttggattaacctgcattaatgctcaacctatatgaaattttattcctttttatggctgaataatgttccactgtatgtatatactacattttgtttatccattcatctgttaacagacacttaagttatttccacattttgggtattataaatagtgctgctgcgaacattggtgtacatgtatctgtttgagtccctgtttttagttattttggttatatacctaggaatggaattgctgatcatatggtaattctgtgtttaactttttgaggaactaccactgttttccacaatggcatcaccattttacattcccaccagcaatgcacaaagatttcagtgtctgtatccttgctaacacttattttccattttttgagtttttttgttttgtttttttaataatagccaatcctaatgggtatgtggtagcatctcatggttttgattttattttcctgactattgatgatgttgagcatcttttcaggtgcttagtggccatttgtccgtcatctttggagcaggaacaatgtcttttcaagtcctttgcccatttttaaattgaattttttgttgttgagttgtatataacaccttttttgaagtaaaaggtgcactgtaataatccagactgtgtttctcccttctcaggattcctacaggaagcaagtagtaattgatggagaaacctgtctcttggatattctcgacacagcaggtcaagaggagtacagtgcaatgagggaccagtacatgaggactggggagggctttctttgtgtatttgccataaataatactaaatcatttgaagatattcaccattataggtgggtttaaattgaatataataagctgacattaaggagtaattatagtttttattttttgagtctttgctaatgccatgcatataatatttaataaaaatttttaaataatgtttatgaggtaggtaatatccctgttttataaatgaagttcttgggggattagagcagtggagtaacttgctccagactgcatcggtagtggtggtgctgggattgaaacctaggcctgtttgactccacagccttctgtactcttgactattctacaaaagcaagactttaaactttttagatacatcattaaaaaagaaaaccataaaaaagaatatgaaaagatgatttgagatggtgtcactttaacagtcttaaaagcaatcgtgtgtatagcatagaattgcttggattggataaacagtggcattatatattttaaaaaataaaagttttgaaagattgaagaatttgggcattacagttctcttaaatctgacaaagctgcataaaactattaaaataatcattattatactattttatattctatttctttgagggtttagttttccaaaaactacatattaagcaaatgaatcactcagtggctatgtcatataataacgagttagcctagttataagaagtttaacattttatttaagaacattgttacagcatgtttactgtatagtctagtaatagaggaaaagacatttgggtgggtggtagtggtagtatttttatagaggagttaccaaatttcagctctattatccaagtttacccagctaatggtgttcggaaccgggaatttgagccaattctgactctgttgtctgctctgctccttcttttgtgctgtgtctttgaaagtcacctaaaattgtgagggaatgtaatttcaccccaaatttagagtttatgcacttgttatattgaaaatgattaacatgtagaagggcttttaatggaataagtggtgtagtaacttcagtgttgcctacctagaaatcaaaatctttctagttgtccactttgttttttgaaaaagtaatatgaaaattatgttaatgctttaattcaggtttttgtaaaatattttttatctttacacatttaacatacgtttctaaaattatagtctgttatatagcactttgggtctagaatttttcagtagtttctgttttactattatgatctacctgcatattaacctattaggttatagttttactatacttctaggtatttgatcttttgagagagatacaaggtttctgtttaaaaaggtaaagaaacaaaataactagtagaagaaggaaggaaaatttggtgtagtggaaactaggaattacattgttttctttcagccaaattttatgacaaaagttgtggacaggttttgaaagatatttgtgttactaatgactgtgctataacttttttttctttcccagagaacaaattaaaagagttaaggactctgaagatgtacctatggtcctagtaggaaataaatgtgatttgccttctagaacagtagacacaaaacaggctcaggacttagcaagaagttatggaattccttttattgaaacatcagcaaagacaagacaggtaagtaacactgaaataaatacagatctgttttctgcaaaatcataactgttatgtcatttaatatatcagtttttctctcaattatgctatactaggaaataaaacaatatttagtaaatgtttttgtctcttgagagggcattgcttcttaatccagtgtccatggtactgcttttggctttggtttctttctacattgaaaatttctcttcaattctgagcacatgttaacatttagaattcaagaggtggggatttttttttcccatggttacatatatatatatatatatatatatatatatatatatatatatatatataaagaacagggcaacaaatttttgcgttttctatttcggtagtacttttaaaccattatgtcatgtttctaggttaaacgttgttgtatttgaagaattttactttggcagaatttttttgaggatgtgtttatttctggagaaaggtctcattaaagaaagacaatacccagaaagccaacagaaattctgttactcatttaatgcatttttctgacaaaaattattgccagagagaacctgaattttgtttcaaaaatcatctttgttttaaaaatgactttttcttcaggtaaaataaaataatttcagttgctattatttaacctgtttgtatgaagagtttaacatataggaaatgaatacataaagataggaaggaattaattgttatatgtagtcatatgtctcttaatgacagggatactttctaagaaatacattgttaggtgattttgtcattgtgcaaacatcatagaatatacttacacaaaccttggtagtataacctactatacacctgggatatgtagtatagtctcttgccccagggatacaaacctgtacagtatgtaactgtactaatgactataaggcaattgttaacacaatggtaagttttgtgtgtctaaacctacacttgggctaccctaagtttatatatttttttaaatttctgttcaataataaattaaccttactttactgtaactttttaaactttttaatttttcctaacattttgacttttgtaatacagcttaaaacacacattatacagctatacaaatttttctttccttatatctttattctgtaagcttttttccatatttaaaattttttgtttgtttttacttattaaacttttttgttaaaaactaagacatgcatgcacattaacctaggcctacacagggtcaggaccatcaatatcattgtcttccacttccacatcttgtcccactggaagatcttcaggggcagtaacacacgtggagctgtcatctcctataataacattgccttcttttggaatacctcctgaaggacctatccaaggctgtttatagttaacttttttttttttttttttttttttttagtaaataggaggagtacactataaaataacaatataggtgctataccattatacaactgacagtgcagtaggtttgtttacaccagcatcaccacaaacacgtgagcaatgtgtcgtactacagtgttaggatggctataacatcactaagcaataggaacttttaaactccattataatcttatgggaccactatcacatatgcaatctcctgtggaccaaaatgtcattatgtggtacatgactgtactaagaaattgatccatctatattccatcaatttgtttagggctttttctggttacatttacctgtgagcccagaaaaccagttttgtagaaattaacttctgtaatgctaggagttaaaaaaaattgctgaacaacttttacattgttaaacatttaaaaacaagcgttctagaagtttatcaaatttcataaaggtgcaaaaatgtaaatgtaaatcattatccagctaatatatatgttgtatttccctagtaggagagcatatgtacctcttcctagttatacaaatttgatatatagtaaagaaacagtaaattctacttcaagtcattttgggaggattaaaaactgaatttctctagtttgaccattgtacagatttatctggcaattttactaaaacctgatttataggttaaacttggtgtatatcatatatcactttactttagaggaattaagatttcacataaatccatttccaggttccaaagaccaggaagaggcttggtttttgtttttctttttactgtctttacagtctccttgacttttcttaggagagaaggtactgagaaaacatgattctaatatttattattttttcttccaacattttcttatgaaacattttcaaatacaaaattgagttttatttaaaacatttgcaaatatactacctagattctaccattgttgttttatatttgctttacttacaacttttaaaagatgctttttataccactgaacattttagcttacatttcacaaagaaaagaaaaaatttaagagactttgcataatgttttaaggggttgcagtaaagaagtgcttcttatattttcttatgcatacaaatcagctgggcttattaaaatccagattctaattcagaaggtttaggtggggaccgagtctgcatttctaacaaactcctaggtggtatttttcttggtacttggaccatactttgagtagaaaagcagtagaggacataaaaagagtcttgttagtcccactttgttgctgtccacttctcatttgataatatcctaaaatagctgtgtctcctttttggtggttgtatgattactacctcagaagtactaattgattcttgctatttgaccttaatactttaatataacacagcattcatatttgatcagaaaactatctggcttccttttataagagatttttaggttttatacagttttgtggccttgggtttttttgtttgatttgtttttttgaaggtatataatatgtaagtagataaacaaatttgatttgtagacatttttatgtggatcatctaattaaaaatggagggatacagtatgaaagaatacttgtacttcttaacagagcactcaacctttcttttacatcctgtttcactgatgttattatgtaatttatgttgctaaactataaattagatatttaatttctgttctttgatttccttttattattaaatggacttgttgatttgcctagaaattaatttgcctttcaaaagtcttattaatcttcctccgttgaaattaatttgatatttgcatgcttctggaagactttaaagagctattccgagtaactgtagagattataaaatgaaatatgggaattttaataaattttacatctccagttactggtgaaaatgtcaagtcctcctttctgcagagtattttgttactcatctgttattcagcttatttatttatttatttatttatttatttttctttctttcttgttttttttttttgagacggagtcttgctttgtcgcccaggctggagtacagtggtgggatcttggctcactgcaggctccgcctcccgggttcacaccattcttctgcctcagcctcccaagtagctgggactacaggcacccgccaccatgccttgctaaatttttgtatttttagtagagacgggtttcactgtgttagccaggatggtctcgatctcttgacctcgtgatccacctgcctcggcctcccaaagtgctgggattacaggcatgagccaccgcgcctggcccttatttgttttttaaacaaaattagtgtgcatatccttgttgtattttatcggcaagttgttttatgccctaacttttggggtcttgatcatgagcctaaaacacgtaaacacccaaaaagaattatattccggttaaaggaacaaaacattcatttagaagttctcatccatgtaaatcagaggctggcaaatattttctgtaaagggccaagatagtaaatgttttaggctttgagggccacaagtggtatctgttgcatttttttttaattatgaccctttaaaatgcaaaaatcgttgttagcttgtgcatagtataaaaataggctggccgcatgctgtggctcatgcctgtaatcccagaaatgaggtgggaagccgaggtgggcacaccacctgaggtcaggagttcgaggccagcctggccaacgtggttgaaaccccgtctctactaaaaatacaaaacttagccaggcgtggtggcgggtgcctgttatcctggctactcaaggggctgaggcagtagaattgcttgaacctgagaggcagaggctgtagtgagcccagatcaagccagtgcacaccagcctggacgaccgagcgagactctgtctcaaaaaaaaaaaaaaaaggctgtggctgcatttggtccattggctgtaatatgctgattcctaattctctgggtaactttagtgtttgattagctactagaagttaggttaaacttttgtattttacaggctaactttaataatcttaaagtaaaacttaacatagttcatggaaaggaaatagaaattttaccctagtactcttttttttttttttttttttttttgaggcagagtctccctctgtcacccaggctggagtgcagtggtgggatcttggctgattgcaacctcctcctcctgggttcaagcaattcttgtgcctcagcctcccgagcagctgggactacaggcacgcaccaccacacctgactgatttttgtatttttagtagagacagggtttcgccatgttggccaggctggtcttgaactcctggcatcaagtgatcctcccatctgagcctcccagtgtgctgggattacagacgtgagtcactgtgcctggtctctagtattttttttttttttgagacggtctcactgttgccaggctggagtgcagtggcgcgatcctggctcactgcaacctccgcttcccggattcaagcgattttcctgcctcagcctcctgagtagctgggactatgggtgcacaccaccacgcccagctaatttttgtatttttagtagagacggggtttcaccatgttggccaatatggtctcaatctcttgacctcgtgatctgcccgtctcggcctcccaaagtgctgggattacaggcgtgagccactgtgcccagctgtactttttaagataagaattgcagggtatatatttttaccaacttaataacttataattttaaaaagctaattacttggctagaatataatgcgttacatattctttacactcagttcagtccatatctgaaaggcaaatagaattattttctgctagtacattgtgtagtccctatgttcctagtgtataaggactgttacctagttcacatttatctgggttgttgacagattttcctggtccctttggacagtgcatggccatgttggcaaaagctgtcaaaattgaaacattgacaccatgagaattgtgtgttttccagtctgctaaaatcaaaagtgggagggttcagtaaggtgaataacagaagcagagttttcggggtatctgttactcctcattcggcttttctgctctctgggggtctcaatttaaatataatgtgaaaattagttttacgaacctaaaaatgttgagtgattcatttcctggttttgttgttaatttctagatatttaaattaattgttagaagaaccccgttaaagaatgctttgcaaaacaacctccttatgtgctatgtctctgtttaatagtagttgagtttgtgtacatgagatcaatattttgaactatagctttttatgagttaaaaattgacggaacagttactgtgcacttgctgtgcaccatggtagtctcccaagtagtggtttttctgcatttcaatagtacatgagataggctgtgggtggcaaggtttcttgagaaagtgagggatgcacagttgggttttagaatacatcttgttcctccatgcccttccccaccaaaaggctggtagtcttgcatttgtatatagttagggtatttgatgtgttgcttccttgacagagttttgcaagaatttgcagatttaacaggaacaaaaacttacttaaaacaaaatctcttagtaaaagcatagtctagcaagatttagaatgatactttggctaacagtactttctctatatggagtgctttgtttccatagcctcacaagtatgttttcagataatagttgagttgaaaatgttgtcaatctcttgattttaaaaaatttacatatttaaagttgtatacttttgttcctacgtattttcagttgttcttaaagtttaataagtgacatttgaaaatgagtatatgtgtataaaaacaaaagtaggctaggcacggtggctcatgcctataatcctagcactttgggaggctgaggcaggcggatcacaaggtcaggagtttgagaccagcctgggcaatatggtgaaacccccctctactaaaaatacaaaaattagctgggtgtggtggtgcatgcctgtagtcccagctactcaggaggctgaggcaggagaatcgcttgaacccggaggtggcggttgcagtgagccgagattgcaccactgcagtccagcctgggcggcagagcgagactccatctcaaaaaaaaaaaacaaaaaaagaaaaagttaaaaaaaaacaaaaaacccccacaaaatgagtatatgtggcaacaagtcctattctcaaaaaaattattgtgtgctagttaagagcttaatgagtagccagtcggtattaaatatctgtttcagctatattttatctttaaaaattatctacagattttggaatgtgaaaaactagtgttttgtttcataggtatatactgtaggcattttaaaaataagagccagtgccagtggtttacagtgtacacaaggataatgttctcatgttctcttgatgtcagtatgactttaaagcatattatcaagaaataactaagtctgaaaaactgtggtaaataactggtactctaaaacctaagtttcttattactaaaaataagaaatggtaaaagtcaccctgtgctgttaattatatgagccactgaggtcctgacactgaattcttggtggtggataataatctcttctttttaattattggcttccaattctctctgcattgctggaaacaaaaatcatatatttcactattggtggtggggatgctgtcactgaaaaagtagacacattcatattgattttagaaataagttaaaatcaaaatttgcttctgctaaattagtagaggaccaatactgtttttctccttcatagtatgttttggtacttctacattgacattataacttttttttttttaaacagaaatagaagtttacat

SEQ ID NO: 8 - protein, 188 aa, Artificial Sequence [sequence omitted]

SEQ ID NO: 9 - DNA, 5306 bp, Artificial Sequence
  KRAS G12D mRNA
ctaggcggcggccgcggcggcggaggcagcagcggcggcggcagtggcggcggcgaaggtggcggcggctcggccagtactcccggcccccgccatttcggactgggagcgagcgcggcgcaggcactgaaggcggcggcggggccagaggctcagcggctcccaggtgcgggagagaggcctgctgaaaatgactgaatataaacttgtggtagttggagctgatggcgtaggcaagagtgccttgacgatacagctaattcagaatcattttgtggacgaatatgatccaacaatagaggattcctacaggaagcaagtagtaattgatggagaaacctgtctcttggatattctcgacacagcaggtcaagaggagtacagtgcaatgagggaccagtacatgaggactggggagggctttctttgtgtatttgccataaataatactaaatcatttgaagatattcaccattatagagaacaaattaaaagagttaaggactctgaagatgtacctatggtcctagtaggaaataaatgtgatttgccttctagaacagtagacacaaaacaggctcaggacttagcaagaagttatggaattccttttattgaaacatcagcaaagacaagacagggtgttgatgatgccttctatacattagttcgagaaattcgaaaacataaagaaaagatgagcaaagatggtaaaaagaagaaaaagaagtcaaagacaaagtgtgtaattatgtaaatacaatttgtacttttttcttaaggcatactagtacaagtggtaatttttgtacattacactaaattattagcatttgttttagcattacctaatttttttcctgctccatgcagactgttagcttttaccttaaatgcttattttaaaatgacagtggaagtttttttttcctctaagtgccagtattcccagagttttggtttttgaactagcaatgcctgtgaaaaagaaactgaatacctaagatttctgtcttggggcttttggtgcatgcagttgattacttcttatttttcttaccaattgtgaatgttggtgtgaaacaaattaatgaagcttttgaatcatccctattctgtgttttatctagtcacataaatggattaattactaatttcagttgagaccttctaattggtttttactgaaacattgagggaacacaaatttatgggcttcctgatgatgattcttctaggcatcatgtcctatagtttgtcatccctgatgaatgtaaagttacactgttcacaaaggttttgtctcctttccactgctattagtcatggtcactctccccaaaatattatattttttctataaaaagaaaaaaatggaaaaaaattacaaggcaatggaaactattataaggccatttccttttcacattagataaattactataaagactcctaatagcttttcctgttaaggcagacccagtatgaaatggggattattatagcaaccattttggggctatatttacatgctactaaatttttataataattgaaaagattttaacaagtataaaaaattctcataggaattaaatgtagtctccctgtgtcagactgctctttcatagtataactttaaatcttttcttcaacttgagtctttgaagatagttttaattctgcttgtgacattaaaagattatttgggccagttatagcttattaggtgttgaagagaccaaggttgcaaggccaggccctgtgtgaacctttgagctttcatagagagtttcacagcatggactgtgtccccacggtcatccagtgttgtcatgcattggttagtcaaaatggggagggactagggcagtttggatagctcaacaagatacaatctcactctgtggtggtcctgctgacaaatcaagagcattgcttttgtttcttaagaaaacaaactcttttttaaaaattacttttaaatattaactcaaaagttgagattttggggtggtggtgtgccaagacattaattttttttttaaacaatgaagtgaaaaagttttacaatctctaggtttggctagttctcttaacactggttaaattaacattgcataaacacttttcaagtctgatccatatttaataatgctttaaaataaaaataaaaacaatccttttgataaatttaaaatgttacttattttaaaataaatgaagtgagatggcatggtgaggtgaaagtatcactggactaggaagaaggtgacttaggttctagataggtgtcttttaggactctgattttgaggacatcacttactatccatttcttcatgttaaaagaagtcatctcaaactcttagttttttttttttacaactatgtaatttatattccatttacataaggatacacttatttgtcaagctcagcacaatctgtaaatttttaacctatgttacaccatcttcagtgccagtcttgggcaaaattgtgcaagaggtgaagtttatatttgaatatccattctcgttttaggactcttcttccatattagtgtcatcttgcctccctaccttccacatgccccatgacttgatgcagttttaatacttgtaattcccctaaccataagatttactgctgctgtggatatctccatgaagttttcccactgagtcacatcagaaatgccctacatcttatttcctcagggctcaagagaatctgacagataccataaagggatttgacctaatcactaattttcaggtggtggctgatgctttgaacatctctttgctgcccaatccattagcgacagtaggatttttcaaacctggtatgaatagacagaaccctatccagtggaaggagaatttaataaagatagtgctgaaagaattccttaggtaatctataactaggactactcctggtaacagtaatacattccattgttttagtaaccagaaatcttcatgcaatgaaaaatactttaattcatgaagcttactttttttttttggtgtcagagtctcgctcttgtcacccaggctggaatgcagtggcgccatctcagctcactgcaacctccatctcccaggttcaagcgattctcgtgcctcggcctcctgagtagctgggattacaggcgtgtgccactacactcaactaatttttgtatttttaggagagacggggtttcaccctgttggccaggctggtctcgaactcctgacctcaagtgattcacccaccttggcctcataaacctgttttgcagaactcatttattcagcaaatatttattgagtgcctaccagatgccagtcaccacacaaggcactgggtatatggtatccccaaacaagagacataatcccggtccttaggtagtgctagtgtggtctgtaatatcttactaaggcctttggtatacgacccagagataacacgatgcgtattttagttttgcaaagaaggggtttggtctctgtgccagctctataattgttttgctacgattccactgaaactcttcgatcaagctactttatgtaaatcacttcattgttttaaaggaataaacttgattatattgtttttttatttggcataactgtgattcttttaggacaattactgtacacattaaggtgtatgtcagatattcatattgacccaaatgtgtaatattccagttttctctgcataagtaattaaaatatacttaaaaattaatagttttatctgggtacaaataaacaggtgcctgaactagttcacagacaaggaaacttctatgtaaaaatcactatgatttctgaattgctatgtgaaactacagatctttggaacactgtttaggtagggtgttaagacttacacagtacctcgtttctacacagagaaagaaatggccatacttcaggaactgcagtgcttatgaggggatatttaggcctcttgaatttttgatgtagatgggcatttttttaaggtagtggttaattacctttatgtgaactttgaatggtttaacaaaagatttgtttttgtagagattttaaagggggagaattctagaaataaatgttacctaattattacagccttaaagacaaaaatccttgttgaagtttttttaaaaaaagctaaattacatagacttaggcattaacatgtttgtggaagaatatagcagacgtatattgtatcatttgagtgaatgttcccaagtaggcattctaggctctatttaactgagtcacactgcataggaatttagaacctaacttttataggttatcaaaactgttgtcaccattgcacaattttgtcctaatatatacatagaaactttgtggggcatgttaagttacagtttgcacaagttcatctcatttgtattccattgattttttttttcttctaaacattttttcttcaaacagtatataactttttttaggggatttttttttagacagcaaaaactatctgaagatttccatttgtcaaaaagtaatgatttcttgataattgtgtagtaatgttttttagaacccagcagttaccttaaagctgaatttatatttagtaacttctgtgttaatactggatagcatgaattctgcattgagaaactgaatagctgtcataaaatgaaactttctttctaaagaaagatactcacatgagttcttgaagaatagtcataactagattaagatctgtgttttagtttaatagtttgaagtgcctgtttgggataatgataggtaatttagatgaatttaggggaaaaaaaagttatctgcagatatgttgagggcccatctctccccccacacccccacagagctaactgggttacagtgttttatccgaaagtttccaattccactgtcttgtgttttcatgttgaaaatacttttgcatttttcctttgagtgccaatttcttactagtactatttcttaatgtaacatgtttacctggaatgtattttaactatttttgtatagtgtaaactgaaacatgcacattttgtacattgtgctttcttttgtgggacatatgcagtgtgatccagttgttttccatcatttggttgcgctgacctaggaatgttggtcatatcaaacattaaaaatgaccactcttttaattgaaattaacttttaaatgtttataggagtatgtgctgtgaagtgatctaaaatttgtaatatttttgtcatgaactgtactactcctaattattgtaatgtaataaaaatagttacagtgac

SEQ ID NO: 10 - protein, 189 aa, Artificial Sequence
  KRAS G12D protein Isoform A
MTEYKLVVVGADGVGKSALTIQLIQNHFVDEYDPTIEDSYRKQVVIDGETCLLDILDTAGQEEYSAMRDQYMRTGEGFLCVFAINNTKSFEDIHHYREQIKRVKDSEDVPMVLVGNKCDLPSRTVDTKQAQDLARSYGIPFIETSAKTRQRVEDAFYTLVREIRQYRLKKISKEEKTPGCVKIKKCIIM

SEQ ID NO: 11 - DNA, 32729 bp, Artificial Sequence
  Genomic Sequence for KRAS Wild-Type
gattttcctaggcggcggccgcggcggcggaggcagcagcggcggcggcagtggcggcggcgaaggtggcggcggctcggccagtactcccggcccccgccatttcggactgggagcgagcgcggcgcaggcactgaaggcggcggcggggccagaggctcagcggctcccaggtgcgggagagaggtacggagcggaccacccctcctgggcccctgcccgggtcccgaccctctttgccggcgccgggcggggccggcggcgagtgaatgaattaggggtccccggaggggcgggtggggggcgcgggcgcggggtcggggcgggctgggtgagaggggtctgcaggggggaggcgcgcggacgcggcggcgcggggagtgaggaatgggcggtgcggggctgaggagggtgaggctggaggcggtcgccgctggtgctgcttcctggacggggaaccccttccttcctcctccccgagagccgcggctggaggcttctggggagaaactcgggccgggccggctgcccctcggagcggtggggtgcggtggaggttactcccgcggcgccccggcctcccctccccctctccccgctcccgcacctcttgcctccctttccagcactcggctgcctcggtccagccttccctgctgcatttggcatctctaggacgaaggtataaacttctccctcgagcgcaggctggacggatagtggtccttttccgtgtgtaggggatgtgtgagtaagaggggaggtcacgttttggaagagcataggaaagtgcttagagaccactgtttgaggttattgtgtttggaaaaaaatgcatctgcctccgagttcctgaatgctcccctcccccatgtatgggctgtgacattgctgtggccacaaaggaggaggtggaggtagagatggtggaagaacaggtggccaacaccctacacgtagagcctgtgacctacagtgaaaaggaaaaagttaatcccagatggtctgttttgcttggtcaagttaaacccgaagaaaacccgcagagcagaagcaaggctttttccttgctagttgagtgtagacagcaatagcaaaaatagtacttgaagtttaatttacctgttcttgtcctttcccctatttcttatgtattaccctcatcccctcgtctcttttatactaccctcattttgcagatgtgttctacatctcaagagttattacagtactccaaaacagcacttacatgattttttaaacttacagaggaattgtagcaatccaccagctaaccgcctgaaatagacttaaacatgtgcatctcctttttttttttttttttgagacacagtctcgctctgttgcccaggctggagtgcaatggcgcggtatcggctcactgaaacctccgcctcctgggttcaagcaattctcctgcctcagcctcccgagtagctgggactagtaggtgcacgccaccatgcccagctaatttttgtatttttagtagagacagagtttcatcatgttggtcaggatggtctccatctgctctgttgcccaggctggagtgcagtggcgccgtctcggctcactgcaacctctgcctcctgcattcaagcaattctcctgcctcagcctcccgaataactgggattacaggtgtctgctgccatgcccggctaattttttgtatttttagtagagacgggggtttcaccatgttggtcaggctggtctagaactcctgacctcgtgatctgcccgcctcggcctcccacagtggcatgtgcatcttatagctgaagtctaagccttcttaaatcttgagatccatcaaaacagacaggttttctaattgttatacaatgtatatgttatgtttataatagaaatcattttacaaataagttataaatgggaaaggtctatttgtaattatcagctcagaattaaccataaaactggtgtcactgaagtgactgaggtccaaaatgctgactctgcatgttatagactacagatatcaaatatggttgctaacaatagtttactttgagactgtagccatccacagtatatttgcttttaagagatggtagatggtaattcagttttatgaaaaataaaaatgaattttcttccattacaaaattgttggattcgagtccagtccactccttactagcttttctaactctcggtgagggatcccctcccagcccatgatcttcatttggtaagactcctttggaacccagttctctctagtggatttaaatgtgatttggttttaaaaatctcattcaaggaattttttttttttctggaaacaaccaccgcataaacaagtaaaccggaagatacatgtggctctgaattcatatatatacacaaactctaatccaatgtctgtccacagtatttcctaggctagtaaactttttggccttaacgacccctctaccctctttgtttttttgagagagagagtctcactctgtcacccaggccggaatgcagtggcgcgatctcggcccgctactacctccgactctcaggctcaagcgattctcccgcctcagcttcccgagtagccgggattacaggctcccgccaccgggctaattgtatttttagatacgggatttcaccatgttggccaggctggtctcgacctcctgacctcaggtgatccgcccgcctaagcctcccaaagtgctgggattacaggccaccacacccggcctacactcttaaaaattatcgaaggggccgggcacattggctcttatctgtaatcccagcactttgggagactgaggcgggaggatcgcttgaggccaggagttggagaccagcgtactcaacatagtgagaccttgttataaagaaaaaaaaaatccaggattaaaaaaaatctttgatttgtttgggatttattaatatttaccgtattggaaattaaaacaattttttaaaatgtattcatttaaaaataataagcccattacttggtaacatgaataaaatattttatgaaaaataactattttccaaaacaaaaccaaaacttagaaaagtggtattgtttcacacttcagtaaatctctttaatgatgtggcttaatagaagatatggattcttatatctgcatctgcattcaatctattatgatcacacatctggaaaacttgtgaaagaatgggagttaaaagggtaaaggacatcttaatgttattatgaaaacagttttgacctcttgcacaccagaaaagtcttagtaacctgaggggttcctagaccacattttgagaactgttttaggctatgcaaactggttggggggaggttggggtaggcagagagctagaagatacattttagtgtaattctcctcatctattcctaattgctttggcctacatttgaaataaagcgtggaggcaaacgggataagatacatgtttgtagtggttgttaacttcaccctagacaagcagccaataagtctaggtagagcagagtaaggcggggaactatgccgtgaccgtgtgtgatacaatttttctagcctgtggtgctttttgcggcagggcttaggagtaaggttagtatgttatcatttgggaaaccaaattattattttgggtcttcagtcaattatgatgctgtgtatatttagtgtttatctacaatatatgcacattcattaatttggagctactcatcctataataaatagttgtgcatttactcccatttttttctgcatttctctccttatttataattatgtgttacatgagggaaaggaggtgaaattaaacattcatattatttcaaaaaatttgaaacaactaactaaaaaatatgttttattttctgtatggtgtttgttatacaatctgtcaatattcatgcacctcttgggagacagtgtatgaaaagcaaagagtaacagtcacatggattactgattactgagatatattcacttgcatctttttttttttttgagacggagtggctctgtcgcccaggctggagtgcagtggcgtgatctcggctcactgcaagctccgcctcctgggttcacgccattcttctgcctcagcctcccaagtagctgggactacaggcgcccgccaccacgcccggctaatttttttatatttttagtagagacggggtttcaccgggttagccaggatggtcttgatctcctgacctcgtgatccaccctcctcggcctcccaaagtgctaggattataggcgtgagccaccgtgcccggctcacttgcatctcttaacagctgttttcttactaaaaacagtgtttatctctaatctttttgtttgtttgtttgttttgagatggagtcttactccgtcacccaatctggagtgcagtggcgtgatctgggctcactgcaacctctgcctcccgggttcaagtgattctccttcctcagcctccccagtagctaggactacaggagagcgccaccacgcctgattaatttttgtatttttagtagagagagggtttcaccatattggccaggctggtcttgaactcctggcctcaggtgatccacccgccttggcctctgaaagtgctgggattacaggcatgagccgccgcacccggctttctaatctttatctttttttgtgcagcggtgatacaggattatgtattgtactgaacagttaattcggagttctcttggtttttagctttattttccccagagatttttttttttttttttttttttgagacggagtcttgctctatcgccaggctggagtgcagtggcgccatctcggctcattgcaacctcggactcctattttccccagagatatttcacacattaaaatgtcgtcaaatattgttcttctttgcctcagtgtttaaatttttatttccccatgacacaatccagctttatttgacactcattctctcaactctcatctgattcttactgttaatatttatccaagagaactactgccatgatgctttaaaagtttttctgtagctgttgcatattgacttctaacacttagaggtgggggtccactaggaaaactgtaacaataagagtggagatagctgtcagcaacttttgtgagggtgtgctacagggtgtagagcactgtgaagtctctacatgagtgaagtcatgatatgatcctttgagagcctttagccgccgcagaacagcagtctggctatttagatagaacaacttgattttaagataaaagaactgtctatgtagcatttatgcatttttcttaagcgtcgatggaggagtttgtaaatgaagtacagttcattacgatacacgtctgcagtcaactggaattttcatgattgaattttgtaaggtattttgaaataatttttcatataaaggtgagtttgtattaaaaggtactggtggagtatttgatagtgtattaaccttatgtgtgacatgttctaatatagtcacattttcattatttttattataaggcctgctgaaaatgactgaatataaacttgtggtagttggagctggtggcgtaggcaagagtgccttgacgatacagctaattcagaatcattttgtggacgaatatgatccaacaatagaggtaaatcttgttttaatatgcatattactggtgcaggaccattctttgatacagataaaggtttctctgaccattttcatgagtacttattacaagataattatgctgaaagttaagttatctgaaatgtaccttgggtttcaagttatatgtaaccattaatatgggaactttactttccttgggagtatgtcagggtccatgatgttcactctctgtgcattttgattggaagtgtatttcagagtttcgtgagagggtagaaatttgtatcctatctggacctaaaagacaatctttttattgtaacttttatttttatgggtttcttggtattgtgacatcatatgtaaaggttagatttaattgtactagtgaaatataattgtttgatggttgatttttttaaacttcatcagcagtattttcctatcttcttctcaacattagagaacctacaactaccggataaattttacaaaatgaattatttgcctaaggtgtggtttatataaaggtactattaccaactttacctttgctttgttgtcatttttaaatttactcaaggaaatactaggatttaaaaaaaaattccttgagtaaatttaaattgttatcatgtttttgaggattattttcagatttttttagtttaatgaaaatttaccaaagtaaagaccagcagcagaatgataagtaaagacctgtaagacaccttgaaggtcatggagtagaacttccatcccaagcagatgaggatttatttaatctcaaagacctccaggaggggacattccccaactgtccttgttaactcattttcagaacatatttattagcatattttacatgtaatttggatcttcatgttaaatttaacatcagtggagatggaaaataagcatatcgccttgtctttgaaatagccctatattgttagattgtttcttaggcttctttaccctgggttaagcagtcctaatactttagcatttattctacatctagtgtactaatttaaaaaaatcagttctgaaaaatttctaagaactttcttcaagttccaagctgtgaaatctagaacaggtcaaagtgccttattaacgtactgtactgtgtagtgtcttgaagagacactttgcgctgaggcaagttctgagggcattgggtggccttgggaagatatttatgcagtttagaacctggagaattgattagataactaatcataaggaaacgtcacatatttttggtactataaaaaagtggagaaataatgcctatttgcaaagatttgatttaaacatagaaacaactttatttggcttccaattttaagaatttacagcagtaaaggggaacagtctaattgaagtagactgcctatgcaatagtctctgtatatttacttttgacaagttaattcaatgtgtactatagttttgtttctttgaagaggtttgaatagtgcacccattttaatctgtattgcaaattcagggttacttggcagactctactatttaaatcagatgtaaaaggaagttttaatataattcactttatgcctgaaagttttcctgggattttggaaggtgattttactggaaatgctgtctgtcttccctgaaaatctgagaaattccattacactttgtttccaatcagaggtcatgagtgctatatgagtatatacagcatgacgtcatgaatgtgataaagtgggttaggaaaccttttgctaatgattgttaaaatgcaatataaatgttgaagaaataaagctaacagttaagcctttatttgggcggaaggctgaaaaagtttataaacttaaacctataactctgcttatgatttctgccaaaccagaagacttgactctgggaagcattggttacctgtgaactttgaaactgacggtccctgacgtagtttagtcacctgggaaaaggtatctgagattatctcttatctcccaagttacagtgagtctctgagggaactgacacattacattaagttcttggtgtagttaaactgtaagaaaggcaggagaacttagtagttaaatagttggttaaatggaaatgctgactccatgttattgtaaaaagttaaaaatttaggaggatatggggatttcactgccattgcaggttttgattggtatttaccaatccgtgtgggtcagagagaaaattagaaaggatatgactgcacattttggaattattagcagtttttctacatttaaaatggaaataaattttttaaaaatttaaatcaagtaatactgtattttttggtgatttagatttttcaaaatttacactaagagatagtaaggagggtggctattgtttctttcaataatgtctctgagaggttgtaactcatctaaggatacgtagctaataagtggtaggatttcaatttaaattctctgagaccaagttaagtagaatttgcactgtactcttgtataactttttaaaactgaaaattagctatctttcaaattaagaaaatatttactaatggagactaattcagatttgtaagtataccaaaatttgaacttagcctgctatctaatggcaacttagtggcagaggtatgatgtaaaatcattcaggtatgacacatagatggagtatgtttgtattcgaggctgtgcacataatcacctttacttgtattgtgaagtatatattgttatcttttatgaagcccactaaagagataatgaaatacctcgttattagggcaagattattgaaaactcaaaatagcccccaaacacaatacttggctagaaatatatacctttatagttcagagatcatttattatcaaaaccctgaagttttttttctaaggtaaaatttggtggaagaggaaaagtctcgttttaaaaaaatgtaggtagttacagagatcagaatgattagttgatcacttaccaaatatatattaagtatctactgtatataatatgctagtaagaataaatatagcaggaagtattttttcccaggctctaattgtttgacatcagcatgcttttattgtggcacttataattcagttcaagtattatgcccctctttgatggaacagtttcctattcagtaaggaagaccagattaatcattggattggtttgtttcatctttagtgttctgagctgtagagtatttatttaccaaggtttattttaatttttattttatttttatttttccatgttcattgtagaattcattttacctacgaatgaagtatgtagattatagagagaaaatttgtaaaattaaactgatactgaagactggtataagaaaagccttatgtaatttgtaagctgctattcttctgagtttatacatatatctttagtaatcaatgagggatggttgggtgactgccctccaggggacatttggcaacatctggagatgtttttggttgccacaacttggggagagagtactgctactggcatctattgagtagatgctattactttaaatggcaaagctgcagttacctttgcaccaacctaatattaaacttcctgcagtgcacgggaaagcccccacaacagggttatctgaccccaaacctcaatggtgttaagatccaaaccttgatatgttaacctgtagctttaaacatcctttaaattgtcaaattcatgtccctgacataaggtttatgttagattttcaagtataacaaagatttaaactttaacttttgtacgttaatgatatgttagcttactccagtcttctattaaaacattctgtttttaaaatcagagacacacagcaattttataaatcatttctcttcaaggctgtgaagctctccccacttttgtgagtgccctctactggtcaaattatttgctttataacaagtaacagtgaaatcctaagtttgtgtagtttcgctgtttaaattatgggtggcatcaatttataaatatattcgttttatttaaaagtcttatatgattgatttcgtatcatttttgctctctgctaatattaatataaagattactgtctgtattagttaggcctaactaagtaggtgagtatagtgaactaagaaaggaaacgaggcagtatataagaaaatagggtggttcagttgttaacacttactgagcttactttgttgaagggactaaaaggcagcagtgtggctctctgagcttctttgcatgcactcaggagctgcttaatggagtccaaggcttggtggtgtgttacaggggatgataggagggtcctattcagaagtggcaaattgtgaaagtgcacattttgtagagttttataggactgtagaatagttgtgagcacctgatttttagaataaacagaaaactcaggtactgtatttaggtcaaattaagaataagtatttattaagacctgaatataaaactttactggtcatggtttttttctaccttgggtttttataaatccaaagatttaaaaacatacaaatggaagttggtaatggaattaagtgaaaggaaaaaatgattttatggtttggaatctcctaagattctggttttaacaatacaactaattccttaatcctagaaatgttcttcactgcccactttgtaccatgcagtcttcctgtgggctagagatacactgaggcgcaaaacagaccagattcctgccttcatggagcttattagttttaggtatctctagatttcttgtaatacctattacaatgcctgcacatcagttcattcatgtgggttcaacgtagtactcagtacatggcaaattcaagttttacttttcggaacttcatggatttttttcctcagaatatcttttatccataattggttgaatctgtagatgcagtacccatggatatggatggcccactttattttgaagagcagtgtttctaggcaatcatgctaattatatatgacttaatttagaggctttatacttaagagcattacatttctggcgtctcttaaccattattatttcataatgtgtaggttatggaacagttaaattattgggatcttaatatagaaattagtagaaataagccagatatggtggctcatgcctgtaatcttagcactttgggaggctgaggctattcgctgtactattttttactacttttctataggtttgaaattttttcaaaataaaacattgaaaaaagtaaggtaggtagtgtgtccctccttaatcctttcaaatattttattttcactatttctattaatttttttttttgtttttgagatggagtctcgctctgttgcccaggctggagtgcagtggcgcgatcttggctcactgcagcctccacctcctgggttccagccattctcctgcctcagcctcctgggtagctggtattacaggcatgcaccaccacacccaattactttttgtatttttagtagagacggggtttcaccatgttggccaggctagtctcgaactcctgacctcgtgatctgcccgcctcagcagtgtcactgcttctagaccgttttcaaggcacagagcttagaaatgcatgttactaagaaatcaagagttaactatttttcaccttctttctcccgcagtgagaaccctggttctaccctgtttctccttgtgtaaattttaatgctaaactatacacttgtgaaataaaaatgataatgtcattcttaaattatggatcttgcagtgttatctaagtaacatagattgagtgatttaactttaggtttccttatttgtggaatttggataaatatttttcacccttgagaaaagtgagactcctttctcatcatcagagtatccttaaaccattaaggcaaacatttgggaaaaaactgagctatctggctgcataaaaattaagttttctttaacaaagatagaagacaaatgaaaacctagaaaaaccatttggttcaagtaacaggaagctatcttatatatgaattagagaaaagcaaacacacaaatagaaaaaaagggatggggggtactaaagatataaatagcttgtctaccaaaaaagaaataaaataaataacatgaacatataaaaagacacttacttcatgaatgtgatgcaagttcaaacaataaataacatttctgtactttcatattggctaaggttaaaatgataactgctaggaagggtatggagaagtgtgcgccttgcactgtagtgggagtatagaccctcagactttatggaggtcagtctggaaatatgtttcaaaatgtaaactacatgtcctttgaccaggtaattcaacttcttgaaatttatccaaggatttaattggataaatgtttaagatgtatatataagaatgtttactgcagtgttgtttatgattttaaaaaaatggaaatcatcttcatgtctaccaatagagaatgggtgaataaattatggtatgtccatatatacaaattacatagttgttggaaatattaggtagatttagatatactgatgttcaaaaatgtccattatgtaagtgaagctgggtcacagcaccttgtgttgagtatgatttcatctagaaacaaaattactccctcatcctttgttgtgttttagttttttaaaataagcttataccattgggctgggggaaaagtaaatactcgttttggagagagaaaagggcactaaagtttcagataccgttagattatttcatgcttatttttcaagcctcaataaattacataattcacatgtagtcttggattaaggaaattgctattaaggctaaataaataatatgagaggtatataatataaaatatgaacattatattggcattaagattggatccacggtcattccagcctctcattcttacctggacttcaagtgatcacttgtgggcaaatgccatctgacttgaacaggttacacatgtatgctcattatatcgttattttcaaaatttgtcatataaattttccttgagttcattcagatttttgaactagttttttctcttgggagtagtacacacttaattctctctagtactaagctaatgttcaccattcttataattttaagtatccagcatttagtaaagaagtctttgttttctttatccttacttttagtgaatgtcttagtttttaattgaaaattctgccatgaaaataagctctttaacatcttcactccctaatcaaaacagaaatccttcatagccttcagttgtagctatccttccctgtgatttgtccagctccattatatttattttgaaatatggtgaccagttttgcaaaattatttcaactgtaggtgcccagtgattttgtaaggagaagatactgtttctgaacagttctcagtagccagtggcctgcccctactttttggcctgcgtgtagtatataaaataatgcagttaactttttatagcacttttcattttataaagagattttcatggtctttaatattaatctatgtataaagtcctgtatgcagttttacctactttcacagctgaaggaacaatagcttagagaagatgtgagataaagtagtttgcccaagcccatagcacaaataagtgaagttcttcggctgtccatggatcgaagactcccaagtctatctctagcctggacttctgtcctgagcaccagacatgtatgtatatcaagatgcctgcaggtcatatccaccaggacaacccatgagtacagggaattcaacatgcccaatatcactcatcttttccttcgccctcccctttgtactcatcccctgtcggtaagctctgttattttaaaaaattgaaatgtattcacatagcatacaatttacacttttcaagtgtacatggtttttagtatattcacaagggttgtgcagtcattactactaattccagaatgttattatcaccccaaaagtcccacatccattagcagccactccccaatcccttctcccaccagcctctaaaaactgctaatttttccatctctgtggatttgtccactctgattatttcatataaagagaatcgtacagacgtggccttttgtgtctggcatcctccacacaggatgatattttcagagttcgtctatgtttttgcttgttgatcattccttcattcctttttctggctgaataatactctgttatatggatataccttattttgtttatctgttcatttgatgggcatttgagtgatttcctctttttggcaattttgaataatgccactataaacatttatgtacacgtttttgtgtgaccatatgttttcacttctctcgggtgtatatctaaggtacagttgctgggttatatggtagctctgtctttgactttttgaggaactgccaagtggttttggtagtgattgtactgtttacattcctaccaacaattttacctaagtatttctcaaatctatttaatcttttcggtccatactgctgttgctgccttagttcagattttgtcatttcttgtaataattcgtagctcatctcccagtctctgctcccctctctccctccctcccccttcttctctctcttatttccacccatttttaacatttatagaagtcaaaagtctagttcagaaagcagaaaccatactagatatttcagcacagagaactaattaggtgttggaagactgaaaggcaaaaaaacactgaagtaacacagtaacatcaagaatgggcactactcctaagattcagggaatgctgggaagatttggggtttatcagaactggaagctcagaggaggggccccttgtcgctgaggcttaatccctgcagaggtgcctttggctgctactggtgaatctgagtgggtatgatgagtcagtgtctgggaagggccaaaacattttgtccctttctataatttgtcatgataatgctagtaatgaatctgatctcccttcctattttaaaaaccttttagtgattttgtataggatgaagtttaaaactccttacttaatatacacatgaccctccgtaagctggcccctgcttgattgtccagtttcacttcttggtgcttattctaaggcctctaagccttagagatcctctaagcctttgagatccccaaaccctggactgcggactggtacccacctgtgtggcctgtgaggaactgggctgcacagccggaaggaggtgagcattacttgccttagctcctgtcagatcggcagcattagattctaataggagcgtgaaccgtgttgtgaactgcccatgcaaggatctaggttgcatactccttaggagaatctaactaatgcttgatggtctgaggtgaaacagtttcatcctgaaatcacccccaactcggtccttggaaaaattgtcttccacgaaactggtccctgatgccggaaaagttggggaccgctgttctaagctaaagttatatggagctccttggttctgtgtcctcaacatgctgttctatgttttttacattctgtttgctccttcctgcttggaatgtccttcccctccccgtctttcttaatgcatacaaagttgatctctcctgtgtgccaccattgtacttcgtcttgcatatggtgttacattcattttattttaattatttatttacgttcatgtctcttccactcaccttagttgcttgaggtcagaaactatataatgtgtgacacggaatgtgacacctagattttcaataagtgtttctatgatacaagggagactgatgtgggtagatgggaatgaactcatcaacctctgtttacataccctaaattccctgtttcttccctattataattctgacagtctacaaccgtctttgatggcttataaacggaaagtgcggaacacatcattctacagtgaatttaaataacctttcggaagagtaacgtaaagtacttgagcattaattgagtaaaagtttctcatcttttcctacaggtgttattaagcagtatgtaaaaagtccttacaatacttaatacattaagaaaacatacaatttcaagaggaaatccccgagtaatacattattgacattttcagcagttctagttatattgagaagagcatctcatggaattggcagaatgaagatggagattaaatgagatgatgtttgtaatatgcttatgacagtatctggcatataagtaagggctcagtaaatgttgactgctgtaattactattaatagtaatatgattacctttagtaaaagttattagtttctttaggttttttgtttactacaatatagtaaacaaaatctatacttggaatgtatatattgttttgttttgatacatggaatatgtctctgtgtcagagtcactgcctgagttggaaaacccatactcgagtatgttaaaaggtgaacacactgaataatttagttattaattataatggaaaaatgacaaacttgatgttctggttaatgaggttatcttatcttgaatgagttagcttttaaattcctcaaaataaaggcatttaataaaccaggaaacacttcattaaaaaaattatgcaagtcagtgtaaaagaagattaaaattccacatgggcaaaggacacacgttggcgataaatatgcagataagaaaaaaaacctatataacattattactcctcaaagaaattggtatgaaaacaataaaaatgtgtagcttatcaaaccaacaaaaatttaaaaatatgaaatccattttaagtaatgataaaatgggtgcactcttagtgctttatagaatagtagtataatgaacctcatgtgtgtaccaaccagctctttcatatcttaacatttagcaacatttgatttagctctttcttttttccaagatagaaaagttaatattgttgaagactcctgcattcttttccctagtcttattttcttccctcccataaatgtgttaaaatctctgtgtgtattgttttggttgtatttttacataaaactttacatattatataaaatttaattgaaggtaaaatttattaaattattcttaatatatattgtaatttaaaaattaacagcttcattgtcttgataaaatttatggtatcttaaacatgtgcttgtttttctaagagaacattgaaacatagattttaaaacaaattgttgaaagattaaaaaatctgcctttgcacactgttacattgaaagtggggcatttgtcgtgaacattcatttcaaatatgtagtatcttcagaatatttgagaaggatttgtattatataattgaaaaatctgttaaattgtatttatgttaactgcttaattctaataaaatttccattcattttttagtatctgcatatatttacatcaaatggattcattcacttatttaagaggcagtactaattacctatagcgttcaagactgttaggtagagggtgtgtagtggtgagtacaacaggcgtgagccctaccaacacggagtttaaagcctagtagaggatatagacttaaacaatttcacaagtaaatacataattacaaattataatacatgctatgaaggaaacataggaggtaccagagaaggaagagtgctttgcatttttatttttaagaccgaagagtgctattggaggactttgagcaagtgaatgacatgatctaacctaccttcgttcattcattcattcattcattttcttccttcctggctcaagcagtcctcccacctgagctccccaaatagctgggactacaggtacacactaccacacctaatttttttttgtattttttgtatttttgatgggattttaccatgttggccaggctggtcttgaactcttgacctcaggtgatccacctgtctcggcctcccaaggtgttgggattataggtgcctagcccatggtgcctagccctaacctacatttataaactatcacttgctgctgtgtggagactatattgtgagattaacagcagggatacctgctaggaagcaattgctgcagattgcctgagacaaaatagttatcatggactagggggatggtggtggtggtggtggtaggtggttggatgtaggatatattttgaagataggtaaatggtgcaagattatgggtcagttttaaatgcttaagtaaattttctttgtaagacattttaggatgccatgttaagaatctctttataactgtcatttaaaaaaaaaccacatattttcttagcataatttcccatagtaacattactatgtcaaaggctatgaacatttgaatgactttagataaatactgtaattgctttccaaaaatattgtgcttattatgtcaccagaaatgtttgaattctgtctacaattcagtcttgccagtatagtacatttcatttagaaaaattttttactatgtagatggaaaaaataatattttagctgggagtggggggactatggggaataactttccttcatttaatattttattgtgagttagtttaagttactttattttatcgtagtttcctaaggctacaaattagtaaccttggtaacttatgtacctaatttaaaagtttacttttttgaaaggctggaaatactaattaaaaacgtaacaccttcatccttgtctttgctccattattaactagtttcattacagaatctctgtgttttaaaatcagatgggttttcataaccagtactttctcagagtggtaaatttaaaaaaatatataaagagaataaataatatttgttgagaatacttcaaataatgtgaagagttattaacttacagcaggagttggcaaacttttctataaagggccatatgggtctttgtcacaaagtcttgggtttttgtttttgtttttttaaacagctatttaactattcctagctaatgggcaatacaaaaacagtgggcaagatttggcctgtgggcagtagcttgctgaaaccttatttagactctaaattttttgaaagagtctacattgatgcatatttttttttcttcctccaaatacagttgacccttgaacaacatgcgtttgagtgaccatgggtccacttgtgatacacgtttttttcccaaccaaatgcagatatggagggctgacttttcatatacctggatgttcctgggccaactgtaggactagaggctgggggggtcttggaaccaatgccgtgtgtataccagggatgactgtttcttatggcctgacctgaagttggaacagaatctttattaatatataatttttgttgcgtttgttttctctttatatttatccattctttttagatcgtatttcatttaacactttttcttctttagtttttaccaagttgcactgaaaatagctcagtgactaattgcacttctaagagtgaggaccctagttaaaattaactctaaaaatactgaatttttaacctaaaccttttatttctaatcaacagtattatttatgagtaggttatagattactttgaaacggaatgtgtctcagaactttgctatcgatatttttaaggtctggtagggaaaagataataggaatgagatttatcagtgaataggggactgctttcccagtttctcggtcgcactggtgtattcaccatggaagcatcttatgaaatatgtacataaactactaatatcccacattacaggttgactattctttatctgaaatgcttaggacctagaagtatttttggattttggtttttcagagtagggatactcagcctacattggtaagtaaagaatgtgaggtgacaggctgggcgcgatggttgacgcctgtaatcccagcactttgggaggccgaggcggatcacctgaggtcaggagttgaagaccagcctggccaatctgtactaaaaatacaaaaattagctggacacagtggcacgtgccagtagtcccagctactcaggaggctgaggtaggagaatcgcttgaacctgggaggcggaggttgcagtgactcgagatcgtgtcactgccctccagcctaggcaacagagcaagactccatctcaaaaaaaaaaaaaaaaaaaaaaaaaaagaatgtgaggtggcagcaataggtaggaagagtctttggtcagctttacatgctctgtagccatgcctgggtaatgggttgactctaagactctgtgctttgctcccacctcctgctttttcattactctttagaatggtttttaatttgtgatctataggagttctttcaagtatttaataagagaataggctaaattaagtaaatgtcaactgaatgctcaaatctctactaaagagcctcttatttagaaaataaatatccatcttttttttctgactggtgagataattaatttttattacagatggtttggaaaataccatatgctttaaaagataagcacaaaattatagtctaatatgtaggttttcatactttaaaaaattgaaaaccaaagaaaaacatttaacatagcatctagtacaaagaaaagagataagcaagagataaatgtcttttttgggacagagttttgctgttgttgcccaggctggagtgcaatggcacaatctcagctcaccgtaacctccacctcccgggttcaagtgattctcctgcctcagcctcccgagtagctgggattacagtcatgcaccaccaggcccaggtaattttgtatgtttagtagagatggggtttctccgtgttggtcaggctgatctcaaactcccgacctcaggtgatctgcccaccttggcctcccaaagtgctgggattacagacatgagccatcgcacccggccaagataaatgtcttttaaattatctccattaaagacataacctttataacattttgatgtatatattaccagtttttaaacacatagtagatttgtataaatacataaacacatattattgtgatcatgctgcacttagacatctttatattctccttatactgtaaacattttgaaatactttactaacaacatttgtaatgaccattctttctctctttctccctctgatagaatggtctacagagtaattcataaactaaacatactttagaggctgggcgcagtggctcatgcctgtaatcccagcactttgagaggctgaggcgtgcagatcacgaggtcaggagttagagaccagcctgactaacatggtgaaaccccatctctactaaaaaaacagtacaaaaattagccgggcgtggtggcgtgcacctagaatcccagctactcaagaggctgaggcaggagaatcactcgagcccaggaggcagaggttgtagtgagccgagattgcaccacagcactccagcctgggcgacagagcgagactccatctcaaaaaaaaaaaaaaaagatacattaatactatagcctacatgtggaacattaagaaaataattgcttttatgtttatgctttatacctgttgttagccctgcttcttatttcatgatttcatggcttcacattgtaacatccctttaccatattttttgaggactgttttggcagaatgtgtgaaatcttgagcagaagtattacccaaaagtcagaagaaaatcagatttttatttcaagattctgttaaagttacccactcccttcttttacttaatcttatagttgcagttctctctctttttagaaaagaaaaaagaggcccctcaggatttgcagatgaaacaatattgctctttagagatatccatctggctgttagattatttttccacagttttcagaagtggatgaggccattagaatcttgagtattgcccatttccttatgtgtgcctttgactatagataaaatagatgcatgacaattatttataagttgattgatttttcttgtcatttaaatcatcttgaataatagagttggtagagctatcccatttttgaaattattttgttttgtcaataactttttgttaccagcatgtacacttgcattgttgactctccatataatacctttaaaaaatttttttttgtggtaaaatatgcataacataaagtttaccatggtagttttctttcatttgttttgtttttgtttttttgagacggagccttgctctgttgccaggctggagtgcagtggagcgatcttggctcactgcaacctccgcctcccgggttcaagcaattcccctgcctcagcctcctgagtagctgggactacaggcgcccgccaccacgcccggctaatattttgtattttaatagagatggggtttcaccatgttggccaggatgttcttgatctcctgacctcatgatccgcccacctcggcctcccaaagtgttgggattgcaagtgtgagccaccgcgcctagaccatggtagttaattttaagtgttcaattcagtgaccttaagtgtgttcataatgttgtgcaaccatcaccatgttgtctaaccattagcactatctgttttgagaacttttttttatcatcccaaattagaattctgtacctgtcaaatagtccccagtaatcctccctcccccagcccctggtaatctgtagtctacttttcgtctttttgaatttgcctattttaggttcctcatataagtggaattatgtggtatttgtccttttgtgttggcttacttcatttagcataatgttttcaaggttcatctgtgttgtagcatgtatatacaggttgaagcatccgttatccaaaatggttgtgaccagaagtggtttggatttcagattttttttttggattttggaatattcatagatacttaactggttcagcatccctcgtccaaaaatccaaaatcagatggagctcagtggctcatgcttgtaatcccaacacgttgggtggccaaggcaggaggatcgcttgagcccaggagttcaaccagcctgagcaacacaagaccctatctctccaaaaaaaaaaaaaaaaaaaaaaagatgaaagaaaaaaaaatccaaaatcaaatgctccagtgagcatttccttttagcatcatgtcaggctctaaaagttacaggttttggagcattttggatttcagatttttggattaacctgcattaatgctcaacctatatgaaattttattcctttttatggctgaataatgttccactgtatgtatatactacattttgtttatccattcatctgttaacagacacttaagttatttccacattttgggtattataaatagtgctgctgcgaacattggtgtacatgtatctgtttgagtccctgtttttagttattttggttatatacctaggaatggaattgctgatcatatggtaattctgtgtttaactttttgaggaactaccactgttttccacaatggcatcaccattttacattcccaccagcaatgcacaaagatttcagtgtctgtatccttgctaacacttattttccattttttgagtttttttgttttgtttttttaataatagccaatcctaatgggtatgtggtagcatctcatggttttgattttattttcctgactattgatgatgttgagcatcttttcaggtgcttagtggccatttgtccgtcatctttggagcaggaacaatgtcttttcaagtcctttgcccatttttaaattgaattttttgttgttgagttgtatataacaccttttttgaagtaaaaggtgcactgtaataatccagactgtgtttctcccttctcaggattcctacaggaagcaagtagtaattgatggagaaacctgtctcttggatattctcgacacagcaggtcaagaggagtacagtgcaatgagggaccagtacatgaggactggggagggctttctttgtgtatttgccataaataatactaaatcatttgaagatattcaccattataggtgggtttaaattgaatataataagctgacattaaggagtaattatagtttttattttttgagtctttgctaatgccatgcatataatatttaataaaaatttttaaataatgtttatgaggtaggtaatatccctgttttataaatgaagttcttgggggattagagcagtggagtaacttgctccagactgcatcggtagtggtggtgctgggattgaaacctaggcctgtttgactccacagccttctgtactcttgactattctacaaaagcaagactttaaactttttagatacatcattaaaaaagaaaaccataaaaaagaatatgaaaagatgatttgagatggtgtcactttaacagtcttaaaagcaatcgtgtgtatagcatagaattgcttggattggataaacagtggcattatatattttaaaaaataaaagttttgaaagattgaagaatttgggcattacagttctcttaaatctgacaaagctgcataaaactattaaaataatcattattatactattttatattctatttctttgagggtttagttttccaaaaactacatattaagcaaatgaatcactcagtggctatgtcatataataacgagttagcctagttataagaagtttaacattttatttaagaacattgttacagcatgtttactgtatagtctagtaatagaggaaaagacatttgggtgggtggtagtggtagtatttttatagaggagttaccaaatttcagctctattatccaagtttacccagctaatggtgttcggaaccgggaatttgagccaattctgactctgttgtctgctctgctccttcttttgtgctgtgtctttgaaagtcacctaaaattgtgagggaatgtaatttcaccccaaatttagagtttatgcacttgttatattgaaaatgattaacatgtagaagggcttttaatggaataagtggtgtagtaacttcagtgttgcctacctagaaatcaaaatctttctagttgtccactttgttttttgaaaaagtaatatgaaaattatgttaatgctttaattcaggtttttgtaaaatattttttatctttacacatttaacatacgtttctaaaattatagtctgttatatagcactttgggtctagaatttttcagtagtttctgttttactattatgatctacctgcatattaacctattaggttatagttttactatacttctaggtatttgatcttttgagagagatacaaggtttctgtttaaaaaggtaaagaaacaaaataactagtagaagaaggaaggaaaatttggtgtagtggaaactaggaattacattgttttctttcagccaaattttatgacaaaagttgtggacaggttttgaaagatatttgtgttactaatgactgtgctataacttttttttctttcccagagaacaaattaaaagagttaaggactctgaagatgtacctatggtcctagtaggaaataaatgtgatttgccttctagaacagtagacacaaaacaggctcaggacttagcaagaagttatggaattccttttattgaaacatcagcaaagacaagacaggtaagtaacactgaaataaatacagatctgttttctgcaaaatcataactgttatgtcatttaatatatcagtttttctctcaattatgctatactaggaaataaaacaatatttagtaaatgtttttgtctcttgagagggcattgcttcttaatccagtgtccatggtactgcttttggctttggtttctttctacattgaaaatttctcttcaattctgagcacatgttaacatttagaattcaagaggtggggatttttttttcccatggttacatatatatatatatatatatatatatatatatatatatatatatatataaagaacagggcaacaaatttttgcgttttctatttcggtagtacttttaaaccattatgtcatgtttctaggttaaacgttgttgtatttgaagaattttactttggcagaatttttttgaggatgtgtttatttctggagaaaggtctcattaaagaaagacaatacccagaaagccaacagaaattctgttactcatttaatgcatttttctgacaaaaattattgccagagagaacctgaattttgtttcaaaaatcatctttgttttaaaaatgactttttcttcaggtaaaataaaataatttcagttgctattatttaacctgtttgtatgaagagtttaacatataggaaatgaatacataaagataggaaggaattaattgttatatgtagtcatatgtctcttaatgacagggatactttctaagaaatacattgttaggtgattttgtcattgtgcaaacatcatagaatatacttacacaaaccttggtagtataacctactatacacctgggatatgtagtatagtctcttgccccagggatacaaacctgtacagtatgtaactgtactaatgactataaggcaattgttaacacaatggtaagttttgtgtgtctaaacctacacttgggctaccctaagtttatatatttttttaaatttctgttcaataataaattaaccttactttactgtaactttttaaactttttaatttttcctaacattttgacttttgtaatacagcttaaaacacacattatacagctatacaaatttttctttccttatatctttattctgtaagcttttttccatatttaaaattttttgtttgtttttacttattaaacttttttgttaaaaactaagacatgcatgcacattaacctaggcctacacagggtcaggaccatcaatatcattgtcttccacttccacatcttgtcccactggaagatcttcaggggcagtaacacacgtggagctgtcatctcctataataacattgccttcttttggaatacctcctgaaggacctatccaaggctgtttatagttaacttttttttttttttttttttttttttagtaaataggaggagtacactataaaataacaatataggtgctataccattatacaactgacagtgcagtaggtttgtttacaccagcatcaccacaaacacgtgagcaatgtgtcgtactacagtgttaggatggctataacatcactaagcaataggaacttttaaactccattataatcttatgggaccactatcacatatgcaatctcctgtggaccaaaatgtcattatgtggtacatgactgtactaagaaattgatccatctatattccatcaatttgtttagggctttttctggttacatttacctgtgagcccagaaaaccagttttgtagaaattaacttctgtaatgctaggagttaaaaaaaattgctgaacaacttttacattgttaaacatttaaaaacaagcgttctagaagtttatcaaatttcataaaggtgcaaaaatgtaaatgtaaatcattatccagctaatatatatgttgtatttccctagtaggagagcatatgtacctcttcctagttatacaaatttgatatatagtaaagaaacagtaaattctacttcaagtcattttgggaggattaaaaactgaatttctctagtttgaccattgtacagatttatctggcaattttactaaaacctgatttataggttaaacttggtgtatatcatatatcactttactttagaggaattaagatttcacataaatccatttccaggttccaaagaccaggaagaggcttggtttttgtttttctttttactgtctttacagtctccttgacttttcttaggagagaaggtactgagaaaacatgattctaatatttattattttttcttccaacattttcttatgaaacattttcaaatacaaaattgagttttatttaaaacatttgcaaatatactacctagattctaccattgttgttttatatttgctttacttacaacttttaaaagatgctttttataccactgaacattttagcttacatttcacaaagaaaagaaaaaatttaagagactttgcataatgttttaaggggttgcagtaaagaagtgcttcttatattttcttatgcatacaaatcagctgggcttattaaaatccagattctaattcagaaggtttaggtggggaccgagtctgcatttctaacaaactcctaggtggtatttttcttggtacttggaccatactttgagtagaaaagcagtagaggacataaaaagagtcttgttagtcccactttgttgctgtccacttctcatttgataatatcctaaaatagctgtgtctcctttttggtggttgtatgattactacctcagaagtactaattgattcttgctatttgaccttaatactttaatataacacagcattcatatttgatcagaaaactatctggcttccttttataagagatttttaggttttatacagttttgtggccttgggtttttttgtttgatttgtttttttgaaggtatataatatgtaagtagataaacaaatttgatttgtagacatttttatgtggatcatctaattaaaaatggagggatacagtatgaaagaatacttgtacttcttaacagagcactcaacctttcttttacatcctgtttcactgatgttattatgtaatttatgttgctaaactataaattagatatttaatttctgttctttgatttccttttattattaaatggacttgttgatttgcctagaaattaatttgcctttcaaaagtcttattaatcttcctccgttgaaattaatttgatatttgcatgcttctggaagactttaaagagctattccgagtaactgtagagattataaaatgaaatatgggaattttaataaattttacatctccagttactggtgaaaatgtcaagtcctcctttctgcagagtattttgttactcatctgttattcagcttatttatttatttatttatttatttatttttctttctttcttgttttttttttttgagacggagtcttgctttgtcgcccaggctggagtacagtggtgggatcttggctcactgcaggctccgcctcccgggttcacaccattcttctgcctcagcctcccaagtagctgggactacaggcacccgccaccatgccttgctaaatttttgtatttttagtagagacgggtttcactgtgttagccaggatggtctcgatctcttgacctcgtgatccacctgcctcggcctcccaaagtgctgggattacaggcatgagccaccgcgcctggcccttatttgttttttaaacaaaattagtgtgcatatccttgttgtattttatcggcaagttgttttatgccctaacttttggggtcttgatcatgagcctaaaacacgtaaacacccaaaaagaattatattccggttaaaggaacaaaacattcatttagaagttctcatccatgtaaatcagaggctggcaaatattttctgtaaagggccaagatagtaaatgttttaggctttgagggccacaagtggtatctgttgcatttttttttaattatgaccctttaaaatgcaaaaatcgttgttagcttgtgcatagtataaaaataggctggccgcatgctgtggctcatgcctgtaatcccagaaatgaggtgggaagccgaggtgggcacaccacctgaggtcaggagttcgaggccagcctggccaacgtggttgaaaccccgtctctactaaaaatacaaaacttagccaggcgtggtggcgggtgcctgttatcctggctactcaaggggctgaggcagtagaattgcttgaacctgagaggcagaggctgtagtgagcccagatcaagccagtgcacaccagcctggacgaccgagcgagactctgtctcaaaaaaaaaaaaaaaaggctgtggctgcatttggtccattggctgtaatatgctgattcctaattctctgggtaactttagtgtttgattagctactagaagttaggttaaacttttgtattttacaggctaactttaataatcttaaagtaaaacttaacatagttcatggaaaggaaatagaaattttaccctagtactcttttttttttttttttttttttttgaggcagagtctccctctgtcacccaggctggagtgcagtggtgggatcttggctgattgcaacctcctcctcctgggttcaagcaattcttgtgcctcagcctcccgagcagctgggactacaggcacgcaccaccacacctgactgatttttgtatttttagtagagacagggtttcgccatgttggccaggctggtcttgaactcctggcatcaagtgatcctcccatctgagcctcccagtgtgctgggattacagacgtgagtcactgtgcctggtctctagtattttttttttttttgagacggtctcactgttgccaggctggagtgcagtggcgcgatcctggctcactgcaacctccgcttcccggattcaagcgattttcctgcctcagcctcctgagtagctgggactatgggtgcacaccaccacgcccagctaatttttgtatttttagtagagacggggtttcaccatgttggccaatatggtctcaatctcttgacctcgtgatctgcccgtctcggcctcccaaagtgctgggattacaggcgtgagccactgtgcccagctgtactttttaagataagaattgcagggtatatatttttaccaacttaataacttataattttaaaaagctaattacttggctagaatataatgcgttacatattctttacactcagttcagtccatatctgaaaggcaaatagaattattttctgctagtacattgtgtagtccctatgttcctagtgtataaggactgttacctagttcacatttatctgggttgttgacagattttcctggtccctttggacagtgcatggccatgttggcaaaagctgtcaaaattgaaacattgacaccatgagaattgtgtgttttccagtctgctaaaatcaaaagtgggagggttcagtaaggtgaataacagaagcagagttttcggggtatctgttactcctcattcggcttttctgctctctgggggtctcaatttaaatataatgtgaaaattagttttacgaacctaaaaatgttgagtgattcatttcctggttttgttgttaatttctagatatttaaattaattgttagaagaaccccgttaaagaatgctttgcaaaacaacctccttatgtgctatgtctctgtttaatagtagttgagtttgtgtacatgagatcaatattttgaactatagctttttatgagttaaaaattgacggaacagttactgtgcacttgctgtgcaccatggtagtctcccaagtagtggtttttctgcatttcaatagtacatgagataggctgtgggtggcaaggtttcttgagaaagtgagggatgcacagttgggttttagaatacatcttgttcctccatgcccttccccaccaaaaggctggtagtcttgcatttgtatatagttagggtatttgatgtgttgcttccttgacagagttttgcaagaatttgcagatttaacaggaacaaaaacttacttaaaacaaaatctcttagtaaaagcatagtctagcaagatttagaatgatactttggctaacagtactttctctatatggagtgctttgtttccatagcctcacaagtatgttttcagataatagttgagttgaaaatgttgtcaatctcttgattttaaaaaatttacatatttaaagttgtatacttttgttcctacgtattttcagttgttcttaaagtttaataagtgacatttgaaaatgagtatatgtgtataaaaacaaaagtaggctaggcacggtggctcatgcctataatcctagcactttgggaggctgaggcaggcggatcacaaggtcaggagtttgagaccagcctgggcaatatggtgaaacccccctctactaaaaatacaaaaattagctgggtgtggtggtgcatgcctgtagtcccagctactcaggaggctgaggcaggagaatcgcttgaacccggaggtggcggttgcagtgagccgagattgcaccactgcagtccagcctgggcggcagagcgagactccatctcaaaaaaaaaaaacaaaaaaagaaaaagttaaaaaaaaacaaaaaacccccacaaaatgagtatatgtggcaacaagtcctattctcaaaaaaattattgtgtgctagttaagagcttaatgagtagccagtcggtattaaatatctgtttcagctatattttatctttaaaaattatctacagattttggaatgtgaaaaactagtgttttgtttcataggtatatactgtaggcattttaaaaataagagccagtgccagtggtttacagtgtacacaaggataatgttctcatgttctcttgatgtcagtatgactttaaagcatattatcaagaaataactaagtctgaaaaactgtggtaaataactggtactctaaaacctaagtttcttattactaaaaataagaaatggtaaaagtcaccctgtgctgttaattatatgagccactgaggtcctgacactgaattcttggtggtggataataatctcttctttttaattattggcttccaattctctctgcattgctggaaacaaaaatcatatatttcactattggtggtggggatgctgtcactgaaaaagtagacacattcatattgattttagaaataagttaaaatcaaaatttgcttctgctaaattagtagaggaccaatactgtttttctccttcatagtatgttttggtacttctacattgacattataacttttttttttttaaacagaaatagaagtttaca

SEQ ID NO: 12 - protein, 188 aa, Artificial Sequence [sequence omitted]

SEQ ID NO: 13 - DNA, 5306 bp, Artificial Sequence
  KRAS Wild-type  mRNA
ctaggcggcggccgcggcggcggaggcagcagcggcggcggcagtggcggcggcgaaggtggcggcggctcggccagtactcccggcccccgccatttcggactgggagcgagcgcggcgcaggcactgaaggcggcggcggggccagaggctcagcggctcccaggtgcgggagagaggcctgctgaaaatgactgaatataaacttgtggtagttggagctggtggcgtaggcaagagtgccttgacgatacagctaattcagaatcattttgtggacgaatatgatccaacaatagaggattcctacaggaagcaagtagtaattgatggagaaacctgtctcttggatattctcgacacagcaggtcaagaggagtacagtgcaatgagggaccagtacatgaggactggggagggctttctttgtgtatttgccataaataatactaaatcatttgaagatattcaccattatagagaacaaattaaaagagttaaggactctgaagatgtacctatggtcctagtaggaaataaatgtgatttgccttctagaacagtagacacaaaacaggctcaggacttagcaagaagttatggaattccttttattgaaacatcagcaaagacaagacagggtgttgatgatgccttctatacattagttcgagaaattcgaaaacataaagaaaagatgagcaaagatggtaaaaagaagaaaaagaagtcaaagacaaagtgtgtaattatgtaaatacaatttgtacttttttcttaaggcatactagtacaagtggtaatttttgtacattacactaaattattagcatttgttttagcattacctaatttttttcctgctccatgcagactgttagcttttaccttaaatgcttattttaaaatgacagtggaagtttttttttcctctaagtgccagtattcccagagttttggtttttgaactagcaatgcctgtgaaaaagaaactgaatacctaagatttctgtcttggggcttttggtgcatgcagttgattacttcttatttttcttaccaattgtgaatgttggtgtgaaacaaattaatgaagcttttgaatcatccctattctgtgttttatctagtcacataaatggattaattactaatttcagttgagaccttctaattggtttttactgaaacattgagggaacacaaatttatgggcttcctgatgatgattcttctaggcatcatgtcctatagtttgtcatccctgatgaatgtaaagttacactgttcacaaaggttttgtctcctttccactgctattagtcatggtcactctccccaaaatattatattttttctataaaaagaaaaaaatggaaaaaaattacaaggcaatggaaactattataaggccatttccttttcacattagataaattactataaagactcctaatagcttttcctgttaaggcagacccagtatgaaatggggattattatagcaaccattttggggctatatttacatgctactaaatttttataataattgaaaagattttaacaagtataaaaaattctcataggaattaaatgtagtctccctgtgtcagactgctctttcatagtataactttaaatcttttcttcaacttgagtctttgaagatagttttaattctgcttgtgacattaaaagattatttgggccagttatagcttattaggtgttgaagagaccaaggttgcaaggccaggccctgtgtgaacctttgagctttcatagagagtttcacagcatggactgtgtccccacggtcatccagtgttgtcatgcattggttagtcaaaatggggagggactagggcagtttggatagctcaacaagatacaatctcactctgtggtggtcctgctgacaaatcaagagcattgcttttgtttcttaagaaaacaaactcttttttaaaaattacttttaaatattaactcaaaagttgagattttggggtggtggtgtgccaagacattaattttttttttaaacaatgaagtgaaaaagttttacaatctctaggtttggctagttctcttaacactggttaaattaacattgcataaacacttttcaagtctgatccatatttaataatgctttaaaataaaaataaaaacaatccttttgataaatttaaaatgttacttattttaaaataaatgaagtgagatggcatggtgaggtgaaagtatcactggactaggaagaaggtgacttaggttctagataggtgtcttttaggactctgattttgaggacatcacttactatccatttcttcatgttaaaagaagtcatctcaaactcttagttttttttttttacaactatgtaatttatattccatttacataaggatacacttatttgtcaagctcagcacaatctgtaaatttttaacctatgttacaccatcttcagtgccagtcttgggcaaaattgtgcaagaggtgaagtttatatttgaatatccattctcgttttaggactcttcttccatattagtgtcatcttgcctccctaccttccacatgccccatgacttgatgcagttttaatacttgtaattcccctaaccataagatttactgctgctgtggatatctccatgaagttttcccactgagtcacatcagaaatgccctacatcttatttcctcagggctcaagagaatctgacagataccataaagggatttgacctaatcactaattttcaggtggtggctgatgctttgaacatctctttgctgcccaatccattagcgacagtaggatttttcaaacctggtatgaatagacagaaccctatccagtggaaggagaatttaataaagatagtgctgaaagaattccttaggtaatctataactaggactactcctggtaacagtaatacattccattgttttagtaaccagaaatcttcatgcaatgaaaaatactttaattcatgaagcttactttttttttttggtgtcagagtctcgctcttgtcacccaggctggaatgcagtggcgccatctcagctcactgcaacctccatctcccaggttcaagcgattctcgtgcctcggcctcctgagtagctgggattacaggcgtgtgccactacactcaactaatttttgtatttttaggagagacggggtttcaccctgttggccaggctggtctcgaactcctgacctcaagtgattcacccaccttggcctcataaacctgttttgcagaactcatttattcagcaaatatttattgagtgcctaccagatgccagtcaccacacaaggcactgggtatatggtatccccaaacaagagacataatcccggtccttaggtagtgctagtgtggtctgtaatatcttactaaggcctttggtatacgacccagagataacacgatgcgtattttagttttgcaaagaaggggtttggtctctgtgccagctctataattgttttgctacgattccactgaaactcttcgatcaagctactttatgtaaatcacttcattgttttaaaggaataaacttgattatattgtttttttatttggcataactgtgattcttttaggacaattactgtacacattaaggtgtatgtcagatattcatattgacccaaatgtgtaatattccagttttctctgcataagtaattaaaatatacttaaaaattaatagttttatctgggtacaaataaacaggtgcctgaactagttcacagacaaggaaacttctatgtaaaaatcactatgatttctgaattgctatgtgaaactacagatctttggaacactgtttaggtagggtgttaagacttacacagtacctcgtttctacacagagaaagaaatggccatacttcaggaactgcagtgcttatgaggggatatttaggcctcttgaatttttgatgtagatgggcatttttttaaggtagtggttaattacctttatgtgaactttgaatggtttaacaaaagatttgtttttgtagagattttaaagggggagaattctagaaataaatgttacctaattattacagccttaaagacaaaaatccttgttgaagtttttttaaaaaaagctaaattacatagacttaggcattaacatgtttgtggaagaatatagcagacgtatattgtatcatttgagtgaatgttcccaagtaggcattctaggctctatttaactgagtcacactgcataggaatttagaacctaacttttataggttatcaaaactgttgtcaccattgcacaattttgtcctaatatatacatagaaactttgtggggcatgttaagttacagtttgcacaagttcatctcatttgtattccattgattttttttttcttctaaacattttttcttcaaacagtatataactttttttaggggatttttttttagacagcaaaaactatctgaagatttccatttgtcaaaaagtaatgatttcttgataattgtgtagtaatgttttttagaacccagcagttaccttaaagctgaatttatatttagtaacttctgtgttaatactggatagcatgaattctgcattgagaaactgaatagctgtcataaaatgaaactttctttctaaagaaagatactcacatgagttcttgaagaatagtcataactagattaagatctgtgttttagtttaatagtttgaagtgcctgtttgggataatgataggtaatttagatgaatttaggggaaaaaaaagttatctgcagatatgttgagggcccatctctccccccacacccccacagagctaactgggttacagtgttttatccgaaagtttccaattccactgtcttgtgttttcatgttgaaaatacttttgcatttttcctttgagtgccaatttcttactagtactatttcttaatgtaacatgtttacctggaatgtattttaactatttttgtatagtgtaaactgaaacatgcacattttgtacattgtgctttcttttgtgggacatatgcagtgtgatccagttgttttccatcatttggttgcgctgacctaggaatgttggtcatatcaaacattaaaaatgaccactcttttaattgaaattaacttttaaatgtttataggagtatgtgctgtgaagtgatctaaaatttgtaatatttttgtcatgaactgtactactcctaattattgtaatgtaataaaaatagttacagtgac

SEQ ID NO: 14 - protein, 189 aa, Artificial Sequence [sequence omitted]

SEQ ID NO: 15 - protein, 25 aa, Artificial Sequence
  KRAS fragment
QYRLKKISKEEKTPGCVKIKKCIIM

SEQ ID NO: 16 - protein, 24 aa, Artificial Sequence
  KRAS fragment
KHKEKMSKDGKKKKKKSKTKCVIM

SEQ ID NO: 17 - DNA, 12303 bp, Artificial Sequence
  NRas Genomic Sequence
ggggccggaagtgccgctccttggtgggggctgttcatggcggttccggggtctccaacatttttcccggctgtggtcctaaatctgtccaaagcagaggcagtggagcttgaggtaagtttatctcatgcatagtgttcggctttgggctgtggaatgttcaggcgtttcactgatgccagaaatggagcagaatctatcagctggagacaaaggccttgggcgggggtccttccatttggtgcctacgtggggagatctttggagacagaagggagaatgggaaggagttgcggcctggaggcttcctgctagagctgagaagccttcggggagtaataggaagggggatttccattgcttaggctgagggcggggcccaaggactgttgaaaaatagctaaggatgggggttgctagaaaactactccagaagtgtgaggccgatattaatccggtgtttttgcgttctctagtcactttaagaaccaaatggaaggtcacactagggttttcatttccattgattatagaaagctttaaagtactgtagatgtggctcgccaattaaccctgattactggtttccaacaggttcttgctggtgtgaaatgactgagtacaaactggtggtggttggagcaggtggtgttgggaaaagcgcactgacaatccagctaatccagaaccactttgtagatgaatatgatcccaccatagaggtgaggcccagtggtagcccgctgacctgatcctgtctctcacttgtcggatcatctttacccatattctgtattaaaggaataagaggagagaaagtaaaaagttattttgggtatacattcagttatgcaataagcttaacgtgtttatagagaacagttcatttttattagctgctgaagtttctaaaacctgtccagtttttaacagttctgtaaactattgcaaactcagtgttgagttcattcatgagtttcttcatatataacagctctattacatgagaaacacaggccatagtagcgagactgtctgattgtatgggagataataggatggagataaaggattcagagatgagtgttcttcaatatttatttattagctagttgaagcagctgagaccagatgattggagtagcaagaacttgagatttttagtctttatgcctaggattttggtccctgtttgcagtttatttagttgtgtgatattgagcaactgaatctctcccaacctcattttcctcatgttttaaattaccataaacttgtcctgcctaccacacagggatgttatggaaagttaaataatatatttaagttatttatgaatggtaaagcactatgtaatagtacttagggattctattgttattatgagagttcatggtacagattgtcttcagtaagtggcacctaaggctctttaaataaagggttttgccggacacggtggctcacgcctgtaatcccagcactttgggaggctgaggcaggcggatcacaaggtcaggagttcaagaccagcctgatcaacatggtgaaaccccgtctctactaaaaatacaaaaattagctgggtgtggtggcaggcacctgtaatcccagctactcaggaggctgaggcaggagaatcgcttgaaccagaggcagagggtgcagtgagccgagatcacaccacagacctccagcctgggcaacagagcgagacttcgtctcaaaaaataaataaatagataaataaataaagggttttgtaattttgttcagtttagaaatgcctaactttagagattattttaatcaacacctggcctccctaccatctggctactcgtgtttaattgatgaaaactaactctaatgtagccactataaaaaattggttgctaacccttggcaaaatctttattttgagcttaacagctttaatattttacatgaaatgtttaatattttaattaaatatttttaaatgtttgatttattgagcaatttacataagtaaaatacataaattttatgtctacagcccagtgctttttgcgtttctatatagtcatgtagctaccacccagataacagtatagagcacttccagtactccagagagttctccaagtgtgatgacattaaaatacaagtaaaagtcctgttgccataaaaccaaaatgaaagtattttttatatgatctatgcatgtttgtcttcctgagaaattaaacataactataccttgtttggaacctttaagaatttgattcaggaatatttcccaaaggtacatctgtcatgataaaaaaaaaaccttctctgaaacaaaggtatttgtatatttagtcataaacacaaatgatgtatatagggccaggttataattggtggaggtatgtttagatttctttaagtaaaataaacagcacaaataaaacagtccagttcatagcttagtgaaatacactgggtacttaatctgtagcctcctggctgcagtagagttgtcatttgagttactgtgttttcttaatcttttccaggaacacagtgaccatatttcttttctgcaggcatatagaatttggtgggttttcttttatgtagggtgatattggatactttttgtttgtgattatatattagcaatttgagggacaaaccagataggcagaaatgggcttgaatagttagatgcttatttaaccttggcaatagcattgcattccctgtggtttttaataaaaattgaacttccctccctccctgcccccttaccctccacacccccaggattcttacagaaaacaagtggttatagatggtgaaacctgtttgttggacatactggatacagctggacaagaagagtacagtgccatgagagaccaatacatgaggacaggcgaaggcttcctctgtgtatttgccatcaataatagcaagtcatttgcggatattaacctctacaggtactaggagcattattttctctgaaaggatgatctttgtgttctgaatctttatggggaaatgaggttaccacactagggaagatagagctttttaattatgggaagagttggttttaggttgtttgacattgagaatctagggtaattactgaaagttaatactggaatttattttacataatatactgttactataaagtttgataatacataagtgaagcttgctactgggaatgacttggaaccagagttgttgtaattagagatcacgaaggaatttcagagaggaaaacatctccaagaaacatctttcagtatgtaatggaaaagataggccaggcacagtggctcacacctggaatgtcagtgctttgggaggccaaggcgggaggatcactttcagcccaggagttggagaccagcctgggcaacagagcaagaccctgtctctacaaaaataaaaataaaaaaattagtcacacatggtggcagctactcgggaggcagaggtgggaggatcacgtgagctcaggaggtcgaggcatgctcactccactgcactgctgcactccagcctaatcaacagagcaagattctgtctccaaaaaaaataaaaaataaaatgataggagtaagcaaataggaagtccataaagatgaaaacaaagcaagggaacataaagatagactttgtccatagaaccataaagtttcaaagctagattggaccataaaaattctagtacaatattcttattttgcagaatcagaaacagagttcagaatgtcgtttgttaggttttggagtcaggattgttattagtagcagagccaggaccaaaaacccaaagctcctttttcttagcacagtgttcttaaacagaataatataatggttaagaatgagaactctgcctggattgaaacctagctctgtttattagcgacgtgactcaggggctatgtggctttcctaacctataatatggaaataataatacctacctcatagagttgtgaagattacagttttaataaatacgcaaatcactcagaatagtgcctggcacacagtaaatgctacttaagtgttctgcctaaaggcttgagtcttggcttattttctatccatgtgaagatgtctgctctcaaaagcagattggtccaacactgaattcaagtgttcttttcctaacctgttgtacttcccattttttttttgtctaaaagtaatagcagtacttaataaaatgcccacacttggcatgcatctaataaatgttttttgaatttctagaagtcatttttcttctttcttacaagaaatttattcatttttctatatgccttagctcaaaccaaagagtatttaaaacatcttatgaaaatgcatatagtagagcaagataagattaatgaaaaataggcttaagtgagaccaaaaaaataagggtaaaataaacaaatttaggagtgagcatattctgtgattgtgcatgaagttccagtggctttctaaaggtggactacaaatttggtcactgttgtgaaaaggaaagtagccagctgaaagattcagtatctgtatgctgaaagccgttaagttgctcggactagaaggaaattttcccatggatcctcaaagaggcttgtttaatgtaaaaatcagtagtaacctgacagtgacatggtccaggtactttaggctgtcttatcccttaatgtaggctattaccatcaagcacagttttgcaaatagccagtggaatgtagttcagatacatgactttgtgggtaatccaggggtagagactaaaacagtactgtgcagtatgtggttatttacagttaattaagattaaataaaatttaaaaattagttccttgactaccaaatgctcaatagccactagtaggtaccatgttgaacagtacagatatagaccatttccatcatcacataaagtactgttggattgtgttggtcaagacaatctaaagcaattgtttcccaggtgtgctgtgtggtgtgccttacatgtcattgaaaggggtgctgtcaggagttctagatgcttcagcctccctttactaagagcagttcttatgttttctattttatcgcttgggcttccagatacaatgttttgttttaggtttgttttttttgtttgtttgtttttttttttttgagacggagttttgctctggttgcccaagctggatggagtacggtggtgcgatcgcggctcactgcaacctccgcctcccgggttcgagagattctcctgcctcagcttcccgagtagctggaattacaggcgtccaccaccatgcctgactaattttttttgtatttttagtagacttggggtttcaccatgttggccgggctggtttcaaactcctgacctcaggtgatccacccgcctcggcctcccagagggctgggattacaggtgtgaaccaccgtgcccggcctgttttagttttttagagatggagtctccctctgttgcccaagccagagtgcggtggcatgacactctcagggttcaacctctcagggatcaagggatcctcccacctcagcttcctgagtagctggaaccacaggcacatgtgccaccatgcccagctaatttttgtattttttgtagaagcaaggtttcaccatgttgcccaggctggtctcggactcctaggtcaagtgatcctcccacctcaatctcctagagtgctaagactataggcgggagtcaccatgcccagcttcatctacaatttatttgaagaaaatgtttgagcaccacccatcttgaaaagtgatagactgccttccattaaatactgtcacacctagttatttagcagcagtgagcttcactttttatactttagaccttaatctaaagggtgatttctagttgccagttaaatccagagccaagctctttggagaatccaggagcctcactaggtcatgtatcaggataaaatacccatccactcccattagaaggtgagcttgtacttatggcttcctgatggctgctgcaacaagtctaaagcagtctccttagtatacaatgtcttctctaagtggtagaaaaaagcaaaaatactacaagttaatagggctacataaaatttgctagtttcttttttgccctagccatttattccttcctgaaatcttgtctctctctcgctctctctttctctcgctctcactttctttctctttttcttttctcttttcttttctttcttccctttcttttctttcttttttcctgttgcccaggctggagtgcagtggaacaattatggctcactgcagccttgacctttctggacccaggtgatcctcccacctcagtctcccaattagctgggactacaggcatgcgccaccacacccagctataatatatattgtatatatattttttatttataaatatatataaatatatatttatatgtgtaaattatatatatttatatattataaattatatataaatatatatttatatataatatatataatatatatttatttttatatattttatatatattttttggggggggttgggggggatggagtctcactctgtcgcccaggctagagtgtagtggcgtgatcttggctcactgcaatcttcgcctcccaggttcaagcgattctcctgcctcagcttcccgagtagctgggactataggcgcctgccaccacacctggctaatttttgtatttttagtagagatggggtttcaccatattggccaggctggtcttcaactcctgaccttgtgatctgcccacctcaacctcccaaagtgctgggaatacaggcatgagccactgcacccagcctaatctttgtatttttttgtagagaccgggttttgccatgttgcccaggctaatctcaaactcctgggttcaagcagtctgccctcctcagcctcccaaagtgctgagattgcaggcatgagccactgtacccagcctaatcttgtttttcttatgttctgataatatattcccgtttttagggagcagattaagcgagtaaaagactcggatgatgtacctatggtgctagtgggaaacaagtgtgatttgccaacaaggacagttgatacaaaacaagcccacgaactggccaagagttacgggattccattcattgaaacctcagccaagaccagacaggtatggtacagctttcagcatttgtgcaagagtttgcatcagttgattaactctggtagagatgtgatccatattcatattctttgttgttatgcatttttttcatttttatttttttattttttatttttttttaggcagagtctcactctatcttctaagctggagtgcagtggtgtgatctcagctcactgcagcctctgtctcttgggttcaagtgattctcctgcctcagcctcccaagtagctgggactacgggcacatcatcatgcccggctaatttttgtacttttagtagagacagggttttaccatgttgcccaggctggtctcgaactcctggcctcaagcaatcctcccacctgggcctcccagagtgctgggattacaggtgtgagccaccacgcccagcctgttgttaggcatttttagtagtgttctttttcttaacgcttgtttaaacccaaaatgaacttactaatattctgttatggcatgtttactcctgcattaacatccacaaatatttcttgggaagatccttgactaaaaatatttataaacattagttatttctctgtcaacaccagcccgtttatggcttaagcctcctgaatggagtctttagtttaatgtagttttgttccgtgtttctcacattacccttttcctttgcatgaatgtttatttggcaaaatgtgccatttttatatcagcctgttcttgtgattcaataggaatgtgaaatttagtgttctcttccttaaatcaccatattttattttatcagctattcgtttagtaattggaatcttatgtccacataaagagatacaaatgcaagagagcttataatttggattgtgtccgttgagctagctctctcattttttttcattttttccttttatagggtgttgaagatgctttttacacactggtaagagaaatacgccagtaccgaatgaaaaaactcaacagcagtgatgatgggactcagggttgtatgggattgccatgtgtggtgatgtaacaaggtgagcatatggtttcttggcataattacaaatcttagtatatagtattgggcaatttggaggagtgctggtgttattgtctatatgttttttgagtttctgcctatcctcttctgcacattttccatatgacaccctttctgaaagtactgaggtctaaagtgtttaaaacatttgattattccacaggtatctttatatttttggtaacattagaaattataagacattatttatgaaatgtaggcataccctattcctggcaatgaccaggaatttgaaggatcactactttgaaactagttaataaggacatggtttctgttctttttttacagatacttttaaagttttgtcagaaaagagccactttcaaggtaggacaagtttggaaatgtattctcattcctgttaattttgtatatttgtttttcttatactctgaatgtgtcacttatacaaattctgtttctatttcagctgcactgacaccctggtcctgacttccctggaggagaagtattcctgttgctgtcttcagtctcacagagaagctcctgctacttccccagctctcagtagtttagtacaataatctctatttgagaagttctcagaataactacctcctcacttggctgtctgaccagagaatgcacctcttgttactccctgttatttttctgccctgggttcttccacagcacaaacacacctctgccaccccaggtttttcatctgaaaagcagttcatgtctgaaacagagaaccaaaccgcaaacgtgaaattctattgaaaacagtgtcttgagctctaaagtagcaactgctggtgattttttttttctttttactgttgaacttagaactatgctaatttttggagaaatgtcataaattactgttttgccaagaatatagttattattgctgtttggtttgtttataatgttatcggctctattctctaaactggcatctgctctagattcataaatacaaaaatgaatactgaattttgagtctatcctagtcttcacaactttgacgtaattaaatccaactttcacagtgaagtgcctttttcctagaagtggtttgtagacttcctttataatatttcagtggaatagatgtctcaaaaatccttatgcatgaaatgaatgtctgagatacgtctgtgacttatctaccattgaaggaaagctatatctatttgagagcagatgccattttgtacatgtatgaaattggttttccagaggcctgttttggggctttcccaggagaaagatgaaactgaaagcacatgaataatttcacttaataatttttacctaatctccacttttttcataggttactacctatacaatgtatgtaatttgtttcccctagcttactgataaacctaatattcaatgaacttccatttgtattcaaatttgtgtcataccagaaagctctacatttgcagatgttcaaatattgtaaaactttggtgcattgttatttaatagctgtgatcagtgattttcaaacctcaaatatagtatattaacaaattacattttcactgtatatcatggtatcttaatgatgtatataattgccttcaatccccttctcaccccaccctctacagcttcccccacagcaataggggcttgattatttcagttgagtaaagcatggtgctaatggaccagggtcacagtttcaaaacttgaacaatccagttagcatcacagagaaagaaattcttctgcatttgctcattgcaccagtaactccagctagtaattttgctaggtagctgcagttagccctgcaaggaaagaagaggtcagttagcacaaaccctttaccatgactggaaaactcagtatcacgtatttaaacatttttttttcttttagccatgtagaaactctaaattaagccaatattctcatttgagaatgaggatgtctcagctgagaaacgttttaaattctctttattcataatgttctttgaagggtttaaaacaagatgttgataaatctaagctgatgagtttgctcaaaacaggaagttgaaattgttgagacaggaatggaaaatataattaattgatacctatgaggatttggaggcttggcattttaatttgcagataataccctggtaattctcatgaaaaatagacttggataacttttgataaaagactaattccaaaatggccactttgttcctgtctttaatatctaaatacttactgaggtcctccatcttctatattatgaattttcatttattaagcaaatgtcatattaccttgaaattcagaagagaagaaacatatactgtgtccagagtataatgaacctgcagagttgtgcttcttactgctaattctgggagctttcacagtactgtcatcatttgtaaatggaaattctgcttttctgtttctgctccttctggagcagtgctactctgtaattttcctgaggcttatcacctcagtcatttcttttttaaatgtctgtgactggcagtgattctttttcttaaaaatctattaaatttgatgtcaaattagggagaaagatagttactcatcttgggctcttgtgccaatagcccttgtatgtatgtacttagagttttccaagtatgttctaagcacagaagtttctaaatggggccaaaattcagacttgagtatgttctttgaataccttaagaagttacaattagccgggcatggtggcccgtgcctgtagtcccagctacttgagaggctgaggcaggagaatcacttcaacccaggaggtggaggttacagtgagcagagatcgtgccactgcactccagcctgggtgacaagagagacttgtctccaaaaaaaaagttacacctaggtgtgaattttggcacaaaggagtgacaaacttatagttaaaagctgaataacttcagtgtggtataaaacgtggtttttaggctatgtttgtgattgctgaaaagaattctagtttacctcaaaatccttctctttccccaaattaagtgcctggccagctgtcataaattacatattccttttggtttttttaaaggttacatgttcaagagtgaaaataagatgttctgtctgaaggctaccatgccggatctgtaaatgaacctgttaaatgctgtatttgctccaacggcttactatagaatgttacttaatacaatatcatacttattacaatttttactataggagtgtaataggtaaaattaatctctattttagtgggcccatgtttagtctttcaccatcctttaaactgctgtgaatttttttgtcatgacttgaaagcaaggatagagaaacactttagagatatgtggggtttttttaccattccagagcttgtgagcataatcatatttgctttatatttatagtcatgaactcctaagttggcagctacaaccaagaaccaaaaaatggtgcgttctgcttcttgtaattcatctctgctaataaattataagaagcaaggaaaattagggaaaatattttatttggatggtttctataaacaagggactataattcttgtacattatttttcatctttgctgtttctttgagcagtctaatgtgccacacaattatctaaggtatttgttttctataagaattgttttaaaagtattcttgttaccagagtagttgtattatatttcaaaacgtaagatgatttttaaaagcctgagtactgacctaagatggaattgtatgaactctgctctggagggaggggaggatgtccgtggaagttgtaagacttttatttttttgtgccatcaaatataggtaaaaataattgtgcaattctgctgtttaaacaggaactattggcctccttggccctaaatggaagggccgatattttaagttgattattttattgtaaattaatccaacctagttctttttaatttggttgaatgttttttcttgttaaatgatgtttaaaaaataaaaactggaagttcttggcttagtcataa

SEQ ID NO: 18 - protein, 189 aa, Artificial Sequence
  NRas Amino Acid Sequence
MTEYKLVVVGAGGVGKSALTIQLIQNHFVDEYDPTIEDSYRKQVVIDGETCLLDILDTAGQEEYSAMRDQYMRTGEGFLCVFAINNSKSFADINLYREQIKRVKDSDDVPMVLVGNKCDLPTRTVDTKQAHELAKSYGIPFIETSAKTRQGVEDAFYTLVREIRQYRMKKLNSSDDGTQGCMGLPCVVM

SEQ ID NO: 19 - DNA, 4326 bp, Artificial Sequence
  NRas mRNA
ggggccggaagtgccgctccttggtgggggctgttcatggcggttccggggtctccaacatttttcccggctgtggtcctaaatctgtccaaagcagaggcagtggagcttgaggttcttgctggtgtgaaatgactgagtacaaactggtggtggttggagcaggtggtgttgggaaaagcgcactgacaatccagctaatccagaaccactttgtagatgaatatgatcccaccatagaggattcttacagaaaacaagtggttatagatggtgaaacctgtttgttggacatactggatacagctggacaagaagagtacagtgccatgagagaccaatacatgaggacaggcgaaggcttcctctgtgtatttgccatcaataatagcaagtcatttgcggatattaacctctacagggagcagattaagcgagtaaaagactcggatgatgtacctatggtgctagtgggaaacaagtgtgatttgccaacaaggacagttgatacaaaacaagcccacgaactggccaagagttacgggattccattcattgaaacctcagccaagaccagacagggtgttgaagatgctttttacacactggtaagagaaatacgccagtaccgaatgaaaaaactcaacagcagtgatgatgggactcagggttgtatgggattgccatgtgtggtgatgtaacaagatacttttaaagttttgtcagaaaagagccactttcaagctgcactgacaccctggtcctgacttccctggaggagaagtattcctgttgctgtcttcagtctcacagagaagctcctgctacttccccagctctcagtagtttagtacaataatctctatttgagaagttctcagaataactacctcctcacttggctgtctgaccagagaatgcacctcttgttactccctgttatttttctgccctgggttcttccacagcacaaacacacctctgccaccccaggtttttcatctgaaaagcagttcatgtctgaaacagagaaccaaaccgcaaacgtgaaattctattgaaaacagtgtcttgagctctaaagtagcaactgctggtgattttttttttctttttactgttgaacttagaactatgctaatttttggagaaatgtcataaattactgttttgccaagaatatagttattattgctgtttggtttgtttataatgttatcggctctattctctaaactggcatctgctctagattcataaatacaaaaatgaatactgaattttgagtctatcctagtcttcacaactttgacgtaattaaatccaactttcacagtgaagtgcctttttcctagaagtggtttgtagacttcctttataatatttcagtggaatagatgtctcaaaaatccttatgcatgaaatgaatgtctgagatacgtctgtgacttatctaccattgaaggaaagctatatctatttgagagcagatgccattttgtacatgtatgaaattggttttccagaggcctgttttggggctttcccaggagaaagatgaaactgaaagcacatgaataatttcacttaataatttttacctaatctccacttttttcataggttactacctatacaatgtatgtaatttgtttcccctagcttactgataaacctaatattcaatgaacttccatttgtattcaaatttgtgtcataccagaaagctctacatttgcagatgttcaaatattgtaaaactttggtgcattgttatttaatagctgtgatcagtgattttcaaacctcaaatatagtatattaacaaattacattttcactgtatatcatggtatcttaatgatgtatataattgccttcaatccccttctcaccccaccctctacagcttcccccacagcaataggggcttgattatttcagttgagtaaagcatggtgctaatggaccagggtcacagtttcaaaacttgaacaatccagttagcatcacagagaaagaaattcttctgcatttgctcattgcaccagtaactccagctagtaattttgctaggtagctgcagttagccctgcaaggaaagaagaggtcagttagcacaaaccctttaccatgactggaaaactcagtatcacgtatttaaacatttttttttcttttagccatgtagaaactctaaattaagccaatattctcatttgagaatgaggatgtctcagctgagaaacgttttaaattctctttattcataatgttctttgaagggtttaaaacaagatgttgataaatctaagctgatgagtttgctcaaaacaggaagttgaaattgttgagacaggaatggaaaatataattaattgatacctatgaggatttggaggcttggcattttaatttgcagataataccctggtaattctcatgaaaaatagacttggataacttttgataaaagactaattccaaaatggccactttgttcctgtctttaatatctaaatacttactgaggtcctccatcttctatattatgaattttcatttattaagcaaatgtcatattaccttgaaattcagaagagaagaaacatatactgtgtccagagtataatgaacctgcagagttgtgcttcttactgctaattctgggagctttcacagtactgtcatcatttgtaaatggaaattctgcttttctgtttctgctccttctggagcagtgctactctgtaattttcctgaggcttatcacctcagtcatttcttttttaaatgtctgtgactggcagtgattctttttcttaaaaatctattaaatttgatgtcaaattagggagaaagatagttactcatcttgggctcttgtgccaatagcccttgtatgtatgtacttagagttttccaagtatgttctaagcacagaagtttctaaatggggccaaaattcagacttgagtatgttctttgaataccttaagaagttacaattagccgggcatggtggcccgtgcctgtagtcccagctacttgagaggctgaggcaggagaatcacttcaacccaggaggtggaggttacagtgagcagagatcgtgccactgcactccagcctgggtgacaagagagacttgtctccaaaaaaaaagttacacctaggtgtgaattttggcacaaaggagtgacaaacttatagttaaaagctgaataacttcagtgtggtataaaacgtggtttttaggctatgtttgtgattgctgaaaagaattctagtttacctcaaaatccttctctttccccaaattaagtgcctggccagctgtcataaattacatattccttttggtttttttaaaggttacatgttcaagagtgaaaataagatgttctgtctgaaggctaccatgccggatctgtaaatgaacctgttaaatgctgtatttgctccaacggcttactatagaatgttacttaatacaatatcatacttattacaatttttactataggagtgtaataggtaaaattaatctctattttagtgggcccatgtttagtctttcaccatcctttaaactgctgtgaatttttttgtcatgacttgaaagcaaggatagagaaacactttagagatatgtggggtttttttaccattccagagcttgtgagcataatcatatttgctttatatttatagtcatgaactcctaagttggcagctacaaccaagaaccaaaaaatggtgcgttctgcttcttgtaattcatctctgctaataaattataagaagcaaggaaaattagggaaaatattttatttggatggtttctataaacaagggactataattcttgtacattatttttcatctttgctgtttctttgagcagtctaatgtgccacacaattatctaaggtatttgttttctataagaattgttttaaaagtattcttgttaccagagtagttgtattatatttcaaaacgtaagatgatttttaaaagcctgagtactgacctaagatggaattgtatgaactctgctctggagggaggggaggatgtccgtggaagttgtaagacttttatttttttgtgccatcaaatataggtaaaaataattgtgcaattctgctgtttaaacaggaactattggcctccttggccctaaatggaagggccgatattttaagttgattattttattgtaaattaatccaacctagttctttttaatttggttgaatgttttttcttgttaaatgatgtttaaaaaataaaaactggaagttcttggcttagtcataa

SEQ ID NO: 20 - DNA, 35550 bp, Artificial Sequence
  Pmp22 genomic sequence
agttacagggagcaccaccagggaacatctcggggagcctggttggaagctgcaggcttagtctgtcggctgcgggtctctgactgccctgtggggagggtcttgccttaacatcccttgcatttggctgcaaagaaatctgcttggaagaaggggttacgctgtttggccgggtgagttttattggcaaactgtgcctctgggtgatgtgtgcctatgctttacaagaattgcctaatttcccaccccctgcaagccgcaaatgaaaaggattgcaggagagatggtgcatttgtgttggaattgactggagattcagagggctttttatatccttggttaaaaggtggatatatactctggctggggaggtggggggccatctgagagcatctagaaaccctaatgcatccagattgaaaggaagaaaggaatctagatgctttttcccccatggaaaatagctgtgcacacacagctggcaggtggccttggtaagcaggttagggagaagctgccacctgtggcagagccttggccagccgggctctgggtgtggcaagcctggtcagcaggcactgagtagcacttcctctgccaccattgagaaccaggcaggaggccagaggcagtgagggacagatgggttgggtttacctgtctggcagtatatggtgtggctgtgacctgggtggttattgattaaactattgggttcaaaagaaaggaagaagcgagctgtagcacccaatatatgcacttttctgtatgtgtattagactttattaaaaagtttatttgaaaatcacaaaggaagggaaagaaaaccctgagttagatatgctcatatttctaaagtgcttacttagaacagtcctgagtatgttgtgatcacataagtgttggttaaataaataaatgtccaaatggcataaaacaaagtaataatttctagagcaaatctaacttataaaatgacctgtggaggaaagaaaacactgccatgtctttagacttttttttctacttgcatatgcactttcatttataaatctttatctatctatctatatctatctatctatctatctatctacctacctacctacctacctatcagagttacaagctactttagtgcagaggtggtcaggtcttccctgaaaggttgatgtgagagttaaatgtgatataataatagtggtggcaatttgggcactgggcccttattatgttgcagacacgatgttaactgctttgtacatattgtctccttcaatcaccaccataaacctttaaagcaggcattactatttccttttgcacctgagaaaactgaagctcagtgaacttgagaaattgcccaaattcacaacaaaagtaagcagggtgattaggtttgttggagcccagagccagagtgcctaaccactgcaccatactgcctctcacagaccatgcatataaagtccaggcaaagtgcttggcatataacgggcactgtaaatgcagtgtttacaagtacacttcattttaatctgataacacgatagttttaaaaagatcattgtttgaagatctttttcaaatttatttttacttaccgtaagaatatacaattagctaaaatagcagctcctttcaaatcgtaaaataatatagaattatttgaatcattgagagtgatgagcttctatgacacagtacactagaggtagggaagtgtgtgtgtgtgtgtgtgtgcgcgcgcgtgcgtgaactgctgcattttcaggcagaaacctttaacatccacattcctgctccctgtcccgtgcctcaaggctggcctgcgcacgggagtctcagttgggcgcgcctctgccaagccgagactgaagggggctagcctctctccctgtaacgctgggcgggccacgttaggaggctatgaatcagctgatttccttggctgctccaaccccacctcaaatggccacctcgcacccgcccgccaaaccccatggccaggactccagccaaggctgacagccaagcccgactgctgcaggaacactttgcctagagcttattcggtggtagtctggttttgcctaggctaggaggagcccaatcccagaccatgctatccagtagtcggccggacttttcttcccctaattcgcacccaagaggagcccgctagatcaatccccgccaatcctaggaagctggcatgcttcgtaggtgcagacagtaatagcggggaccggcgcggggcaggtgtgtccggctaagacgccaggacagggcaggggctccaggacccgagaggagagggacttcttccagcgctcaagcgcccgctgccctctattagtgggaaaggaatccagcctcagccccgcgcgggcgcggtcggcgtcggcgggcccagaagcccagccctgggcatccgctgagctacatttggctgggtcttcccagagtgggctgaggagccagtttctcggtcaacactaggtctccacggggccaggggagaagggaggtgggaggtgagaaagctcagccgcctctggtttcgagtaaaagtcgccgcggttttgcagggaccgactttttcttgaggcgcatttaaggccaagtgactgtctcctgccctccctctctcctgccccctctcctccctgagtcccgccctcccgcacacgctgacccagggacacaccctactgcagcgacgcaaacagggcgttgttcccgttaaaggggaacgccaggagcctcccactgcccccttgcttcgcgcgcgcgcagccccgcagcgcagctttggcggcgccagcagcggagccaacgcacccgagtttgtgtttgaggccaccctgaggatcgggacagctgttcctttgggctgtaagtgatttggtggggagagtgaaggagatggaggagaaatgtgggcatcttccagtgagggtgccagaaagcgcagcgcaggcgcggggctttggccagctccctggggcttctgtttaggggcacagggtcccctgtgtgtcctgtttccctccaatgggtcttggagtaatacaacgaggagagcctttatggtctataagaccttacagggcaagggtgatggtgctggtgtctggatagcggataagggcggcccagttctcgccttgctgaagaggcgttgactctgggacacactggcaaaacagtccctgtggcggacatcccgagagtgttggactcctgtggttccccagttcccagcctcctgccatcggcttaattcaaaccctctgggagtcatcagaaatccttgtttatttcttccagtgcattccagagtttctttgaatgtgatgcttgtggagaggaacagaggggcctgggattgggtactttccaaactgggttattgaaacgttgtctccctggcccaagactctgcctaaaatggtccccagagtctcagccagatctttcacagccatgcatgtcctctaacaggtcatcccagccttcagttcccccaaagtttaaaatgaggggcgaggaccgcattacttgggataaatgtcctgccggctctgaccggctgaaattctcggactcagccttttaccctctgtctctctctcccgtccgctggacatctactcccttcggtccaggctcctgggctcctgtcccaccgcacccagaccggagctcaggcttgttggggttcgtgtcctggctttgagtgcctggggtgcagactggacccctaggcgagcacgtgggtctagcgcaagagcagaatgccccctgaccccaggggctgcctggggaagcgcgcggtggacgggaagcgcagggtccgggcaaccctctcgagccattcttttctttccacactactctggctctgcaccacctctccggagccgccagagtctgcgcgaggctgagctggggccaggaccgttcctctacgctggcagagttgggtggaaacttggagacaaacggaatgcggagagcactggggtctgggaaaccagcctcctcgccgctgtctcccccaccgcatgccacggctgtctccaggtctcagacggaaatctgggcacctactcccctcacccctacctccaccccataggggaattcaccatctgaaccggggtctcggagaacgtgacctctcaccttccagggaggtcgccgggaggtgcttggggtgggtggaagcgtgcagtggcctctgctcatattttctggaaacccctccgttccctgggtggttttagacgtgcgaaccgcttgttttgtttccaaaagcaaaagatgttccgttgcaggcgggcccggctgggcgctgggcactgggcgctggtcctgcaggcggctgctgccccctctcggcggcaggcggcgcgaaggctcctgacccgcgcgggcggtcgggctgcgggcgctgggccaggccgggccttccgctagtgcgcgggaccctccctctgcgcgcgcctccgtcgctcggcccagtgcgttcggcctcacgcccagcgctctcctcgcaggcagaaactccgctgagcagaacttgccgccagaatgctcctcctgttgctgagtatcatcgtcctccacgtcgcggtgctggtgctgctgttcgtctccacgatcgtcagcgtgagtgcctggcggggaggctccctgcgcggcccgcccttccccatctgggttcccagcccgtgctcctgctggttcaggactgtgttatttgcagacagttggaagtctcagacgtcccagggaagtttctggcaatctgcccccttccagttgctttgagaaaacgagagcagattcagtgataggaaccaagcgagcgctgggctgggttagctgcgcaggtctctatttaagccaagtaacttcagagccgatctagggtccccgaccttcatttgacaagattgtttaacttttttttttcttgatgcagcctcgttgaagaagaggagtatttatgatttttttttctccaaaccatagtcagatgggtgaattaatttataaaacacccttttaggacttgaaattggaaagttaaaatgggcttttctggaaaagagttcacaggtcccatgtcggctttatggcatgaacacaacacattgttagtaaagcttccactggtaggaacaggccatcagagtaacttctgttacaaaactgtccagcccattagatcttaaagttattttcttggcgatgaagatgagcagacattcaggcagttttccagtggtggctttcacttcttaatttaaggcacattgtaagcatgattttctttttcgttttcttttcttttcttttctttttttttttttttttgagatggagtctccagcctgtcacccgggctggagtgcagtgccatgatcttggcttactgcaacctctgccttccgggttcaagccattctcctgcctcagcctgggattacaggtgcccgccaccacgcctggctaattttttttttttttgtatttttagtagagacggggtttcactatgttggccaggcttgtctcaaactcctgacctcatgatccgcccacctctgcctcccaaagtgctgggattacaggtgtgagccaccgtgcccggcctgtaagcatgattttctagtctctgtgagaaataattatgttggggatttgtgacttagtttaacatttacaagcatcttcacagtatctccattgtgcctggtgatgatgatatcagactgataggagctataaacaaggaaatagactgagagaggcgggcttggggaatgatcccgagatgctgggaggagagaaggcttgaatgcaggtgtctaaggttgagttcatggctccttctactatagtaaacatctctgcacataatcgtttctgtgtgcatgtggaacttctccatttacaaggtgcttttaagtcataaaacgttggctcttaccatgcaggggtgggcggtgtggctaggtggatgcgggtgcttttcgccatccctgggcctttctccttccccttttccttcactcctccctccctccctgactcaggatatctatctgattctctctagcaatggatcgtgggcaatggacacgcaactgatctctggcagaactgtagcacctcttcctcaggaaatgtccaccactgtttctcatcatcaccaaacggtgaggctggttttgtgctccatgagcttgtcctcagacgcctgtaacacgtttctcagcccagagctggaaacgcttattggaagacacaagccagaatgtcgttgctggggtggggtgggatgtgacagggagccatgagtccagggaaaatgggaggggtggtgatctcgctggggaagctgagatcctgggcatcattgtgattcactctacctagagacatgcccttagtgccctcctgatcacttaggataatgctttttgtgattgaaaaaaatatcgacctgggagctgtgaaggtggtatgatagctaagcctttggcagacccccttgggacattggatcaaacgtgtatctttggtttggtggctgtctctattcagaaatgtcctgcccctttctgctgcagtgacagtggggctagctcactgcaccgtcagttacatggacacaagactggctgcctttccaggtcttgggcctcagtgatgccacctagcatcaaaacctttgaatgtttccttgttgcaagatggggacttgaagctatttgcaaaaccctaagctaagccttggggtccttaatccagaagatcgtatttctcctctgtcctcagcatctttgcttgtgagatatggaagccaggcttcatgagggtcaaattaagggataattggcagcagaagcaccaactaggtacccaaggcacccagagggaaaggaacacccagccaggagccctgtgtgtttggatgcagacaggtggaggtaaacaggatgagctgttttggtggctgggtaggccatagcgattgatgttaagagcccgtggacctggatccacatgatcttttgttccagaagatgtgtcctcaggctggaaggacctagagatacagcagagctttcctaacatcctgggtttaaaaggccacggaaatacagctttaaatgttgctggagctactcatagatccagtatatatgttcaagatgctacaccagacgagagaaaccagtttagatccagttcagtaaaacaggcagtgaagtggcctttggtcctggctttgcataatccagttgctttgctggactttccctcttacagctcagtacccagtaatacccaagcatgtccccagctgaagcattataaaccaaattccttgaaccacagtacaaatagaaactgctaaaataataatttggtaatttacatggagaagatacgcaaggagtagaaaaccctgctttatgtttttaccttctgggttggggagggagcagagaaaaggtcccagtcctattggagtgagaacagtgcttaatcttgtctctgagtgtgtgaaaggcattgaattaaagccatcccagaaattacgtggtgggtttgcatggtgagttggcaactgagtaaatgaaatactcatgagtgcctgagaatgtgaccgtagcactgcttgtccccaaagccacagcatccggtttctccccctttagggtctggctgaagttcccggagcactccggatgggagtctccgtactcgctactgacacctggtggttacaagtagtgactcagcccgaaaagggcaggctttggtgctcacaggcgccatccccaagtggcatctggccacgcggcttggcacagaatcctggactcttgggcccggaagggggcagttttggcaggcgtgttaaaacccggcgaagtttcagcagaaacgaggcggcagaggagttgctaagttgtgcttaaaccatctgcaggaaagaaagcaatattgacctgtagcatgttacagattgacatttggtgtcttctgccgttggaaatagctgtcagttggtgctagaagcagatctcaaagaggcactagggttattttaatcaggaaacttcttatctctcaacttgttccttctgtgccaagctcatgttcttgagttcatttacaatgcctccttagtgtgggtttcaaatctgcctcgttgctttccgtgaggaccccagagtgtctgttttccacatctcccttctcagctctcacaatcagggcattttgaaaacatctggacactgcacctgaacatgctgggtttgttttcacgccactcaggcttaatctaaatttgaaatttccatttacacttccccagtagtggttatctctgccgctatcttccccaacgtggcagcacttgctacgacttcagccttaagtggcgaatcctccagggcctctttgattgagtttaacaattgtggctgcagacaataagctgaaaaaaatgtgtactttttaaaacattatactgtctttacaaatgaactatgctcattgcgaaccatttaacttgtctgtatttgctcttagaaagtatatttgaaaaaaaatacttgttaagtaatcaaaagtaatttgttattgacatcgatttgtgaagaatatgttgcaagtgtgaaaaaataaatagtggtgcaatctcggctgactacaacctccacctcctgggttcaagcgattttcctgcctcagcctcccgagtagctgggattataggcgcccaacaccacgcctggctaatttttgtatttttagtagagaggggtttcatcatgttgggcaggctggtctcgaactcctgacctcaggagatccacccacctcacctcccaaagtgctgggattagaggtgtgagccactgcgccatgtgacttggtatttttttctgaaaggactcatttttctggtgcatgaccatgacacttcacctctctctgggggttgccactcatgttgttttctacatgaatggggcctcctggcatcgtgccatgaggcagtctaacatctaggttgtgtagtttgaaagagacacaccagatcttgcccccaggctacatcttaatattagaaatagttttagatttttaactaactgactttgactccgcctgccttctcgtttttctaaatgtgtttgtatactttctggcaccccctccttatctgcctcgtgtgggcagaggtaagagaggcttagtgtggggatattcgttatgatattgtatccagtgcctctccggcccagggaatacaaggatctggaatgcatgggccttgccttgatggtcccgagcctggtcgaagagtcaggagatagatatggaagggtgaatcactcccttggaaggcagagcaggccaggtgcccaaagggaggcaggcagacagcgtctgagttcagggaggaagcggatgggaaatctctggtgggaggtagaatctgatccatcctccaaaggatgggcaggatttaagtcaatacaggcaacggggaggagaatattccctgtgacctaaggtaagggtagaacaaggcaggggatggggtagactggttggctagtgttctggttaggattaggattgattgtgtataagagaacatcttcaaatgataggggcttaagtaagatcatttatttttctctcttttcaaagaagtctggaagtaggtagcctgagagaggtatggaggttccatgaaattgtcagagatgcagacactttctagctcatttctttgccatctcttgggtttggctgtcatcttcaggaaacaaaaggctgctagagctccagccatctcatccatgattcaagcagtagggtggagaaaggaggtggggaagaatgaatctccttttcttttaatgaaatgtgacatggtcacacctacacctatttacaagagaggctgagaaatatagtcattcggccttgggggaagcatggcttttcaaatcatagaaacctggcagcaaatacctctctgtaagcctggtgtggaatactttccttgagggtttgaccatcccctcccatacccaatcatactcttttgcaatagctcagttgggccctatgcagttccataagtcccagttatttcagcattcttcaaagagtccatctctgctgcatcctgggctctgtcagccaccccaccattctcacatgggctcttctcagaaactttaggacctgttgaggcttctctctctctatttctaccacctctccaggtataagtaagtcttattattattattgagacagagtttcactcttgttgcccaggctggagttcagtggcgccatcttggctcactgcaacctccgcttcccgggttcaagcaattctcctgcctcagcctcccgggtagctgggattacaggcatgcgccaccacgcttggctaattttttgtatttttagtagagacgggctttctccatgttggtcaggctggtctcgaactcccgacctcaggtgatccacctgcctcagcctcccaaagtgctgagattacaagcgtgagccaccatgcctggccatcttattattatttaatgagtccagacctctcttctgaatcccagacctgtttatccagctgtctcctggccacttcccttgggatatctaagagaggcccccaagtcactaggccagagacagtccttatcttcctctgccaattcaacccctctgtcactttctagtattttagtgaatgctgcttcaccagccagcaagccaaacatctagagtctgccttgacttgacgcgtttccttctttctcttctcagcattgtcacgggtccctcaggccaccccattgttccaatgcctgttgcccacctgtggtcacgctgcttcctcgtttgtcagaggcgccagggcagcctcctaactagtttgcctgaaccctttcttgctcctctgtgactcatttttcatatggaatccaggctgatatttaaaaaagcacaaacctaattatatcactcctcattttgaaacctttcagaggccgttcattggtcttaatcttcagatgaaaatctttaacaaggcccatcggaatctacctgaatgatccactcctgcttctgttaagtctcacctcccatctctcttcccctcatcttggaatttcagcgttttctcacgtcctgaaatgtgaacttcccacttcgggagtctctccatttctcttctgatctttcatgcaggactatttcttgaacaactctcgtgtaccagagactattgcaggtgctaaggttacaagagtgaacaagagcttatgttttactggacaaaccagtcagtaaacatggagaatttgggggcaatggtaagaactatataagacagggtaatgggataaagagggattgcagtggtgaaggaaggtctccttgaggagtggccaggagccagccatatgaacatctcggggaggttccatacagaaggaccgtcaagtgcaagatcgctggggagggaaggagcttggcgtagttgagggacagagggcagggcagactagtgggaacagagagtgaggggtaagtagaatcacagaccatctcaaaggtaccccccacccccactaggaaggagttgggtgcacatggatgcatttctaatctttgtgatttccttagacctgctgtcttccacgggtttctcagtggtccatttgattccaagttggagtgacagtccagaagcctctataaggcagaatatatcagaaattgtacaaggtagaaatgcatcggtatattttcagtgattattttgggtgacgggattcttatcactttggctgttttctttcttttgctgccttacctgttttcctcattgagatcttttattttcacaatcagaaaataactgtgaacattttatgttagaaaattggttttgagtagtaagtaggttccctctgccttgattaagagagtggagccctggggcatggcacgcagggtccatggcgtcgctttgaatgaggccagttcctggagctttagtttgcaaactcatacaatctggaaggctctggtgagggggaggggtgtgccaagcctcctccccaagaccctatgggtgagtttaaaatctactgacccaaaggattcaggcaaaacatttgccctgctattgaatgaaccagtgctttttgttttgaagtctccaagatccaaatatcaagtccaagttctcacaagcattcccctgctttttgtttaatttgtgtggacctgacgtgtagcagaatgggtcagaatactggaattaagccacaggcggcttgggagcccaagagctagaagggcacagtcctggcttgccctggcccctggctggtcttcatcagcttcagtgatgaggcaggacccaggcagtttgtcttcagtaaaatctgtctctcagggcctgtccctgctcacaaagtcctctcttgtctcagaagaaaaggtagttgataaactttttcatgctgaggtgttaggcacaaaaaatgtgcccctttttgaatcacttttgtttttaaaaaggaggccagtgctcaacaccaaagcatgaagggaattgttgagctttcctgtaatctgtccccaaacgtccttggccacctccattgtctaagggcagtacctgcagcccctcatttcccagtgacaacaggtgggtctgctctgccacagtgtgtgggcgggaccagcaccagacgctgagaagatgaccacttactactcttcttttccatttaaacagcagcagcagcagcagcagcagcagcagcagcagcaacagcaaactcatgactatcaataggttgtgtgaggaattagatcaatgctttgggttgaaaattagagaaactaaatcttgccagtctcagcagcccccaacctgagcccttggtggtctcctatcatcgctgtcttcaaaacgatcccagacttgtttatcaatttggtgacactgtcattttggcaaggacaccagacaatttccttgtctgtggctcagcttttggccagattttagaaaacacgggagaccttctgcatttatgggttcatgttttacattttaaaatcttcgtggctccctcagccaacccataatctctacccaaggaatggctctggattttacaggctcttatgagatgctgagaccctggtggtacaagggaggtacagaggacggaatgtgttgtcaacatgccaggatttcaacccttagggtttctctgatgccaatacccaggaattagtatgaaatgtttgtttgaacctgtgtctgaactgtatgacctggaatctatagtctttgctttaaaaaaacttcaattgtatccccaagatttcaccagcaccaagaaaacatcccttgcatttcaggagcagggactggccatggtgcagcctgaggttgtggatgttgatctttggtgcccgagagaaggctgtctgggatgaagccttctgactgtggtcaggtccctgccagtgctgggggccacatgagtgtgcagtcatccacacacaagtggcccccaacactggcagggacccggagtcatctggcccatccctccttcctatcccatcgagccacagacccctctgcaatatgcctaccacatgttcatcctaccactgatggggaacttattaccttcaagagagcctcttttgtttttgaagagctaatagtgagatccattcatgtgttcttcaactctattgagcctgtcctatgtactgggcactgttctagaaatggggtgcacagagatgaacaagaaagagcaggtccctgccattgtgcagctcacaaggagttggaggaaacaggcaatacacaatacatgcatcactatgggtagtggaacatgctctgcaggaaacaaatagggtgatccaatggaaagtcatcactggaggaatgagctgctcagggaaggcctcttccttccatagtgatgtggtctgagatttagaagacagggaaggaccagttataggaagaaccatgggaagaaaattctaggaggtaaagggaagaaccaaggccctgagttagctgaagaaaggagggtggggaatgcgggagagagggatgggagcaggatcgctggtgcctcacaggctgtggtactgagaaggacagttgggacatcattgaagggttttaagcagaagagtgtcatgatttgattcatgttttgtaagctcattctggctgttgagaatgaattctggggagaggcaagagtggaaactggggaccagtgaggagtttgtggtcatagtccagactggacatgatgatgacactgagatgacaatgatgacaatgacaatgatgttaagaatacaaacagctcacgtaagtgccaggcattctttgaaaagcaatgcatttaatcctcacaagaactctaggaggtagctggtggcttagctagggaggggaagtagagaagaaaacaggtctcatgacagggtttgctgatgggttagatgtagggagttagggaagaatgattctagatgactctacgttttgggcttgagcaactggtgtgtaactgaatcttggactgagatggggagactggaggaggaacagaagatttgcgggaaggtgtagaaatcaggatttatattttgaccatcagagaggtcagcaaatcacttcaatttagaagtctttggcttaggggagaggtctgggctggaaattcaaagtcaagagtcattcctctataccgaagggtattcaatgttgtggtgctgaatacagttacttggggaggagttgagagcagaaggcagaaaaggggaacagggttcagagctaagtcttgggcatgccaggggttaacgagggtacaggaaggagaggagactggggatgaacagccagtgatgagggaggaatgccaggagatattgtcacttaagaaattacctcggctgggcgcggtggctcacgcctataatcccagcactttgggaggctgaggcgggcggattacaaggtcaggagattgagaccatcctggctaacacggtgaaaccctgtctctactaaaaatacaaaacaaaattagccgggcgtggtggccggtgcctgtagtcccagctactcgggaggctgaggcaggagaatggcgtgaacccgggaggcggagcttgcagtgagccgagatcgcaccactgcacgccagcctgagcgacagagtgagactccgtctcaaaaaaagaaattaccttgttaaacccaacactgcccctcttttgtccattcacttctagttgccttcattcatgcctgatgtgctggacttgggttttatcaagttgcttggcacgtccttaaagaatttaaatctccacagtgcctcctggacaatgactgcagggtgacccccgtctctcctctacacgatgactcttcaaacagttgacgattgcagtttttctttccttccttctttcagtggcttctctggtgctggtcccagctgcataagcagggcctcttcttgcccttctgaagtttggtcagtggtttggcttggcaggctgatgagcagagaataagggaagccgctctctctttgccacaccattctccttccaccctctctagtttttgtggattctaagtctgaagaatggtggtagaataatttaattcattagattgcaagcatatcattgacttctctgcacccccagtgtgttgtagtggaaaaactagtagtctgggcatcagggaatccttgtttttctgcaccgggtctgcctgtaacaaattaggtaacctggggcaggtaccctggtttcctaaaagcagagcaggcattgaggtaggacctgaagttgaggtaggacctgcacattgcatgggtcccggagcctctgttcatgttcaggatgtaattgtggcatcgagggatcctaaaaggaggtggcctctgagctgggccttggcaatggggtagaattgcagtaggcagagggagcagagatgggttttgtgcttgtaaacgggcattggtttactgtcactggtgggggtagcagctcttttgttctagctcttcatttccataatgcgtgttcttttttcatactttaggggaaagaaggaggagaactctattatttctatggggagaattcctcctaaacctgaagatcttaaaactaagcgaattattccctgttcattctccactgatgcagttcatgactgcaattgcaactgcctttcccgtcattttctatggccaaactcagtgtttttaagtgagctcttcttttaaaaaacaaaaacaaaaacaagtctcctgataaatccgtttgaaagacactaagttttgaaagttaagcaggctttgatcattcatggtacattgtgaattaccaaggagggagattgatatccttcatcgtacaatgcactcccctcctttttcttttgtatctggtggagtaagtcttccaagagcaattcttagagaaacaaagcctactctgtttccctgtttctagagttttccaacaagggtataaaaaagcctcagacagcttactattatccagtaacctcaggtacctcagtggctgcgtgttattccctttagaagtccaaaaactcactagcagagcaagaatatggatgtcaaagtgcagaactagaccctgacaaactagctctgtgcctgccacaaagcctcttaattaggaatgcagttcattgaataactgtatcaaagttagctggaataccttgacatgaagattccttccacttactgagcagtttgtgcccactagtggccagacacaggctttgctctagctaaaatacccccaggattacctgttgagagagccgcccacgtcaccttcatcgcctttgtgagctccatgctggcacatagttgtctccatctgttttgctttccgcatgaatcataggcaaagttagcctgaccagcaagcccatttcaaagccaccagctgggggagaagttgaagcccagggggcaagacccacgctgggctttgggcatgtttgagctggtgggcgaagcatatgggcaaaggccacattgtttaggatggaggcctttcagagactcagctatttctggaatgacattcatactgagaaataaggaaaatggcgatctgtgtgatggttgtgggttgggaggtttgggcgtgggagtcctggtcttggggtcatgtgttttgaaaacagtctagcactatgcaaatgggaggtgttaataactctttgcctctgtgatttaccctctcatggctttttctctcttggcctctccaaggtctcttctgactcttgcaactgtccttcctttcactttcaacaaaacctgttctcttgagtcagaacagttttatgaattgcccagagtgggacttgatatggggcagggttggttccatgctggtaatgaaagatgcacataaactgttacattgaaaagtgcttcatactttctgagcccttaactcactaggttgtaggccctgggctaagaatatagctgagggggctgatgtatttccttcattgctcagctgctcctacagcaggaatctgaccttgaaatgagctttgatctttgtgcaactcgagcttcccactatctgctgggggagctaggtctgggtgctgccacggcccatgtcagaaagctgtcagcagctcttataccggacactctcagaacaggaggcctgcaaagagctttagctttagttttgttgttgttgttgtttttgagacagtctcgctctgtcgcccaggctggagtgcagtggcgccatctcggctcactgcaagctccacctcccgggttcacaccattctcctgcctcagcctcccaagtagttgggactacaggtgcccgccaccacgcccagctaattttttgtatttttagtagagacgaggtttcaccgtgttagccaggatggtctcaatctcctgacctcgtgatccacccgccttggcctcccaaagtgctgggattacaggtgtgagccacggcgcccggccttttttttttttttttttttgagacgagtcttgctctgtttccaggctggagtgcagtggtgtgatctcggctcactgcagtctccgccttccgggttcaagtgattctcctgctccagcctcccaaatagctgggattacaggcacatgccaccacacccagctaatttttgtatttttagtagagacggggtttcaccatgttggccagtatgatctcgatctcctgaccttgtgatccacccgctttggcctcccaaagtgctgggattacaggcatgagccaccacgcccggccagagctttagtttttaattccagtgctcagcaccaaggttggatattggcttaaaacttccactggaaactccacaaatgtttagcaggcctccactttgcaccaggaactgagtgtggcctggaggacagcaggtactcaacataagttctactatttattgcatacttgcaaattgggtggggcgtggggaagagtatcgccacactggggcttgtgttaatctatagtttagccacttgggatgttggtgtcacactaggtttgatctaaatagaacaggtttgtaattgacagcattttcacttgcattatatttctctgaactcgaatcattattttctgtacagctgacttgttttgctgtagcagagtttggcagataatagcttgcatgtcgaatccaacctgcttttgtaaataagattttattggataaatggctattgaaggaatgggtcacacccactcatttacatcttgtccatggctatggctgattttgtgatacaaaggcagaattgagtagttgttaagaagaccgtatgacctgcaaagcctaaagtatttgctctctgattctttatagatagtttgctatctgtgcagatatttgcactctgactctgtagcacccttatgctggagaggagatatgaattgataccaaagttgtatcaaaacacttttggagttctggccaatgtgctaataacctggcttgtgtgaacattgtggctctcattttcttttttcttttttttttttttgagacgagtcttgctctgtcgcccaggctggagtgcagtggcgcagtggcgcgatctcggctcactgcaagctccgcctccagggttcacgccattctcctgcctcagcctccagagtagctgggactacaggcgcccgccaccacgcccggctaatttttttttttttgtatttttagtagagacgggttttcactgtgttagccagcatggtctcgatctcctgacctcgtgatctgccctcctgggcctcccaagtgctgggattacaggcgtgacccactgcgcccggcctgtggctcccattttcatactgcttggtgtgacccagatggaaatgctccagaacctggcccctcaataacagcctgtaaatgcttgtttaccctgttttctcacatcagccttttaggtggggttatttgcactatcctttaacagcgcttcaataacaactcttttgtttgatcattatgacaacccaataaaatatattagtgcctcaagtacgtaaagcagaattcaaggccaaaaaaatgtatgtggcaagttaggtgggcggtcagaagaacttggcaacagagcccagccctgcctgggctgtcctaaccagagcacataaatgctggagagagtcaggctttgcacgtgctcacacgggacccttaccttggacaggatcaaagccctgtcatttctggagtgtgtgatatctgctgtctcttactgcgctggttgttacctgtctattccagttctgatgaatggctctgattggggagcagcatcatctgagcttagaaatgtcctcagggccctgtggggttccctttgagcaacaacgagagctcttgaatcttgcaccagccttttggagctggaatggagtttgctttctcctgggctgggctctgttttttttcctctcgctgtccttgtgtagcttttgatcaatggcactggaggaaaggaaaatcccttgttgttttcctgggcatgtggaagcccagtcctgcccagaattccactagccctttgagttttggaatcctgactcttagtaagtcaatagagtgctgcatctgtttttacctttgtaatcttttaaattggttttaattatttaagtaatacaagtattataatacatgaaaatatcctcaactgaaaggcttcttgaccaaactcttcttcgttgcaacagtagttcctgggggaacccactgacatcaatttgacacaactttggctctttctctacgaatatttgcatgcctgtggatgtctatacgcaattacatagttttttggtgtttgttttcataatgatgacatgttgtgtgtgcaccttactcttttcattgtcttggagacctttcaaagactcttcattttctaactcatgatttttttaactgctgcaaaatatttcattgtgaggatataccataatttattttccctcatagaaatgctacaatcaatgtccttatttattttcctctgagtatatgttcactgtttttccaggatatagtagataagcacttgaacacatatagtgtcattacgctagaggtgttacaatttttaaactacttttaatggcaaaaattacaattacttttgtatcaacctaatatattctgccacaaaatggctggtcacaaaaggattataataataatattattattattcctgtgaatggtgtctgcaggtagctatcacttatttgttctgctgatattatccattttttttgaattttgcctattggctggatgaaaattggtgtcaccctcctcatgggtttctcttgcatttccttggttgctagtgaggttgggcaccttttacgatgtttattggctgttcatatttctcctttgctaatcacatggcttttcaattttatacttagctgttttctctttgttctgtctgtaatttaattttgttaatgatgcgaactagagatttaattttatgttttaccaaatgaatagccaacactatgtattgtctgttgtatttttccccactggtttatatgatgttgtgtattatctaccaaatttacatgtatgcttccaaagtcttattccatcccattcttttatttttctttcatgattaacaccatatttttgaattgctaaaactttataatataaatataagctttgtatgtctataaataaaatacattttattaattataattatatgttatataattataatataagcacttgaacatatatacttctataattatatattatataattatatatcatacttctatgatatgttctataattatatattgtatatatcatagttctatgatatgttctataattatatattataaagttacaattaattgtatatttaatttataccatatactgtaataagcaaaatatagaaatatgttttaaatctggtaggtggtatcttgactcattggttttatatgtttttctgattttctttttgttcatttgttcgttttggtttttagttgctgttgtgtttacttcaaattttttcttatctgtcattgctcattgttttttagatgaatttttaattgatttttttccagttccagttgcaatatggattaggacagcattgaatttgtagattattttggatgaaattggcatctttataactttgagtgtttctatccaggaacttagtatgtttctttagtacttcttttatgtacttgaataaaatttgtctaacttgttgatgtatccccaaagaaccagacatttttattaaatgtattttaatatttttttctgtctcattagtctgtgcttttatccatattaagtcaattaatttttggacttatttcattgttttttttctggcttcttgagttgaaagtgtagttcactctttttaaggatttttctagcaaatgcttagaagtgtatacattgtcctctgagaactgctttggttacaacccacaggtgtgccatgtggctctctatataattccttgctgaagaagtttttacttttcatcttgttttttttaatccgaggaattatctggaacactgtttttaaatttccaaatttattttggctagtttgtttttaatgtctaatttctgtttgcctttaggtatatgttgagcctacatcatttctgcttctatatttattgagatattctttgttgcccttatagtcagtttgaaaagctgtcccatgtgtgtttgaaaataactttgctatatagacacaagttttctatacatctattaggacagatttgttaatcctcttatgtaatctatattctttcttctttttggtctacctgacatctattttgaggaaggaagctaaagtcttctactgttattgtgattttaacaatttcttctcatattttgattactttttgattttaactttttcaggccatgttattatatgcataatgatttattttcttcagtcatagatcatgtaaaccagaagtaaagatcaaataaaccaaatctttcctctatgaaacaaccaaacaactctctggccacttttatcctttcaacataagttctattttttattattaatttatcttctttcttttttgttaacatttgcctgaagcttcttttcagaatcttttttgtttttgactgttgcttgttttaggtgtatctattatattagaatatagctacaatgtctctcttttttttttttttttttttttttgagacagagtctctctctgtgcccaggctggagtgcagtggtgtgatcttggctcactacaacctccacctcctgagttcaagcgattctctgcctcaacctcccaagtagctgggactataggtgtccaccagcacacctggccaatttttttgtatttttcgtagagatggggttttggcatgttggccaggctggtcttgaactcctggcctcaagtgatctacctgcctcagcctcccaaaatgtcttaatcaaagataaaattccatatcttatgagtgccttgaacccattcacatataatgtggttgatgatagacttactatcttaatgcatgtgttttatttattgtgcttatggttgaaaaccatcttcttcatctctggatcatcagagtcaaccagagggcttggctcaaagcagtaggtattcaacaaatgctcattgaataaaaatgtccttgatcctctaattctgatttgattcgagaaataacttatggcaaagagctcaattgtaatggggttgggactaaaattcaagttaatgttgaaagatgtttcaagaagtatttaggttatattattaaatattagacactttctgtttatatagatttaacatataaagattttaagttttctgtgtatgtgaggtctcgtagtagtttctgctgaaaatgacaggggcgcggggttaagggtgaagacagtatctcaggattggagaaggaaatctaagatattgtctccaccagccatactcctcatgaacatgcacatggaaggacatttcccagccaaagtgaatccctttatttgttttagtttcagatttgagtctcagatttctttgtaattccagctgcatctaccaaagtgctagataatttttttattttaagcaaacaatattatgagaacattatctttattgcaaagtgctcctccagaagaacctctatgctggataaagacaaacatttgattaaggttatgtaagagtgaaatcaggatggctcacaacccattagccgtcattttcttactttaattgacaaagaaattgaaaaaatgaaagaagcatatgttgtgcttgaatgtgaagagtgctagactagaatcaaaggcctcttagatttggctgtgtcatttgggctcatgaaaacacctctggaaatctctttcagtgcaaaggagctggactagttgatctctcaggtttcttccaactctaaaatatctccagtctgtgccttggaaacatcttaggtgaaaatctaggaacagttaacctaatttgcacccttaaaattctgccatgagctgcttacaactcaaaacaagtttatcttactcagttactaattataaaccatccagatttcagagctgtgagtactgggtgaagcattgaaggtatgcttttgaagccattacatatggcagttactgagctgaaaggattaaatgctgcagcttccccagttgcccttcctccatgagagcagtgcctgcccccagcattctgtggcacttggaagacaagacagaggccaaatgcagatttttaccctgggcttccctctacagtgtggaactcaggttgtttcttctttcctccctgaaatgacatgagtttgcagcggatggtgaactgaagaaaccataggaggctctgtcttcttgcctgaatttcagttggaagcttggagatttggggttcaacagagataaggaagtgtaagccttcatcccgtctggtggttggcgatcacacaccgctctgtgctgaggctaatggccatgatcagagttgaccaaaaaaaaaaaaaaaaaaaaatacgggttgtccaagcaaattgatttccatacctatagagagcatacctttcttcatcagtattttcttccattcttccaaaaaattactttgggctctaacagccattcccgtgatctttacctctccttggggaatgcagataatttgaatagtggttttaagctatttttcttggaatacagaagttctgataagcccttcaaagacccctgagggcaagaagagggaaggtagtaggcagggctcaggccctctttaacacagacacatgtacataagtaacacatttgcaccaacactggaaggaaattcaatatattttaaaatgactttaactcctagtgatggaactatagatatttttttacagcccttccctgaatgttcacatgtgttttttatatatatgtgtgtgtcacgtatttgtatatgtgtatatacacatatatatagaaacacgtacatatttgtatgcatatttgtacatataggtatatatgtatgtaatgtgtacatattggcacatgtgtgtgtttgtatatgtatatatcagtacatatagatgtatgtatatatgtatatattttttcctccaaaataaacaataaagaatgtcttcttagattgcaaaagtgaattgtctgagttctgctaaggaaaaaggacttctgcttctgctgcctgtgaggactgtgctgtcagcagtcatggcccttcaggccctgcacctcgaggcagagccctcccccggccatggccagctctcctaaccaagtgtctctttcccccagaatggctgcagtctgtccaggccaccatgatcctgtcgatcatcttcagcattctgtctctgttcctgttcttctgccaactcttcaccctcaccaaggggggcaggttttacatcactggaatcttccaaattcttgctggtaagttgtggatggtaaagtccatgtggaagcggggtgcatccaagtctgcggaatgattagtttagtagaaggatgtggcctcagaatgactgatgttcatgagtctccccactggatgctttccataaagtgagggtgggtgcttgtatgtgtgggtgtgtacctgtatgtgtcttagaacttgggacttagaactctccccttctccctggaatgagatgcatatgaaagagaacttagaggatctggaaggaaggtccccacccaagccaggcgtatcaacaggaatgaaactgcaatctggacacataatcagaggtgaatactgaggctatctgtagagcaaaggtcaggcttgagagctgtttctgtagattacattatgcctccagaaaatggccctgatgtgctaagaactagcaaagtagttatcaggtatgtgtcttccaccaataggtagtgatgaagccacactgacaaattctcaccttccttgcttccagttcctagattctactgggctttgattgactgttgtcatcctctggtgtcttcattttgacactcttgtgtcacatattgtcatttccaaacatggggctatgacaacacatgaaaacacatgagaggtctccttaatctcctgcctaaactgtcttcaagttccctctttaaatacgttattaatatgcatagtgtgcagagtcctagaaacttctgttacacagggtgacatcttccaactttgtctctggattctgcctagcatcttacatgcttacatcttacatcttacatcttacatcttgcattctgcctagcatcttacattagctcttacatgtctgtctgttgacttactgttgactgaaccagcagggcattggagagaagtaagagctagatgtagtggtggattctgtggtccaaattcatagatcacaaacttcatatgtaccagagtatgtctaggtactgggagatgttctcaattctgaccctctgagagggcaaaggatgtagcatctcttctctgagttggttgtcagaatgcccatggtaccatttcaccactctgtccccaggagcagtcattggaaggttgacgtaaatagggttgtatgggaagacacagcccaaggttagatgttggtgaccttgtctagaagacagagagttcccctttcctgaaaaaaggaagtaaatgattaaccacttctcattaaacactcaaatacaacatttcaatactcatggttttgagatttcaaaaccagacagtgctttgctacttacacatgtcttatgacaccaagccaagctcctggatggttgctggctctgttaaatgactaattatgcaaggagatatcatttctaggtacgttaaagtgaagagttacccttactcaattttcagttggaataaaaacaactgtaacatattctggggtttctttttttttttctcactcgttttagtttgatatcaaatcaaataatgatcatatccattgcatcagtggatatgccctcaagataatatggatttagaaccagaactttcataatgtatttctattgaaatgttagtttcataagcgatgattgggttttcatgcccatgtgtgagatgtgcctcgctcaaaccttgttatgatttggcacgttacccatctgatgtgaaaaaaattacattttatttgtacaggctcgttattttactgatgaataatttgagcccaccagaggataaatgaatgaccaaggtcacccagctcatgacagggacggttgagtgttacactgaatatagtgaggtacttcttatattttaaagacagaatgcaccaaaaaatttaaagaacacaaaatccaaggcagaagctctgccttttatattatcttttattggaactgatttacaatggaaggtaaatgcaaatttgcaccatgtattattctgaagttccaaacatctgtgatgaatacaagcctgtactataagacccagtcacattgaaaatatggagctgagaagaggtaagctgctgttgaatgggctccttgggatagccagtaccttcatcttcattcatcctgctgagctgtttcggctttaagttctttaacaatgtctttttagcaacatcattacatcattttaggccaaaactcaaagtccagagataagaacccttaagtcactcatgtaactgcactgtgtgttaaaagtatttcagttcagccaaacactcttctcctaggtattgcgatttaagtatatttactaatccactcttgcttcactattttcattctcctccaaagtcaatacaagatgtttagaactgtgctggaagtgcagaattccgaatgtaaaagcgcatgactttgtcctctttatcccctttacatctagctgcttacgtctcatgaaactgaattttcagttatctgttggtccacatttgaataagaaattatcttgaatttgaaatgctgagctgtaatagcagttgtaatttgtaagtcctgagagtgtcctgtcctccgttgttaatcccagtcaagatcatctgagagttggtctccagggaacctcagatctctaggatgttgcactggaaatggctgcaggatctttccactaattctgagaactgaaagagttaggaactctatttggagagttcctggttcccttatcgtgtgacagttctaagtcaattttgtcatgtggttttctgactcacagactagtaagaagttagtaattagagagctaagtagattagggttgttggagatgagaaacccacgttttgggaaaacctggcaagtgacaacttaacatcaaggaagtagtcagaaaagctaaaactgacaaacagaaggtagaagaaagtagctccacactcatgggatgtgaaatctacaagcgtgcatgcccggcaaatgcctctccaatgcactggagcgttttaagtggaaaccactagaatctctgtgtagtctccggaagtggctgtgagggctgcattatctctgcacagcttcctcttggtgggcccagctgtgatctttatggatggcacacatcagctttcaggaaaagcacatgaaaggtgctagggctcttggagctgactgtaggtttgggagttgtctgtctccttgctctagattacagctctgtgtgttgtgtggggtctccatggtttgccaaattatctcttcctcacttagccacaaggctgacagttaggaactatctcttcttgattgcattaggttggctgcttcctgaatgcatatcaaaaggctccttcctttagttcagtgctttcaacctgagctgtgcatcagaatcacctgaggtcctttaaaaaaaaaaaaaagacagtgggcggggcgcagtggctcacgcctgtaatcccagcactttgggaggctgaggtgggcagatcacttgaggtcaggagttcaagaccagcccggccaacatggtgaaaccctgtctctactaaaaataaaaataaaaaaatagccaggcgtggtggtgcgtgcctgtagtcccagctacttgggaaactgaggcagagaagaatcacttgaacctaggaggtggaggttgcagtgagccaagatcatgccactgcactccagcctgggggtgacagagtaagactgtctcaaaaaaaaagaaaaaagaaaagaaaaaagacagtattcaggtctcatccctggagactctcatttaatagttgtgggatggatccactgcctaggtgactctgatgtgcatttagggttgggaaccactgacatagccattaaactgtccctaatcccactgtaaggttttctaggatattttcccagaaataactaaaccaccttcttagagaaggaacatcctgatcctgcgtctggactttggagtcattcttattttcagaacctatagccatctattccttgacaagatctgttgggttgggttgcactagactggaaaacatcaagaaattaatctagacacagacctaaaaggaagatttgcacgttttgatttattttactgcttacacccagcatcaagctccatgtggggcacatagaggagcctgaataaaactattattggttggatgattagataattgtgtttcctcggcagaatcaaactcaagtcaaatgtgtggttaccgggattaagaacagaaagaatagaggggactcctgagtgagtttcactttctctctctttttgttattgttgttcatttgttttgttaatagaaagatcaatatagctatagagcatttaaaataaaaggatttgggccaggtgtggtggcgaatgcctgtaatcccaacactttgaaagactgaggtgagaggattgcttaaagccaggagttcaagaccagcctgggcaacaaagcgagatgccatctctacaaaaaatgatttaaaaattagtggggtgccttggagcacgcctgtggtcccagctattcaggaggctgaggcaggaggattgcttgaggctgagaggtcaagactacagtgaactatgatcaggcccctgcacttgctccagcctggtgacagagtgagaccctgcctctctaggaaaaaaaaaaaaagaatttggtggggggggattaataaaagttcagtgccatcctgttcagagtgattcaaaggtggcttaagtcaaataccacatttagaaatttttgttagggacggatgattatggatgtctcactggccatgcccaaatcagagtcaatgctatgggtggctttctaggcagcaatggtcatttggatactgaaaatgtaaaaggagtgggcttcaatcacagaaacacagagaagtctcttgctttcagaggaacaggcctcacagccccttcctgccctcccttgttgccctgaggatgaagtgggagggagaaaaaggcacccactcatcaacccaacatcatagctgcaccttccagtgaccaccctggtggtctcactgacatccctttccagccaacttctctctgacttctgccccaggctctcaaatgaaagtgcttttgcgaggttaccaaagtacactttgaagtctttaatttgttggatcactctgctcctttcaatactgttagctacttactctttgaagctctattcccctggcttctgagacatcgctgtgttcccacttgcctgagtgaacacaccaggcggtcatgctggcctctcctctctccctcaccccacagccagccttctactgaatcctgcatttgggtagcatcctccgtaggcattacgcccatttctttgtcttgactcactaaccccagtgcagctatgcaaaggcctcctcatgcaccttccagctacctgccttgtccctgcccctgaatccattttctgcaccatggccagagtgatcattctaaaacgtgcgtctgatcatgtttctcctctgctgaagtttcctcagaggcttctcatcacagcttccttaacatgtcatgtaaggccctctctttcctgacccttagtgagctaatcagcctattatatgagagtccgtgtggcttctccagttctccagtttggactcagcgcccgtctatgctcttggggcatctggtgcatttccttccctctctcgaaattccatcgaactatattgaaattatatgcaaatgtctgtcttctagacacacagtccttaaggtaggagccatgtctcacttatcttggtacatctagagcagcagctagaacagggcccgcatgcaataggcactcattaaatgttcactgaaccaaagggaatggagatgataaggatgtactgggaattccctcagctacttcctttgaccttggccccttgggtgcttccttccagaggctctgggctctaatcactctcatggggttgcagtcactgttaaaggagcttaagactttctcttcaaaagggctttaggcagaacttgcaggaagttgttgcagacctacccatcctgagacagggagaaactcttgtaagttgaatgctcagcacatttgtattgtctggacagggtcagtgtccttctgcttaaagatgacctatgctcccagactcaggcccctaccagggagtcccggtcattgccaaagagcagaacatctgcctgtgcctcagggcctcacttacccttgccacagggacctggtgatacatctccacctactggttgctgagaaagtgagtcacagtccacttactaggggtatttggcttttggagatgactactggatgacattaactgtcttgggttgcagacagagggaacccagccaaagaatcatccttttctctatttcagggtacatctattgctttacatgcagacaatcttgtaataatatattccctaaaacatcagtctcatgacaacaatcatataaagtgtgtatcctctctttggctttgtagatatctaagtttactgcttatcacggttaagcttagagtcattcacttctgagattctactaagatgaaagtcatacacattaagctgtgtagttagtcgctgcacttctctatactgcctctttctatccctcttgttcaaggatggaatctggtatctcctcttagtcagtgaaatcggggagtagctggtccactcagctcctgaggcatttctcatgccagatctggttagacagcccatttgggagccctgcctgcatgatgataagtgttgtcctgccctgctagcactctgttaacacctttctctctgccaaggtcatgtttccttttttatagccctgccttcattagataagtcagacagagcccaagagacaacttcagtatttcttaaagacaagagttagcactttggagatgcaagccgtggaagagtggggcaagataattaaggatcctggacctcaaggcaaataaagtgtgtccccagcagatcaaaactgctgttttctgcaatcaacaattaacccgcaatgatttcgctcctgacatggccatctttgctgtcttctgaacttcctgtaggtggcaggtcctggatgctgtcccattttggttccaagactattgtgtggctctcttgacaggggccagtcaagtggcagttttctcctctgagttgcaggaggacaggcttaacagggtggttcatgtggcgtattcccacttctgcactgtcttcaaacaaagttgcagtgtccagtaaaacagcagcccaaatagcagtgaggttagatgtaggtggccgggcggtgggggggcgcgggtgcattgggaactctggaactgcatgaatcccacacggcatactggatttataatagagtcactcagagcttctcaaagaccctgttttcagggaggaaacagaccaggctttgtgcagctccaggctggggtgctgacatcactggacccctccttgtggggggacgctgtctgtcacgtgagctggggccatcagtttgagcgtggctgctccacagggcccaagatggaggcttttcttctctttccaacaccgaagggctgcattggtgggccagggagggtggcctgacccacctgcatatccagtgccctttagccttctttgggcttcaaatgcaaccttggggcacccagggaaatggagcttgcctttgatcatcttccccctctgcagcgtggcttcccagtcatactgtcggctgcatccttattcctcactttctttttccctctccacacatttctttgtctgtttggcagtgcccataggcattgcttgcttcacctggtatgtggcaactctgttagggggaccataggcccctgtggtctgcatggagcttaatccttttaccatggcgtgactccaataatggtaaaatgtcacttcacttccattggctttaggtaatgccaccactcacttgtagagtggcatatagatttccaggggtttccatacccaaccacccttggaaagagacaggtaggtttttcttgcagcctgaatgcctgctggccatgtagtgtggcctgggaattggtgacagtgaaagaaagagaaatagggcagaaaatgtaaagaaaaccctcaggtattaaggcctaggtggccaagattggaaatagagagcaagttgttttccttgttcccatatttttgtgctacctcctttcaattctggacctggaagcagatttccttccagaggtagaaatgttcttcctacccagcaattgtcagcatccggggtggcggagagggggccgctctgccatggactctccgtcacccagcttgtccctctccttccccaggtctgtgcgtgatgagtgctgcggccatctacacggtgaggcacccggagtggcatctcaactcggattactcctacggtttcgcctacatcctggcctgggtggccttccccctggcccttctcagcggtgtcatctatgtgatcttgcggaaacgcgaatgaggcgcccagacggtctgtctgaggctctgagcgtacatagggaagggaggaagggaaaacagaaagcagacaaagaaaaaagagctagcccaaaatcccaaactcaaaccaaaccaaacagaaagcagtggaggtgggggttgctgttgattgaagatgtatataatatctccggtttataaaacctatttataacactttttacatatatgtacatagtattgtttgctttttatgttgaccatcagcctcgtgttgagccttaaagaagtagctaaggaactttacatcctaacagtataatccagctcagtatttttgttttgttttttgtttgtttgttttgttttacccagaaataagataactccatctcgccccttccctttcatctgaaagaagatacctccctcccagtccacctcatttagaaaaccaaagtgtgggtagaaaccccaaatgtccaaaagcccttttctggtgggtgacccagtgcatccaacagaaacagccgctgcccgaacctctgtgtgaagctttacgcgcacacggacaaaatgcccaaactggagcccttgcaaaaacacggcttgtggcattggcatacttgcccttacaggtggagtatcttcgtcacacatctaaatgagaaatcagtgacaacaagtctttgaaatggtgctatggatttaccattccttattatcactaatcatctaaacaactcactggaaatccaattaacaattttacaacataagatagaatggagacctgaataattctgtgtaatataaatggtttataactgcttttgtacctagctaggctgctattattactataatgagtaaatcataaagccttcatcactcccacatttttcttacggtcggagcatcagaacaagcgtctagactccttgggaccgtgagttcctagagcttggctgggtctaggctgttctgtgcctccaaggactgtctggcaatgacttgtattggccaccaactgtagatgtatatatggtgcccttctgatgctaagactccagaccttttgtttttgctttgcattttctgattttataccaactgtgtggactaagatgcattaaaataaacatcagagtaactcact

SEQ ID NO: 21 - DNA, 1828 bp, Artificial Sequence
  Pmp22 mRNA
agttacagggagcaccaccagggaacatctcggggagcctggttggaagctgcaggcttagtctgtcggctgcgggtctctgactgccctgtggggagggtcttgccttaacatcccttgcatttggctgcaaagaaatctgcttggaagaaggggttacgctgtttggccgggcagaaactccgctgagcagaacttgccgccagaatgctcctcctgttgctgagtatcatcgtcctccacgtcgcggtgctggtgctgctgttcgtctccacgatcgtcagccaatggatcgtgggcaatggacacgcaactgatctctggcagaactgtagcacctcttcctcaggaaatgtccaccactgtttctcatcatcaccaaacgaatggctgcagtctgtccaggccaccatgatcctgtcgatcatcttcagcattctgtctctgttcctgttcttctgccaactcttcaccctcaccaaggggggcaggttttacatcactggaatcttccaaattcttgctggtctgtgcgtgatgagtgctgcggccatctacacggtgaggcacccggagtggcatctcaactcggattactcctacggtttcgcctacatcctggcctgggtggccttccccctggcccttctcagcggtgtcatctatgtgatcttgcggaaacgcgaatgaggcgcccagacggtctgtctgaggctctgagcgtacatagggaagggaggaagggaaaacagaaagcagacaaagaaaaaagagctagcccaaaatcccaaactcaaaccaaaccaaacagaaagcagtggaggtgggggttgctgttgattgaagatgtatataatatctccggtttataaaacctatttataacactttttacatatatgtacatagtattgtttgctttttatgttgaccatcagcctcgtgttgagccttaaagaagtagctaaggaactttacatcctaacagtataatccagctcagtatttttgttttgttttttgtttgtttgttttgttttacccagaaataagataactccatctcgccccttccctttcatctgaaagaagatacctccctcccagtccacctcatttagaaaaccaaagtgtgggtagaaaccccaaatgtccaaaagcccttttctggtgggtgacccagtgcatccaacagaaacagccgctgcccgaacctctgtgtgaagctttacgcgcacacggacaaaatgcccaaactggagcccttgcaaaaacacggcttgtggcattggcatacttgcccttacaggtggagtatcttcgtcacacatctaaatgagaaatcagtgacaacaagtctttgaaatggtgctatggatttaccattccttattatcactaatcatctaaacaactcactggaaatccaattaacaattttacaacataagatagaatggagacctgaataattctgtgtaatataaatggtttataactgcttttgtacctagctaggctgctattattactataatgagtaaatcataaagccttcatcactcccacatttttcttacggtcggagcatcagaacaagcgtctagactccttgggaccgtgagttcctagagcttggctgggtctaggctgttctgtgcctccaaggactgtctggcaatgacttgtattggccaccaactgtagatgtatatatggtgcccttctgatgctaagactccagaccttttgtttttgctttgcattttctgattttataccaactgtgtggactaagatgcattaaaataaacatcagagtaactca

SEQ ID NO: 22 - DNA, 483 bp, Artificial Sequence
  Pmp22 Coding sequence
atgctcctcctgttgctgagtatcatcgtcctccacgtcgcggtgctggtgctgctgttcgtctccacgatcgtcagccaatggatcgtgggcaatggacacgcaactgatctctggcagaactgtagcacctcttcctcaggaaatgtccaccactgtttctcatcatcaccaaacgaatggctgcagtctgtccaggccaccatgatcctgtcgatcatcttcagcattctgtctctgttcctgttcttctgccaactcttcaccctcaccaaggggggcaggttttacatcactggaatcttccaaattcttgctggtctgtgcgtgatgagtgctgcggccatctacacggtgaggcacccggagtggcatctcaactcggattactcctacggtttcgcctacatcctggcctgggtggccttccccctggcccttctcagcggtgtcatctatgtgatcttgcggaaacgcgaatga

SEQ ID NO: 23 - protein, 160 aa, Artificial Sequence
  Pmp protein sequence
MLLLLLSIIVLHVAVLVLLFVSTIVSQWIVGNGHATDLWQNCSTSSSGNVHHCFSSSPNEWLQSVQATMILSIIFSILSLFLFFCQLFTLTKGGRFYITGIFQILAGLCVMSAAAIYTVRHPEWHLNSDYSYGFAYILAWVAFPLALLSGVIYVILRKRE

SEQ ID NO: 24 - DNA, 16 bp, Artificial Sequence
  proviso seq
atcttcaatcaacagc

SEQ ID NO: 25 - DNA, 2108 bp, Artificial Sequence
  CEBPb  NC_000020.11:c50192690-50190583
ttactgcccccaaaaggctttgtaaccattctcaaaaaaaagtttattaaaagtgttcttaatgcttgaaacggaaaagattcccaaaatatacagacgcctcttttctcatagaaatagattattttttataatacaaaaaaagaccaaaaaacaaaacaaaacaaaacatcaacagcaacaagcccgtaggaacatctttaagcgattactcagggcccggctgacagttacacgtgggttgcgtcagtcccgtgtacacacgcgttcagccatgtttaaaccgattgcatcaacttcgaaaccggcccgcccgccggcgcctggagaggggcagagggagaagcagagagtttatcattcatctgtacacatagacgtttcttctttaaataacaccacgggcgggagccccatctgcatgtgcggttggtttggacaaaaatatagatatatatatataataaaatattaaaattaccgacgggctccccgcgctgccaagtgccccagtgccaaagttttgccggcgccgccgggggcgggggcgagggcgcgggcgcgggcgctccccggagtctcagccccggccggcagggggacgcgcgcgggggccgcgctagcagtggccggaggaggcgagcaggggctcgggcagctgcttgaacaagttccgcagggtgctgagctcgcgcgacagctgctccaccttcttctgcagccgctcgttctcggccgtgagctccaggaccttgtgctgcgtctccaggttgcgcatcttggccttgtcgcggctcttgcgcacggcgatgttgttgcgctcgcgccggatcttgtactcgtcgctgtgcttgtccacggtcttcttggccttgctcttgacctgcgagggcgccggcgcggcccccgcgtagcaggcggtcgggggcgccttggcgtcagcggggctcggcgtgccgggcgggctggacgaggaggacgtggagaggctcccgctgctgccgctcggcaccgcctggtagccgaggtaagcgcgcagcgcgtacgggaagcccgccgccatgcctgcgccgccgcccggcgccccggcctcctccttccgcttgcagtccgcgggctcgaagcccggctccgccttgagctcggcgggcggcggcggcggcgggggcggtgggtgcaggggcgcgaagcagccggggtgcagcgcgcccttggcggcccccaggcgccccaggctcacgtagccgtactcggccggcttcttgcagttcttgcccccgtagtcgtcggagaagaggtcggagaggaagtcgtggtgctgcccggaggaggcgggcgcgggggcgggcgcgggcggagccgcctcgaaggtgtccgtggccgtggcgggcgccggggcctgcggcgcgcccagcggctccaggtacgggctgaagtcgatggcgcgctcgtggtcgccgatgctgcccagctcgccggcgggggggcgcggcccgggtctggccgcggggggcgccgcgggggccgccttgccgccgtacgcagcagccaagcagtccgcctcgtagtagaagttggccacttccatggatttaaaggcaggcggcggcggcggcagggggagacatgctgggtcccaggccaccaggcgttgcatgaacgcgggtgcccggggagggggcctggggctgcccgctccggccggcccgcaggtggcgcggcctccctgctctgagctgtcgccgctgcgtcgctgctgctgctgccgccgctgccggggtggccgctattagtgagggggctggtggctggaccctcgggtgggtccccttcccagtcccgtgcgcggctctgactcgctaaagtttctcctgagcccggttatttataagggcggcccgtagcaaccgctgcgtcacgccggcccctcccgccgcgccgccgggacgcgaaggacacggccgcggccgcccgagacccccgggaggacggcggcagggcgcagcggagggaccgggcacccggagcgcgttttcggggggcccccgggacgcaggggcggcctcacgccccctgcccacccccgcccggccgccccgggattggga

SEQ ID NO: 26 - protein, 345 aa, Artificial Sequence
  CEBPn Amino Acid
MQRLVAWDPACLPLPPPPPAFKSMEVANFYYEADCLAAAYGGKAAPAAPPAARPGPRPPAGELGSIGDHERAIDFSPYLEPLGAPQAPAPATATDTFEAAPPAPAPAPASSGQHHDFLSDLFSDDYGGKNCKKPAEYGYVSLGRLGAAKGALHPGCFAPLHPPPPPPPPPAELKAEPGFEPADCKRKEEAGAPGGGAGMAAGFPYALRAYLGYQAVPSGSSGSLSTSSSSSPPGTPSPADAKAPPTACYAGAAPAPSQVKSKAKKTVDKHSDEYKIRRERNNIAVRKSRDKAKMRNLETQHKVLELTAENERLQKKVEQLSRELSTLRNLFKQLPEPLLASSGHC

SEQ ID NO: 27 - DNA, 2113 bp, Artificial Sequence
  CEBP NM_005194.3
tcccaatcccggggcggccgggcgggggtgggcagggggcgtgaggccgcccctgcgtcccgggggccccccgaaaacgcgctccgggtgcccggtccctccgctgcgccctgccgccgtcctcccgggggtctcgggcggccgcggccgtgtccttcgcgtcccggcggcgcggcgggaggggccggcgtgacgcagcggttgctacgggccgcccttataaataaccgggctcaggagaaactttagcgagtcagagccgcgcacgggactgggaaggggacccacccgagggtccagccaccagccccctcactaatagcggccaccccggcagcggcggcagcagcagcagcgacgcagcggcgacagctcagagcagggaggccgcgccacctgcgggccggccggagcgggcagccccaggccccctccccgggcacccgcgttcatgcaacgcctggtggcctgggacccagcatgtctccccctgccgccgccgccgcctgcctttaaatccatggaagtggccaacttctactacgaggcggactgcttggctgctgcgtacggcggcaaggcggcccccgcggcgccccccgcggccagacccgggccgcgcccccccgccggcgagctgggcagcatcggcgaccacgagcgcgccatcgacttcagcccgtacctggagccgctgggcgcgccgcaggccccggcgcccgccacggccacggacaccttcgaggcggctccgcccgcgcccgcccccgcgcccgcctcctccgggcagcaccacgacttcctctccgacctcttctccgacgactacgggggcaagaactgcaagaagccggccgagtacggctacgtgagcctggggcgcctgggggccgccaagggcgcgctgcaccccggctgcttcgcgcccctgcacccaccgcccccgccgccgccgccgcccgccgagctcaaggcggagccgggcttcgagcccgcggactgcaagcggaaggaggaggccggggcgccgggcggcggcgcaggcatggcggcgggcttcccgtacgcgctgcgcgcttacctcggctaccaggcggtgccgagcggcagcagcgggagcctctccacgtcctcctcgtccagcccgcccggcacgccgagccccgctgacgccaaggcgcccccgaccgcctgctacgcgggggccgcgccggcgccctcgcaggtcaagagcaaggccaagaagaccgtggacaagcacagcgacgagtacaagatccggcgcgagcgcaacaacatcgccgtgcgcaagagccgcgacaaggccaagatgcgcaacctggagacgcagcacaaggtcctggagctcacggccgagaacgagcggctgcagaagaaggtggagcagctgtcgcgcgagctcagcaccctgcggaacttgttcaagcagctgcccgagcccctgctcgcctcctccggccactgctagcgcggcccccgcgcgcgtccccctgccggccggggctgagactccggggagcgcccgcgcccgcgccctcgcccccgcccccggcggcgccggcaaaactttggcactggggcacttggcagcgcggggagcccgtcggtaattttaatattttattatatatatatatctatatttttgtccaaaccaaccgcacatgcagatggggctcccgcccgtggtgttatttaaagaagaaacgtctatgtgtacagatgaatgataaactctctgcttctccctctgcccctctccaggcgccggcgggcgggccggtttcgaagttgatgcaatcggtttaaacatggctgaacgcgtgtgtacacgggactgacgcaacccacgtgtaactgtcagccgggccctgagtaatcgcttaaagatgttcctacgggcttgttgctgttgatgttttgttttgttttgttttttggtctttttttgtattataaaaaataatctatttctatgagaaaagaggcgtctgtatattttgggaatcttttccgtttcaagcattaagaacacttttaataaacttttttttgagaatggttacaaagccttttgggggcagtaaaaaaa

SEQ ID NO: 28 - protein, 322 aa, Artificial Sequence
  CEBPb Iso 2
MEVANFYYEADCLAAAYGGKAAPAAPPAARPGPRPPAGELGSIGDHERAIDFSPYLEPLGAPQAPAPATATDTFEAAPPAPAPAPASSGQHHDFLSDLFSDDYGGKNCKKPAEYGYVSLGRLGAAKGALHPGCFAPLHPPPPPPPPPAELKAEPGFEPADCKRKEEAGAPGGGAGMAAGFPYALRAYLGYQAVPSGSSGSLSTSSSSSPPGTPSPADAKAPPTACYAGAAPAPSQVKSKAKKTVDKHSDEYKIRRERNNIAVRKSRDKAKMRNLETQHKVLELTAENERLQKKVEQLSRELSTLRNLFKQLPEPLLASSGHC

SEQ ID NO: 29 - protein, 147 aa, Artificial Sequence
  CEBPb Iso 3
MAAGFPYALRAYLGYQAVPSGSSGSLSTSSSSSPPGTPSPADAKAPPTACYAGAAPAPSQVKSKAKKTVDKHSDEYKIRRERNNIAVRKSRDKAKMRNLETQHKVLELTAENERLQKKVEQLSRELSTLRNLFKQLPEPLLASSGHC

SEQ ID NO: 30 - DNA, 75245 bp, Artificial Sequence
  STAT3 Genomic Sequence
gaattatgcatgacggcgtgcctcggccaggctggggctgggcgaggattggctgaaggggctgtaattcagcggtttccggagctgcggcggcgcagactgggagggggagccgggggttccgacgtcgcagccgagggaacaagccccaaccggatcctggacaggcaccccggcttggcgctgtctctccccctcggctcggagaggcccttcggcctgagggagcctcgccgcccgtccccggcacacgcgcagccccggcctctcggcctctgccggagaaacaggtgaagggggtgcagggtggggccgttggggaggcctggggacccgggggctccgcagcggcagggggcctctgggaccttggggatgttgtgatggacgctgcagtggggccgggagagatgaagagacgcggagggtcgccctgagggaagactcttcgggatgacaggagcgggcctcggaagggactcggggcgctggagggaagtttcgttcttcggagaaacagaacgcgctcgagggggcaccgtggggcgagggcgcactcggttgcggcggcaggagtgagggacagtcccccgatttcctgctccctggggccctggggacgttccggccaccggagcgactgtcacgccgacggggatcaccggcgcgagtggggggtcggaaagcgcctcctccccgcccggtcggcggctcccgctgagccacttcctccgcttgccctgttcccgctccttcaggagacagctgtgcccttttggaggcaggaataggtgtgtctgtcgcctgcagccttacgggctggctggtcgtgggtaggctttattgcataagaatcaagtttcctgtagggaaattgacagaccggtactctttctaaattccctcgcatctttttctaggttaaattatgctccccccacgtccccgccttgtaaaaaagagaaaaaaagacaaaataaaatccccatcaacccgtcaagccagctctagagagagaaataaacctcttgacattgtccttttccaaatacctggtaaagtcggccagaagataaataattgagccattgcatttactggattgtggtgttgcttaattgcataggacggaatgaaccaattgagagtgggagttttctgtctcagagccaagatcttgggtaaatgcagaggagagggaaacaaagacaggctggccttgaaaaaaccatgtgtgcaaactttacatgcatttggggggtgtggttgcactgaagttaacaagattcaaaccgtcgcccaagttggtatttccatgtttggtacacatcactctgtgccatatcaggtcgttgttaagtgtggtgacaaaatcagtggttagtcatttttttaattaaaaatgtgtatagtgtgtacctgctggtcttactgtatgtgcaactaaaggtttacatagtctgtgtatgggttgtaaatttttggctggctgtgctgataaagcattgggcttgaataaagcaaagcagaaaatcatctcaatcttttatatgtggatttagactgtgttatgacttggttcagccagttttctatcttattttatattaaatatgtctgtgttctctgagtcagcacatttatttccttattacatgttccagacaggagtgctagcccagtttttgttcagtttgcacagtgggatggggaaacaagtctggaatttaaaaaaaaatgttttagaggttggagccttgattttagtctctatattagcacatccatcacaaagaaccattagtaaattcatgaatcttttgttttttatgtagttcatttgagaagaataatcacttagaaatatccacagtgccaggcatggtggtgcacacctctgatcccagctaattgaaggctgaggtgggaggattccttgagtccaggagttgagtctggtctgggcaacatggtgagaggccaggaattgggtctagagtctagtctaagcaccataatgagaacccatctttaagaaagaaagaaaggaaaggaggaagaaaggaaagaaaaagaaatacccacagcacagttatgaattaacccacaaaggacttgtgaggtgggtagttcacataacaattaccctaatatcgtagataagaaaattgaggccaaaggatcaagacacttggccaacgcagcagagtgccatagtggtggaatttgtgcctccttctgtatattttgtgaaaagtatcagtgaaattctttttttttttttttttgagtcagagtcttgctctgttgcccaggctagagtgcagtggcgcaatcttggctcactgcaacctctgcctcctgggttcaagcgattctcctgcctcagcctcccaagtagctgggactacaggcgtgcgccaccacgcccagctaatttttgtatttttagtagagaccggggttttaccatattggccaggctggtcttgaactcctgaccttgtgatttgcccacctctatctcccaaagtgctgggattacaggtgtgagccaccgcgcccagtaagtatcagtgaaattctaacatatatctgaacagtaaaataccaccaataggctgaaagacttcatgggaggtaaatattcaataaacaggtgaaaaaagaaatacaaatggagcttgcttagattatttttctaattgctatgtctaacttgggaagtgaggaactgtttttggtcagcataatttaccatcagaatttagctatttactaatgaaaagaaatactaatctaggtttgttttagattaaggacagtcatgacctaaatgtcatttaaaccagagtgcattgtggcttgatcagtggtcatttctgtctctagaaagttgctttaacttctctgcctctacgtgtctcttgacattcagatatgaggtggggtagaggtggtgaccaactttccagacgcctgagtccaaaccttcttagcttatggttttcttaggtgatgtgcaaatcaacaaatatatacttttttttttttttttttgagttggagttgcactctatcacccaggctggagtgcagtggcatgatcgtggctcactgcaacctcctcctcccgggttcaagtgattctcgcacctcagcctcctgagtagctgggattacaggtgcccgccactacgcccggctaatttttgtatttttagtagagataaggtttcactatattgaccaggctggtctcaaactcctgacctcaagagatctgcccacctcagcctcccaaagtgctgggattacaggcgtgaaccaccttgcctggccaacatatatataccttttgcaactttgtcagagttgctatgaagaataagttgtatcttgttcacagaaattgcagtctactgggggagctgataaatgttttaaccatccaatgtaacatgttgtcatcaaagagatggtgagactttacacttgtgctaacaaggtagctgttctacataaaagaacatacagtacagatgtagaacttttctgttatcatagaacgttctattggacagtgctaggctgaatgctacagatcttcagagaaaggagaggttatgaggcctggagttgtctagaaagtctttttgccaaagagggatttcaactgggtcccaaataatgggtggaatttgataggtgtaaagaatttgcggtggtttatgcctgtaatcccagcactttgggaggctgaggcaggaggattgcttgagcccaggagtttgagaccagcttgggcaacgtggtaaaactccctctcccctaaaaataaaaaaaattagccaggcctggtggcgtggacctgtagtcccagctactggtgagactaaggtgggaggatcacccaagccccgggggttaaggctgcagtgagccgtgatcccgccaccgcactccagcctgggtgacagagtgagaccctgtctccaaaaaaaaaaaaaattcctggtagcccggtagactaggagggtaagtaggggagaagtgattacttacaaaagacattgaatacaggaccaaggaatttcagttctgttcttttgtaggggaagcttttaaaactttcggggcgccgggcgcggtggctcacgcctgtaatcccagcactttgggaggcccagacgcgcggatcacgaggccaggagatcgagaccatcctggctaacacggtgaaaccccatctctactaaaaatacaaaaaaaagtagccgggcgttgtggcgggcgtctgtagtcccagctactcgggaggctgaggcaggagaagagcgtgaactcgggaggcggagcttgcagtgagccgatatcgcaccactgcactccagcctgggcgacagagcgagactccgtctcaaaaaaaaaaaaaataaataaataaataaataaataaaactttggagccgaagcactgatgtttaatcatagagtgcttactatgtgttaggcacaggcctgattgcctgatgctggttaatttgtacaaagtaaatcagtgcatatgccctctgccctaggggagttattaactggagtctgacattgtacaaaggtaggtatcctgactagtttgatttggtactttgggtgaaaaaagtatagtgtgcttaagtgcagaagtgttttttgaggatttttgattggatacaaaccaccactcatattttatgtctttggcacttaaaaatttcaccataacttttgagtcatttataaaaaccactgaaagagtacttgagggacatccccgaatcctgaagaacttctggtgttctggagcagcctcagtgagatccaggaggatggcattgctgggctggcccagcccttattgattatggtgtaaagaattaatatggtggttatatactctttgttagacaccttggcttacaagacgtaagcgtaaagtgtagtgcgctttagtcagtatggccacatggtcctttggtggtaaattgtttgagatgcctccagtttttaaaaggagtagcatatcgggccaggagcagtggctcatgcctataatcccagcactttggaaggccgaggcaagaggattgcttgagcccaggagttcaagaccagcctgggcaacatagtgagaccactttgtttctttaaaaaaaaaaaaaaggcaaaaacaggctgggcatggtggctgatgcctgtaatcccagcgctttgtgaggcagaggtgagcggatcacttgaggtcaggagtttgagaccagcctggccaacatggtaaaaccccgtctctactaaaaatacaaaaattagccaggtgtggtggcacacgcctgtagttccagctactctggaggctgagccaggagaattgcttgaacctgggaggtggaggctgcagtgagccaagatcctgccactgcactccagactgggggacagagtgagacattctgacagtgctacactgaatgctacatgtcttcagaggaaggagaggttatgaggcctgggaataacatatggaagaatgaatttctgttatggtcagttctcatttgtcatgttaggattactgcaactcttacccagccgggtgtggtggctcatgcctgtaattccagcactttgggaggctgtgggcggatcacgaggtcaggagatcgagaccatcctggctaacacggtgaaactccgcctctactaaaaatacaaaaaattagcccagcgtggtggcagacgcctgtagtcccagctactcaggaggctgaggcaggagaatggcatgagtcctggaggcggagcttgcagtgagctgagatcgtgccactgcactccagcctgggcaacagagtgggactccatctcaaaaaaaaaagaaaaaaaaaaggattaccgcaactctttaattcagatcagcaaacatgttgagagccaggtattgcgtcaggcaggatccaaggataatgaaatattgtccgttttcatgaaactggagatgttgcagggaccgaggtgtgtgctatgccagtatggaagtaggacaggggagacgacagggcagtgagtggttcaagactctggctctgaagtcaaacagatctgggactgaatcctggatctgccacttcctagtcagaatctgagcctctattttcttatctgtaaaagaagattataacagtgcttatcttgtaggtactgttgacgattcaataagataatgtggataaaatgcttagcatagtgcctggcacatagtaagagctcggtaaatctaagttcttactaaatatccaagaaaagagattaattcttttcaggagtgagagaaagtcatcattattgaggggctttatcagatgggaacacctgaatagggttttataggatgaataggaattctttccacgaagttgcgttacaaaaagttgcattcaaggctgaaggaacatgagggtgcagaggcttaaaacagccttgtgtgttcagggagctataagtagaagttcttaatttaggagaactaaaccaaggggaaaggaggccaaggaaccacagttcttatcccttttctgttaataattgggtttaaatgtcattaaaataagttattttgtcctttttagaaaagtaataacatgctattataaaaaaaaagacttgtaggaatataaaatgtgtgttttacatgtatcctgttaattgacttgcttttattcagattttttgcagccctttctgtttaccaggttatcttggagacatatttattccaaattcctttttttttttttttttgagatggagtctcgctctgtcgcccaggctggagtgcagtggcgctatcttggctcattgcaagctccgcctcccgggttcacgccactctcctgcctcagcctcccgagtagctgggactacaggcgcccgccaccacgcccagctaatgtttttttttttatatttttagtagcgacagggtttcaccgtgttagccaggatggtctcaatctcctcacattgtgatccgcctgcctcggcctcccaaagtgctgggattacaggcgtgagccagcacgcctggccttccaaattccttttaacagcctagcaaaagaataataaggaaggtaaatctgcccctacaagaaaataatgcttcgacgatccggctttccttcctgctacccccagccataagaataaatgaccttgctcatcactgaaattttacctgacctttgaatttttaactgcgtcagccaaagaacttatattttgagtattcctaaggtgattgctattgtagttttgaaacacttggttggtatgtttgagggtttcatggtccaaagttactatagcagttaaaagagtggactatcaggtcagacctattgggctttaatcccagttctgccttctcttagaccttgggcctgttgttttcacttctctggttttcagtttctctgtccacaattgtggaaacgaggtccacttgtagagtaattgagaggatgaagcaagatgatgcatatcaagtactttgcatagtgccgggcagacaggtaacattcaagtgctaataattactattattactatttattttttgagacaggttctcactctgtcacctaggctggagtgcagcggtgagatcacagctcatgacagccttgacctcctaggctcaagtgatcctcctgcctcagccttcggggtagctggggctacaggtgtgtgctaccaccctcagctaattttctaatttttttgagtcaggatctcgtcacgttgcctaggctgaattactcttattaaaaactataatatcaggccgagtgcggtggctcacgcctgtaatcccagcactttgggaggccaaggcgggtggatcacctgaggtcaggagttcaagaccagcctgcccaacagagtgagaccccccccgtctctactaaaaatataaaaattagccagttgtggtggtgggcacctgtaatcccagctactcgggaggctgaggcaggataatcgcttgaacccgggaggcggaggttgcggtgaaccgagatcgtgccactgcactacagcctgggtgacagagtgagactctgtctcaaaaaaaccgaaaaacaaaaagcataattagggtggtaacgcttatacataggggcaggtggaataaaacataattaggaggtcgggcatggtggctcacgcctgtaattccagcactttgggaggccgaggcgggtcaggagttcaagaccagcctgcccaacatagtgagaccccgtctctactaaaaatataaaatttagcctgttgtggtggcgggtgcctgtagtcccagctacccgggaggctgaggcaggagaattgcttttgaacccaggaggtgggggttgcagtgagctgagatcgcgccgctgcactccagcctgggagacagagcaagactccgtcacaaaaacaaaaaacaaaaaactgtcatatcaaaaactaaactaaaatggtaatatctgttagatattacaaagtcaggcaaattatgattcatggcagccactaatgacccaaaggagagaaagaataattagcagattctaacctaatgggaaaaaaactaaatgaatagggatgggggacttacattctgttagaggaaattgaggctgtcatataaaaggaataggtaaggcaaactgtaaattcctgtttacacaaatgcccttctgataaatctctgcattgcccacagtccatgattacctctcccttattttaagtaatatttaacacattaaaaatggattaccacccaaggaattgctcccgacccagaaagtgcaggtagtgttgaaggtttgaggggaagaggaatgattagagttggttgtgtctcaggaagaagccaacaggaggaaccttattttgagtcaggtaaagaaggtgggagtgaggaggcatcccggtggccaggtatgaagctgggagctgattgctgcacattactcagctgaattaaatgtgccctcacatctgtgtgtgtgcgtacatgcaaatgtacatgtgtatgagttagttggaggggtagacctttattttcctgtcctgtaactttcctttgcaaactaatctgtattcagaacagtgttgcagttaagaaccacccagcttgtccatgaaacaggttctctcaccccatctccccagttttagagaaggcaggaaagaaaaggcagtgcttttcttttttcctggccgtatgcggggcaggaagaagccagcagagcttgaaagagaaagtaaaccttctgggaaataaacggcttggcttccctattgtggaggaggagtgcaaattattagggggatgtttgggtagtttttgtagaagccatttctgaaaactgatttggattagtgaaggtaagcccaatttaggaaaaccctgcccagtctggtgtcagccacctgtttcccgctttgtttgattgatttgattagtttgtggtattctgacctctcatttttattacaagagttggaagatttgagtctgaacttgagcacctgcttcggtgaaagcttcctaaaatgcatgttttttcacattttttctcatgttcattttgttttgctttttagcaaacactttttctgacagaatctaaaagcattagacttttcttgttttccccttctctccccacaatgtaatcttgaaaacccaaatgttagctgtgtaaattacctctcccgtaaaccaaacaaagtgcaatattgcattgagttagcattgaaatagtcggcctttgaatttttttctacttgtggtttagacataataaatatttcatctcagactgactttctcgacaaatcagttttgcatttgggcctcttttcatcagtatgtttagggaaagcacatttattgaaacattaaccaaaatgaaacataattaggaggccgggagcgatggctcacgcctgtaatcccagcactttgggagaccaaggcatgtggattgcttgaggtcaggagttcaagaccatccttgccgacttggtgaaatcctgtttctactgaaaatacaaaaaactagctgggtgtggtgacgcgtgcctgtaatcccagctactctggaggctaaagcaagagaatcgcttgaacctgggaggcagaggttgcagtgagtcgagatcgtgccactgcactccagcctgggcaacagagactccgtctcaaacaaccaaaaaaacaaaaacaagcataattagggtggtaacgcttatacataggggcaggtggaataattgaagcattctggagccagaaataatcaactgattaagaataatctggctgggtgcggtggctcacgcctgtaatcccagctactcaggaggctgaggcaggagaatcgcttgaacctgggaggtggaggttgcagtgagccgagatcgcgccattgcactccagcctgggctatggagcaagactccatctcaaaaaaaaaaaaaaaaaaaatcctgtttctgcagaaatatcccaggtgtcctgggtcagcagtgccccatagattccacggacgtttaccctaagttttccaatgggagttcatacctctatacccagtgagaatattttctgagtaatgggaatgagattggagatgtagggtagagaagatccatacagtctttgggttaaactttttcctctttgcctaggaaagattaatgctaatcttaaccacagatttgtagtaagaatgtatcagttttgtcattcagttctagactccagttttctttattgtaataccaatattttagagtaaattttgaaatgaatcagtacaaaagatatgtagtaagtggaaagttagtccgcaccttatccttgggactctttcccagggacagctagttacctactatttatctctcctgagttacttcatatgtatgcatgcaaacatgttattctctgggtgttgttccttccatatatagcagcaaatacaccaaactctgtattttgctttttgtcactttatcttagagaatactcaatgcaaatacatgtgtatatacctcatgtttaaaaaatctacatagtaaaattagccaggcatggtagtgtgtgcctgtaatcccagctactcgggaggctgtggtgggagaatcacttgaaccctgagatcacaccactggactccagcctgggccacagagcaagattctgtctcaaaaaacaaaaacaaaaacaaaaaaactacagagtagtattctaggctatgcatatcataaatttgatttcctaatgataggcatagatgatttgcctgggcggcaaattagcgttggctgtgtctcaggaagaagccaacaggaggaaccttattttgagtcaggttccaaagacagaaacattgtctgacatttgtttttgggcttatatgaataaatctgtacacatatatttttaatgttttaatcgtaatatgtatactatttggaaatgtggctttttagttaacagagtgcatgttttaccccattgcacttaaacattaacttggggataattaaatgagtctgtcacttggacaggcaggaattgtaccccccacaaacccataaaccgccaattttttttttttgagacagagcctcattctgttgcccaggctggagtgcagtggtgcgatctgggcccactgtaagctcagcctcccgggttcatgccattctcctgcctcagcctcccaagtagctgggactacaggcgcccgtcacaatgcccggctaattttttgtatttttagtagagtcggggtttcaccatgttagccaggatggtctctatctcctgaccttgtgatccgcccgctttggcctcccaaagtgctggaattacaggtgtgagccaccgcacctggccggtttttttttttttttttgagatggagtcttgctctgttgccaggctggagtgcaatggcatgatctccgctcactgcaacctccacctcccgggttcaagtgattctcctgcctcagcctcctgagtagctgggactacaggcgtgtgccaccacgcacagctaatttttgtaattttagtagagatggggtttcattaataatcattaatattagacaactgtcagactcacagtggtggatacaaactttctcaaattctgatttttactctaaagctcaaattttatcattggcaacaaatattgtcagttgctttccctgaacagacagcttcccttctttcatttttgagaaaatatctgccagtatcccagttggtttatcaatcattctttctctttttttttttgagacggagtctcactctgtcacccaggctggagtgcagtggcatgatctcggctcactgcaacctccacctcccaggttccagcaattctcctgcctcagcctcccgagtagctgggattacaggggctagcagccacacctggctaatttttgcatttttagtagagacagggttttaccatgttggccaggctgatcttgaactcctgacctcatgatatgcccaccttggcctcccaaagtgctgggattacaggtgtgagccattgcgcccggctctattatttcttttctttctttctttttcttttttttttttgagatggagtttcgctcttgttgcccaggctggagtgcaatggcgcgatctcggctcaccacaacctccgcctcccgaattcaagtgattctcttgcctaagcctcccgagtagctgggattacaggcatgtgccaccacacccgtctagttttgtatttttattagagatgggggtttctccatgttggtcaggctggtctcgaactcccaacctcaggagatctgcctgcctcagcctcccaaagtactgggattacagttttgagccacctgacccggtttgcttattatttcttttaaatttaaaaaataataaataaaggggccatgagagcgaagagtttgagaaaggttggtctaaaggttttaacataagaatccctgggttatttgcttaaaaagaagaaagaatctatggatctgcctgagagggtctgatgtagtttatctggggtcatcctcacaggcatagcagatattctgattcagatggtccttggtccttagtttgagaaatgtggctttacaaggcccatagaatataaagtcttctttggattagtgaagtcatgtccacagggtttagaaaatgtttttgttttagagataaaggtaagtggaagagtagacatgtagtgaatgagggaaaatgttttagagatttctttttattctgtttactcttcttggtatgcacgtacctgaatattaaggatattttatgaagtcatgacattaccagattaatgttggttttgttttaaggtactttctgactgctggggttaattcctacagacgattctggtaaagaatagcctttaagttttaaaagtgttgacttatttcagatgtcttaataaagttaacttccagttattacatgtaacgtatataaagctctcattttcctttattctcgttaattgtttgcataacaaattcaaagggaaatttgcttggcagagatcagatagcagagatgagatttaaaaacaggtaatttggctactagcctgggagtttgaagattccaagtttgcatccatgtgtagtcacttaacatttctgtccttatctgtaaatgggaataacacctacttgatagggttgttacattatcttggccacctcaggttctctttggctgagtgattgactggaaaacgcaatgtgaattcatgcttcagactgggttcttttttttttttttttttgagatggagtttcactcttattgcccaggctggagtgcaatggcacgatctcagctcactgcaacctctgcctcccaggttcaagcgattctcctgcctcaggctcccgagtagctgggattacaggcatgcaccaccatgcctggctaatttttttgtatttttagtagagacggggtttcactgtgttggtcagactggtttcaaactcctgacctcaggtgatccacctgcttcagtctcccaaagtgctgggattacaggcatgagccaccgcacccagcccaggctaggttctatatgggtgtgctttttagaatttagatcatgggctatccccaacacaaactggataatgtttctttctagattctctctaagcgtgtattctctttctttcctaggcacagccaccacttcacttacattgtgggattataatttcatgagtagtggaatttccttaaccttctcttgtgtgggagctgaaggacaaaatgagatattctctgaagagtggttacatcatgcaaaactatgatgtgtaatgaggtcacttagttttctaagtacattatacattttgataagattttcatagaaaagcttgtctccttggggagatcactcatcttccatcttgactattatttaaactttatgggtcagatttatctttttaaaaacttaaccataaagctcaattaattttttttttttttttttgagacggagtctcgctctgttgcccaggctggagtgtagtggcgcgatctcggctcactgcaagctctgcctcccaggttcatgccattctcctgcctcagcctcctgactagatgggactacaggcgcccgccacgatgcccggctaattttttgtatttttagtagagacggggtttcaccgtgttaggatggtctcgatctcctgacctcgtgatccacccgcctcggcctcccaaagtgctgggattacaagcgtgagccaccgcgcccggctcaattaatatattttaaaaattaatagactttattatttttattttattttatttttgaggcagagtctcgctctgtcacccaggctgagtgcagtggtgtgatcttggctcactgcaaactccacctcccgggctcaagtgattctcctgcctcagcctcctaagtagctaggattacaggtgcctgccaccatacccggctagtttttgtaattttagtagatacgtgttttctttcttttcttttcttttttttgagatggagtttcactctttttgcccaggctggagtgcaatggcatgatctcggctcactgcaacctccgcctcccaggttcaagtgattctcctgcctcagcctcccaagtagctgagattatagttgtctgccaccacgcctggctaattttttgtatgtttgatagagacagggtttcactatgttagccaggatgtctcgatctcttgacctcgtgatccgcctgccttggcctcccaaagtgctgggattacaggcgtgagccactgcggccagtctagactttattttttaaagcagtgttagttttacagaaaaattatgtggaaagtacagagagtttccatataccccttactttctcccacaacttctattattaacatcttgcattagtatagtacgtcccttacaactaatgaaccaactcgatacattattattaaccaaattcctgagtttattttatttctatttttattttattattattattttttagaggtagggtctcactgtgttgtccaggccaggttgcagtggcatcatcatagcttgctatagcctgaaactcctgggctcaagcaatcctcctgcctcagtctcccaaagtgttggaattacaggtgtgagccactctgtccagcctgaagtccatagtttacattacatttcactctgttgagcattctatggattttgacaaatgtgtgatgatgtatatttgccagtacacaattatataaaatagttttactgccctagaaaccccctgtgctccacctattcattcctctgctgaaccactggcaaccactgatcttttataatatctccatagttttgtcttttccagaatgtcatatagttggacatacagtgtgtagccttttcagattggcttctttcagtaaatgatatgcatttcaggtttcttcatgtttttttgtggcttgataggttgtttcttttcattggtgagtaatactctattgtatggatataccacatgttgtttatcaaacattcacctgaaggatagacatcttggttgcttccaagtttgagcagttatgaataaagctgctataaacattccagtgcaggacttttcacctcctctggataaatatcaaggagtgcaattgctagatcatatggtaagagtatgtttagttttgtaagaagctatcaaactatattcaaagtgactgtaccattatacattcccatcagcagtgagtgagagttcctgttactccacatcttcaccagcatttagtggtgtcagtgttttggattttagccattttaatgggtgtataatggtatacctattaaaattggttttttttggagacagagtttcacagtttcactcttgttgccctggctggagtgcaatggcgcaatctcggctcactgcagcctccgcctcccagtttcaagtgattctcctgcctcagcctcccaagtagctgggattacaggtgcacgccaccatgttctgctaatttttttgtattttagtagagatggggtttcactgtgttacccaggctggtcttgaactcctgagctcaggtaatccacctgcctcagcttcccaaagtgttaggattacaggcatgagccaccgcacctggcctcaatttttttttttttttttttgagacagagttttgctcctgttgaccaggctggagtgcagtggcacaatctcggctcactgcaacctccgcctcctgagttcaagcgattctcctgccacagcctcctgagtagctgggattataggcgcccgccactacgcctggctaattttttttttttttttaattagagacgaggtttctccatgttggtcaggctggtcttgaactccccgttctcaggtgatccgcctgcctcagcctcccaaagtgctgagattacaggtgtgagccaccgtgccccgcctgttttggcttttactgtgaagacgtgttagccgctgtgatgactagcaagtgtggccctccacccagtcgctctgggctcccagctcctgcatcctgctgcaaacttgacatcttccctcaagtaacttgtagttgtctcctgtctacttgcccaaaatataactcttaaacttttctctctgcaagtttgtgcctctctccctgtctgacttccccatctaaataaatggtagaccaccatctactcctttgtgcaagccagaaatctaggaatcatccttaaattccctgttctgtcttatctctgctttcattcaaagcatcagcaaatcctgttggttctacctctgaagttttctcaaatactgttacttgactcatcctgacttttgtttctgctttatgttaggctaaatgccctgaaaactcttttgtacaaaacacctagaaatactggataaactgggcttaacagggaggcccggtgtggtggctcacgcctgtaatcccagaactttgggaggccaaggtgggtggatcacctgaggtcaggagttccagaccagcctggccaatacgtagtgaaaccccacctctactaaaaaaaaaaaaaaaaattagctgggtgttgtggtgcacacctgtaggtggtgcatgcttgaacttgggaggcggaggttgcagcgagctgagatcgcgccactgcacttcagcctgggtgacagagcaggattctgtctcttaaaaaaaaaaacaaaaaaagaaaaacaggaaaatcttcagaagcaaaaaccaaacaatctcaccaaagaaatgagaagatggctgggcgcggtggctcacgcctgtaatcccagcactttgggaggccgaggcgggcagatcacccgagatgggcagatcacccgaggtcaggaattcgagaccagcctggccaatatggtgaaaccccgtctctgctaaaaatacaaaaattagccaggtgtggtggcaggcgcctgtaatcccagctactcaggaggctgaggcaggagaatcgcttgaacctgggaggcggaggttgcagtgagccgagatcatgccactgtactctagcctggacgacagagcaagactctgtctcaaaaaaaaaaaaggctgggtgtggtggctcatgcctataatcctagcactttgggaggccaaggtgggcggatcacttgaggccaggtgaacatggcgaaaccccatctctactaaaaatactaaagttagctgggcatggtggtgggtgcctgtaatcccagctactcgggaggcgaggcaggagaatcgcttgaaccaggaggtggaggttacagtgaaccgagatctcgccaccgcactctagtctgggcgacagagcaagactccgtctcaaaaaacaacaacaaaaaaccaacacatggccaaagtgcagtgacttacatctgtataatcccaatgttttgggaggctgaggcaggaggatcgcttgagtccaggaatttgagaccagcctgggcaacatagacctcatcaccaaaaaaaaaatattttttaattagctgggtttggcagcatgtacctgtagtcctagctactcaggaggctgaggtgggaggatcacttaggcccaggagtttgatagttcgaggttatagtgagctatgatcctgccactgcactccagcctgggccacagagtgagaccctgtctcttagaaacaaaacaaaacaaaaaaaagaaactgaattaaaaacaacaagaacaaaaatgctgctttttgttattgagttgtagcccaagtttcttgagggtaaagcattgaaaagcaggcagtaatagatttgctgtttaaagagatttacttgcagcactattcacaatagcaaagacatggaatcaacctaaatgcccatcagtgacaaattggataaagaaaatgtggtacatacactgtggaatactatgcagccataaaaaacaacgagatcatgtttttgtttgtttgtttgtttgtttgtttttgagatggagtcttgctctattgcccaggctggaatgcaggtggcacgatttcagctcactgcaacctccgcctcccaggttcaagcaattctctgcctcagcctcccgagtagctgggattacaggtgccctccaccatgcctggctaatttttgtatttctagtagagatggggtttcaccgtgttgggcaggctgttcttgaactcctgacctcatgatcctcccacctcggcctcccaaagtgccgggattacgtgtgagccaccgtgctcggctgagatcatgtttttgcaggaacatggatggagctggaggctattatccttagcaaagtaatgcaggaacagaaaaccgaagaccacgtgttctcacttataagtgggagctaaatgataaggacttgtgaacacaaagaaggaaaccacagatactggggtttacttgagggtggagagtgggaggagggagaggaacagaaaagataactattgggtattgggcttaatacttaatattttatcaaaataagctgtacaacaaacccctctgacatgagtttacctatataacaaacttgcacgtgtaaccccaaacctaaaataaaagttaaaaaaaaaaaaaaaggctggttgcattgggaggctgaggcaggcagagcacttgaggccaggaattcgagaccagcttggctaacgtggagaaaccctgtctctactaaaaattcaaaaattagccaggtgtggtggtgcatgcctgcagtcccagctaccagggaggctgaggcaggagaattgcttgaactcaggaggcagaggttgcagtgagctgagattgcaccactgcattccagcctgggcgacagggcgagaccttgtctcaaaaaacaaaacaaaacaaaacaaaaacctgtcactttgggaatatctcaaacctagtcatccaagtggttgtacgattttagtgtctgcatatcaatatttagtgtgatctactttcttagattctcaaatactgccaatgggcacatgtcatgaaataatgtcttttagaggacaagagagtgctaaagtctcattattgcagtttaagaaaaacaattctgtaacagtttaactttataggaaatgccttttgtttatttattttttttcttttgaggcttagatttttatttttatgtttttagagatggggtcttcctatgttacccaggctggccttgaattcctgggctcaagtgatcttcctgcttcagcctcctgagtagctgggactagacgtccactactgctcctggctggaagtttagattttaatttaaactcttctattgggaaactttgtatgtttgctttaccacttaacatttgcatgcattattgtacctattgtctcctacttaaggaagggcagtttatgctgttatatgaagtgaattaacctcctatggtacttcagttttctctatgctaaaagtgtgttctagatttttgaaaaacttacttaattttcattcatttattcaaatatttgagcattctgtagttgctggggaaatagcagtgaactgaagaatgtctttgttcttatggggcttaagttcctagttgatcatattggaaggagatacatgaaaaaagaaatatatgaacaatggagggcgatgagtactgtaaaggagaattcagcaggggagatgttgctgttttagatagaggggtgtcaagagacattgtgcagagacctgaacgaagtgagggagcaagccatggagatatctagggaaagagcctatcaggtggagagaagagtcctagggcagaaacgggcaaggtgtgttccaggagcagagaggggacagctgtgagcaaggggagagttgtagggaaggaggcaaagagagacatctggggcaaaatggattgactggtgggccgtggtaggactttggattttttcctgagtgggttttgagcaggggaatgaaatgatctgactctggttttttttttttttggagacaaaatcttgctctgttgccgaggctgaagtgcagtggcgcaatctcggctcattgcaacatctacttcctgggttcaagctatgctcctgcctcagcctcccgagtagctaggattacaggcttgggccaccatgccggcgaatttctgtttttatttttattttttatttatttttatgtttatgttttttgagacggagtctcgctgtgtcacccaggctggagtgcagtggcgcgatctcagctcactgcaacctctgcctccccggttcaagcaacttctcctgcctcagcctcccgagtagctgagattacaggcgcctgccactacacctggctaatttttgtatttttagtagaaacgggatttcaccttgttggccaggctggtctcgaactcctgaccttaatttatctgctcgccttggcctcccaaagtgctgggatgacaggtttgagccaccgtgccagccaggactcttattttgaaaggatctgtaatgtggagaatagaaggtagagggacaaggatgaaagcatccaggccagttagcctagtccagctatctaggtaagagatgctggtggcctggattaaggctgcgtcagtgggaggttgtgagaaaggctcaccttccttttttttttttttttttttttttgagacaggatcttactctgtctcccaggctggagtgcagtggtgcaatctcagcttactacaacctccgcctcctgggctcaagtgatacccccacctcagcctcccaagtagctgggatcacaggcttgcgccactatatccggctaatttttgtatatttcgtagagacagggttttgccatgttgcctaggctggtctcaaactcctgagctcaagtgatccacccgcctcagcctcctaaagtgctgggattataggcctgagccattgtgcccggtcacttccagattttgaagacagagccaacaggatttgttaatggattaggtgtggcaggaggagggggaggaagagagagagagactggagttgaagttaaggctcatttcaaggtttttagcctcaacatgtgcaggaatggagttgtcacttgctagaatgggggagactggaggagaagccggctgggagaggtttttaatgaaggggttggctttggatacattaagtttgacatgcattttagacatccaggtggagatattgaagaggcagttggctataagtgtctgatgttcatattagcggatggggctagagacataaatttgagaattgtcagtgtataaacgttgttttgaaagaaagtggggctgaataatttagaaaggagtgcatagagaaaataagtttactattaaaatagctttaacaggccgggcacggtggctcatgcctgtaatcccagcactttgggaggctggggtgggcagatcaaaaggtcaggagtttgagaccagcctggccaatatggtgaaaccctgtctctactgaaaatacaaaaattagccaggcgttgtaccgggcacctgtagtcccagctacttgggaggttgaggcaggagaatcacttcaacccgggaggtggaggttgcagtgagccaagatcacgccactgcactccatcctgggcaacagagcaagactccgtctcaaaaaaaaaaacaaaaaaaaacaaaaaaaaaaaactttaacagcaaagcctcttcctttaaaattatgaatttttttcttatggaagttggactctttcattattaagtctacattcaatcactatgttagtaaaaatgttgttctagttgccgaatgcaataaaccagctcagacttagtggcctaaagcagcaatcatttgactatgttcgaagatgccgtgggcaggaatttagataacagcagggatggcttgtctttgctctgcgatgtctgaggtctcactgagaaaactcaagcggctgggggtaataatcatctggaattttctttactcctgtatctgatgtctgggctgcgatgactcaaaggctgatttcagctgagactgtagaccacgtgcctacttgtggcctccccttttgccttgggtttctcacagaatgtggctggttctggagaatgagacttccaatgaaatcaggtggaaatgacatctcgccgctttcagcatgctctattggttggaacagttatggacttagctagattcaaaggaagggaacaaagaccccctcctctcagagagtggggcataatgagagaatttagggccatgttatccaaccaccacaaatgccttctgaatttgaggttctgcctcaaaagttcatagttcctttgactgaaggacttctatatatccaagcatcgtcagccccaggtatattgttccatgtaagtgaccaggactaccttagtatttcgtatagggaaagtgacctgaataaatttgagaaaagaatcttccttctctccagtaagcactgaggtaagcattgagccatattataggtttatgactttgagactcagaaatttaaattcttggccaggcgcagtggctcacgcctgtaaccccaacactttgggaggccaaggcaggcagatcacttgaggtcaggagtttgagaccaacctggccaaaatggtgaaactccatctctacgaaaaatacaaaaattagccaggtgtggtggcgggcacctgtaatcccagctacttgggaggctgaggtaagagaatggcttaagttctctttatctgctttatttcagttgcctctcttagatgaatattaatgacttacatagcattttagatcagtggatgtttttgtgattcttttatttgagctttggccaaagataacagtacccacaggttttttccagctactcgctcttctcccttcagtggccctcgagcctggaaaatctgacatgacaatgtgcttgctcaacctaccactgtttttcttttgaaaagtttggcagcctgtttctgactcctatgaaggtgaattcctcagcattcacagtttattagaaaaatactttgcttctctccaaactcgaaattcaagataaccaaacctatatataggctgatctttcaggatgcagttgtcatgttgatgccatgcttttcagtatcgtggccatcatctgttcagtaggggaggtgtacttctgtaatgggaggtggtggttatgtgtgtgtgcaagtgtttatttggtgtcttaagttagcctgtgggaagttctaaatcaggatggtacgtggttgccagcagagagctgctcctcaagtgaaggaggtagaatcaaagccaataggaaagagcctcagatgcttatatatgtaccgtggggattcagagtgaaagcagtcattggactaggggtggggttagggagagcctgtctgacagacacaagaaagggatggataacgccacccagagaaaaaagcattttaggcaagaacaaatatgaaaaaggaacaaagtctgtgggtggggggcaaggaggagataagttgacttgaaggaagacaacacttatgaaagtcacctggaggctgggtgccatggctcatgcctataatcgcagcactttgggaggccgaggtaggaggacaacttgagcccaggagttcgagaccatcctgggcaacatggtgagactgagtctctaccaaaaaaaaaaaaaaaagaaaattatccagacatggtggcatgtgcctgtaatcccagttactcaggaggctgaggtgggagggttgcttgagcccaggaggttgaggctgcagtgagctgtgatcgtattattgcactccagcctgggtaacagagcaagaccctgtctcaaaaaatgaaagtcatctgtaggctggagagaggaactggaaggggctaaagttggctgagtagttacagagcctgagataagggtaaagattttgcattggacaatgagatgttagtgtgtgtttttgagctggggagtgctgtgattttactcttattgaagaatcactgaaggattattcttgaatcagtgattcttgatcattcttgaatttttcaaacagcaaaactggaagagttggcctattcctcagaatattttctaattgggcgcagtgtcctcacttgggagaacctggctacacactttagttgtaattcactccagtcgttcattcattcaatacctattttttcagcacctattatgagccagacactatgctggatgccagggttcagggtaggacacgctagtgagcaaaagccaagactcttcttgtcttcatggggctttcagtccagcatagtggttatgagtccaagttaatggagtcacagtacttgggtgcaagtcatggtgatggtgatagaaggaaggcatgtgtgagggccagtggcaggcaggagcctggtgtttttgaggacctgaagaaggagcagagtgagtgccaggaacttagccaccagctggtaccagccatacgagaggggcagagccagccaggatgtcggtcatgctagtaatgagtacaaacacttacatgctgcacgctattgggctcctgagtgctacgtgttcattagctcgatgaatttgtacagcaaccctgtgaggtaagcactgttctctcccctttctatagatgaggaaattaaggcacaaagaggataaataactggcaccagctacacgctaagtgatcgaagtggtggaaccaggattcaaatccatgctattctgccttaagataacaaatcttgttttttagcctaagaacagagcagtcatcaggagggttttaagtaggggtgtggcaagatcaagtttgtgtcttgaaaaggtctctctacccacagtgtggaaaatggcctggaggcaagcacacagatgttgggagacagttaacagctcttgccatggccccctatgcattttggctctgatgtttctgcctgatttttctcttgcctctgcctcttttcctgaggggatggcaggttttaccattcagctggagtacaaaccctgaaccctttttggttaaatatctacttgcttttcctacagtattattttgagttgctgtggctgtaatgtcttgagggaatcgagcttgacagtaatttatagaacaaacagtttttagagactgtgtggcccaattgccctctcaatgttggcactcctgccatgacatttaccatgctgagcatgtgaccgccatctgaataccaaatgccacaggaacctgggaggttgtcacttactcctccctttctctgagtcacctttgcccttcagtcagtcaccaagtcccatcacatgtagctctgtaatgtcacagaagatggatgtctgcctcaaaacacttacaatgctgctacctaaattgggcagccacgacctcccaccaggattattgcagcctgagggatctttttgaaatgtaaatcaaactatcacttgtctgtttaaagcttttcaaagacttaccccattgcccttggaagaaagtgcagatatcttgacaggagagccttctccagcctcctcttctgccgtggtctccttgtacagtctctacagtgtactgcttcattagaaccctggagattattatttgctagttctgggctaagaactggcacctggctttgtagagctcctcaggagattctgaggcgtattcagagttgagccctgatctctgctctgatttcgaggttctcgttatatttattaatgatcacgaaaaaatttattattattctttggcctcactttagcatcatctgaggaatttttttttttttttgacagagttttgctcttgttgcccaggctggagtgcaatggcgtgatctcagctcactgcaacctccgcctcccgggttcaagagattctcctgcctcagcctcccaagtagctgaaattacaggcatccaccaccatgcctgctaatgtttttgtattttttagtagaggtgggctttcacagtgttggtcaggctggttttgaactcctgacgtcagctgatccacccacctaggccccccagagtgctgggattacaggtgtgagccaccgtgcccagccgtagctttcgaaatttgaaacctggtcccactgtcagaggttccaatttggcactggtttggttcccaggcatctttcttgctgtatatattttttagtgtcagccagggtggagacctctgtattacttcatggggaagaatttgggagaagatgttgtgaggagacaggttctagtcctagagtgatttatcctttctcgtacagatttccaggtatttgaggggccactcttctgtaattcatgtttttctctcctaacctcactcctgttgcctgcatcttcttgctgagcaaaatattcaaggtcttcaactcctcacaccctggttgtccctccctggatgtgtttggttgttttagtgttccatttcaattttgatacacagaattagaatagcatccagatgtgggtctgttacagctagactactagatccttcaaaatccaagtactagtatgtctattaaaataccataagatcacattggctagttacaatggttggtttgtgggttacttaaaaatcaactaaaattctttttttttttttgagatggagttttgctcttgttgcctaggctggaatgcaatgacacaatcttggctcactgccacctctgcctcccaggttcaagcaattcccctgccttagcctcctgagtagctgggattacaggcatgtgccaccatggccagctaattctgtatttttagtagagatgaggtttttccatgttggtcaggctggtctcgaactcccgacctcaggtgatccacctgcctcagcctcccaaagtgctgggattacaggcgtgagccactgagcctggccaaaattcccactttctaatactcctgtagtagctgggtacggtgggtcacatctgtaatcccagcacttttggaggctgaggctggaggatcgcttgagcctaggagttcgagaccagcctgggcaagatggccagacgccatctctaatttaaaaaaaagaaaaaacaagactcctatagtggtgaagaacagacattccgaaaacagactgtgcgttatgattccagctccatgcctttactacctgtgttgtgactttggataaatcacttaaaaatcttttttttttttttttttttttgagacggagtcttgctctgccgcccaggctggagtgcagtggcgcgatctcggctcactgcaagctctgcctcccaggttcacaccattctcctgcctcagcctcccaagtagctgggactgcaggtgcccgccactacacctggctaattttttgtatttttagtagagacggggtttcaccgtgttagccaggatggtctcgatctcctgtcctcgtgatccacccgcctcagcctctcaaagtgttgggattacaggcgtgagccaccgcacccggccaaatcacttaaaattctgtgcctcagtttctcctctgtaaagtgggataaaaatagtacctatctgatagggttgttacaattatgaaatgagcaaataagtatgtcaagtgtttaaaacagcgcctggcttcttgtaaaaagtgctatataaatcatagctataatcattacttatttcgactgctctttaaccaaggttcttatttttcatctttttcttttgttttgaatatcacttagtgttttcaccttttactctttttaggacctagagccatcctaggtgaaatacgtatggagatatttgatcaggtcaccacccagctctcctgacctcccttctctccttaaattaacatgccaaatcacagcatcactgactccttccctcccgatatgataagagtgtgcattgaaatgcatgtattttacttagcagggaaagctgattagtgattatcacacttaacccctagtgaatctgatggattaacctgctttccaggacactaaggaaatgggtttaagataagaaatatctggctgggtgcggtggctttacgcctgtaatcccagcactttgggaggccgaggtgggcagatcacgaggtcaggtgattgagatcatcctggctaacacgatgaaaccccctctttactaaaaatacaaaaaattagccgggtgtggtggcgggcgcctggagtcccagctactcgggaggctgaggcaagagaatggtgtgaacccaggaggcagagcttgcagtgagctgagattgtgcccaccgcattccagcctgggcaacagagtgagactacatctcaaaaaaaaaaaaaaaaaaagtaagaaatgtccatgaaagggagaccctgggggaaaggaacaataactgcagctctgaggatctggcaccagcagcaccagcacagagggatgctgtacaaccattattgattttaactttacaacagttcttcaaaggagagagagttccctgttttactgaagagaaagcccatttggtagtgaaataccattcccaaagacaaatagctaataaatgtcaggcagggttttgcacccaggcccatccagctcccgtctctactgtcctttcccccacaccacactgatacagaggaatgtgtctggttggggaagtggaagtgttcccaagtggggaggtcatctgatgcacaaatttggtctgttttgtgggttttcttgttttagttttagtttttgtagagctcagacctgttcttaggcagctttaacaatcaactgtgcactcagtaattgacaaatcatgtttgttacttttaatttagagggaattaggtttgttaagctcttgctccttctttagagatggggtctagctctgtcacccaggctggagcgcagtggtatgatcacagctcactgcagtctcaatctgctcaagtgatcctcctgcctcagcctccatgggactacaagcatgggccaccatgctaggctaattttaaaaaaatttttttgtagaggcaaggtctcacggtgttgcccaggctggtcttgaactcctgagctcaagcaatccctcttccaccttggcctctcaaagtgctagaattataggcatgagccaccatgcctggcctttacttctttcatatattcaaattttgtcatattagtagggaactataactcaagttttcttatagattgatgttcatttttacaagcttgatcgtcattggtttttaattttaaagcaaatcctgttatatgtaattgaacattacagtaattatagtaatttgtttcagattgggcactcaagtgttaatattttgtctctttaggaaatcaaaactagatttatatatagacttcttattgcaagtatctagtcttaaatcttacaaaggtactatttggacttaaaactatgaaattgtgtgcttactatataagtgtacttattttgagttatgttttaaacttgaaattccattcttaatgtctagagtaattatgaatggttaaattatgaatgactctaatagtttaaagctacagtatttatttatttatttatttaatttattttttgagatggagtttcgctcttgtcgcccaggctggagtgtagtggcaccatcttggttcactgcaacctctgcctcgcgggttcaagtgattctcctgcctcagcctcccaagtggctgggattacaggtgtatttcaccatgcctggctaatttttgtatttttagtagagacaggcttttgccatgttagcctggctggtctcgaactcctgacctcaggtgacctaccctcctcagcctcccaaggattacaagcatgagccaccacacctggcctacagtattttaatgtggactctctgtcatccattatgctgtttatcctgtggtgaaaattttatgaagattgaatgtttttctctagcgtgaattgctttctcttacttttctcatttttttccttcctaatctacttgcagatacttcagattatttttagaacgtggtatggtgagaacaaataaattggggtttccaaatcttaataaattatgtggccctcagtgggattagcagggttgtattgaaaacaccaatagaaacaaaatagttcttttatgcgctttaaataaaaatttcttttcaggccaggcgcagtggctcacacctgtaatcccagcaccctgggaggctgaggcaggcagatcacctcaggtcaggagtttaagacaagcctggccaacatggtgaagcgccgtctctactaaaaatacaaaaattagccgggtatgatggcgcatgcctgtaatcccagctactccagaggctgaggcatgagaatcacttgaactcaggagatggaggttgcagtgagctgagatggtgccactgcactctagcctgggcaacagagtgagattctgtctcaaacaacaacaacaacaataacaaaacatctcttttcaggccaggtactgtggctcacgcctgtaatcccagcactttgggaggccaaaacaggagggtcgcttgagaccaggagtttgagaccagcttgggcagctggtctctatttgaacaaacaaacaaacaaacacaatactcttttcatagaaaaatgtttactacacaataaactttaaaagaatatgcagctgtattaatgctatgactccaatgtaaaaaaaaaaaaatatatatatatatatacacacacacaaacacattctgaaatagatttaaaggaattacatcaacatgtcaatttttattttttcggagacagggtctcgctgtgtcacccaagctggagtacagtggtgcaatcacagctcactgcagccttgacttcctggcctcaagtgatcctcccccctcagcctcccaaagtgctggggtcacagaccaccacacctggcaacatgtcagtttttgttctgcatagtgggatggtgggatatggatgtttttatcttttattttcttttttatatttttctaaattttccacattgaacattattttataatctttcaaacatatctcttaaaaggactggttcctatagaattcagtgcaagaaatcttctgtgtttctttatactttggttgccttgatcactgggcctttcctgacagcaaagaagaggttagtgtaggcagcagataaaacacaggtatgctctatttaaaatgcatgtatttataataaaagtataggtggtacccaaaggaaaatgtcatgacacattgcaaagtggaacagaagttatctttagatcactttctgttctggattattgtatgagcctgattttcgtctctctttccgccttccctcaccctcgttgtaaatccactagtgcatggatgtgaagtacaagtcttaactttaaaaagttttatgaagctgtgtagtaaatcccttttgtaagtggtcttgactgcgtttctcaatatatcttttggtttcattagattcaagtatataaatgagaactgtaactttggacagactttttcagtcatctttacggtaataagttcccaattagacaatagttatttgttttatgacttgctgttggtaggttatccccaagggactgagaaattcctgttttgaaaagtccaaaaagtctttgatgacttgctgtttcatttttttcttttctcttcagttatagaaaacaggattacacccaccttgcctttgtacagtgcatctactatctgctgacttaacctgagtaaatgctttgaattgagccccatataatgtcctaaggcagcctatatggagtaatgaattgtcttctctcttatgcacccagagtggtagttggcactcaagttgttcctcagataactttgtgtgttctggggctcaatgaagtagttattaagtcacaggcttggggagaacattcatcctatggcattgaatgaagtgttgcccaattctagaatgtctaataaaatttttttaaaaacccacaggcttagaattattccgtagatatgaagtaatgtagttagaacttagtggagttctttagattaacttgtaatttgaaaaaccaaaattgaaattgtgaaataacatgggctctttgaggtcttttccagtaaaacagttacagtaaagctgcttggcagtgattttcctagacactttggctagtcatctcctgtgactgctgttaattaaatatggtttgtagctaagcagcctgtaaggagaagactatggaagtatttgcatattctctccttgaaaatactacctggtctttggctttaagttatacttttattttcccctgtagaataactattaaagtattacctatggtgattagactaagaagtaaaacatgaaatcagtcattgttggtgccctggtgccttcttttttttttttttgagacagagtctcactctgttgcccaggctggagtgcaatggcacgatcttggctcactgcaacctctgcctcccaggttcaagcgattctcctgcctcagcctcccaagtagctgagactacaggcgcccaccaccacgcctggctaatttttgaatttttagtagagacagggtttcactatattggctaggctggtctcaaactcctgaccttgtgatccgcccacctcagcctcccaaagtgctgggattataggtgttagccactgtgcccagcctggtgctttaattttatggaaaaaactactagctggtttctgttttaagaaataacacaggccgggtgccatgacttgcgcttgtactcccagcagtttgggaggccgaggcgggcggatcacgaggtcaggagtttgagaccagcctggccaacatagtgaaaccccgtctctactaaaaatacaaaaattagccgggcgtggtggggcatgcctgtagtcccagctactcgggaggctgaggcaggagaatcgcttgaacctgggaggtggaggctgcagtgagccaagatcgccccactgcacaccagcccgggtgacagtatttcatctcaaaaaaaaaaaaaaaaaaaagaacacaattattgtactacttactagccctcctctgtccccagctaaaaataagaacagcaacaaccaaaaaatccttagttatgtactggaaatgaattagataattttcaataacttacacgtttttaggatatgttagtttgaaaatgcaaatattcatgcatgaccccagtgttaatctatgatggagcaggtatagtgggatgctgtttcatgatttaatttggaccttcagggagtagactgtgatgcctctgcatttgtatccaagacaaataattaaatagtctatttttggctgggcatgatgcctcatgcctgcagtcccagcactttgggaggctgaggtgggaggatcgcttgaggccaggagttcaagatcagtctgggcaacaaaatgagaccttgtctctacaaaaactacaaaaaattagctgaacattgtggcttgtgcccctagtcccagctactcaggtccctgagttaggaggattgcttgagcccaggagttggaggttacagtgatctatatttgccactgcactccagcctgggtgacagagagagaccctgtctcaaaaaataaagtctgtttttaaaattaattttaaacactggagtttattacaaaaagcagttggttctttttttaaatcatttttttttaggagaaccaccgctttttggctacattgtctagagtagcagtgttcaataaaaataagatccaagtcacatatgtaatgttaagttttcttttagtttctttttcttttcttttcttttctcttctttctttctttctttcttttttttttttttgatatgcagtctcactctgttgcccaggctggagtgcagtggcacgatctcggcccactgcaacctccgcctcccgggttcaagcaattctcctgcctcagcctcccgagtagctgggactacaggcatgtgccaccatacccagctaatttttgtatttttagtagagatggagctttgccatgttggccagtctggtctcaaactcctgacctcgggtgatccacatgctttggcctccctaagtgctgggattacaggcatgagccaccatgccctaccaatgttaagttttctagtagccatattaaaagaagtaaaaagaaatgggtgaagttaattttaataatatattttatttaacccaatatatctaaaatattatcatttcaacatgaacaagatactttacattcttttgtttttcactaagtcctcaaaatccagtgtgtattttatattgacagcatagttcagtttgaagcagccacatttcaagtgctcagtagccacatgtggctagtgactccatactggactgtgtaggtttagagtttcagtaaatttgtatgcaatagaatctacataaattggcatattatgcagatttctttgtatgcacatcagttcttgcatagcataagtcaggtcatgatgcttttagtctatgaggcagatttttttttttttttttttgagacagagtctcacttggtcacccaggctggagtgtagatgcacaatcttggctcactgcaacctccatgtgaggcagattttaacttggccctaatgcaaatattgtaagagagatctaatggcctttgatttcttacagagggcaatcaatacatgccatggttacaatgcttcagcatatagtatgcacgtcagccactgcttttactctggctagtgcttagtgtacctgtaccactgcccaggcagcatttgtcctgtggcaggtgaatcttagggtggaaggtggcaagtaacattgcttttttttgagagggagtcttgctgtattgcccaggctggagtgcagtggtgcgatctcggctcactacaacctccacctcccgggttcaagtgattctcctgcctcagcctcctgagtagctgggattacagacggccaccaccatgctcggctaatttttgtatttttagtagagacggggtttcactatgttggccaggctggtctcgaactcctgacctcgtgatccacccgcctcggcctcccaaagttctgggattacaggtgtgagccaccgtgcccagcctacatttttaaattaattaattataagcaggatctcactgtgttggccagactggtcttgaactgataagagttcaagaccagcctaggcaacatggtaaaaccctgtctactaaaaaatacaaaaaaaaaaattagctgggcatggtggtgcgtgcctataatcccagctacttgggaggctgaggcaggaaaatcgcttgaacccgggagactgaagttgcagtgaggtgagattgcaccactgcactccagcctaggcgattccatctcaaaaacaataacaacaaaataacattgttggaatatttagttaatttatagaagcgtattggcctaattggggcaaataccttattctgacattctctctatttgctttactgagctttttcaccagtggaatttaagcccttgatacatgaggagggaaaataccttggagctgtgctgcacatgtaaagtacacaggagatttagaaaacttcgtagcaaaaaaaagagtgtaaagtatctcattaatagtttttgtgggctggacacggtggctcaagcctatactcttggcacattgggaggctgagatgcatgagtctaggagtttgagaccagcctgggcaacacagtaggaccccgtctctacaaaaataatcagccagatgtggtgcgcatctgtagtcccagttacttgagaggctgaggtgggaggatcgtttgagctgggaagttgaggctacagtgagctgtgattgaaccactgcactccagcctgggtgacagagtgcctgtctccaaaaaataaataaataaataataatatgttttgtatgttcatatgttgcaataacattttggatatattaaatgaaataaaatacattaaaattaatttcacctgtttcttttcttttcttttttttttttttttttgagatggagtctcgctatgtcatcaggctggagtgcagtggcacgatctcggctcactgcaacctcctcctcctgggttcaagcgattcttctgcctcagcctccctagtagctgggattaaaggcatgtgccaccacacccagctaatttttgtatttttagtagagacggggtttcaccatattggccaggatggtctcgatctcctgacctcatgatccgcctgccttggcctcccaaagttctgggattacaggcgtgagccactgcacccagcctcttttaactttttaagtatggctaccagaaaatttaaaatgcatgtgtggcctgtattctatttctgttggatgctgctgccttagattattaattattcaatgtaaagactgctgggaggtactacctgcacttccctgaatatatgcttgagagctccaccagccgtcttcacagtagcaagaggggtattctgagtctgtcccccaaagagggagggagaagtgcagccctctcaggttctgtcagaaaacctgatcccaggccaggcgtggtagcttacgcctgtaatcccagcactttgggaggttgaggcaggaggattgcttaagcccaggagttcgagaccagcctgggcaacacagtgaagaccctatctctacaaaaatttttttaaaaaaattagccaggtgcagcaatgctgcctgtactcccagctgcttgggaggctgaggtaggaggattgcctgagcccaggagttagaggttgcaggagttagaggttccacgatcgcacctttcattccgttacatttgctgccttgagaacagaagacctgctggttttgttgccagtttgctcagtcatttttatgaaaaagccagtgctaactaggtgcttcttcgtgccttctctgagaatcaagaactctagtatgtttgcgtgtgttcagtctctcattaaatgttctcactatcccagagaaccatctcattggaccttggtctgtacataccttcatctttggctctgacttgtaattatttttagaacttctctttttttttttttggagacagagttttgctctagttgccagactggaatgcagtggcacgatctcagctcacctcaacctctgccttccaggttcaagcaattctcctgcctcaacctcttgagtagctgtaattacaggcatgtgccaccacgcctggctaattttgtgtttttagtagagacagggtttctccaagttggtcaggctggtctcaaactcccgacctcaggtgatctgcccgccttggcctcccaaagtgctgggattacaggcgtaagccactgcgcctggcctaattttagaacttgttaaaacaacttggcctctattgatatttccatgacccatgctattcagaaagaggattacaggtaattagctggctgggtttctcataccagagcatttcactgggatgttcctgaacctgggacaacttttatgcctggcatttttctttccttctctgttgtcccagactaagcaatttttaaaatagttattatttgttgagtaggagaatctcaggcagatcttcctggatcctcatttatacttttaaacctgtagtcttggaattagtgctctgtcccccaaccccaaacatccaatttctacattttggctacagtacaggtttactgtgtataactaaaagggctgtggaggagaaagaaaggaaccgacatttgttgggcatctgttatgtgccatgcactgagctggatgctgtaggaatatctcaatacctctgaggagtgggaattattatctctattttatagacaagggaatagaaatctgggagttaagtaattttttaatttcacacacttctggtagataatggattctagaacctggcataatagccacttgtcatcccagtgtaaaagagatgtgtggccagatggggtggctcacatatgtaatcccagcactttgggaagccgaggcaggaggatgacttgagcccaggagttcaagaccagcctgggcatgttttgtttgtctcacgaaacattttttaaaaaatgagtgtggcatggtgttgtgtgcctatagtcccagctcctcgggaggctgaggtgggaggatctcttgagcccatgatcatgccattgcactctagcctgggccacagagcaagactctgtcttcaaaaaataataaaaaggagctgtgattatcccaaggtggggattgtgaatgtgtttgtattgttctaaactgggagaaacaggctgggtgtgttggcttatgcctgtaatctcagcactttgggaggccaaggtgggaggatcacttgagtccaggagttcaaggccaccctgggcaacaggcaaaaaatagagaccccatctctattttttaaaaataaaataaactgggagaaagaagcagggtcctccccagagcatctttatccctagtcacagacctgacacctgtgttgggcaatggctacttctagattgtttacccctactgggacttgtggtgaacatatgcacactttggtttacagttgggacccctgattttagcaggatggcccaatggaatcagctacagcagcttgacacacggtacctggagcagctccatcagctctacagtgacagcttcccaatggagctgcggcagtttctggccccttggattgagagtcaagattggtaagtccttcttaagtgactctccaaattgttaggtttcagtttgagtcaagagacatgaactcttaatgtcatgccttgctgttccattaaaaaatgtatgggtacaggtgatggggaaaatgagatcaggagataaaggggcaccctttggtcttgtaaagccttttttatcttagaagggcatgtgggcaactgtctttgacacattgaaaccgcctgtatggtggtggatgtcttgaaggttgatttggacctcatttacttgggcagatcctctatatattctgataatccagtgatgtggtagacatattttttctctgaatgtgaattctgtcatagctagaactttgggttgatacttgtaattcccctttagttaaaggaaggagccacaggggtgtattagtctgttctcaatttgctataaagaaatacctgagactgggtaatttataagaaaagaggtttaatcggctcatagttctgcaggctatataggaagcatagcagcatctgctgctggggaggcctcagcaagcttccaatcatggcggaaggcagagagggagcaggcaggtcacatggccacagcaagagcaagagagcaagggggaggtgccacacacttttaaactatcagatctcacaagaactcactgtctcgaggacagtatcaacagggatggtattaaaccattcatgagaaacccacccccatgatccagtcaccttccaccaggccccacctcaaacagtgggggttacatttcagtatgagatttgggcagggatgtagatccaaactagatcacaggataagggaagtagattccattcatagagcagataatggcacagatgtccagcaactattttcttcactttaatatgctcaggctcactactgattttggtttaattcaggccagtgttaatatgacctggtttttccagaatgcatactctgatttggtgaagggccaggaggtgattcacagatgttggagataggccatcccagcctgggattacttatttgtactaataaatctgaccagagttaattgagggtttaaagcaaaacagcatatctgtctactttgctcaaatattttacaaatacaacagattatgagagtgggtaataatatctggaataattgtttttttgttttgtggtttttttttttttttttttgagatggagtctggctgtagcccaggctggagtgcagtggtacagtctcggctcactgcacctctgcctcttggattcaagcgattctcccgcctcagcctcccgagtagctgggattacaggtgcccaccaccacacctggctaattttttatttttagtagagacagcgtttcaccatgttggccaggttggtctggaactcctgacctcaggtgatccgcctgcctcagcctcccaaagtgctgggattacaggcatgagccaccatgcctggcctggaataattgttaataattattacattgatggcattttattgctgagcaagaagaatctaacatgatgaatgggttatagcatcaggtttgctttgtttttttgtttttttcctctttcttgatggtgatttctgtgtttgtgtgtatgcgtcggcttcagagccattctttatcattcttccttttcctagggcatatgcggccagcaaagaatcacatgccactttggtgtttcataatctcctgggagagattgaccagcagtatagccgcttcctgcaagagtcgaatgttctctatcagcacaatctacgaagaatcaagcagtttcttcaggtatgatgagaaactgaggacaaggagaaacaggacccgcagagtcgggtgttagtgttctttcctggaagcatctcttttctcatttggctaagtaacgagaatctatcttgtattttcaatcacaggagaagtaattagccctttctcaaagctctgtatacttacccgtgagcatcattacctgagaatcacttctcttgtcacagttgaagtaataaagtgattgttatgttaatcatacatgttagcatgttaacgcggtccactgataggaagatgactctcactgttacatgttaaatgtttgaccataatgggatacttcttgactaagtcagtagcttccctgcaagaccaggatagtatactgtgtaaagactcagacaaggccaggcatggtggctcacgcctgtaatcccaacaccttaggaggttgaggtgggaggattgcttgagcctgggagttttgagaccagcttgggcaacataacaagacaccatctctacagaaattttttttaaaaactagctgattgtggtggcatgcacctgtagtcccagctactcagaaggctgaggtgagaaaattgtttgagcctgggaggtcgaagctgcaataagccgtgattgcgccactgcactccagcctggcggacagagtgagagccagtctcaaaaaaaaaaaaaaaagactcaggctaatgtgccttctgttacagaaatagtaacgacctccccttcgccccccgccgacagagagccttcacccaggctctgaagcctttgttccgttgtttcctagaataaatgctttccttgatgaatacattagttttaaggtgccacagttcagtccacatctccatggtctgctgctgatttttattctctttctctcctacttatagagcaggtatcttgagaagccaatggagattgcccggattgtggcccggtgcctgtgggaagaatcacgccttctacagactgcagccactgcggcccaggtgagacctgagacaaaacaaatccctggtctgggaggaatggaaaatcaaacaactttataatgagataaattattagatctactaaaaaagaaggaaaagaaattaaatagatcaataatcataaaaatacattgaaaaactctaaaaaaaaagaaagttccaccccccaaaatacattgaaaaactctaaaaaaaagaaagttccaccaaaagaatccaacagacccaatggtttaaaagttttgttttgttctgacaaattttctttgtttttctttttttttttttctgagacagagttttgctcttgttacccaggctagagtgcaatggcgcgatcttggctcactgcaacctccacctccagggttcaagtgattctcctgcctcagcctcaagagtagctgggattataggcgtgtgccaccacacccagctaattttgtatttttagtagagacggggtttcttcatgttggtcaggctggtctcgaactcctgacctcaggtgatccgcccgcctcagcctcccacagtgctgggattacaggcgtgagccactgtgcccggcctgttctgacaaactttcatagtacagattattccaatatcattcaaacttttccaaagtataggaaaacaagggatgttttcagcttattttatgaggctggaaaaatcctcatatcaaaacctaaaaaacagccaggtgtagtagctcacgcctgtaatcccagcactttgggaggctgagacgggcagattgcctgagcctcaggagttcgagaccagctggggcaatgtagcgagacctcatctctctttttttttttttttgagacagagtctctctctgtcgtccaggctggagtgcagtggtgccatcttagctcactgcaacctccgcctcccaggttcaagcgattctcttgcctcagcctcccgactagctgggactacaggtgtgtgccaccaagcctggctaattttttgtattttttttagtagagatggggtttcaccttgttaggcaggatggtcttgatctcctgacttcatgatccaccggccacagcctcccaaagtgctgggattataggcatgagccaccacgcccagccttttttttttttttgagacagagtcttgctctgttgccaggctggagtgcagtggcgtgatctcagctcactgcaacttctgcctcccaggttcaagctattcccctgcctcagcctcccaagtagctgggactacaggcgcgcgccaccacacccagctaattttttgtgtttttagtagagatggggtttcactgtgttagccaggatggtctcgatctcttgacctcgtgatccgcccgcctcggcctcccaaagtgctgggattacaggcgtgagcaaccgcacctggcttaattaaggatctttctaaacacaagaaagaatatttatcagaaaccaaagggagcatgatgcacagtggtgaaacactattctcagtaaaaacagcaaaagataaggatgtcttttaccattgatacttttctgagggatccagcctatgcaaaaagaaaaagaaatgagggtacaaatattggaaagcaagggacagaactcttattatttacagatagataggtcttcctcgaagatccaagagaaacaaaactaacaataacaattggaactagcaaggtttagaaaggccattgtatacaagataaatatttttagaatctgcagttcccctaatcagtagcagcagtaacctgttagaagatgtaatgaaagtaaagatctgggccaggcacgatgtctcacgcctgtaatccaagcactttgggaggccaaggtgggcagatcatgaggtcaagagattgagaccatcctggccaacatgatgaaaccccatctctactaaaaatacaaaaattagctgggtgtggtggtacgcgcctgtagtcccagctactcgggaagctggggcaggagaatcgcttgaacctgggaggcggaggttgtagtgaaccaagattgcgccactgcactcctgggcgacagagcgagactccgactgaaaaaaaaaaaaaaaaaaaaagaaagatctgattcatagtagtaaaactaaatgtatgcaatttgcatatactattggtatgtatgggaaaatatctggaaacacatatactaaatcattaaagtagtcggtcataggagacttttttactttctgtgaggggttttaccgtctttaatatcctataatcagggacattttttctttttctccgtgaccccctgctttttaaaaaattgtggtgaaatacacataacattacatttcaaatttacctttgtaacctttgttttttttttttttttttgagacagtctcactctgtcacccaggctggagtgcagtggtgtgatcacagctcactgcagcctcaaccacctgggccctagcgatcctcctgcctcagccttatgagtagctgggactacaggcacatgccaccatgcccagctaattttttttttttttttttttggtagagatgggctcttgccatgtttcccaggctggtgttgaactcctgggctcatcaactgatgagaaagagctctccaggcagaaagaagatcatgttcaaagacagaaacagaaatgtgtattcttgggagaagtgtagaaagttcagcatctgattgggtcggggaagacaagctagtcaaggccacatgatgttttaattagtcatgcctaacagtggggccctggaagagcagtttaccacaaggggccaactgcttcggtttgaacccgcagccctgccacttgctctgtaaccttaagtaaacaatttttactctctctgttcctccaatgggagtgataacaataccttcttcatagaattaattcatacatgtaaaatgcttagaacagtatctgacacataaatgcaaaataatttaactgctttctgctgctgctgacatcactatcatcaccctcaccattactgtaggaaatggggacccagtgaagaattttttttttttcttttgagacagagtctcactctgtcacccaggccggagtgcagtgacgcgatttcggcccactgcaacctctgcctctcaggttcaagcgattctcatgtctcagcttcccaagtagctgggattacaggcatgagccaccacactgggctaattttttgtatttttagtgagatagggtttcaccatattggccaggctggtctcaaactcctgacctcaggtgatccatccacctcggcctcccaaagtgctgggattacaggcataagccactgtgtccggccctagtgaggaattttaagcagaaaactgatatgctcaggtgtgagcgaggtggtaggtaacacttactgtgcagtgccctgtagcccaagaggttagcacacaggcatttgctcaggcagcactaggattttctgctgtggaaaacctttgtattttatcctgctccacaagataaaaataagtggtttaagtcaatttggatagaggctccaacttaccatgggaggtaggaaagccaaagttatcccaaggatgttttcaatcgtacggattaggggtctgcaaactgtgagcgtggcccaaatccagcctgctgcttgtttttgtaaatgaggttttttcggaacccagccacactcatttatttatgcattatctgtggctgctttggtgctgcagtggcagggctatttgtggcagggactgtatgacccaggaaaccaaaaatatttaccctctgtcccttagagaaaaagtttgcaacccctgatataaagctataagttggttatttgtggcctcaacccaggcctcactgctattttttctgtttacaatacctggcatgctcttaagtgtctagaattggttaaagatagaagagtggatgtaatccctgctaccaagggctgtcaggctagttgggattataagtacacaaacactcaaagtgagaaaaacacagaaaaggatgtgtgtcattttgtctaaggaagttgaataagatttctcaggaaaagaaacatttgaactgaatttgaaggtgagtgagttcaggtgtgtttgggctgaagcccaggccatgctgagtggatagcgggtgggaagagagtgtggaaacacactgcatgcagggaagagttgggagtctggggtgaccaaggcacagggagggaaagttgaagttatcaattgtgtgaaacagctttctgtgttggcctgagatgtttatagctggaagcagtggggagccaatacagttttttacgaaggtattagaggtgggtttctgtgggtgatcgttaatcatgttttctccctttaagtgtagtcctgcttgagaaatagacatgagaaaggaatgaaggttaaaacatcagctgtattgttggtaaaactagaatggaaagtgtggcttgagctggtaaccataggggctttccaatgcctgtgccctgagttagatcttggggtagagagactggatgtgcagagcagcacccccaccccaccccagccatccatatggagcttcagctgccatagaccaacaaggcagagggataggcctctagacctgcttctagaaaccaggctgctgctcttgcttatggtgggccctaggaaggcaagagtgagaggagggaggcaccagcttaggtgctgggttctttgaagatctgtgtgtacacagagtctttctctccatcttaccaatcagatgagtcactgtcactgtgggaagaagtaggggcatgggtcaccttcccaaaacttctaagaagtttgtattctgtgggcttggatagggaccatgggaaaggaagagaatggttgcccataaaactggctgtagtgtggcctcaaacttctggacttaaatgatcctcccacctcagcctcccaagtagctagaactacaggtatatgccaccatgcccagctagttaaaaaaaaatttttttttttttttggttgagatgaggtctctttctatgttccctgggccggtctcaaactcccagcctcaagtgatcctcctgccttggtttcccaaagtgctaggattataggtgggagctaccatgcctagcccaagcctgtaattttttttttttttttttgagatggagtttcacttttgttgctcaggctggagtgcatggcgcagtcttggctcaccacaacctccacctcccgggttcaggcgattctccttcctcagcctcccgagtagctgggattacaggcatgcaccaccaagctcagctaactttgtatttttagtagagatgggtttctccgtgtcggtcaggctggtctcaaactcctgacctcaggtaatctgcccaccttggcctcccaaagtgctgggattacaggcatcagccaccgcacctggcacgaacctgtaatttttaagtttcatatgctatttattttttgttatttctttaattcattcattcatttattcattcgagatggggcctcactatgttgactaggctagttttgaactcctggcctcaagcagtcctcccacttcagccttcccaagtgctgatattataggtgtgagctgctacatccagccttctttcttctttttctttttccatgtgctatttgacattttccaaggtaccagcctccccttctccccaagataatatcttttaatatggaatttcatccctagggcaggactttttttttattatccctcagaaatatactggacaccacgtttaagtagacatccaacatctgctgtcataaattgttttgaattttttgacatacttgcccatgaggtttttgaaggcatagaccatgtcttagctgaacatgtggtctcttagtgccataaagggggtttatggtatgacctgtgtagtgtcacctgtgtagtgacagcaccactgcctctgtttcccttcctcttgtgatggcagcagcgtctcaagccaaacaagaagggtagttagggtgggatggaagctgggtagaggtattcctctccccatagttctgtgttcacatgtgcattgacctcctttttggcagcaagggggccaggccaaccaccccacagcagccgtggtgacggagaagcagcagatgctggagcagcaccttcaggatgtccggaagagagtgcaggtgatgcaagttacaagcctcgggcagggagctttcattaatttttttttttttttttgagacagggtcttgctctgccactcaggctgggctgcagtggcatgatcacagctcactgcagcctcgacctctcaggcccaagcgatcctcctacctcatcctcccaagtagccgggaccacaggcatgcaccaccacgcccagctaattaaaaaaaaaaaatttgtagagatgggggtctccctgtgttgtccaggctgatcatgaactcctgggctcaagtgatcctcccaactcagcctctcaaagtgctggcattacaggcgtgagccactgcacctggccaacagggagccttctcttggggatactgcctgcaggtcctgcatgtatcttttttgaggttttggcttcatttgaattctcctcagaaactttatattttctgttcccaaggaaatctttctttacttctgtttttttgtttgcttattttaaacaggatctagaacagaaaatgaaagtggtagagaatctccaggatgactttgatttcaactataaaaccctcaagagtcaaggaggcaagtgaatattagagatgttaaaatctctagaaagtgagtttgtgttgttgagttgaaagactcatttgtcttaactctgtttagatcttaaggcgggcggggcgcaagggaggtacgggtcctcaaaggagcctggtcattaaggacaggagtattccctcaggtccaggagtattccctcaggtccaggagtattccctcaggtcaaggagtattccctcaggtcaaggagtattccctcaggtccaggagtattccctcaggtccaggagtattccctcaggtccaggagtattccctcaggtccaggagtattccctcaggtccaggagtattccctcaggtcaaggagtattccctcaggtccaggagtattccctcaggtccaggagtattccctcaggtccaggagtattccctcaggtccaggagtattccctcaggtccaggagtattccctcaggtcaaggagtattccctcaggtccaggagtattccctcaggtccaggagtattccctcaggtccaggagtattccctcaggtcaaggagtattccctcaggtccaggagtattccctcaggtccaggagtattccctcaggtccaggagtattccctcaggtccaggagtattccctcaggtccaggagtattccctcaggtccaggagtattccctcaggtccaggagtattccctcaggtccaggagtattccctcaggtcaaggagtattccctcaggtccaggagtattccctcaggtccaggagtattccctcaggtccaggagtattccctcaggtcaaggagtattccctcaggtcaaggagtattccctcaggtcaaggagttttttcttccttcgcagacatgcaagatctgaatggaaacaaccagtcagtgaccaggcagaagatgcagcagctggaacagatgctcactgcgctggaccagatgcggagagtaagggcataggtcggaccacttcccccatgtgtctcgctcacttgcgggatttcagcgtcttgtggcagaacttgcttggtttctaagaagttcctgctctggagttgactaaagaatgtggttagagacagtctgaggaaatgttttctgactttgttttggtttccaaccagagcatcgtgagtgagctggcggggcttttgtcagcgatggagtacgtgcagaaaactctcacggacgaggagctggctgactggaagaggcggcaacagattgcctgcattggaggcccgcccaacatctgcctagatcggctagaaaactggtaaaggatgaaagaagcttttcctttctttctcgaaagctagattgaattctgatcttaactgcaggcccacagaattggtactatatctccaacgtggggacttttccatattcaaatttagcccaagaattaaagtttttactttatttcggccaggcgctgtggctcacacctgtaatcccagcactttgggagaccaagatgggcggatcacttgaggtcaggagtttgagaccagcctggccaacatggtgaaaacacatctctactaaaaacataaaaaaattagccgggcgtggtggtgcgcacctgtagtcccagctactctgggcggctgaggcaggagaatcacttgaacctgggatatggaagttgcagtgagcggagatcttactaccgcacaccaaccagcctgggagacagagtgagactccatctcaaaaaaataaaaataaaataaagtttttactttatttggagaaactttgttttaaaaaatgtatttatattattatattttaagtatattttacttaataattcaattaaggcttttggtttaactgtatttaacagatagacaaaccttttaattttagttattttagtaatctaaaatgacacatgccctttttaagggaaaaaattcaaatacagaaaattaatcaagagaagaaaaaatttttaaatgaaatcatcagcagtactagtagttaaaatttagttgatgctcaatctagacatctgtcattatgtatatacacattatgtatatacacataaagatagaaatttatacagtttatattaggatcatttttttttctttttttggagtcagggtctcactgtgttacccagtctagagtacagttatgcagtcatggctcactggagccttgacctcctgggctcaggcagtcttcccaccttagccttctcagtagctgggactacaggcatgcaccaccacacctggctaatttttaaattttttatagagacagggtcttactttgttgcctgggctggtctcaaattcctgggctcaagggatcatcccacttcggcctctcaaaagctctggaattatagatgtgagctgccgtgcccagcccaggatcttcctttatatgcttttctgtaatttgcacttttaccttcatccagcatatcttactgcaacccttcctgtgcaaggccctatagtgagcatgttgcaccagcttgccttaggagaaacttgagatacagagcctgcactggaaatttagcgcaactctacatgagaatgcctgtctattcatatcctcactaaccctgagtgttgttaatttactgaaagcagttttaaatgcttcctgaccagggaacgaagaagcttaagttctgggaatgggaggatagaagtgccagaaaagagctcaggagttcagaaatccctgcagcggtccccctccctctcctttcactttctgtctttctggtcttttggtctttgttacactagtgataaaccatcaaagaatgatggaatgatgctaacttctctctttttttaatttttttgagacagagtctcactctgtcacccaggttagagtgcagtggcatgatcttggcttactgcaacctcctcctcccaggttcaagcgattcttagtcacaaccttccaagtagctgggattacaggcccatgccaccatgcctggctatttttttgtattttagtagatcgacctgcctcggcctctcaaatttttgggattacaggtgtcagccactgcacctggcctaatatctctattcttggagatagatttaatgagctttttctccctctctattcacttattccttgtgcatgttatcaatattttgaaacataatgtcatgtcctttgatcagttgaaggctgacattgaaaaggcttatggggattgggtgttgtggctcacgcctgtaaatcccaatgctttgggaggcagagtcgggaggatcacttgaacccaggagtttgagaccagcctgggcaacaaagtgagatcccatccctacaaaaatttaaaaaactagacatgtgccattacacttcagcctgggtgacagagtgagactccatctcaaaaaactaaactaaactaaacaggcatggtggcacacacctatagttctagctactcaggaagctgaggtaggaggatcactcatgtccaggagttggaggaggcagtgagctatgatcatgccattgcactgcactaggccacagagtgggaccctgtctcaaaaaaaaaaaaagaaagaaagaaaagaaagggctcatgtagttcaagcccttctcttcatgcaaggggatgctaaggcccatgatggtgaagggcctggcaaagcttgcacagatagtgtgtgacagagctggctcaaacccatctttgggagctgtctaatctctttttctgagtctttatgttcatagacaagttaggatgagtaaagtaagtgctaaattccatatttcgtgttctgcatatctgggctcagatgcttgtcattttccagtgataactccatcaatgcctcctagtggtataaattttaatacttcttgtgtgcccagccccctcttagaaatttgagattttaggaagggactagtaataaaaggtaaaataaattattttctggccaggcatggtggctcacacctgtaatgccagtacttcgggaggtcgaggcagatggatcacctgaggtcaggagttcaagaccagcctggccaacaaggcaaaatcccatctctactaaaaatgcaaaaattatccgggagtggtggtgggtgcctgtaatcccagctacttgggaggctgaggcaggagaatcacttgaacttgggaggcggaggttgcagtgagctgagactgtgccactgcactccagcctgggcaacagagtaagactctatctcaaaaaaaaaaaaaaaaaaaaaaaggccaggcgcagtggcttacacctgtaatctctcaggaggctcaggcaggagaatcacttgaacccgggaaatggaggttgcagtgagccgagattgcaccactgcactccagctcaaaaaataaataaataaataaattattttctttttttatttattttttcagcatccacccaacatggtgaaaaattcctcttttcttaatgtcactgaactgtaaacttaagatgaaaaattgtaaatttcatgctatatatatttcaccacaataaaaaaattccttgttcttattgtagtggtctccatgtcttcagtatttccttccccttctccatctcacctgtatacattcactttggtaattagcatctttcttaatttattggcaggataacgtcattagcagaatctcaacttcagacccgtcaacaaattaagaaactggaggagttgcagcaaaaagtttcctacaaaggggaccccattgtacagcaccggccgatgctggaggagagaatcgtggagctgtttagaaacttaatgaaaaggtaatttagcatccttgtccctttccctcatctaaaaaatacctaaagactcacgtggtagagtgagaggcgggctgacttctggtcatggccgtggcgcgtgagcccatcttctctttcctcagtgcctttgtggtggagcggcagccctgcatgcccatgcatcctgaccggcccctcgtcatcaagaccggcgtccagttcactactaaagtcaggtaggccatgccacttccatttccagtagagattttactgagggacactgttagggtgagggtagagttggtggccagggtcattctttccaggtgtggtgtcacaggcagtacactgttgcggggttgaaatttgttgccatactatctgcttgctctctgattctgatgtcaaaagcaaaagagcagtcatctttttgaaggtacctgggcatattcctatgattgtagacctggagtctcaggccacagcttctccttctgcccaagggacaaaataatgtcatctattttctgttctttgaggctactcttccctgtggattttaagggaaagagtaaggcttagtgatggggaagctgagaggccccagggcaggtgggtggtgggcctgtagggtgaggtgttactttcacactcaagtcagaacaggtgtgctggggttttgaccttctgcagcaaaatttccctcctcagaaacttagtatggtgttcggtttcaggattaatagaacaaaatgccagctgcacagcatgtgttcctgtaatatttttcattatatggctttgattatccttttgtgaatctctcacaactttaagttgttagttcttagatgttttctcagtacctttggcttgaaggagtgatactcatcttttgtttttgtttgagacagggtctcactctcacccaggctggtgtgcagtggcatgatctcagctcactgcaacctccatctcccaggttcaagtgattcttgtgcctcagcctcctgagtaactgggaatagaggtgcgtgccaccacacccggctaatttttttttttttgagacagagtctcgctctttcggccaggccagagtgcgtgttgcaatctcaactcactgcaacctccacctcccaggttcaagcgattctcctgccttagcctccctgagtagctggaccggcacactccaccatgcccggctaatttttgtatttttagtagagacagggtttctccatgttggccaggctggtctcaaaactcctgacctcagtaatccacccaccccggcctccaaaagtgctgggattacagatgtgagccaccacgctcggcctttttttttttttttttttttttgagatggagtctttctctatcacccaggctagagtgctgaggtgtgatctcggatcactgcagcctctgcctcctgggttcaagtgattctcctgcctcagcctcccaagtagctgggattacaggtacctgccaccatgcccggctgatttttgtatttttagtagagacggggtttcaccatcttggccaggctggtctcgaactcctgaccttgtgatccacctgccttggcctcccaaagtgctgggattacaggtgtgagtcaccgcacccagccctattttaatttttttaaagagagagataggggccaggcacggtggctctcgcctgtaatcccagcactttgggaggccaaggtgggtggatcacctgaggtcgggagttcgagaccatcctgaccaacatggagaaactctgtctctactaaaaatacaaaattagctgagcgtggtggcgcgcgcctgtaatcccagctacttgagaggctgaggcaggagaatcacttgaacccaggaggcggaggttgcggtgaacggagattgcgccattgcactccagcctgggtaacgagagaaactgtctcaaaaaaaaaaaaagagaaagagagataggatctcgctctgtcatctaggctagagtgcagtggcatgatcatagatcactgtagccttgaactcctgggcacaagtgatcctcttgcctcagcctcccgagtaactgcgactacaggtacatgctaccacaccccgctaatttttaaattttttatagatgtgggctctcactttgttgcccagactgttatggaactcctgggctcaagggatcctcccagcttggcctcccacagtgctgagattatagatgtgagcctgtaattatagacagcttggcctatttacctgttggaaatgaagaattatgaattttacatttcttcaagaaaaggttatgggagagttactgactttttttccttggattttttctttttaaataggttgctggtcaaattccctgagttgaattatcagcttaaaattaaagtgtgcattgacaagtaagtactcctatcttagctctgtttttcaaatgaggaatagaaaaatgagaactttgacagacatcatttgaactagagactctgtctttattcagagatcttcattttgtggacaaaagttttcaaaagccttggggtgcattgtcatttacgtgtctgaacaaagccacaaagctgggggtacagatttgatttgtggttgctattgtgacaaccagtccctcttttccttgtttagttttttacttgtacatgtcattcatgcatattatatataagactgagatcatgtgttaattaacgactgggatacgttctgcaaaatgtatcattaggcaattttgttgtgcaaatgttgtagagtatatagtccttacacaaacctgggtggcagaacctactgcacacctacgctatgtggcagagcctactggtcgtaggctgtaaacctgtacagtatgttactgtgctgaataccgtaggcaattgtaacacatctcaatgaagtaggaatttttcagctccatgataatcttatgggaccaccatcatatatgcattttgttgttgaccgaaacgtcgttatatattctttccatacatagcatgtggaaagaatagatctcttttttttaattgttccacactttaccatataatggaatacgcaaaatttcacaatacctttcaggatgtaaaatacatataccctttgacgacattagaaaagagaaaatgtgggccgggcgcggtggctcatgcctgtaatcccagcactttgggaggccgaggcgggcggatcacgaggtcaggagatcgagaccatcctgggtaacacggtgaaaccccgtctctactaaaaatacaaaaaaactagctgggcgtggtggcgggcacctgtagtcccagctactcaggaggctgaggcaggagaatggcatgaacctgggaggtggagtttgcagtgagccaagatcacaccactgcactccagcctgggcgacagagactccatctcaaaaaaaaaaaaaaagaaaagaaaagagaaaatgtggctgggcgcggtggctcacgcctgtaatctcagcactttgggaggctgaggtgggcagatcacctgaggtcgagagttcgaaaccagcccgaccaacatggagaaaccttgtctctactaaaaatacaaaattagccaggtgtgttggcgcatgcccgtaatcccagctacacgggaggctgaggcaggagaatcacttgaactcaggaggtggaggttgtggtgagccgagatcacaccattgcactccagcctgggcaacaagagcgaaactatctcaaaaaaaaaaaaagaaaaaagaaaagataaaatgcattcttatttttagttgatgtaattatgtggaaatttcatgaggatgcactggaaaataatgaaataagggagttgacgaaggtggtaggtttaataagtacatatgcaatatgaaacataggttccccttcctatggggaggcaaccaactgtgcctgctacgcagaggtgttatgttgcgctgatcaactgtaactgaatagtttaaagaaatgcccaggagcacagaggttttttcatgacagtaaataacaggtggtcaaagtaggctttttgaagaaacacagagcctattttattaacaacagtctgtgttcttacagagactctggggacgttgcagctctcagagggtaagttcagcctagaggcttccttttgttccgtttaacctaacttcatcctccggctacttggtcacctacatagttgattgttcccctgtgattcagatcccggaaatttaacattctgggcacaaacacaaaagtgatgaacatggaagaatccaacaacggcagcctctctgcagaattcaaacacttggtatgtgggaggagctccccttcacaaagggcctctggctgccggagagggctagggagagcctcacaggacacctgcctttttcttttcttacagaccctgagggagcagagatgtgggaatgggggccgagccaattgtgatgtaagttttgttggggatgaaagacaactggggtgttttccttgagggagagaggggtaaagatccttcttaatccccagaattagaaacatcaacctgttctttcagctgtagttattccaaaaagtcacttcaggccaaagtgacatgaacagaagttccatgtgccatggagctctctggcttggaacatttccgtgaatatctgggagttggctcctccttaaggagaagtggaaagtcccttgctgagttgttctccacacccatgtggtataaagcagctttccaccttgcctggggctttccaaattccccatccagctcctgcggctgaccctgcttggctccatttttagtgccctgtttttctctcccactgaggtgggatagagggtgtaaaagcaacagatttgagttaaactttaaaataaatgaccaccttgcattagcttgcttaggaaaagagtacataaaataaaatgaacaaacaaaaacccatcttgttctttatcccccttattttctgcttttcattgattcagattattggattcttattgtcaagaataaactttaaacaaacaaacaaaaaaaggtaaatgtgacggaaggctagttttcagtcatttttaaaaattgtgatgccccgttctttttcttacatttgtcccctgaacaattcttcctctttaaaatgtagcagtcctagctgggcgtgctggctcacaccccgtactttgggatgccaaggcaggctggtcacttgaggtcaggagttcaagaccagcctggccaacatggtgaaagcccgtctctactaaagatacaaaaattagctgggtgtggtggtgcacgcctgtagtcccagttactggggaggctgaggcatgagaatcgcttgaacctgagaggtggagcttgcagtgagccaagattttgccactgcactctagcctgggcaacagagtgaaactctgtctcaaaaaaataaataaaataaaatgtagcagtcctttttaaaaatgtggaattttacttgacagtagagtgaagtagcctgtatgcaatgatatgggaaaatgtacatgacatattaagaaaaagcaaaatgtaaaataatttgaatagtattattagtatatgtgttttaaaaatacactatactcttatgtgtattcatatgtatattaagaaattctggaggaatataccagcagtgctatgtgtattagtgctgctgttggtatccatggctattctagactgtctctgtgatatttgcattttaaactgaatatattacttttataatcagaaaaatagtattaaaaatgaattataatttaatttcttttttcttttttttttttgagtcggagtctcgttctatcggattgcagtggtgcgatctcagctcactgcaacctctgcctcctaggttcaagcgattctcctgtctcagcctcccaagtagctgggacgataggtgcatgccaccacgcctggctaatttttgcatttttagtagagacagggtttcaccatattggtcaggctggtcttgaactcctgacctcgtgatccacccatctcggcctccgaaagtgctgggattacaggcatgagccgctgtgcccagactagaattcaatttttgagaattcattgacaactcttacttaaaataaggttgctgtactgatgtgagacattgttgtagtcagtttggaaaacaatttggcagtataaaaatgaacatacctgtaaaccaacggtgccattcccaggatttaatagcagagaaatctttgcatatatgtcccaggagacatatataaagtggacatcagcctgattataagctctaaatgcaacccaaataaatacccatcaacattagaatgaatacattatttgtggtatagacacaatggaatactccgcagctgtgaaaaggaatacactgcagatacacataaccatgtggattcatttcacatcaagtgaaaagtgaatcccaaaagaattcattggagtccataagtgtaaggttcacaaatgtcccaaactaaacaatacctgcattgcttagataaacaaatatggtaaaactgtaaaaaaacaaaacaaaacaagacaaaaagggctaggaaatgataaacccaaaagacaaaatagcagttatttctgagggaggagggaaggggatggggttggggaagggcacccagagaattttaggagtgatggacttttccttaaattgaatggtgggttcatattgttttgttattctttgtgccttacgtattttacaaataaccaattggatctatgtaatattataatacaaactgagtaaaggattaggttgaggatcacagcattggaagttcttggtgttgaagagagtaagtgccgagcaagttgtgtccctggcagtttgtttgtgaccacctggtggcttacccttcttggtgtggtgaggcttggcatgtcactttccttggctgtggctgttagtactgaatgccattctctctgaggaaaagtgtccttctcttttttattgattgactgattgattgagacagagtctcactctgtcacccaggctggagtgcagtggcgtgatctcggctcactgcatcctctgcctcctgggttcaagcgattctcctgcctcagcctcctgagtagctgggactacaggcgcccactaccacacccagctaatttttgtattcttagtagaaacggggtttcaccaaattattggccaggctggtctcgaactcctgaccatgtgatccacctgcctcggcctcccaaaatgctgggattgtaggtgtgagccatcacgctcagcctttttttttatttaatttaatttttttttaagacagggtctcactctgtcaccccagctagagtgcagtggcacaatcatagctcgctgcagcctccatctcctaggctcaagccatcctcccacctcagcctctcgagtagctggggctataggtgtgcaccaccacacccagctaatttttgtattttttgcagagatggagttttgctgtgctgcttagactggtctcgaactcctgggctcaggcaatcctcctgccttggcctcccaaagtgctgggattacaggcatgagccaccacacctggcctaagagtgtccttctcgttactgtaggcttccctgattgtgactgaggagctgcacctgatcacctttgagaccgaggtgtatcaccaaggcctcaagattgacctagaggtaagttctgcagcagaatcggtgagaggctacgtacaggggtgactcaggacaaaaacttccactgggatttttacaagagaaggtggaatgattactgtttgcttaacactgtgtttatttttgcttacttttctccaaaaaaatccttggcatcccatctggcaataaagtcttgcttgaatgcttagaagatgtgtgtatattcagctttcagcaaacttgatatgaaaatctctatttagaaattgattggccgggcgcggtggctcacgcctgtaatcccagcactttgggaggctgaggcgggtggatcacgaggtcaggagttcgagaccagcctggccaacatgacgaaaccccgtctctactaaaatacaaaaattagctgggtatggtggcggacgcctataatcccagctactcgggaggctgaggcaggagaatcacttgaacctgggaggcagaggttgcagtgagctgagattgtgccattgcactccagcctgggtgacagagtgagactccgtctcaaaaaaaaaaaaaagaaattagaactgactttataaagtttgggcataagagtcttagcagccagtgtgtttagtatacagaaaattgtggcaatgacattctcctttcccaactttcttgatttttaaattaagatatacctagaaaagcaggaatcctggtctttgattcctgagacctccctgtttcatgtgaagatacagcttcaagtcttggagaatgcctccaaggtcttaaaaatggggaatctgtggattgtgagtcaagctttgagcaagtcaggttttacaagggaccggtatattccgactgcagcctgagttgtgtggccacgctgggcattctttccactatgagtgctcactgagctgactcactcacactcctcgcctagagttggcagcaggtgtggtttatggcatgtcctttcattctgagccccgtgagatgcgggtgaagagatttccaaggctgtgagagcccctctgcctccccagctcagtccccactccctccgcagacccactccttgccagttgtggtgatctccaacatctgtcagatgccaaatgcctgggcgtccatcctgtggtacaacatgctgaccaacaatcccaaggttagtgccccctccttttagttggtgccccgggatctcttgcgacttaggggtacctagtatagacaatgagcaccatccctcatctaaacaagcaaatgtgttctttccaatagaatgtaaacttttttaccaagcccccaattggaacctgggatcaagtggccgaggtcctgagctggcagttctcctccaccaccaagcgaggactgagcatcgagcagctgactacactggcagagaaactcttgggtccgcatttcaccccttctccctcccgcccacccgcccagaaaagggatccggcccatagggctgttcatttgggccatgtctactgagcattaggccatgtttctttcctgagcaaggcgctgtgctggtgccaggaaacaggggagttggggagttggggtgcagagacagtttgcagttttcagtcgaggtgatcatttttgaggtgggaggtagatttcttttctcctggttgctgtctcattcacccactctatctaactttagaagatcttttaagtgtgtgttggaaggtggcactaaaggcttgacattccctgtccatttttttaataaactataggctagttggttttttttgtcttattttatttatttatttatttttttgagacgagtcttgctctgttgcccaggctggagtgcagtagtgtgatctcggctcactgcaacctccgccttctgggttcaagcgattcttctgcctcggcctcccgagtagctgagactacaggtgctcaccaccacgcccagctaatttttgtatttttagtagagacggggttttaccatgttggccaggatagtctccgtctcttcacctcgtgatccgcccacctcggcctcctaaagtgctgggattacaggcttgagccactgtgcccagcgtaggctagtttttaaaaaagaattagtggaatattttatgtgccacctgggctagaagtagctttgttctaataaagctgttgccaccaaatacacctgtctgacacccgatgtcagcttgttagtgagtgctgctgttggttcccagcctaccacccgaggttgggaagagcagggggacttgttatatcaccctccatccctgctgggctacccagcaacacaagtgagtcaaatgatgggatagtgtttgtcctcatgtgcacacacacaacagtgcctaccttcaaagatgtgaaagctgattattttgtggcccattgtgggatgaatgtgtgtgtgttctgttttaagaaataacctcttgaccccaagctgaaaatgtactacttgactctttttctttccttcaggacctggtgtgaattattcagggtgtcagatcacatgggctaaattttgcaaagtaagcaatcttgttaaattctcgtgggaatgggaatgctcacctgcacggctgtcgttgagggctctggcttgaaggccctgaactcttggtccagcggccagtaggacctgcctgaaggtagacgggcctgaggatttgggtgatgcactgcacccctaggaagggaagggctgggatggcagtagacttggctttcccattactcttttctccaggaaaacatggctggcaagggcttctccttctgggtctggctggacaatatcattgaccttgtgaaaaagtacatcctggccctttggaacgaagggtaggttggacagagtgtgcacagatgtaaccaagtcccctgctctcagcaagccagtggcaggggatggatgccctgttagcaataacaacattgttcctcctccttggctccaggtacatcatgggctttatcagtaaggagcgggagcgggccatcttgagcactaagcctccaggcaccttcctgctaagattcagtgaaagcagcaaagaaggaggcgtcactttcacttgggtggagaaggacatcagcggtaagggaggctcccacccaccccacctgctggtggctgctgaggcctcatcactgcttctagttgcaagcacctactgccccctggtgggtggagatggccttgactccctgtttcactcagactcgcaaaacacatttgcgtgacttctaaatccttccagctgaaggattggtttgctttgttttgcttgctccagtgactatttgttgagaattttgcaatttaaattgtattcttcatctctttttctacttaaccctgttaatatatcttacgcaagtagttatattcaagtttattttctatgacccaactagtagcctcttcttaattagaagccagcctgaatatttccacagtgccaggccactgaacagggtgttcagggtctcaacactagggtggcttaagtcttttccccttcgaggaaagaaaaaatgggcagttttctctgagatgacctagctgtaggttccatgatctttccttcccatgtcctgtgacaggtaagacccagatccagtccgtggaaccatacacaaagcagcagctgaacaacatgtcatttgctgaaatcatcatgggctataagatcatggatgctaccaatatcctggtgtctccactggtctatctctatcctgacattcccaaggaggaggcattcggaaagtattgtcggccagagagccaggagcatcctgaagctgacccaggtagttgttgattttccatgttcctggcatttaatttttgggaaaagttggaaattttgggatccttggaggatagataggcaaatgcctgaataacctgggggataattatttctccttatgggaaagaattgtagtgagtgcttttgttggggtgaccgatgggatttgagaggagaatcagaatcacttagagtagtgtagttcctgctccacagagagtgcatgagtctaaagaggggatacagcctgggcaatatggtgaaacctcgtctctacaaaaaatccaaaaaaattacccggtgtggtggcacgcatttgtagtcgtagctacttgggaggctgaggtgggaggatcacctgagccaaggagttcaaggctgtagtgagcggtgatcatgccaccgcactccagcctggctgatagagtgagatactgtgtcaaaaaataaaaataaagaggggatcaatacacatacgtcccccaaaacatgcctgaaacacgagaagggaaagtgagggcagttaacaggatgccctgctggcacagtgcttcttagtagatgctagaaggtttgaggcccagatttcagcccagcatatggctttttgcctgtaactgaaccatgtcagtgtgccagatggtctgaagaaagggtttctggaggaaattattattagctgcatgggagtatggtttacactagagtagaagagctgggagcatcacgtttgaaggggaagacagtgactgggtggaggggcaagggattagtatttagagtgtgcaactattgaaaataaggtatattttaatgtgtaagaggacatgtacttatatgttatatataaattattttagctgggtgaagtggctcatgcctatagtcctagcactttgggaggcccaggcgggaggatcacttgagcctgggagtttgagaacagcctagacaacatagtgagaccctatctatacaaaaataattttttttaaattagccacgtgtggtggtttgtgcctgtagtcctagctactcgggaggctgaggtgggaggattgcttaagcccaggaggttgaggctgcagtgagccatgatcgcaccactgcactccagcctgggtgacagagcaagaccttgactcaccaaaaaaaaaaaaaaaaaaaagagagagaaattaaaaatactgtaatctcagctgggcatgggggttcacacctgcagtcctagcactttgggaggctgaagcaggaggatcacttgaggccaggaactcaagaccagcctggcaacatagcaagaccccactacacacacacacacacacacacacaaagaagagaaagaaaaaaacgaaacaaaactgtaatctctgcagctgtcctcagtgtggagggggtagccctgtctgttccccttcagcacttgctgttttgactctctgggttctttgtgcaggtcttgatggggagtctctggtttgccattctttgtttgatttaactttctgtaatcataaagccaatgatgggctttttttttttttttttttttagactaagtcttgctctatcacccaagctggagtgcagtggcaccatctcggctcactgcaacctccacctcccggttcaagcaattctcctgcctcagcctcccgagtagctgggattatgggcttgtgccaccatgcccagctgatttttgtattttttgtagagaaagggtttcgccatgttggccaggctggcctcgaactcctgacctcaggtgatctgcccacttcagcctcccaaagtgctgggattacaggcgtgagccactgtgcctggcctaatgatgggctctttaatgtgatcctttagggttggcgccttgccctagttgctgttgaaaaaactatttttgtccaaatagcacacacacagaaacctaccaacttccctcccactttttcctaggaattccttctgagggatttcttgagatggggcagaatggggcttggaagagggagttggagctaattgaccgttgcctttctcctttgttggggtcctgagtcttgttcctgctgtaagagttactcacttcctgtctgccacctatctccctttgcatgtgtgcttcagttgggagatctgtttatcagcccctgccacacggctctttgttccttctgcagaggacgttggggtcccacggctggtccttttgactcattttgctttcaaggtcccacctcccagtctgaggctgcatcctccattaccatcgcccttcctgtgggctgggaggccaggtcctttcctgcccagcgatgtcagcgtttcctcaggggccaggcactcatcaggagaaaggaactaattacttgagtaatttgccttgccttgctgagaggagtgtgccctgagggactccatgtgagtgtggtgacgggtgtgggggtgtccctgtgttattttaaaatgggtgccttcaggacgatgagcatgtgaccatttcctctctatttccatcacaagagtattatggtatgagggtctcaggttagattatcctcccaagactcttctctcttccttctctactggaagcccacatagcatttccttatggcttgagggagaggttcggagccacttacaaattagataaagtacatttacaatcttgtacaaagccacacaatgaagtcatttttctcagctttttttttttttttttttttttttttgagcctgagtctcgctctatcgtccagactggagtgcagtggcgcgatcttgcttcactgaaacctctgcctcccaggttcaagagattctcatacctcagcctcctgagtagctgggattacagacatgcaccactatgcctggctaatttttggatttttagtagagaccgggtttcaccctgttggccaggctggtctcgaacccctgacctcaagtgatcttcccgcctgggcctcccaaagtgctgggattataggtgtgagccacagtgcccagccttgtttttgtttttgttttgttttgacagtctgtcactctgtcacccaggctggagtgcagtggtgcgatctcacctcacttcagcctctgcctcccaggttcaagtgattctcctgtctcagcctcctgagtagctgggattacaggcgtgccaccacgcccagctatttttgtaatttcattaaagacagggtttccccatgttggtgaggctggtcttgaactcctggcctcaagtgatccacctgcttcagcctcccaaagtgcagggattacaggcatgagccactgtgcctggcctcagctatcttgaatgctggagaattaaatccttttctgtctagggtgtcagctccctaagggctgggccaaaacagttggatttataagacactagagtcttgcctcagtagctcctttgaattctgcactgaattgatcagtttcttggcccaaagtaaactcagatggcagcccaagagccactctgcagtgccttctttcacatggtcatcatgctctctgatccctcaggttctgtctaagcctcatgttttatgaccgtgctgttctcagcccacctcaccctgccccatgccttctcaatggtttgttcacctgaattccccagatttcatgccagtatccccaaggttccttgacctcttggtgtaagcattcagcatctaaaattcattttattcccgtcaacgcatttctaactgtagaacaagaattataaatgacaaagctcatagaaaattggcaccttgtcttccccctccctcttattttatacataaaagagaatatgggctgggcattgtggccaaggctgggcatgatagctcatacttgtaatccagcactttgggagggtgaggcagatggatcacctgaggtcaggagttcaagaccagcctggccaacatggtgaaacctcatctctactaaaattacaaaaaaaaaattagctaggcatggtggcagatgcctgtaatccagctactcaggaggctgatgaaggagaatcacttgaaccctggaggcagaggttgtagagagccaagatggcgctactgcactccaacctgggcgaaagagagcaagactccgtctcaaaaaaaaaaaagacaaaaattagccaggcatggtggtgccacctgtagtcccagctgcttgggagcctaaggcaggagaatcgttttgacctgggagtaggaggttgcggtaaccgagattgtgccactgcacttgagcctgggcaacagagtgagactctgtctcaaaacaataagaacaacagcaacaaaagagagagaccatgccttgctccaggtctcttagctattgaagatgtacctggacccaggtctccggtcttctagttgaagcaattgtactgccttacaaagtcacattctctttggtgctttttgattgacgtatttatccaactagaaagttactcatgccctcatccaaaaatgtggtagaggccagattagtgctggtaggaataagagatataacctttggctttggaaccacaagcattagcagtctccatgttctttaaagacttggtgatattggtatttaggctggacaccatgcaaagactacacaggctcggttcctgcatgcagagaagttatctaagagatatgaccaggccggaatagaatgctcagaccacgtggaggctgttaaacttttacataatctagggaaagaagggacacaaggtggcattagtctagggtcaggtgggaaaaggttatgctgaaaagtctctgcagctcaggacagctttgtgcaaagaactgaagttcacagctgctagtgcctgggagatcaaatagtataaatgagggcagacaaccctgaggggcagatggagctttccagacaatcttggcatgaggatgagtgagtttcaaatcagtcctgccgaggcagatggcttcctccagctctgcttactgaatgcgaagtcacagtcagtaagaaaactggttttcttcttcccaggcgctgccccatacctgaagaccaagtttatctgtgtgacaccgtaagtggcttcctttccccgttttgccttcatttctaatatcctcagttatccctgggaatgggacactgggtgagagttaatctgccaaaggttggaagcccctgggctatgtttagtactcaaagtgaccttgtgtgtttaaaaagcttgagcttttatttttctgttggagaccagagtttgatggcttgtgtgtgtgtgttttgttcttttttttttttccattgtgtcttgtcaaccccccgtttcccctcctgctgccccccatttcctacagaacgacctgcagcaataccattgacctgccgatgtccccccgcactttagattcattgatgcagtttggaaataatggtgaaggtgctgaaccctcagcaggagggcagtttggtgagtatttggttgacagactttgtccctataagggaagttggtcccctttgtgtgatgctctcacatgtacacaccgagagctggtcactcggaatggtaggagattctagagctttgctttccaaaagagatggtatgaatgccacatgtgtgagtataaatcttctagcagccacactggaaatagacgaacttaatttttacaatatattttatttaacccactaaatccaacatactctcaatttaacatttcagaaaaagttgaggctgggtgagtggctcatgcctgtaatcccagcactttgggaggccgaggtgggtggatcacttgaggtcaggagttcgagaccagtctgaccaaaatctctaaaatataaaaattagctgggcatggtggcgcatacctgtaatcccagctactcaagaagctgaggtgggaggatcgcttgagcctgggaggtggaggttgcagtgagcagagatcgtgccactgcactccagcctgggcgacagagtgagactccatctcaaataaacaaaactaaactaaaaagaaaaagttgagacctttttttattcttttttttcatactaagcctttaaaatccagtgggcttttgacagccacagcacagctcagtttggacaaaccaaatctcaaatgcttggtggccacgtgtgtctcggggctcctgaattaaacagtagatcaagggcagaagatctcaggacagccttagagcttctgtaaacatggagctctgggaatcagttaaggtgggaatgagaaaggacccttcccgaggcagggtcctccagggaggagggtaaatctggcttttctgaccatccctgggccttaaggggcaggagattggatagcagtggtagcctgggccctgtcctctgaagggctgggggcgtggcctgccagttgcagagggtggacaactgaactagttttccctgtctgtccctccagagtccctcacctttgacatggagttgacctcggagtgcgctacctcccccatgtgaggagctgagaacggaagctgcagaaagatacgactgaggcgcctacctgcattctgccacccctcacacagccaaaccccagatcatctgaaactactaactttgtggttccagattttttttaatctcctacttctgctatctttgagcaatctgggcacttttaaaaatagagaaatgagtgaatgtgggtgatctgcttttatctaaatgcaaataaggatgtgttctctgagacccatgatcaggggatgtggcggggggtggctagagggagaaaaaggaaatgtcttgtgttgttttgttcccctgccctcctttctcagcagctttttgttattgttgttgttgttcttagacaagtgcctcctggtgcctgcggcatccttctgcctgtttctgtaagcaaatgccacaggccacctatagctacatactcctggcattgcactttttaaccttgctgacatccaaatagaagataggactatctaagccctaggtttctttttaaattaagaaataataacaattaaagggcaaaaaacactgtatcagcatagcctttctgtatttaagaaacttaagcagccgggcatggtggctcacgcctgtaatcccagcactttgggaggccgaggcggatcataaggtcaggagatcaagaccatcctggctaacacggtgaaaccccgtctctactaaaagtacaaaaaattagctgggtgtggtggtgggcgcctgtagtcccagctactcgggaggctgaggcaggagaatcgcttgaacctgagaggcggaggttgcagtgagccaaaattgcaccactgcacactgcactccatcctgggcgacagtctgagactctgtctcaaaaaaaaaaaaaaaaaaaagaaacttcagttaacagcctccttggtgctttaagcattcagcttccttcaggctggtaatttatataatccctgaaacgggcttcaggtcaaacccttaagacatctgaagctgcaacctggcctttggtgttgaaataggaaggtttaaggagaatctaagcattttagacttttttttataaatagacttattttcctttgtaatgtattggccttttagtgagtaaggctgggcagagggtgcttacaaccttgactccctttctccctggacttgatctgctgtttcagaggctaggttgtttctgtgggtgccttatcagggctgggatacttctgattctggcttccttcctgccccaccctcccgaccccagtccccctgatcctgctagaggcatgtctccttgcgtgtctaaaggtccctcatcctgtttgttttaggaatcctggtctcaggacctcatggaagaagagggggagagagttacaggttggacatgatgcacactatggggccccagcgacgtgtctggttgagctcagggaatatggttcttagccagtttcttggtgatatccagtggcacttgtaatggcgtcttcattcagttcatgcagggcaaaggcttactgataaacttgagtctgccctcgtatgagggtgtatacctggcctccctctgaggctggtgactcctccctgctggggccccacaggtgaggcagaacagctagagggcctccccgcctgcccgccttggctggctagctcgcctctcctgtgcgtatgggaacacctagcacgtgctggatgggctgcctctgactcagaggcatggccggatttggcaactcaaaaccaccttgcctcagctgatcagagtttctgtggaattctgtttgttaaatcaaattagctggtctctgaattaagggggagacgaccttctctaagatgaacagggttcgccccagtcctcctgcctggagacagttgatgtgtcatgcagagctcttacttctccagcaacactcttcagtacataataagcttaactgataaacagaatatttagaaaggtgagacttgggcttaccattgggtttaaatcatagggacctagggcgagggttcagggcttctctggagcagatattgtcaagttcatggccttaggtagcatgtatctggtcttaactctgattgtagcaaaagttctgagaggagctgagccctgttgtggcccattaaagaacagggtcctcaggccctgcccgcttcctgtccactgccccctccccatccccagcccagccgagggaatcccgtgggttgcttacctacctataaggtggtttataagctgctgtcctggccactgcattcaaattccaatgtgtacttcatagtgtaaaaatttatattattgtgaggttttttgtcttttttttttttttttttttttggtatattgctgtatctactttaacttccagaaataaacgttatataggaaccgtc

SEQ ID NO: 31 - protein, 770 aa, Artificial Sequence
  STAT3 Amino Acid Sequence
MAQWNQLQQLDTRYLEQLHQLYSDSFPMELRQFLAPWIESQDWAYAASKESHATLVFHNLLGEIDQQYSRFLQESNVLYQHNLRRIKQFLQSRYLEKPMEIARIVARCLWEESRLLQTAATAAQQGGQANHPTAAVVTEKQQMLEQHLQDVRKRVQDLEQKMKVVENLQDDFDFNYKTLKSQGDMQDLNGNNQSVTRQKMQQLEQMLTALDQMRRSIVSELAGLLSAMEYVQKTLTDEELADWKRRQQIACIGGPPNICLDRLENWITSLAESQLQTRQQIKKLEELQQKVSYKGDPIVQHRPMLEERIVELFRNLMKSAFVVERQPCMPMHPDRPLVIKTGVQFTTKVRLLVKFPELNYQLKIKVCIDKDSGDVAALRGSRKFNILGTNTKVMNMEESNNGSLSAEFKHLTLREQRCGNGGRANCDASLIVTEELHLITFETEVYHQGLKIDLETHSLPVVVISNICQMPNAWASILWYNMLTNNPKNVNFFTKPPIGTWDQVAEVLSWQFSSTTKRGLSIEQLTTLAEKLLGPGVNYSGCQITWAKFCKENMAGKGFSFWVWLDNIIDLVKKYILALWNEGYIMGFISKERERAILSTKPPGTFLLRFSESSKEGGVTFTWVEKDISGKTQIQSVEPYTKQQLNNMSFAEIIMGYKIMDATNILVSPLVYLYPDIPKEEAFGKYCRPESQEHPEADPGSAAPYLKTKFICVTPTTCSNTIDLPMSPRTLDSLMQFGNNGEGAEPSAGGQFESLTFDMELTSECATSPM

SEQ ID NO: 32 - DNA, 4953 bp, Artificial Sequence
  STAT3 mRNA NM_003150.3
ggtttccggagctgcggcggcgcagactgggagggggagccgggggttccgacgtcgcagccgagggaacaagccccaaccggatcctggacaggcaccccggcttggcgctgtctctccccctcggctcggagaggcccttcggcctgagggagcctcgccgcccgtccccggcacacgcgcagccccggcctctcggcctctgccggagaaacaggatggcccaatggaatcagctacagcagcttgacacacggtacctggagcagctccatcagctctacagtgacagcttcccaatggagctgcggcagtttctggccccttggattgagagtcaagattgggcatatgcggccagcaaagaatcacatgccactttggtgtttcataatctcctgggagagattgaccagcagtatagccgcttcctgcaagagtcgaatgttctctatcagcacaatctacgaagaatcaagcagtttcttcagagcaggtatcttgagaagccaatggagattgcccggattgtggcccggtgcctgtgggaagaatcacgccttctacagactgcagccactgcggcccagcaagggggccaggccaaccaccccacagcagccgtggtgacggagaagcagcagatgctggagcagcaccttcaggatgtccggaagagagtgcaggatctagaacagaaaatgaaagtggtagagaatctccaggatgactttgatttcaactataaaaccctcaagagtcaaggagacatgcaagatctgaatggaaacaaccagtcagtgaccaggcagaagatgcagcagctggaacagatgctcactgcgctggaccagatgcggagaagcatcgtgagtgagctggcggggcttttgtcagcgatggagtacgtgcagaaaactctcacggacgaggagctggctgactggaagaggcggcaacagattgcctgcattggaggcccgcccaacatctgcctagatcggctagaaaactggataacgtcattagcagaatctcaacttcagacccgtcaacaaattaagaaactggaggagttgcagcaaaaagtttcctacaaaggggaccccattgtacagcaccggccgatgctggaggagagaatcgtggagctgtttagaaacttaatgaaaagtgcctttgtggtggagcggcagccctgcatgcccatgcatcctgaccggcccctcgtcatcaagaccggcgtccagttcactactaaagtcaggttgctggtcaaattccctgagttgaattatcagcttaaaattaaagtgtgcattgacaaagactctggggacgttgcagctctcagaggatcccggaaatttaacattctgggcacaaacacaaaagtgatgaacatggaagaatccaacaacggcagcctctctgcagaattcaaacacttgaccctgagggagcagagatgtgggaatgggggccgagccaattgtgatgcttccctgattgtgactgaggagctgcacctgatcacctttgagaccgaggtgtatcaccaaggcctcaagattgacctagagacccactccttgccagttgtggtgatctccaacatctgtcagatgccaaatgcctgggcgtccatcctgtggtacaacatgctgaccaacaatcccaagaatgtaaacttttttaccaagcccccaattggaacctgggatcaagtggccgaggtcctgagctggcagttctcctccaccaccaagcgaggactgagcatcgagcagctgactacactggcagagaaactcttgggacctggtgtgaattattcagggtgtcagatcacatgggctaaattttgcaaagaaaacatggctggcaagggcttctccttctgggtctggctggacaatatcattgaccttgtgaaaaagtacatcctggccctttggaacgaagggtacatcatgggctttatcagtaaggagcgggagcgggccatcttgagcactaagcctccaggcaccttcctgctaagattcagtgaaagcagcaaagaaggaggcgtcactttcacttgggtggagaaggacatcagcggtaagacccagatccagtccgtggaaccatacacaaagcagcagctgaacaacatgtcatttgctgaaatcatcatgggctataagatcatggatgctaccaatatcctggtgtctccactggtctatctctatcctgacattcccaaggaggaggcattcggaaagtattgtcggccagagagccaggagcatcctgaagctgacccaggcgctgccccatacctgaagaccaagtttatctgtgtgacaccaacgacctgcagcaataccattgacctgccgatgtccccccgcactttagattcattgatgcagtttggaaataatggtgaaggtgctgaaccctcagcaggagggcagtttgagtccctcacctttgacatggagttgacctcggagtgcgctacctcccccatgtgaggagctgagaacggaagctgcagaaagatacgactgaggcgcctacctgcattctgccacccctcacacagccaaaccccagatcatctgaaactactaactttgtggttccagattttttttaatctcctacttctgctatctttgagcaatctgggcacttttaaaaatagagaaatgagtgaatgtgggtgatctgcttttatctaaatgcaaataaggatgtgttctctgagacccatgatcaggggatgtggcggggggtggctagagggagaaaaaggaaatgtcttgtgttgttttgttcccctgccctcctttctcagcagctttttgttattgttgttgttgttcttagacaagtgcctcctggtgcctgcggcatccttctgcctgtttctgtaagcaaatgccacaggccacctatagctacatactcctggcattgcactttttaaccttgctgacatccaaatagaagataggactatctaagccctaggtttctttttaaattaagaaataataacaattaaagggcaaaaaacactgtatcagcatagcctttctgtatttaagaaacttaagcagccgggcatggtggctcacgcctgtaatcccagcactttgggaggccgaggcggatcataaggtcaggagatcaagaccatcctggctaacacggtgaaaccccgtctctactaaaagtacaaaaaattagctgggtgtggtggtgggcgcctgtagtcccagctactcgggaggctgaggcaggagaatcgcttgaacctgagaggcggaggttgcagtgagccaaaattgcaccactgcacactgcactccatcctgggcgacagtctgagactctgtctcaaaaaaaaaaaaaaaaaaaagaaacttcagttaacagcctccttggtgctttaagcattcagcttccttcaggctggtaatttatataatccctgaaacgggcttcaggtcaaacccttaagacatctgaagctgcaacctggcctttggtgttgaaataggaaggtttaaggagaatctaagcattttagacttttttttataaatagacttattttcctttgtaatgtattggccttttagtgagtaaggctgggcagagggtgcttacaaccttgactccctttctccctggacttgatctgctgtttcagaggctaggttgtttctgtgggtgccttatcagggctgggatacttctgattctggcttccttcctgccccaccctcccgaccccagtccccctgatcctgctagaggcatgtctccttgcgtgtctaaaggtccctcatcctgtttgttttaggaatcctggtctcaggacctcatggaagaagagggggagagagttacaggttggacatgatgcacactatggggccccagcgacgtgtctggttgagctcagggaatatggttcttagccagtttcttggtgatatccagtggcacttgtaatggcgtcttcattcagttcatgcagggcaaaggcttactgataaacttgagtctgccctcgtatgagggtgtatacctggcctccctctgaggctggtgactcctccctgctggggccccacaggtgaggcagaacagctagagggcctccccgcctgcccgccttggctggctagctcgcctctcctgtgcgtatgggaacacctagcacgtgctggatgggctgcctctgactcagaggcatggccggatttggcaactcaaaaccaccttgcctcagctgatcagagtttctgtggaattctgtttgttaaatcaaattagctggtctctgaattaagggggagacgaccttctctaagatgaacagggttcgccccagtcctcctgcctggagacagttgatgtgtcatgcagagctcttacttctccagcaacactcttcagtacataataagcttaactgataaacagaatatttagaaaggtgagacttgggcttaccattgggtttaaatcatagggacctagggcgagggttcagggcttctctggagcagatattgtcaagttcatggccttaggtagcatgtatctggtcttaactctgattgtagcaaaagttctgagaggagctgagccctgttgtggcccattaaagaacagggtcctcaggccctgcccgcttcctgtccactgccccctccccatccccagcccagccgagggaatcccgtgggttgcttacctacctataaggtggtttataagctgctgtcctggccactgcattcaaattccaatgtgtacttcatagtgtaaaaatttatattattgtgaggttttttgtcttttttttttttttttttttttggtatattgctgtatctactttaacttccagaaataaacgttatataggaaccgtaaaaa

SEQ ID NO: 33 - DNA, 32729 bp, Artificial Sequence
  Genomic Sequence
ttttttaaaattaagaaaaggaatcaatttaattaaataccaaaaagttttacatattcctgaattttcaaccagctacaaaaagcatggatttttcttattagaaaacaaaactgttacaaaaaatttaaataaataaatagctgccataaaatttcaacataatatatagtcaactagttctgtgttatggtcagttaatagaaagatagcgggaatgatgatatgagcaaaagtaaacagaacaaagaagaaaaaagataggaaaaagaaagttagacagagaagagaaaaataaagaaagtgctttattgaatgagctaattacatgaggtcaccaagaggaacatcctctaactgaggcgctgtgatgacaacaacacccgatgctgtcattgtcctggtgtcttcctcaccctggcgtaaaggagatgcccaagctctgcacaggaaggcatcgtcggcaagctctcttctccgacactccaccggaaggatcacagagctgtggtcttggcctggatggatcgcagctctctccacctgagggcccccagctggagggaccggagaacactggcgtctggcagccccgtttccactcctaccaagaaggctcaaagacgacggtcagctcaggcttttcttcttgaagtgtttctaacgcactttttgtctcataattgaaatacatttcagacaacctgtaaaagcaaatagaaagcctgggttgcactcttcagataactctgtcagagtcgttaaccttaaaagtctcatctcttcatttccctaaactccacacacttctaaaatgtaaaaaaaaaaaaaaaaaaaaaagagggaccacaactcccagagtgctccgcgtcctcgccgccgtcgccgccgccgagaccaagatggccgcgagactccgcaccttcttcaagaatgcctgggccaaggagccggtgctcgtcgtgtccttcgtcactgggagcctcagacccccaggaccccagcctggagtggctgaagaaactgtgagcacctccaatgacagaggaggcccctcccacggctcccaataaaaatgtggggaaaaaaaaaaaaaagctctaagtgcccaatgtggttcctgttatatttttaactatctagttgggaaaatgttaagcatacataaaagtatagaaaatagtataatgaaccccctgtgtccattacccaagttcgacaattaaacaggtcatgtcaacttgtttcttctattgcccacccactcctcccacccatggattattttaaatactgcatttaatgcatctatcaataattcactttgtgacactaaaatataattacaatgtcactatcacaccaaaatcgtttaacaataatttcttagtatcactgtatgtccagtcagcatttacgcttcctcaactgtcttgtaaatttttttaccttatgttcatttagtcactaacctgatcaattctacacattgcatttgcccaggatgcctctcacatcttcgatgtaagttcttcctcctctttaataaagtttcccttgcaacttaactaataaatccacccatttgtcctgcaccatttataaccatctcaatttggtggtgttatatactgaatgtttgtcttccttaacaattcccatgatgaagcccgaacccctaatgtacggtacttaaaggtgaggcccttgggaagtagttagagttagatgaagttgtgagggtggggccctcagtatggggtgagtgcccttacaggagagatatcagagagtttgttctttctcccctgtcttctctcccttgcctcccctccctccatgcaatcacataacaagaaggtagccatctgcaaatcaggaagaggactctcgccagcaaccaaattcatcagagacttgattttggactttctagcctccagtattgtgagataataaatctgtgtttgagtcacacagtctaaagcagcttgttatcgcagcctgagaaaacgggttgattgcattcatggattcttcaatctattttgagcctgtccctcagcctgggtccagaatgtccctcagggctaggtcagtgatgctacatgtagcagtgtccccagctttgacctgaccaatcctttgtttgttcccccatctctcttagctctgggaatattggcttgtcctgcagcaaatgtgctccattatgttggcacaaggatgcaaggctgattcaaacttgtatttattcaaacctgcattccaacaagttctcagccttgagatcattaatatggacagaagtccctggactaatggaatttatattttgggagcagagatagataataaataaacaagaaaatgacatagcacataagatgtgctacactgcagaggagaatgagaagagaagaaaaagtgcttctattttcagtagaatagtcaaagacagcctcgcagagaagacctttaagcagagaatttaggaaggtacagggaataatgcaggtggatactgaaggggagagagttctaggccagaagaaaagcaagtgcaaaaatccagagatgacagtgttcttgcaaaacagcaaggagatcactgtactggggcagaataagcaagggttgggagaagcggaatcttcggaagcaggagaggctggattatgtggggcatggaagccaccatgagtttgttgctctgattatgaaagtgataagaagacgatgttgacaagagtgatatgatgcgagttacgttttagctgaatcccttgtctgctaaaatcagaataacagatgcagggtgacctgtcagaatgccaccatgacaatccagacaccaggtgatggtggcttgagccaaggaagaagccgtgaagctggcctgaagtggtcagggagtggccaagctgggaaggcagagctcacaggatgtgctgacacattggacatgattataaggaaaaagagacagtgacgacagaaccagaaatgttttggcccgagcaacttggaggaagtgaccatcgactgaaatggggaagaatcaggtttcgggtagaagagagtagcaagggtgtggatctagatgtgacgtttgagaggtttattaaaccttcaagaagaaagatcagccaagcacggagacacagaatttatggacatataatctggaggccacagcacacatatcatgaagccagaagaccagataatttaaatgagggagaaagtgtagggaagaaaaattagcccagcgactaagctctgaggattcaacacataagggtcaggatgatgaagaagaggccagaaaggagactgagtagaaggatctgatgaaataggagaaaacccaggagagcatgttggccttaaagccaagcagtgaaaacgtcttcagggaaaagtgcaatcatcacggctgacagaaccgtgggactcgccaggaagctcttgctagagaggagacgactacctcagtagtatcacagaggtgggctggcaatatcctgacacactgtcgaatttcgtgtaatttcccatcttgctattcctggagcactcttttcccatttagaaatcctcagaaaccgccaggcacggaggctcacacctgtaatcccagcacttggggaggccgaggcaggcagatcacgaggtcaggagatggagaccatcctggctaacacagtgaaaccccaactctactaaaaatacaaaaaattagccgggtgtggtggcaggcgcctgtggtcccagctacttgggaggccgaggcaggagaatggcgtgaacccgggaggcggagcttgcagtgagccgagatcatgccactgcactccagcctgggcgacagagcaagactctgtctcaaggaaaaaaaaaataaatcctcagaaacaaaacaacaagatccccactatgtaaagacccttccaatttggatgacccatagacgagttctacgaagttcggttccttgtgtagaacagaatcctccttggccatgatcgcatgagggcttgtgtttctttggggaatgtgggtgaaatccagcttagccttggtgattctaaccatctcagtgaagtggaatgtgtagtttaaccccatattctctattttaaaatatccaccacaactgacccaggcccaacctaatcttgagtggctgcaaatgaagcgagagccatcctggattttgataacagtcaacgtttcctgagaactcagagtcccaccacgggcatctctgcagagcacactcaccccaggttctgcaggaggcagctctgctgtttcagcacttcacagaacatcatgacccccaggtcgcccaggtcattgttgcccaggctcagctttcgcaggctctggctggaggtcagaagtgtggaaagatcccagcagcagtgtgacgtgaggttgcagttgtctaatctgcaaaaagggggtgatttaaagaaaatgtccccttaaccatccccctagctccccaagattttagcatcttagcctgtcttgtttcaggtggaaaaaaaaaaagcacaggagcacaggactaactagcttcaagcagccttgtatgctggtaattattcttctctctctttttcaaatccactgcattgcacagatcaaattagtaacagtggtttgttcattgatttaccaaattctgtgcctttccctacatttccataaaatgtaagtgtcatactgccctccttgttttgtggtacagaaaactgtgatggtaaggactcaagttcctacatctatatcatctggaaggactcctcccagtcccatgatcctgtaacaaggcaaacactaagaagacacctcacttctaagatacagattatcttgtggccactctgcctaaacgtccctccacccttggccaccatgtgttctcattgctgtaataaaccaaaggacttactccaacacctgaagcttgcagtcggggtgcaagagtccctcacagagtagtttgatccccttgtctccgagagtgttgcctcgcaggtaaaggtgcgtgagattctgattagtgctgagtaccgaggacaaagctgaacaacagactgacgtaaggccagaattcaccaacctgtagaaggacagggagaagagtcctcagtacccagctgttccccaacattgtgcagctgctttgactcagtgcctcgtcctctctcagcagctgcagccttcagctcagagagcaggagccagcatctcagatatgatctggggagagcaagacctgctgtctctggctgtcacaggagacacaaatgatgtctcagcagatgctttgctgtatgagtccgacagaaagagccaaggcaaactgagccagttaccccatactcctcctcctcctcacacagctttcctccggccaggagtgctcctcagcaccacttcttccagaaacacatcccagtggttatcctcaactaataatccccgtaacactgcagacacccacactgcaggggcctttttttttttttttaagagagacaggaaaaaaaaatcctcctcatgggaagtcggtgctgatttaaacatcaaagacaacaggtgaacgtccattgtgaccttctaagctgtagctagggctgtgacaggaacacggcggggcccttagcaattgccacctcccgccttcctgcgcccccaaatgcccctttcacatctttctcgctgcagccctcaaccacgttggagaggtgggaggatcgcttgagtccaggaagtcgaggctgcagtgagccatgattgcgctgccacactctagcctgggtgacagagtgagaccctgcctaaataaataaataaataaggccaggtgcagtggcttatgcctgtaatcccagcactttgggaggtccagcactttgggagggtggatcacgaggtcaggagttcaaaaccagcctggccaacatggtgaaagcccatctctactaaaaatataaaaattagttagggtggtggtgggcacctgtaatcccagctacttgggaggctgaggcaggagaattgcttgaacctgggaggcagaggttgcagtgagccgagattgccactgcacttcaacctgggcaacaaagtgagactctgtctcaaaaataaataaataaatagaaaaagccaggctcttgctcagtcacccaggccaagtgcacagctcactgcagtcttaaactcctgggctcagacaatccacccaccttggcctcccaaagtgctgggattacaggcatgagccactgtgcctgacccagagaccagtcttatttgattattatatcaacctggcaaggaaggagtgcagctaaaactattacatacattttacatattagaaatctaaggcttataaaaattacatgtttctctcaaggccacagagcaggtgtgtggtggggagggatccagacctggactttccaccttttagtctcatcttctccccactgccctttctgtccacctctctcttccttctgcacagcaaaaggccttttagagcataaaaccccaaaaatgcatcaatctcgatggaattaagagttttgatgtactattcttgagtcaaattaagcccattctatcacccaggaagagcataagagctctaaaatcactggtggcgtaattcctaggagcacagatgcttctattccatgaagccaggaatagcgcaggtgattgcctccttcctgccagagtccttggcaatggcatgttttttaagctctttggtgtctacgaggcaggaaaaatagaaatacagaaaaagtgtattcagacagtaaagcatgaacagatgaccagcaggaaaaagtgattatccatccactggtttctatcttcccaattaaggaagagtcaaactgaaaagacacagtaagtaagactaataggcaaatgaagcccaagagagacagacaaaaacaaagcaagttttgagtggcttctactaagctctcatccccggtaagaattctatcagagggttgttgttaattaacatgcagaagggattagtagcattcctggcaaaggccagggacattctagtagaatggggatggtcttcaaagaggaaaagagaaaatattttttaaattatgtaattaaagttatgcaggctttaccactatttccaaaaaggagtagaatggattattcaacagatgtttggggagcactacacagtagtagtagaaattgcaacagacggtgcagttttgttaagaaaacgtcatatccaaattgtgaaaatgctggtaactattaagcaacggttacactgaacacataataaaatgtttaaagaatcaaacaaccatgtcccaccaaccaatccttggattagaggaatgtgattgacatctcgatttcaaccaatccacctaactgagctctacatttaccaagcacggatatcttgccatgtactgtattaagttaattggttggggatttttatttattaactacctgcctatgtcacaaaactgtctcataatgaaaactgaatcccagtgctttgggaggccaaggtgggaggaccacttgaggccaggagtttgagaccagcctgggcaacatagcaagaccctgtctctacataaaaaattttaaacattttaaacattacccaggcatggtagtacacacctgtagtcctagctagtcagaaggctgaggcaggaagattgcttgagcccaggagagttcaaggctacagtgagctatgatcctaccactgcactccagtctgagccacagagcaaaaccctgtcttaaaaaaagaaaagaaaagaaaggaaaataaggaaaggaaaggggaaagggaaaggggggggggaggggaagggaagggagaaagagaaagaaagaaagagagagagagagaaagaaagaaagaaagagaaaaagaaaaagagagaaagaaaggaggaggaggaagaaggaaggaaggaaggaaggaatctgaagaagaagatcaaacattttttgagtatttattgtgtgcttgacatggatgacgactttaaacagggttatctcattgaatgatcacaacctcaagatgggaatgttagttttatccctgcttttaaatggacaaaatgaggatcacagtaattaaaaaataagtaggagcttcttagatggatagtagaaagtgggaaagtgggggtaaccttccaggcaaaaggaaaagagtagcaagaataaggaagattaaaagaaccaccaagatgtttcaaaactaattcatagctgggcacagtgatgtccacctatagtcccagctacttgggcggctgagacgggaggattgcttgagcccaggagtgcagatgagatcaggcactctgggtggtatggctgtagatgaacccaggaattcaaattcagcctgagcatcatagcaagtccccatctctaaaacagcaaaacaaaactcatccaatatgactcaaaatggagtgcaaggtatggcaggagagagggcagtatcagggacagccttgtgtgccaagctaagatgtcactctgactgcagagaagaacttttgaagatttttgaacaaagggtcaatattttcaaatttgcatcttaaaaagttccctctggtgtagtgatgagtggtagagggaaccgaaagcagagcatttaggaccgtcccccgtttactcactcagcagcctcctggaaagccccactattcaatgaggcaggaggaagagggcaggagcaggtcagagaacgggggtggaaggtggggtatgataattaaaccaatgttgcaaatgctcagcatgtgtgacccttgagcagtattgagacaggcagtacacaatatgcagccagagatgaggacccaaagttcgagagaaaaaaatgtagctatacctaacacataggctatacctaacacataggctatacctaacacgtaggctatacctaacccataggctatacctaacacacaggctatgcctaacccataggctatacctaacacacagccacatgtatggctgtacctaacacataaaatgcataaaagtctcgactgattaatgccacttatagatacctatctcaaagcaaatacacatgcataaaactatatatacaaatgtgctttttgcagagttgtttgtaatagtggaaaagaacagttatcccaaaatgcatgatttgattaaataaattatggtaaagcacactatgggatattatgccccaatcgatagatctacacaaatcagcatggaaatttatccatgataaatgaaaaaaggatatcacagaaaaatatttatattatggttctagtttcaatagatagggtgttatggattgaattgtttcctctaagactttatatgtggaagtcctaggccccagtacttcagattgtgaccttatttggtgatacggttactgaaaatgtaattagttaagatcaggtcgttacaaatctaacatgacttgtgttctttcacagggaaacttgggacatggagaaagacacacacagacacagggaagacaccacgtagagataaaggcaatggtgtggcagaggcatctacaggtcaaggaatggcaaaatgtgtcagcaagatgacattccaccagaagccaaagagaagcatgaacagattccccacagccctcagaaggacccagcctgctagcatcttaatctcacacttctggcctccagaactgagggacaataaatttctgttgtttaagctgctctgtttgtgatactttattacagtagctctaacagactaggcatttaaaatactacataacaatgtattacaaatgcaacatgaaaatcacataggtcttcattcacattactgatataaataccacccagatcagcatatacaggaaatccatttgtccataattagcaaccaatatatgttcacaaagctctgatactcccttggatggattgatggatggatggatggatggatggatggatggatggatggattgacggatggaaaatagagggatggatgatggatggatggatggatggacagatgaatggattatataacaatctattgtattaaaaaaagtctggatggttgttcatcagactattgtaaatggctctctcagaagagggctgagaaggagctttcactttccactttgtctgtactatgatatgtttacaccaagcatgtgttacttttctaataaaaagtttgtgaatgatatctgggtttgagacctactgttgttgaaattgagaggtatatgagaattctcagggagtttagaaatatttagtaacaacaacaacaaaaaaggtaaaccaggcgggtgtgtggctcacgcctgtaatcccaacactttgggaggccaaggcaggcagatcacctgaggtcagaaattcgagaccagcctggcaaacatggtgaaaccccgtatctactaaaaatacaaaaattagccaggcatggcagtgcacacctgtagtccctgctactcagaaggctgaggcagaagaattgttggaacccgggaggcagaggttgcagtgagccaagattgcgccactgcattttagcctgggtgacagagtaagactccaactcaaaaaaaaaaaaaaaaaaaaaaacacaactaaaccagtcgtgaaatccccagaccacaggaagagaagccaatgcaggatccagggagggggaagctataacattagcaggaaagactaagtagtgacctaaaaataagagcgaagaaggcttccaaagaggaagagtgaaatgaattaaaggcagcagatgtcaactaaagtaaggactgggaaggacctgtacgacctataaggacccagcctgctgatgcctcagtctcagactttggcctcctgaactgagaggcaataaactcttgttgtttaggccgctctgtttgtgatactttattacagcagctctaccaggttaggtattgacaatagtaactacatagagcatattacagatgcatcaggcacatttgtaattggcttgtttgtcatgtggaatttggaaccaggatcactgagagtcacctgagtgcctacgcctgggcctcttcggttccatctgctttgcctggagggctcttccggctccttcacagcccatcccacgcttcactgagcacctgctccaatgtcacccgctcggagaggcactcgccaaacgtgagcagagaagcacccctcgccgtcactccagtttttcttatagctcttatacacagggtatattgtttagcatgtctattatctgttatcacttccctaaaagaacggttgtgaaaacaggattttggtctgttttactcactgctgctgtcagtgcccaccacagagcccccagagggcctgcaaaatgaagggacaaaatcatgtctgttgaacaaacttagagaagcagaagtcaaattgccaaggaagagtaatattctaaggcgatttgctaaggaagggtaataccctaaggcgaggaaatgaaggcactgcaggaagacttcatagaaagagatatggtcacatctgaggattggctgatgggagaggtccaaggaagtatcagagctttgtgaacagaggttggttgttaattatggattagtggattactcctctgggaagacctttcctgccaaattttgtcttgaatgctgatctggctggtatatatattaataatgtgaatgaatgaagacctatccaatttgcttattgtatttgtagatattattgtcagaatgaagattcaaaactgcctagtcaatgggtcaaaagacaggtaagatgaggtttagcaaagctaaattggaggtcccacccttaagctgagagccagatgaagaagccctgtagagagcccattagcaacatctcctaaggcaatgcactgggaattaaggcagtggcttgggaggtcacagacgtttgtctacactgagttccactaccttctctctgagtgtccttggacaaagttatgaggctccctgaattttattttctcctctttaaattggagacacagataccctaccctatagcatctttctgaagccaactgagaaaatccatgtaagaacatgaaagagcaggtgatacagggaaagtgatacaggaaagtggtacagggaaagtgcatgattattagtgggtattccctactactgtttactgcagaattccaacatgaatcaaaaggcttatgtaactgccaaaaaaaacaaggaaatcagagattccaccagtgaaaccatagttctctgcaacaggaggtaaaacatccaccatgcatcatcaggtctgggcaccacatttcaaagacagacactaacaaaccagcctgtgtacctgggagagcatggctacataggtgaaggtgctgagccatgacactgttgaggatatagaggctgcagtgtaagagtcctctcctagtgtagaggctgcagggtgagagctctttcctagtgtagaggctgcatgcactatgcgataacttgcatgcttgcaagcatgcacacataaaatgggtgactattcatgtgagtgtcttggaagcaagtttttccctcaacaggcaattgggctgcaccatctctaaggtttcttccaacactaagaaactctagttctataatcataaattagcataaattatcttattagcagcagtatacattatatgcctccagtccttcaaagcatttctgatgtttttacctccttactctaccttcagctctgcctgaccaaagtaacccccatccacattttccaaataattcacctctgaaaagaagttacttttctggtaagacacccatgaagacttaccccagtttctgcaggttacactgtggattcttggctttttcacataaaattgcgactcctgagtctcccaaggcattctcccccacatagagtctggtcagggaatggctggtgctcaatactgatgcaagatcctgacaacatgctgatgtgaggcagcagctgaccaaccttccatagagatggcagaatgtcagtcatgtctctcacccacgctccaccatggacaaggaagcacccgtacctgccactgcctctactccagtttacacatggaaagggagtggacacaagctctatgtacacttctgatttccttttccatttggtggaataacaagtaagcattctccaagctcccaccaatactacatcttcccagctccctacattcagctttattgtggtaaaatacgtgtaaaataaaatttaccattttaaccatttttaagtgcacaattaatggccttaagcacttcacattgttgtgcaaccatcaccaccaccatctccagaactcctttcatcttgcagaactgaaactccataaccattaaacaatgtcttcccactctccgccctcccattgcctgcaaccacgtttcttcctgtctctatgaatctgtctgttctagacacctcctataaggacaatcagagtatttgccctttcgagtctagcttatcttacttagcataatgtccccgaggctcatccatgttgtagtgtgtactagaattctttttaaagctgaatgtacatatatagcacttttcaacacccttcatccgttgaaggacgtttggttatttccaccttttggctatttctaatagtgttgctatggacatagatgtacaaataacatgtttgagttcctgccttctgttttttttaatgcttcctctgtcacccaggcgggagtacagtgacgggatcttgactcactgcaacccccgcctcccaggttcaaaagattctcttgcctccaccccgagtaactgggattacaggcatgcaccaccatgcctggctaatttttgtatttttagtagagacaaggttttactatgatggccaggctagtctcgaactcccgacctccagtgatccacctgcctcagcctcccaaaatgctgggattacaggtgtgagccaccgctcctggctgagttcctgctttgaactcttttgcagatatacccagcagtggaaatgctggctccagtagtaattctgtatttattttttaggaattgctgtgctgttttccatagtggctgcatcatttacattcccaccagcaacacacaatggcttccatttctccgcacccacaccaatacttgttgttttctagttttcttgcttttgtttgataatagccatcctaatgggtgagaaatggcccttccatttttaagtggttttttctctccttcaaaatgcaagtctcccagaagcactcagggaagggctgcatacaacatcgagggtctgcattgctttagcaccatttttcttatacaatatgaggacccagggcttgtcatgaagttctaaaactcctctaaagcaatgcattacactgattttttctttttgtcagctaggcagtaggcaccctaaaggcagacatcttctttttgttattatttatgctccttgtcagggttgagtgtgtggctttccccacgacaaacactcactgaccgcaatgctagacaccccaagacaagcacacgcagtcacccgagccgccaaggccattctcactcaaaccccagcccaccgggcctcactgaagccagagtgcgcagcacgcctcgctggcagaacttccttaggggaacgggctcgactcaccagagcttcttcagattgcacaacaggtgcttcagtcccacacacagaagtctgattccgaagtcaccgagggcgttgtcactcaggtccagctccaccagcttctggttgctgctgaggaccaaggagatgtcgaagcagcactcatgcgagaggccacagcgccccaaccttcatgccaagaacagaggcagaaagcatcagaacacacctgaccagagagctccagaacagaggaagcatcaggacacacctgatcaggaagctccggaatagagaaagcatcagaacacatctgatcagagagctccggaatacagaaagcatcagaacacacctgaccagagagctccggaatagagaaagcatcagaacacatctgaccagagagctccagaatagagaaagcatcaggacacacctgacaagagagctctggaatagagaaagcatcaggacacacctgaccagagagctctggaatagagaatgcatcaggacacacctgaccagagagctccggaatagagaaagcatcaggacacacctgaccagagagctccggaatagagaaagcatcaggacacacctgaccagagagctctggaatagagaaagcatcaggacacacctgaccagagagctctggaatagagaaagcatcagaatacacctgaccagagagctccggaatacagcacaaggcacattgggaggtcagcccccagtctccccagtcacagcagagggatcacctgtcagtgaactcccggccgtaaacagtgccgggtgcattgagatcaccccccagacatgtgaatggtgcgctcctggtttgtaagtgaagcgggcggtgtgggcctgtgcacccacctccttccctcgtgttcctaaccattgacgtgcccgcagtcggcactgccctcgccagtgctgcactcagctatttcttgtcttcaccaacattgtcaccccattgtgtttgacgatttcatcccagccctccatctatattgaaaggaaaagcagctctgattctttttcttttcttttcttttctttttttaaagacagggtctcactttgttgcacaggctggagtgcactggcgagatcatagctcactgccacctcgaactcctgggctcaagggatccacctgcctcagcctcccaagtggctgcaaatacaggcatgtgctaccatgcttagccattttattttatttatattttatttttattattattattatcttctaaagacaaggtctcaccagcttgctcaggctggttttgaactcctgggctcaggtgatctgcccacctcagcctctcaaagtgctgggattccacatcccgctgcagctctgattcttgattagtttccccgtcacacacatgcacacaaacacacacgcacatcactaccaccgtcaccaccaccaccagcaacaaaaactatactttatccctgtcatgggggcaagaacaacattctagcttctttccagggcaatagttcataggtcctggagcctgttagaccaccttcctttctgtccctatccttacaccaacttcaagcaaatggacaaatggatctctacttctctgcgaagcatctcactgtcccctacccttccctgtttgtgtctgcctctccagaatcatacaggggcaatggcagtggggagagaatttgggcatgaagttggagaaataaggttaaatgtcccaaacaaccagtctccatggcactacgatttgaaatttaccaaaagagcaaagatgaagagtgtgatctatatacataatggaatactgctcagccatagaaaagaatgaagtcacatctttgaagccacacagatggaactggaggccattaccttaagtgaaacaactcagaaacagagtcaaataccacacgttctcacttacaagtgggagctaaacaaagggtaacatccatagagcatggaatgatagacactagagcctcagaagggtgggagggtgggagccaggtgagggctggaaaattatttattgggtacaatgttcactatttgggtaagagttacactaaggccgggcacggtggctcacgcctgtaatcccagcactttgggaggccgaggcgggtggatcacgaggtcaggagtttgagaccagcctagccaatacggtgaaaccttgtccctactaaaaatacaaaaatcagctgggcgtggtggcccatgcctgtaatcccaactactcgaagaattgcttgaacccaggaggtggatgttgcagtgagccgagatcactccactgtactccagcctgggcaacacggcgagagtccatctcaaaaaaaaaggggtagttacagtaaaagcccagacactaccactgtgcagtaacatatccatgaaacaaagctgctcttgcgccccctacatctacaaaaataaatacataaagtaaaaaataaagagcagagcagacagaaagcatttaagccaccgaacagcacaatcgaatcagaattttctaaaggaccatcttacttttgtgcagagaatggtcgggtgagggaaaaaggcagacacagggagaccaaagagccaacattcattcagtgcgtgcttttgaccactgatgggtactaagatgtctgtccaggcgtggcaaagatgacagcaagacaaacaaacgcaaaccccatccccggggagctgatggtctaggaggtcactgcgtgtccaggcaagtggtgacagttgctggacctgggctggtggggtgaggacgaggaaaagtggaaaacagctcgggtaggaggaaaaattgataagactggtgacaaggtgagtgtgttgagccggagagggaggtagcaaaatgtcctagagtggcggactttaacacttgctgtgcagctcctcaaaaatgcagacgcctgcatgcgtccacagagcagggaatgaaacagagctagtgaggcggcccaggcaccagcgcggtggggcgtgtgaatctgattcatggtgtgggagaaagcaagcacattttttattattattattattattattattttgaaatggaatctcgctctgtcacccaggctggagtgcaatggcacgatctcggctcactgccatctccgcctcccgggtacacacagttctcctgcctcagcctcccgagtagctgggactacaggtgtgagcaagcacattattaataaagtcacaggagattccctgtgacatttcaacccatacaaagcattctgaccaggctgggcaacgtgatgagaccacatctctacaaaaaaaatacaaaaattagccagcatggtggtgcatgcctgtagtcccagctactcgggggagctgaggtgggaggattgcttgagcctgggaggtcgaggctgcagtaagctgtgatcacacactccagcctgggtgacagagagaggtcctgtctcaaagaaaaaaaaaaaaagtattttcatagtttttaggtgaggttgccattgttgtaaatggcaaattctccaactctcatctatgaacatggcccatgaggaaatggaatatatcgagcatcatggttgtttcaagaaatgactttttttttagttcctcattcattcttccccacacaaaacttccccagctggcctccaacccattctaccttctcacttgttctgggctgaactgtgcccccccaaaaatttacatgttgaagccctaatcctcaagacctcataatgtggctgttttgggaaatggggtctttaaaggagtgactagattaacattaggtcttgtgtagtcatgcctgactgtgcctaatccatcaggactgctgtccctgtaagaagaggagactaggccactcttccccccaaggcaagatggcatcagtacacagggagaagggggcatctacaaaccaaggagggcggcctcagaagaaaccaaccctgctgacaccttgatcttagactttcggcctcagaactgcaagaaaatgaatttttgttgttgaagccattcagtctgtggcactttgttacagcagaaaccacaccaccggccgggtgcggtggctcatgcctgtaatcccagcattttgggaggccgaggcgggcggatcacctgaggtcaggacttcgagactagcctggacaacatgatgaaaccccatctctactaaaaatacaaaaaattagctgggtatggtggtgggtgcctgtaatcccagctactcaggaggctgaggcaggagaatcacttgaacccaggaggcagagattgcagtgagccgaggtcacggcattgcactccagcctgggcaataagagcaaaactctgcctcaaaaaaagaaaaaaagaaaaagaaaagaaagaaaccacaccagcaacctggtcctgaagatctttctccagtctgtttctctctctctctctcatatgaacttgcactcacacagatcacatgcacggggactcaccacaatctccgaatgttacagccaggatgctggagcgtttcacacaacactctcatccctgggtcccccagagaattgtcactgaggtccaattcagttagactctggctggtgctcagaactgaaaagaggccccggcaaaaactggaagtgaggtggctgttcaccaatctaggaattagaaggaagacagacagaaaagaaatcagcctcgaataataactaactggagctgggggccggggtgcctggcaccagttcagagaaatgccttccggggattaagaaatgggtcacgaaaccaaaaattgttcccagagaaatgaagagggctggatgagccttggtaaaagcagttctgcctcctctcggacggagagcatgagcctgtgactgtggcggactgtggcaccctacagcctgctccccagtgtcctcctctcgcccttaccagtccactgtcccaacatggccctgaacgttctgtgctgggtgatcagagggcagtcctcactcctggctacacaacagcatcaggagtgctcacaaaaatcctcaggccaggctgggcatggtggctcacacctgtaatcccagcactttgggaggccgaggcgggcagatcacctgaggtcaggagttcaagatcagcctggccaacatggtgaaaccctctctctactaaaaatacaaaaattaattgggtgtggtggcacgagcctgtcatcccagctattagggaggctgaggcaggagaatcacttgaacctgggaggtggaagttgcagtgagccaagatcatgccacagcactccagcctgggcaacagagcaagacttcatctcaaaaaaaaaaaaaagaaaaagaaaatcgcaagcccaggccacatccatggaaataaaatcagaagctctgaggtggaactagatgaattttttaaattttttttcagatgaaacccaagctggaatgcagtgccatgatcatagctcactgcagcctcaaactcctgggctcaagcaatcctcttgcctcagcctcccgagtagctgaggttacaggcacgagtcactgtgtccagctatatggatcttttttatttaaaaaaagccaggtggctccaacatgcagtcacatttttgcttttgtttttctgtagagaggtgctctcactttgctgctcaggtaggacttgaattcctggcttcaagcaatccccccatcttggcctcccaaaacctaggattacaggcaagagccactgcacccacacatgcagtcacctttgaatcacctgtagctctcattcaaatgcaaagtctagctctctaggtctaagattgggtccacaatcctgcatttctaatagatgctcaggcttctggttctcagaagggactggaacatacaaagcaagctcctgccctcagagtaaggcagctgccatctagaaagatgggtgctgagccccctaccagggctccagtcagagtctgtcctcagagtaaggcaggtgccatctagagggatgggtgctgagccccctaccagggctcccgtcagagtctgtcctcagagtaaggcaggtgccatctagagggatgggtgctgagccccctaccagggttccagtcagagtctgtcctgaggaaggaaggtgctatctagagaaatgggtgctgagcctcctaccggggcttcagtgagagtctgtcctcagaggaaggaaggtgctatctagagaaatgggtgctgagccccctgccagggctccaatcagagtctgtcctcagaggaaggaaggtgctatctagagaaatggttgctgagcctcctaccggggcttcagtgagagtctgtcctcagagtaaggcaggtgccatctagagggatgggtgctgagccccctgccagggctccaatcagagtctgtcctcagaggaaggaaggtgctatctagagaaatgggtgctgagcctcctaccggggcttcagtgagagtctgtcctcagaggaaggaaggtgctatctagagaaatgggtgctgagccccctgccagggctccaatcagagtctgtcctcagaggaaggaaggtgctatctagagaaatgggtgctgagcctcctaccggggcttcagtgagagtctgtcctcagagtaaggcaggtgccatctagagggatgggtgctgagccccctaccagggctccagtcagaatctgtcctcagaggaaggaaggtgctatctagagaaatgggtgctgagcctcctaccggggcttcagtgagagtgtgcaaaccttcctcacagatgtgtgatcttcataaggtctccctgccctctccaccttccacctcactcttaatgagtagttctgcctacttttctctctgtcttactcttcttctcccatttctatggtctgaatgtttgtgtgccccaaaatccatacgctgaaatcctaaccctcaacatgacgtatcaggcgatggggcctttgaggtgtggttaagttatgagggtggagccctcaggagtgggattgctgtccttaggaaagggaccccagagagctgccttgcctcttcaccatgtaaggacacagtgagaaggcaccatcgaccagggaacaggccctcaccaaacaccagatctgccagagcctggatcatggacttcccagcctccagaaccgtaaggtgaaccttccttttgcttataagccaaccagcctgcagtgttttgttatggcaacctgatgaatgaagacaactgtcttttttccagtcactcggaactgtttgctgccgtagaaaccgtaccctgctttcccacacctgccctctctctcaacaccgtaagcccccagcctggctgcccctttccttctctcactctctcactgcccatcctccggaagctggctgagcggggacacccacccgtgccccgctggtgaacaggttcgtccccttgtgctttggatactctgcaagtttccttgtcagagcccatgaccccctccccgacatctgcacttgtttccggactgtcccacagccagacctcaagtccctgtgaccaggacctgggtcttcaccaccactgcggccctgtgggcagtcagtccttcatggccaaaccatgactaggaaggtggtcctggtcatggtaatgtcaacggatcaagaaagctgaaactcattgttgcctgtggaagggccaagcctcctgtttcccttaattttgccccacgtcaagtgtcttctatccaggctaaactcacacatcacagggtggccaccttcctacaaccactgtgggtggtccttctgcaggaggcactgaacgataaacccaaaagggactcagaagtcaggtgactcaaccacttcattgcacagacttggccactagcttccaaccacccagcaagtgtgtgaacagacccgaaaacggggttttggcaatgcccagtgcagagcaacatgggggcctagaaagagggtctccacatttctgctctatttcccttgatttaccttcatcatgtttttttccaaggaaactgtgtctctctccactgtcacctgcacacactttttctcagactgcattcatgatttggctcataccagtcttcagtgcagaattcctttaatttcttctctatgcgcccaggtcccaccattccttaaaggaggcttagattgcacatttctaagaaacatccccccagcctccagctctgaggccctctgtcccctcgctcctgggacacagactctctggcattgttctgccccacagacattgactgactcttaggcactagtgctccaagtagcttacaagaaatttcagttgacaaatatttgtaggcaatcctacatcctacttaataccttgtgctaaactggcattccccaaacatttgttccttgttttattttttttttcctcatcccatttatccacctaccatacatcaatctttgctcatgaaggagtctcaaacagacagtggtggcattatgatgtagctgtggcaacagtatttggaagatagttgaaaagagatgagaggaggcaagcgccaagaagaagctggcgaggaagcaggaggaagcacctggaagccgagtttccttacccatgagaacaggcagcatgagaggagcttgggaggacacactgcaccatatcaaggtgtcggccttccttttcctcctcctcttcctccttgggcatgttatggagaaaccccagggacagtgactccacccgatgacagttctcaatgcaaaaggaagaaaccatgtggtccattctggtggagagattgatctcaatcttggggaaatagtccatggccctttgcacgaagtcctcctcctgcatctcgtacaaacagtagaacaattccagctggctgggctggatctgcagctttttagctttggctttcacttcaatccatttcagcagctccagcctgatttgctgagagatcttgcaacttaatttcttctccaagtaggaggtcctctcctggtttaccaggccaaagaggaaacgtacaacaaaaatcaaataccccttttcgaatttgccatagttttccagaaggactgtcacgtctcggctgggaagcttcaaacgactccctggaacgttcgtccttccttccttttcctcttccagcaggtagtacatggcggcaaagaactcctggaaagtcatgtggatgaagctgtagaacttctcgcagtccacttccttttggaacaggttcatcctcaggaaagcagacacatccgccttctgcagtccatgattcctgaggtcggactcctcaaacaggattttctggttccagattccatctgcagccaaagagcagagcccccagaggtgggcgcagaggccgtgctcctggctccctccccggggctgcagcaaactggaaaggaagaagacgtacaccgcggtggtggtcttggatgtctgggcaaggctcttgccactctccatctgctgtttcagtccagtgcacacgatccagcagaccagggggatgaagcacatggtgaagaggacctcgttctcctgaatcagactgaaggctgccctggcttgggcctcatcagagaagtacttgaagaagtactctttccttttggcctcggagaaacccaggatctccacatgccgaggatggtccagcaagtgctgcagtttctccagggccacaggtctcgtggtgatgagcagagaggcctcgggaagcagcttctttctgatgaggctgctcaggagaatgtctccccgctcggccttctgccagtcagtgcagagcggtcctatgtgctcgtcaaaggcaccttgcagctcatcgaagccgtccatgaggaagaggattctggagggttttctcacgatcttgtggatgggtgggtttgggtcggggcagcagctcatgatcaggtcccccaggctcctctgtgtcacaaggctcacctctcgacagtggatatagaacagatagtcaaacctgtcttggtagagtgtccccgacgcccagtccaacatcatcttcctggccaggattgttttcccaatccctgccgccccctggaacaccacggtgtgcacaggctcagaatgctcatcatcggggtcaaacagcaactccatcttaatgggactcacggggctctcacacgtcttggtcttgccgatggccagaagctcctgctccctctcctgctggctccggtgctccttgatgagacgcagtcgtgtgtagcgtttgttgaggctcacactctcacccagacgggcattcctgtcttcaatgcactggaatctgcttctcacgtactttctgtacttcttacggtaatctacggcaaagacaggaagttagggggaaagtatacacacatccacctgagatgcgctctcagctggggcctgtcatcggaagcgagtggtaaccggaatggagaaatggaaggtgcagctcctccccactgggtaggaaaggtgccgagaatctctggtgtcaagtttttaagatacacagctgagcagaaggcccatctctatgtgtagctaccagcccaaagatcatttgaatcaatcttattcctttaagtaatctgcatcctatgccttatcaaacttgaaacgcttaatcaccgccgctggctctgggactgcaagagccacacaaacatgaatttgtttcttcaactgacaatggatttcctgagacaggcctttgcattccaaagagcaggaacctatagtatggccaagttacccagctgctcagcttcccagagcctcctgaaccaggtcttaaaactcaactagaagcaccaccccagtcgcttacctttcttcattttacaaatagagattctcgaaaggtactccagtaaacccatccactcctcttcaatgctgtcttcctggcatatcacagtgggattcgaaacacgtgcattatctgaacctaaaagggaaaaaaaaggtgtcaaaacccagaactattatcacagaggatgcaattgaaacctggcctaatatttggcatgagagaggagaccccaaacatcccccaaatcaaaacatggctctgagttgcagaggacaggtatccagtcaaaagtctggttgggagcatttctgcactcctagtttcaaaacaacttctgctgtccacctgccaagcatgtgttcccactgtccccagtctcagaatctcttcctcaggcctggaaatcaatcagcaaacatgcgaagcaggctaagtttcttttaccctcgtttgcttttgcctgcccctggcagcctgattgtgagggcatctccaagctctcctatatccccaacacggctgtgggctaagaaaggtcacccttccctgaccgcagttccctgcaatccattttacacacgtcttctattgtcaagtctagatgtctggttcttcaagagtgagaacgaccagtctatttcgtgcctaatctagtggttgggaatcctggctgactttagaatcacccaggaagctttaaaaatatggacttcaggactgcacgcccagaggttctttttcagtccctctgaggtgaggcccaggaaccatcacatactaaaagctcccaggtgattccaacatgcatctgtgttgagaatcacaaatccaaacagtcactagatagcatatcttaagaaggcattctataggagaaattcaggttaggtaaaacaagagttagtcactaggggaaatatataagacagataacttcaggtgggcaggaatctacaagtaacataaatgattttttttttttttttgagacagggcctcactctattgcccaggctggagtgcaatgacacaatcatggctccctgcagcctcaacctcctgggctcaagtgatcctcccacctcagcctccagaacagctgggactattgacacgtgccaccacacctaactaatgtttgcattttttgtagagacaggttctcactatgttgcccaggctggtctcaaactcctgggctcaagcaatcctcccatcttggcctcctgaagtgctgggattacaggcataagccactgcgcccagcccataaaagacctctgacagctgtctacttggtaaccatatcacaaaataaaatccaaaaaatctaagccaaaaccaaaatcttattctttttttttaagagacagagtcttgctttgtttccaaagctggagggcagtggcatggtcatagctcactccagcctggaactcctgagctcaagtgatgcacccacttcagccacctgagtaactgggactcaggtaggagccatgacagtaaattagccaaagtctattacctaaaacctaaccccaccccaggaaacaaacaaacaaacttctaaccctagttataacttttctgcctcaaaatccagatatggaagcaaagacggtgtagtggttaagagccaggctttgatcagagacatgccctgctttttaccccagctctggttatggctagaaataaaccatgggccagttaggatctcttccaggctcacctcattcacttgcaggagggataataccagaagctgtttcatgggtttcttgaatgtgccataaaatccataaaaactgcttagcaaagtacttctacagttgtgattatgacactttcatttgggtatgtgagtatataagtactgacacaatgataattgctttatttacttagagatgaggtctccctatgttgctcaggctggttttgagctcctgggctcaagcgatcctcctgccttagcctcctgagtagctgggactacaggtgagagccattgcagcaactggtttctgacctcccccggctgcacactgctgtctgtttccccagtgtcattacacccacactgctgccctgccttaacatgtgtctccctatccactgactcatttgtactcctccttcccatcaccaccagctctacatcatcatcctgcaataccctgcccttctctgagccctacctttgcctagaacacaagacaaaagaaagaaccttatccccaatgtgtacatggggattaagagaatttcttttacattccaattcccaaagtggtggtgaaaggaaaggcttctgccccaaactccacggttcttcaaggagagaggctgccctctgggccataggaagcagaggcccaagcctgctgaccacacagcagatactggacaaaacatgtggtctgagaagctggatggagaattggaggcaggtctaggcactgctgagattcagataaagagggactaatcatggcaggtgcccagggggtaggtacagtctgcatcagctttttaaaggagttagagaaagcaaacagtttgcctccaccttctcatagcactaccgtgagaggggaaaagagaaaaaaccaagacaatacaagaaaaaaaaatttttttttgaaacagggtcttgctctttagcccaggctggagtgccgtggtgcaatctcagctcactgcaacctccactccccatgttcaagcaattctcctacctcagcctcctgagtagctgggattacaggtgcccaccaccacacccggctaattttttttgtatttttagtagagatggggttttgccatgttggccaggctggtgttgaactcctgacctcaggtgatccacccacctcagcctcacaaagtgctggaattacaggcatgagccaccatgcccggccatgatttaaaaaaaaaaaaatcatactaacttctgtgcatcaaaggacacagttaaccaaatgaaaagacaacccacagaataggagaaaatatttgtaaatcatatatctgatatggggttaatatctagaatacataaagaactcctacaaggcaacaacaaaagccaaacctggtctgaaaatgagaaaagaacttgaacagaactttctctgaagaagctctataaatggccaacaagcagtgaaaatgtgctcagcatcacttatcattagggaaacggaaatcaaaactacagtgagataccacctcacactcattagaatggctactataaaaaagaaaaaataaataaaaataacgtgttcttaggatatggagaaattggaacccttgtgtgctgttggtgggaaatggtgcagatggtatctaaaacagtagagcagttcttcaaaatatttaacagaattaccgtatgattcagaaatttcacttctgagtatataccccagagaattcaaagcagggtcttgaagagatatttgtgcaccaacactcataacagcattaacaataacaaaaaggtagaagtaatccaggtgttcatcaacagataactaaacaaaatttggtatatggtaccatggagtatttatacagtcttttttaaaggaagggaattccgacacatgctacaacatagttgaacccggaggacattatgctgagtgaaataaactactcataaaggaaaaaatgctgtatgtttccacttatatgaggtacccagagtagtaagattcacagagatggcaaatagaatggtggttaccagggctgggagaatgaggcaatgaggagttatcattcaatgggtgaggagtttcagttttgcaagatgaaaacagttctggagactggttgcacaatgtgagtgtacctaacactactgaactgtacatttaaaaattattacggccgggcgcggtggctcacacctgtaattccagcactttgcgaggccgaggcgggtggatcacctgaggtcgggagtttgagaccaacctgaccaacatggagaaaccccatctctactaaaaatacaaaattagccgggcgtggaggtgcaatgcctgtaatcccagctacttgggaggctgaggcaggaaaatcgcttgaacccgggaggtggaggttgcagtgagccaagatctcaccattgcactccagcctgggcaacaagagcaactccgtctcaaaaaaaaatatatatatatatatatataaagatggaaaattgtacactatgtgcacttggccacaattttttttaaaagtcttccttccactcaccccacttcggctcatctctttttgctttctcataaaggtctctcctgttgatcgcagcgaagatccacacggccatggcccacgccttctcctccccattgaagtcgatcattagcgtggctagatccacatggtctgccttctctgtctgacccctcgggagggggatgcagcccttctggggaggatagtcctctaagtgcatcttaaatttcttcaagtccacatcctccaggtcctccaggtacctggccagcttgcagcgggtgcttgccatcttcatctgcagctgttttcagggtccttaggcttcggtccacactaagataccaggcagtgaacacggcacacggatgagtcttttttaaagtctccactttgagagatataaattatcaaaaactcagcaaacagaaagaaaaaaatgtcacatgactgtaacaagtcaaaatctttaattttgaaaagttagccaaggccgggcacagtggctcacgcctgtaatcccagcactttgagaggccaaggcaggcagatcacctgagctgaggaattcaagaccagcctggccaacatggcaaaactgtgtctctactaaaagtacaaaaatgagccgggtgtggtggcgggcgcctgtaatcccagctactcaggaagttgaggtaggagaattgattgaacccgggaagtggaggctgcagtgagccaagatcacgccactgcactccagcctaggcgacacagcaagactccatctcaaaaaaaaaaaagttagccaaatgcttaccagaaagttctcctgttggctcgatccaggagtgtgtcctgagccatggaagaaaggtttccctatggagggaaaaatatgcaaacaaatccataaacaggattgtattacagtttacggtgaacaaccacttcacgatgccatcttgacccatcagcaagaaaatttttgtcccgttgattacggggctatgacattggacaaactcttcactattcctcaacttcagtttcctcatctacaaaatgagaaagcagaagagaatgttttcagttcctccaaactgaaggctctggctctttgcttctgtttttgtgagggaagagggatgagagacaatagaaggagaaggccaggaggtgagtaagtgtgttgataacagaacaggacgtggctagggagagaggagagagaacataaaagcttgcagaggaggggacagtctttgactgcacttctatcaaccagtggattgaagtgagatgaagctgggagtgcataatggagaataataaaaacatacatccctgtaatcccagcactttgggaggccgaggtgggcggatcacctgaggtcaggagttggagaccaggctcaccaaacaacagggagaaatcccgtctctactaaaaatacaaaaattaaccgggcatggtaccaggcacctgtaatcccagctactcgggaggctgaggcaggagaatcgcttgaacccaggaggcggaggttgcgatgagccaagatcacaccactgcactccagcctgggcaataagagcaaaactccatctcaaaaaataaaatagaataaaataaaataaataaaaacatacatcctttaatgtctccttgcaaaattcgcaattgttatcattataattcacattaatttagagctttccacaggctaggcactcactgatgtttttccccatctaacctgcacagagctctatgaggtgcacctattcctagccccattttatagatgcataaactgagtcttagggggactaggaagcctgccgaggggtttagaaccaggaaggaacagagccaggattttgaccagagatatgagaccatgtcttccatcacttgtttcagtcagacaaagacaaagacaacaaaatagatgactaaaagacacacttccccagcatttatcacaggtgtatcactgcagcattcaccaacatagtcttcccaactagactgtgagttccacaaaaactagcaatcacctgctgtatctttagatcttccatatctcctagagtccggatggatgaacaagttggctttgtttggaattgttccctccttgatcccttgattatactctatttggcaaagcacctcaacctaaagccataaataacactcaagggaggcagagagcctggaaaacggtggagctctccaaattggaatttctgtgactgcagttcaatgtcaagatgcctcagactcactcatctctcccgtcccatctccattcctgcctatctactcctcgcctcctgagccctgcaaacccagccctgtgcatcctgaggtgactgctctccagacagccctattagctccgcataccctcccagctcctgcccatcctgaggtgactgctctccagacagccctattagctccgcataccctcccagctcctgccccatcagtccttccatctgcatcaggattctgcctttcttctgtgctccttccaccctaacaccagcacaaaaatctgctgccctttggtctttaaggaggtttgtttccttctgtatatcccatccatcttctcccctgggagggatactgggcaaatctgctgaagtcgtgggtgtaaactatggttgctgccgctgtcctccccgcttccccccgccacatacacacacacga

SEQ ID NO: 34 - protein, 1036 aa, Artificial Sequence
  NLRP3 Canonical
MKMASTRCKLARYLEDLEDVDLKKFKMHLEDYPPQKGCIPLPRGQTEKADHVDLATLMIDFNGEEKAWAMAVWIFAAINRRDLYEKAKRDEPKWGSDNARVSNPTVICQEDSIEEEWMGLLEYLSRISICKMKKDYRKKYRKYVRSRFQCIEDRNARLGESVSLNKRYTRLRLIKEHRSQQEREQELLAIGKTKTCESPVSPIKMELLFDPDDEHSEPVHTVVFQGAAGIGKTILARKMMLDWASGTLYQDRFDYLFYIHCREVSLVTQRSLGDLIMSCCPDPNPPIHKIVRKPSRILFLMDGFDELQGAFDEHIGPLCTDWQKAERGDILLSSLIRKKLLPEASLLITTRPVALEKLQHLLDHPRHVEILGFSEAKRKEYFFKYFSDEAQARAAFSLIQENEVLFTMCFIPLVCWIVCTGLKQQMESGKSLAQTSKTTTAVYVFFLSSLLQPRGGSQEHGLCAHLWGLCSLAADGIWNQKILFEESDLRNHGLQKADVSAFLRMNLFQKEVDCEKFYSFIHMTFQEFFAAMYYLLEEEKEGRTNVPGSRLKLPSRDVTVLLENYGKFEKGYLIFVVRFLFGLVNQERTSYLEKKLSCKISQQIRLELLKWIEVKAKAKKLQIQPSQLELFYCLYEMQEEDFVQRAMDYFPKIEINLSTRMDHMVSSFCIENCHRVESLSLGFLHNMPKEEEEEEKEGRHLDMVQCVLPSSSHAACSHGLVNSHLTSSFCRGLFSVLSTSQSLTELDLSDNSLGDPGMRVLCETLQHPGCNIRRLWLGRCGLSHECCFDISLVLSSNQKLVELDLSDNALGDFGIRLLCVGLKHLLCNLKKLWLVSCCLTSACCQDLASVLSTSHSLTRLYVGENALGDSGVAILCEKAKNPQCNLQKLGLVNSGLTSVCCSALSSVLSTNQNLTHLYLRGNTLGDKGIKLLCEGLLHPDCKLQVLELDNCNLTSHCCWDLSTLLTSSQSLRKLSLGNNDLGDLGVMMFCEVLKQQSCLLQNLGLSEMYFNYETKSALETLQEEKPELTVVFEPSW

SEQ ID NO: 35 - DNA, 4470 bp, Artificial Sequence
  pyrin
gtagatgaggaaactgaagttgaggaatagtgaagagtttgtccaatgtcatagccccgtaatcaacgggacaaaaattttcttgctgatgggtcaagatggcatcgtgaagtggttgttcaccgtaaactgtaatacaatcctgtttatggatttgtttgcatatttttccctccatagggaaacctttcttccatggctcaggacacactcctggatcgagccaacaggagaactttctggtaagcatttggctaacttttttttttttgagatggagtcttgctgtgtcgcctaggctggagtgcagtggcgtgatcttggctcactgcagcctccacttcccgggttcaatcaattctcctacctcaacttcctgagtagctgggattacaggcgcccgccaccacacccggctcatttttgtacttttagtagagacacagttttgccatgttggccaggctggtcttgaattcctcagctcaggtgatctgcctgccttggcctctcaaagtgctgggattacaggcgtgagccactgtgcccggccttggctaacttttcaaaattaaagattttgacttgttacagtcatgtgacatttttttctttctgtttgctgagtttttgataatttatatctctcaaagtggagactttaaaaaagactcatccgtgtgccgtgttcactgcctggtatcttagtgtggaccgaagcctaaggaccctgaaaacagctgcagatgaagatggcaagcacccgctgcaagctggccaggtacctggaggacctggaggatgtggacttgaagaaatttaagatgcacttagaggactatcctccccagaagggctgcatccccctcccgaggggtcagacagagaaggcagaccatgtggatctagccacgctaatgatcgacttcaatggggaggagaaggcgtgggccatggccgtgtggatcttcgctgcgatcaacaggagagacctttatgagaaagcaaaaagagatgagccgaagtggggttcagataatgcacgtgtttcgaatcccactgtgatatgccaggaagacagcattgaagaggagtggatgggtttactggagtacctttcgagaatctctatttgtaaaatgaagaaagattaccgtaagaagtacagaaagtacgtgagaagcagattccagtgcattgaagacaggaatgcccgtctgggtgagagtgtgagcctcaacaaacgctacacacgactgcgtctcatcaaggagcaccggagccagcaggagagggagcaggagcttctggccatcggcaagaccaagacgtgtgagagccccgtgagtcccattaagatggagttgctgtttgaccccgatgatgagcattctgagcctgtgcacaccgtggtgttccagggggcggcagggattgggaaaacaatcctggccaggaagatgatgttggactgggcgtcggggacactctaccaagacaggtttgactatctgttctatatccactgtcgggaggtgagccttgtgacacagaggagcctgggggacctgatcatgagctgctgccccgacccaaacccacccatccacaagatcgtgagaaaaccctccagaatcctcttcctcatggacggcttcgatgagctgcaaggtgcctttgacgagcacataggaccgctctgcactgactggcagaaggccgagcggggagacattctcctgagcagcctcatcagaaagaagctgcttcccgaggcctctctgctcatcaccacgagacctgtggccctggagaaactgcagcacttgctggaccatcctcggcatgtggagatcctgggtttctccgaggccaaaaggaaagagtacttcttcaagtacttctctgatgaggcccaagccagggcagccttcagtctgattcaggagaacgaggtcctcttcaccatgtgcttcatccccctggtctgctggatcgtgtgcactggactgaaacagcagatggagagtggcaagagccttgcccagacatccaagaccaccaccgcggtgtacgtcttcttcctttccagtttgctgcagccccggggagggagccaggagcacggcctctgcgcccacctctgggggctctgctctttggctgcagatggaatctggaaccagaaaatcctgtttgaggagtccgacctcaggaatcatggactgcagaaggcggatgtgtctgctttcctgaggatgaacctgttccaaaaggaagtggactgcgagaagttctacagcttcatccacatgactttccaggagttctttgccgccatgtactacctgctggaagaggaaaaggaaggaaggacgaacgttccagggagtcgtttgaagcttcccagccgagacgtgacagtccttctggaaaactatggcaaattcgaaaaggggtatttgatttttgttgtacgtttcctctttggcctggtaaaccaggagaggacctcctacttggagaagaaattaagttgcaagatctctcagcaaatcaggctggagctgctgaaatggattgaagtgaaagccaaagctaaaaagctgcagatccagcccagccagctggaattgttctactgtttgtacgagatgcaggaggaggacttcgtgcaaagggccatggactatttccccaagattgagatcaatctctccaccagaatggaccacatggtttcttccttttgcattgagaactgtcatcgggtggagtcactgtccctggggtttctccataacatgcccaaggaggaagaggaggaggaaaaggaaggccgacaccttgatatggtgcagtgtgtcctcccaagctcctctcatgctgcctgttctcatggattggtgaacagccacctcacttccagtttttgccggggcctcttttcagttctgagcaccagccagagtctaactgaattggacctcagtgacaattctctgggggacccagggatgagagtgttgtgtgaaacgctccagcatcctggctgtaacattcggagattgtggttggggcgctgtggcctctcgcatgagtgctgcttcgacatctccttggtcctcagcagcaaccagaagctggtggagctggacctgagtgacaacgccctcggtgacttcggaatcagacttctgtgtgtgggactgaagcacctgttgtgcaatctgaagaagctctggttggtcagctgctgcctcacatcagcatgttgtcaggatcttgcatcagtattgagcaccagccattccctgaccagactctatgtgggggagaatgccttgggagactcaggagtcgcaattttatgtgaaaaagccaagaatccacagtgtaacctgcagaaactggggttggtgaattctggccttacgtcagtctgttgttcagctttgtcctcggtactcagcactaatcagaatctcacgcacctttacctgcgaggcaacactctcggagacaaggggatcaaactactctgtgagggactcttgcaccccgactgcaagcttcaggtgttggaattagacaactgcaacctcacgtcacactgctgctgggatctttccacacttctgacctccagccagagcctgcgaaagctgagcctgggcaacaatgacctgggcgacctgggggtcatgatgttctgtgaagtgctgaaacagcagagctgcctcctgcagaacctggggttgtctgaaatgtatttcaattatgagacaaaaagtgcgttagaaacacttcaagaagaaaagcctgagctgaccgtcgtctttgagccttcttggtaggagtggaaacggggctgccagacgccagtgttctccggtccctccagctgggggccctcaggtggagagagctgcgatccatccaggccaagaccacagctctgtgatccttccggtggagtgtcggagaagagagcttgccgacgatgccttcctgtgcagagcttgggcatctcctttacgccagggtgaggaagacaccaggacaatgacagcatcgggtgttgttgtcatcacagcgcctcagttagaggatgttcctcttggtgacctcatgtaattagctcattcaataaagcactttctttatttttctcttctctgtctaactttctttttcctatcttttttcttctttgttctgtttacttttgctcatatcatcattcccgctatctttctattaactgaccataacacagaactagttgactatatattatgttgaaattttatggcagctatttatttatttaaattttttgtaacagttttgttttctaataagaaaaatccatgctttttgtagctggttgaaaattcaggaatatgtaaaactttttggtatttaattaaattgattccttttcttaattttaaaaaaaaaaaaaaa

SEQ ID NO: 36 - protein, 922 aa, Artificial Sequence
  NLR family pyrin domain 2
MKMASTRCKLARYLEDLEDVDLKKFKMHLEDYPPQKGCIPLPRGQTEKADHVDLATLMIDFNGEEKAWAMAVWIFAAINRRDLYEKAKRDEPKWGSDNARVSNPTVICQEDSIEEEWMGLLEYLSRISICKMKKDYRKKYRKYVRSRFQCIEDRNARLGESVSLNKRYTRLRLIKEHRSQQEREQELLAIGKTKTCESPVSPIKMELLFDPDDEHSEPVHTVVFQGAAGIGKTILARKMMLDWASGTLYQDRFDYLFYIHCREVSLVTQRSLGDLIMSCCPDPNPPIHKIVRKPSRILFLMDGFDELQGAFDEHIGPLCTDWQKAERGDILLSSLIRKKLLPEASLLITTRPVALEKLQHLLDHPRHVEILGFSEAKRKEYFFKYFSDEAQARAAFSLIQENEVLFTMCFIPLVCWIVCTGLKQQMESGKSLAQTSKTTTAVYVFFLSSLLQPRGGSQEHGLCAHLWGLCSLAADGIWNQKILFEESDLRNHGLQKADVSAFLRMNLFQKEVDCEKFYSFIHMTFQEFFAAMYYLLEEEKEGRTNVPGSRLKLPSRDVTVLLENYGKFEKGYLIFVVRFLFGLVNQERTSYLEKKLSCKISQQIRLELLKWIEVKAKAKKLQIQPSQLELFYCLYEMQEEDFVQRAMDYFPKIEINLSTRMDHMVSSFCIENCHRVESLSLGFLHNMPKEEEEEEKEGRHLDMVQCVLPSSSHAACSHGLGRCGLSHECCFDISLVLSSNQKLVELDLSDNALGDFGIRLLCVGLKHLLCNLKKLWLVNSGLTSVCCSALSSVLSTNQNLTHLYLRGNTLGDKGIKLLCEGLLHPDCKLQVLELDNCNLTSHCCWDLSTLLTSSQSLRKLSLGNNDLGDLGVMMFCEVLKQQSCLLQNLGLSEMYFNYETKSALETLQEEKPELTVVFEPSW

SEQ ID NO: 37 - protein, 719 aa, Artificial Sequence
  NLR family pyrin domain 3
MKMASTRCKLARYLEDLEDVDLKKFKMHLEDYPPQKGCIPLPRGQTEKADHVDLATLMIDFNGEEKAWAMAVWIFAAINRRDLYEKAKRDEPKWGSDNARVSNPTVICQEDSIEEEWMGLLEYLSRISICKMKKDYRKKYRKYVRSRFQCIEDRNARLGESVSLNKRYTRLRLIKEHRSQQEREQELLAIGKTKTCESPVSPIKMELLFDPDDEHSEPVHTVVFQGAAGIGKTILARKMMLDWASGTLYQDRFDYLFYIHCREVSLVTQRSLGDLIMSCCPDPNPPIHKIVRKPSRILFLMDGFDELQGAFDEHIGPLCTDWQKAERGDILLSSLIRKKLLPEASLLITTRPVALEKLQHLLDHPRHVEILGFSEAKRKEYFFKYFSDEAQARAAFSLIQENEVLFTMCFIPLVCWIVCTGLKQQMESGKSLAQTSKTTTAVYVFFLSSLLQPRGGSQEHGLCAHLWGLCSLAADGIWNQKILFEESDLRNHGLQKADVSAFLRMNLFQKEVDCEKFYSFIHMTFQEFFAAMYYLLEEEKEGRTNVPGSRLKLPSRDVTVLLENYGKFEKGYLIFVVRFLFGLVNQERTSYLEKKLSCKISQQIRLELLKWIEVKAKAKKLQIQPSQLELFYCLYEMQEEDFVQRAMDYFPKIEINLSTRMDHMVSSFCIENCHRVESLSLGFLHNMPKEEEEEEKEGRHLDMVQCVLPSSSHAACSHG

SEQ ID NO: 38 - protein, 979 aa, Artificial Sequence
  NLR family pyrin domain 4
MKMASTRCKLARYLEDLEDVDLKKFKMHLEDYPPQKGCIPLPRGQTEKADHVDLATLMIDFNGEEKAWAMAVWIFAAINRRDLYEKAKRDEPKWGSDNARVSNPTVICQEDSIEEEWMGLLEYLSRISICKMKKDYRKKYRKYVRSRFQCIEDRNARLGESVSLNKRYTRLRLIKEHRSQQEREQELLAIGKTKTCESPVSPIKMELLFDPDDEHSEPVHTVVFQGAAGIGKTILARKMMLDWASGTLYQDRFDYLFYIHCREVSLVTQRSLGDLIMSCCPDPNPPIHKIVRKPSRILFLMDGFDELQGAFDEHIGPLCTDWQKAERGDILLSSLIRKKLLPEASLLITTRPVALEKLQHLLDHPRHVEILGFSEAKRKEYFFKYFSDEAQARAAFSLIQENEVLFTMCFIPLVCWIVCTGLKQQMESGKSLAQTSKTTTAVYVFFLSSLLQPRGGSQEHGLCAHLWGLCSLAADGIWNQKILFEESDLRNHGLQKADVSAFLRMNLFQKEVDCEKFYSFIHMTFQEFFAAMYYLLEEEKEGRTNVPGSRLKLPSRDVTVLLENYGKFEKGYLIFVVRFLFGLVNQERTSYLEKKLSCKISQQIRLELLKWIEVKAKAKKLQIQPSQLELFYCLYEMQEEDFVQRAMDYFPKIEINLSTRMDHMVSSFCIENCHRVESLSLGFLHNMPKEEEEEEKEGRHLDMVQCVLPSSSHAACSHGLGRCGLSHECCFDISLVLSSNQKLVELDLSDNALGDFGIRLLCVGLKHLLCNLKKLWLVSCCLTSACCQDLASVLSTSHSLTRLYVGENALGDSGVAILCEKAKNPQCNLQKLGLVNSGLTSVCCSALSSVLSTNQNLTHLYLRGNTLGDKGIKLLCEGLLHPDCKLQVLELDNCNLTSHCCWDLSTLLTSSQSLRKLSLGNNDLGDLGVMMFCEVLKQQSCLLQNLGLSEMYFNYETKSALETLQEEKPELTVVFEPSW

SEQ ID NO: 39 - protein, 979 aa, Artificial Sequence
  NLR family pyrin domain 5
MKMASTRCKLARYLEDLEDVDLKKFKMHLEDYPPQKGCIPLPRGQTEKADHVDLATLMIDFNGEEKAWAMAVWIFAAINRRDLYEKAKRDEPKWGSDNARVSNPTVICQEDSIEEEWMGLLEYLSRISICKMKKDYRKKYRKYVRSRFQCIEDRNARLGESVSLNKRYTRLRLIKEHRSQQEREQELLAIGKTKTCESPVSPIKMELLFDPDDEHSEPVHTVVFQGAAGIGKTILARKMMLDWASGTLYQDRFDYLFYIHCREVSLVTQRSLGDLIMSCCPDPNPPIHKIVRKPSRILFLMDGFDELQGAFDEHIGPLCTDWQKAERGDILLSSLIRKKLLPEASLLITTRPVALEKLQHLLDHPRHVEILGFSEAKRKEYFFKYFSDEAQARAAFSLIQENEVLFTMCFIPLVCWIVCTGLKQQMESGKSLAQTSKTTTAVYVFFLSSLLQPRGGSQEHGLCAHLWGLCSLAADGIWNQKILFEESDLRNHGLQKADVSAFLRMNLFQKEVDCEKFYSFIHMTFQEFFAAMYYLLEEEKEGRTNVPGSRLKLPSRDVTVLLENYGKFEKGYLIFVVRFLFGLVNQERTSYLEKKLSCKISQQIRLELLKWIEVKAKAKKLQIQPSQLELFYCLYEMQEEDFVQRAMDYFPKIEINLSTRMDHMVSSFCIENCHRVESLSLGFLHNMPKEEEEEEKEGRHLDMVQCVLPSSSHAACSHGLVNSHLTSSFCRGLFSVLSTSQSLTELDLSDNSLGDPGMRVLCETLQHPGCNIRRLWLGRCGLSHECCFDISLVLSSNQKLVELDLSDNALGDFGIRLLCVGLKHLLCNLKKLWLVNSGLTSVCCSALSSVLSTNQNLTHLYLRGNTLGDKGIKLLCEGLLHPDCKLQVLELDNCNLTSHCCWDLSTLLTSSQSLRKLSLGNNDLGDLGVMMFCEVLKQQSCLLQNLGLSEMYFNYETKSALETLQEEKPELTVVFEPSW

SEQ ID NO: 40 - protein, 1016 aa, Artificial Sequence
  NLR family pyrin domain 6
MKMASTRCKLARYLEDLEDVDLKKFKMHLEDYPPQKGCIPLPRGQTEKADHVDLATLMIDFNGEEKAWAMAVWIFAAINRRDLYEKAKRDEPKWGSDNARVSNPTVICQEDSIEEEWMGLLEYLSRISICKMKKDYRKKYRKYVRSRFQCIEDRNARLGESVSLNKRYTRLRLIKEHRSQQEREQELLAIGKTKTCESPVSPIKMELLFDPDDEHSEPVHTVVFQGAAGIGKTILARKMMLDWASGTLYQDRFDYLFYIHCREVSLVTQRSLGDLIMSCCPDPNPPIHKIVRKPSRILFLMDGFDELQGAFDEHIGPLCTDWQKAERGDILLSSLIRKKLLPEASLLITTRPVALEKLQHLLDHPRHVEILGFSEAKRKEYFFKYFSDEAQARAAFSLIQENEVLFTMCFIPLVCWIVCTGLKQQMESGKSLAQTSKTTTAVYVFFLSSLLQPRGGSQEHGLCAHLWGLCSLAADGIWNQKILFEESDLRNHGLQKADVSAFLRMNLFQKEVDCEKFYSFIHMTFQEFFAAMYYLLEEEKEGRTNVPGSRLKLPSRDVTVLLENYGKFEKGYLIFVVRFLFGLVNQERTSYLEKKLSCKISQQIRLELLKWIEVKAKAKKLQIQPSQLELFYCLYEMQEEDFVQRAMDYFPKIEINLSTRMDHMVSSFCIENCHRVESLSLGFLHNMPKEEEEEEKEGRHLDMVQCVLPSSSHAACSHGLVNSHLTSSFCRGLFSVLSTSQSLTELDLSDNSLGDPGMRVLCETLQHPGCNIRRLCNQKLVELDLSDNALGDFGIRLLCVGLKHLLCNLKKLWLVSCCLTSACCQDLASVLSTSHSLTRLYVGENALGDSGVAILCEKAKNPQCNLQKLGLVNSGLTSVCCSALSSVLSTNQNLTHLYLRGNTLGDKGIKLLCEGLLHPDCKLQVLELDNCNLTSHCCWDLSTLLTSSQSLRKLSLGNNDLGDLGVMMFCEVLKQQSCLLQNLGLSEMYFNYETKSALETLQEEKPELTVVFEPSW

SEQ ID NO: 41 - DNA, 15 bp, Artificial Sequence
  STAT6 Antisense Oligonucleotide
gaaaggttccgtcgg

SEQ ID NO: 42 - DNA, 16 bp, Artificial Sequence
  STAT6 Antisense Oligonucleotide
ggctagtaacgtactg

SEQ ID NO: 43 - DNA, 17 bp, Artificial Sequence
  STAT6 Antisense Oligonucleotide
gaaaggttccgtcgggc

SEQ ID NO: 44 - DNA, 17 bp, Artificial Sequence
  STAT6 Antisense Oligonucleotide
ctgagtcgctgaagcgg

SEQ ID NO: 45 - DNA, 20 bp, Artificial Sequence
  STAT6 Antisense Oligonucleotide
cgctcacaccgcttgatctt

SEQ ID NO: 46 - DNA, 20 bp, Artificial Sequence
  STAT6 Antisense Oligonucleotide
agaagaaggctagtaacgta

SEQ ID NO: 47 - DNA, 20 bp, Artificial Sequence
  STAT6 Antisense Oligonucleotide
gagaaaggttccgtcgggct

SEQ ID NO: 48 - DNA, 20 bp, Artificial Sequence
  STAT6 Antisense Oligonucleotide
gcaagatcccggattcggtc

SEQ ID NO: 49 - DNA, 20 bp, Artificial Sequence
  STAT6 Antisense Oligonucleotide
gtgcgtgtgcgcgctgcagg

SEQ ID NO: 50 - DNA, 20 bp, Artificial Sequence
  KRAS Antisense Oligonucleotide
gcccttgtacttttgcatag

SEQ ID NO: 51 - DNA, 14 bp, Artificial Sequence
  KRAS Antisense Oligonucleotide
ccatcagctccaac

SEQ ID NO: 52 - DNA, 14 bp, Artificial Sequence
  KRAS Antisense Oligonucleotide
gccatcagctccaa

SEQ ID NO: 53 - DNA, 14 bp, Artificial Sequence
  KRAS Antisense Oligonucleotide
cgccatcagctcca

SEQ ID NO: 54 - DNA, 15 bp, Artificial Sequence
  KRAS Antisense Oligonucleotide
ccatcagctccaact

SEQ ID NO: 55 - DNA, 15 bp, Artificial Sequence
  KRAS Antisense Oligonucleotide
gccatcagctccaac

SEQ ID NO: 56 - DNA, 15 bp, Artificial Sequence
  KRAS Antisense Oligonucleotide
cgccatcagctccaa

SEQ ID NO: 57 - DNA, 16 bp, Artificial Sequence
  KRAS Antisense Oligonucleotide
ccatcagctccaacta

SEQ ID NO: 58 - DNA, 16 bp, Artificial Sequence
  KRAS Antisense Oligonucleotide
gccatcagctccaact

SEQ ID NO: 59 - DNA, 16 bp, Artificial Sequence
  KRAS Antisense Oligonucleotide
cgccatcagctccaac

SEQ ID NO: 60 - DNA, 16 bp, Artificial Sequence
  KRAS Antisense Oligonucleotide
acgccatcagctccaa

SEQ ID NO: 61 - DNA, 17 bp, Artificial Sequence
  NRAS Antisense Oligonucleotide
gcctacgccatcagctc

SEQ ID NO: 62 - DNA, 15 bp, Artificial Sequence
  NRAS Antisense Oligonucleotide
ggattgtcagtgcgc

SEQ ID NO: 63 - DNA, 15 bp, Artificial Sequence
  NRAS Antisense Oligonucleotide
attcggtactggcgt

SEQ ID NO: 64 - DNA, 20 bp, Artificial Sequence
  NRAS Antisense Oligonucleotide
ggattgtcagtgcgcttttc

SEQ ID NO: 65 - DNA, 20 bp, Artificial Sequence
  NRAS Antisense Oligonucleotide
gacttgctattattgatggc

SEQ ID NO: 66 - DNA, 20 bp, Artificial Sequence
  NRAS Antisense Oligonucleotide
tactcgcttaatctgctccc

SEQ ID NO: 67 - DNA, 20 bp, Artificial Sequence
  NRAS Antisense Oligonucleotide
atcaactgtccttgttggca

SEQ ID NO: 68 - DNA, 20 bp, Artificial Sequence
  NRAS Antisense Oligonucleotide
gcgtatttctcttaccagtg

SEQ ID NO: 69 - DNA, 20 bp, Artificial Sequence
  NRAS Antisense Oligonucleotide
gttttttcattcggtactgg

SEQ ID NO: 70 - DNA, 20 bp, Artificial Sequence
  NRAS Antisense Oligonucleotide
aacagggagtaacaagaggt

SEQ ID NO: 71 - DNA, 20 bp, Artificial Sequence
  PMP22 Antisense Oligonucleotide
cagttgctactttagagctc

SEQ ID NO: 72 - DNA, 17 bp, Artificial Sequence
  PMP22 Antisense Oligonucleotide
caaacagcgtaacccct

SEQ ID NO: 73 - DNA, 20 bp, Artificial Sequence
  PMP22 Antisense Oligonucleotide
agcaccgcgacgtggaggac

SEQ ID NO: 74 - DNA, 20 bp, Artificial Sequence
  PMP22 Antisense Oligonucleotide
tggacagactgcagccattc

SEQ ID NO: 75 - DNA, 20 bp, Artificial Sequence
  PMP22 Antisense Oligonucleotide
gtaaaacctgccccccttgg

SEQ ID NO: 76 - DNA, 20 bp, Artificial Sequence
  PMP22 Antisense Oligonucleotide
ctcattcgcgtttccgcaag

SEQ ID NO: 77 - DNA, 20 bp, Artificial Sequence
  PMP22 Antisense Oligonucleotide
ctttaaggctcaacacgagg

SEQ ID NO: 78 - DNA, 20 bp, Artificial Sequence
  PMP22 Antisense Oligonucleotide
ttggggtttctacccacact

SEQ ID NO: 79 - DNA, 20 bp, Artificial Sequence
  PMP22 Antisense Oligonucleotide
cacctgtaagggcaagtatg

SEQ ID NO: 80 - DNA, 20 bp, Artificial Sequence
  PMP22 Antisense Oligonucleotide
tccagtgagttgtttagatg

SEQ ID NO: 81 - DNA, 20 bp, Artificial Sequence
  C/EBPBeta Antisense Oligonucleotide
tcacggtcccaaggagtcta

SEQ ID NO: 82 - DNA, 15 bp, Artificial Sequence
  C/EBPBeta Antisense Oligonucleotide
gctcgtggtcgccga

SEQ ID NO: 83 - DNA, 15 bp, Artificial Sequence
  C/EBPBeta Antisense Oligonucleotide
cgtagtcgtcggaga

SEQ ID NO: 84 - DNA, 16 bp, Artificial Sequence
  C/EBPBeta Antisense Oligonucleotide
tcgtggtcgccgatgc

SEQ ID NO: 85 - DNA, 16 bp, Artificial Sequence
  C/EBPBeta Antisense Oligonucleotide
tcgcgccggatcttgt

SEQ ID NO: 86 - DNA, 17 bp, Artificial Sequence
  C/EBPBeta Antisense Oligonucleotide
cgctcgtggtcgccgat

SEQ ID NO: 87 - DNA, 17 bp, Artificial Sequence
  C/EBPBeta Antisense Oligonucleotide
ccgtagtcgtcggagaa

SEQ ID NO: 88 - DNA, 17 bp, Artificial Sequence
  C/EBPBeta Antisense Oligonucleotide
tgcccccgtagtcgtcg

SEQ ID NO: 89 - DNA, 17 bp, Artificial Sequence
  C/EBPBeta Antisense Oligonucleotide
cggatcttgtactcgtc

SEQ ID NO: 90 - DNA, 20 bp, Artificial Sequence
  C/EBPBeta Antisense Oligonucleotide
taagcgcgcagcgcgtacgg

SEQ ID NO: 91 - DNA, 20 bp, Artificial Sequence
  STAT3 Antisense Oligonucleotide
cgcgccggatcttgtactcg

SEQ ID NO: 92 - DNA, 15 bp, Artificial Sequence
  STAT3 Antisense Oligonucleotide
atttgttgacgggtc

SEQ ID NO: 93 - DNA, 15 bp, Artificial Sequence
  STAT3 Antisense Oligonucleotide
cgacaatactttccg

SEQ ID NO: 94 - DNA, 16 bp, Artificial Sequence
  STAT3 Antisense Oligonucleotide
gaactggacgccggtc

SEQ ID NO: 95 - DNA, 16 bp, Artificial Sequence
  STAT3 Antisense Oligonucleotide
cacaattggctcggcc

SEQ ID NO: 96 - DNA, 20 bp, Artificial Sequence
  STAT3 Antisense Oligonucleotide
cgtagattgtgctgatagag

SEQ ID NO: 97 - DNA, 20 bp, Artificial Sequence
  STAT3 Antisense Oligonucleotide
gccacaatccgggcaatctc

SEQ ID NO: 98 - DNA, 20 bp, Artificial Sequence
  STAT3 Antisense Oligonucleotide
agttttctagccgatctagg

SEQ ID NO: 99 - DNA, 20 bp, Artificial Sequence
  STAT3 Antisense Oligonucleotide
cgacaatactttccgaatgc

SEQ ID NO: 100 - DNA, 20 bp, Artificial Sequence
  STAT3 Antisense Oligonucleotide
aggtaggcgcctcagtcgta

SEQ ID NO: 101 - DNA, 20 bp, Artificial Sequence
  NLRP3 Antisense Oligonucleotide
caggtaggcgcctcagtcgt

SEQ ID NO: 102 - DNA, 20 bp, Artificial Sequence
  NLRP3 Antisense Oligonucleotide
ctccgagagtgttgcctcgc

SEQ ID NO: 103 - DNA, 20 bp, Artificial Sequence
  NLRP3 Antisense Oligonucleotide
gtaaaggtgcgtgagattct

SEQ ID NO: 104 - DNA, 20 bp, Artificial Sequence
  NLRP3 Antisense Oligonucleotide
gtcgaagcagcactcatgcg

SEQ ID NO: 105 - DNA, 20 bp, Artificial Sequence
  NLRP3 Antisense Oligonucleotide
agtccatggccctttgcacg

SEQ ID NO: 106 - DNA, 20 bp, Artificial Sequence
  NLRP3 Antisense Oligonucleotide
gcagtgtgacgtgaggttgc

SEQ ID NO: 107 - DNA, 20 bp, Artificial Sequence
  NLRP3 Antisense Oligonucleotide
cgagagtgttgcctcgcagg

SEQ ID NO: 108 - DNA, 20 bp, Artificial Sequence
  NLRP3 Antisense Oligonucleotide
atcgcagcgaagatccacac

SEQ ID NO: 109 - DNA, 20 bp, Artificial Sequence
  NLRP3 Antisense Oligonucleotide
atcttaatgggactcacggg

SEQ ID NO: 110 - DNA, 20 bp, Artificial Sequence
  NLRP3 Antisense Oligonucleotide
gatctccacatgccgaggat

SEQ ID NO: 111 - DNA, 20 bp, Artificial Sequence
  NLRP3 Antisense Oligonucleotide
tccgagagtgttgcctcgca

SEQ ID NO: 112 - DNA, 20 bp, Artificial Sequence
  NLRP3 Antisense Oligonucleotide
tggttgctgctgaggaccaa